European Patent Specification EP 3 230 314 B1, published May 3, 2023. Title: USE OF MARKERS INCLUDING FILAMIN A IN THE DIAGNOSIS AND TREATMENT OF PROSTATE CANCER. Applicant: BERG LLC AKMAEV, VIATCHESLAV R. The sequence listing filed with the application follows.

SEQUENCE LISTING (49 sequences)

SEQ ID NO: 1 - protein, 520 aa, Homo Sapiens
MIARQQCVRGGPRGFSCGSAIVGGGKRGAFSSVSMSGGAGRCSSGGFGSRSLYNLRGNKSISMSVAGSRQGACFGGAGGFGTGGFGGGFGGSFSGKGGPGFPVCPAGGIQEVTINQSLLTPLHVEIDPEIQKVRTEEREQIKLLNNKFASFIDKVQFLEQQNKVLETKWNLLQQQTTTTSSKNLEPLFETYLSVLRKQLDTLGNDKGRLQSELKTMQDSVEDFKTKYEEEINKRTAAENDFVVLKKDVDAAYLNKVELEAKVDSLNDEINFLKVLYDAELSQMQTHVSDTSVVLSMDNNRNLDLDSIIAEVRAQYEEIAQRSKAEAEALYQTKVQQLQISVDQHGDNLKNTKSEIAELNRMIQRLRAEIENIKKQCQTLQVSVADAEQRGENALKDAHSKRVELEAALQQAKEELARMLREYQELMSVKLALDIEIATYRKLLEGEEYRMSGECQSAVSISVVSGSTSTGGISGGLGSGSGFGLSSGFGSGSGSGFGFGGSVSGSSSSKIISTTTLNKRR

SEQ ID NO: 2 - DNA, 2147 bp, Homo sapiens
actcaccggcctgggccctgtcacttctctgatagctcccagctcgctctctgcagccatgattgccagacagcagtgtgtccgaggcgggccccggggcttcagctgtggctcggccattgtaggcggtggcaagagaggtgccttcagctcagtctccatgtctggaggtgctggccgatgctcttctgggggatttggcagcagaagcctctacaacctcagggggaacaaaagcatctccatgagtgtggctgggtcacgacaaggtgcctgctttgggggtgctggaggctttggcactggtggctttggtggtggatttgggggctccttcagtggtaagggtggccctggcttccccgtctgccccgctgggggaattcaggaggtcaccatcaaccagagcttgctcacccccctccacgtggagattgaccctgagatccagaaagtccggacggaagagcgcgaacagatcaagctcctcaacaacaagtttgcctccttcatcgacaaggtgcagttcttagagcaacagaataaggtcctggagaccaaatggaacctgctccagcagcagacgaccaccacctccagcaaaaaccttgagcccctctttgagacctacctcagtgtcctgaggaagcagctagataccttgggcaatgacaaagggcgcctgcagtctgagctgaagaccatgcaggacagcgtggaggacttcaagactaagtatgaagaggagatcaacaaacgcacagcagccgagaatgactttgtggtcctaaagaaggacgtggatgctgcctacctgaacaaggtggagttggaggccaaggtggacagtcttaatgacgagatcaacttcctgaaggtcctctatgatgcggagctgtcccagatgcagacccatgtcagcgacacgtccgtggtcctttccatggacaacaaccgcaacctggacctggacagcattattgccgaggtccgtgcccagtacgaggagattgcccagaggagcaaggctgaggctgaagccctgtaccagaccaaggtccagcagctccagatctcggttgaccaacatggtgacaacctgaagaacaccaagagtgaaattgcagagctcaacaggatgatccagaggctgcgggcagagatcgagaacatcaagaagcagtgccagactcttcaggtatccgtggctgatgcagagcagcgaggtgagaatgcccttaaagatgcccacagcaagcgcgtagagctggaggctgccctgcagcaggccaaggaggagctggcacgaatgctgcgtgagtaccaggagctcatgagtgtgaagctggccttggacatcgagatcgccacctaccgcaaactgctggagggcgaggagtacagaatgtctggagaatgccagagtgccgtgagcatctctgtggtcagcggtagcaccagcactggaggcatcagcggaggattaggaagtggctccgggtttggcctgagtagtggctttggctccggctctggaagtggctttgggtttggtggcagtgtctctggcagttccagcagcaagatcatctctaccaccaccctgaacaagagacgatagaggagacgaggtccctgcagctcactgtgtccagctgggcccagcactggtgtctctgtgcttccttcacttcacctccatcctctgtctctggggctcatcttactagtatcccctccactatcccatgggctctctctgccccaggatgatcttctgtgctgggacagggactctgcctcttggagtttggtagctacttcttgatttgggcctggtgacccacctggaatgggaaggatgtcagctgacctctcacctcccatggacagagaagaaaatgaccaggagtgtcatctccagaattattggggtcacatatgtcccttcccagtccaatgccatctcccactagatcctgtattatccatctacatcagaaccaaactacttctccaacacccggcagcacttggccctgcaagcttaggatgagaaccacttagtgtcccattctactcctctcattccctcttatccatctgcaggtgaatcttcaataaaatgcttttgtcattcattctga

SEQ ID NO: 3 - protein, 469 aa, Homo sapiens
MSIHFSSPVFTSRSAAFSGRGAQVRLSSARPGGLGSSSLYGLGASRPRVAVRSAYGGPVGAGIREVTINQSLLAPLRLDADPSLQRVRQEESEQIKTLNNKFASFIDKVRFLEQQNKLLETKWTLLQEQKSAKSSRLPDIFEAQIAGLRGQLEALQVDGGRLEAELRSMQDVVEDFKNKYEDEINHRTAAENEFVVLKKDVDAAYMSKVELEAKVDALNDEINFLRTLNETELTELQSQISDTSVVLSMDNSRSLDLDGIIAEVKAQYEEMAKCSRAEAEAWYQTKFETLQAQAGKHGDDLRNTRNEISEMNRAIQRLQAEIDNIKNQRAKLEAAIAEAEERGELALKDARAKQEELEAALQRGKQDMARQLREYQELMSVKLALDIEIATYRKLLEGEESRLAGDGVGAVNISVMNSTGGSSSGGGIGLTLGGTMGSNALSFSSSAGPGLLKAYSIRTASASRRSARD

SEQ ID NO: 4 - DNA, 1753 bp, Homo sapiens
cagccccgcccctacctgtggaagcccagccgcccgctcccgcggataaaaggcgcggagtgtccccgaggtcagcgagtgcgcgctcctcctcgcccgccgctaggtccatcccggcccagccaccatgtccatccacttcagctccccggtattcacctcgcgctcagccgccttctcgggccgcggcgcccaggtgcgcctgagctccgctcgccccggcggccttggcagcagcagcctctacggcctcggcgcctcacggccgcgcgtggccgtgcgctctgcctatgggggcccggtgggcgccggcatccgcgaggtcaccattaaccagagcctgctggccccgctgcggctggacgccgacccctccctccagcgggtgcgccaggaggagagcgagcagatcaagaccctcaacaacaagtttgcctccttcatcgacaaggtgcggtttctggagcagcagaacaagctgctggagaccaagtggacgctgctgcaggagcagaagtcggccaagagcagccgcctcccagacatctttgaggcccagattgctggccttcggggtcagcttgaggcactgcaggtggatgggggccgcctggaggcggagctgcggagcatgcaggatgtggtggaggacttcaagaataagtacgaagatgaaattaaccaccgcacagctgctgagaatgagtttgtggtgctgaagaaggatgtggatgctgcctacatgagcaaggtggagctggaggccaaggtggatgccctgaatgatgagatcaacttcctcaggaccctcaatgagacggagttgacagagctgcagtcccagatctccgacacatctgtggtgctgtccatggacaacagtcgctccctggacctggacggcatcatcgctgaggtcaaggcgcagtatgaggagatggccaaatgcagccgggctgaggctgaagcctggtaccagaccaagtttgagaccctccaggcccaggctgggaagcatggggacgacctccggaatacccggaatgagatttcagagatgaaccgggccatccagaggctgcaggctgagatcgacaacatcaagaaccagcgtgccaagttggaggccgccattgccgaggctgaggagcgtggggagctggcgctcaaggatgctcgtgccaagcaggaggagctggaagccgccctgcagcggggcaagcaggatatggcacggcagctgcgtgagtaccaggaactcatgagcgtgaagctggccctggacatcgagatcgccacctaccgcaagctgctggagggcgaggagagccggttggctggagatggagtgggagccgtgaatatctctgtgatgaattccactggtggcagtagcagtggcggtggcattgggctgaccctcgggggaaccatgggcagcaatgccctgagcttctccagcagtgcgggtcctgggctcctgaaggcttattccatccggaccgcatccgccagtcgcaggagtgcccgcgactgagccgcctcccaccactccactcctccagccaccacccacaatcacaagaagattcccacccctgcctcccatgcctggtcccaagacagtgagacagtctggaaagtgatgtcagaatagcttccaataaagcagcctcattctgaggcctgagtgatccacgtgaaaaaaaaaaaaaaaaaaaaaaaaaaaaaaaaaaaaaaaaaaaaaaaaaaa

SEQ ID NO: 5 - protein, 511 aa, Homo sapiens
MNGVSWSQDLQEGISAWFGPPASTPASTMSIRVTQKSYKVSTSGPRAFSSRSYTSGPGSRISSSSFSRVGSSNFRGGLGGGYGGASGMGGITAVTVNQSLLSPLVLEVDPNIQAVRTQEKEQIKTLNNKFASFIDKVRFLEQQNKMLETKWSLLQQQKTARSNMDNMFESYINNLRRQLETLGQEKLKLEAELGNMQGLVEDFKNKYEDEINKRTEMENEFVLIKKDVDEAYMNKVELESRLEGLTDEINFLRQLYEEEIRELQSQISDTSVVLSMDNSRSLDMDSIIAEVKAQYEDIANRSRAEAESMYQIKYEELQSLAGKHGDDLRRTKTEISEMNRNISRLQAEIEGLKGQRASLEAAIADAEQRGELAIKDANAKLSELEAALQRAKQDMARQLREYQELMNVKLALDIEIATYRKLLEGEESRLESGMQNMSIHTKTTSGYAGGLSSAYGGLTSPGLSYSLGSSFGSGAGSSSFSRTSSSRAVVVKKIETRDGKLVSESSDVLPK

SEQ ID NO: 6 - DNA, 1807 bp, Homo sapiens
attcagcaaatgtttgcggaatgaatggggtgagctggagccaggacctgcaggaagggatctccgcctggttcggcccgcctgcctccactcctgcctctaccatgtccatcagggtgacccagaagtcctacaaggtgtccacctctggcccccgggccttcagcagccgctcctacacgagtgggcccggttcccgcatcagctcctcgagcttctcccgagtgggcagcagcaactttcgcggtggcctgggcggcggctatggtggggccagcggcatgggaggcatcaccgcagttacggtcaaccagagcctgctgagcccccttgtcctggaggtggaccccaacatccaggccgtgcgcacccaggagaaggagcagatcaagaccctcaacaacaagtttgcctccttcatagacaaggtacggttcctggagcagcagaacaagatgctggagaccaagtggagcctcctgcagcagcagaagacggctcgaagcaacatggacaacatgttcgagagctacatcaacaaccttaggcggcagctggagactctgggccaggagaagctgaagctggaggcggagcttggcaacatgcaggggctggtggaggacttcaagaacaagtatgaggatgagatcaataagcgtacagagatggagaacgaatttgtcctcatcaagaaggatgtggatgaagcttacatgaacaaggtagagctggagtctcgcctggaagggctgaccgacgagatcaacttcctcaggcagctatatgaagaggagatccgggagctgcagtcccagatctcggacacatctgtggtgctgtccatggacaacagccgctccctggacatggacagcatcattgctgaggtcaaggcacagtacgaggatattgccaaccgcagccgggctgaggctgagagcatgtaccagatcaagtatgaggagctgcagagcctggctgggaagcacggggatgacctgcggcgcacaaagactgagatctctgagatgaaccggaacatcagccggctccaggctgagattgagggcctcaaaggccagagggcttccctggaggccgccattgcagatgccgagcagcgtggagagctggccattaaggatgccaacgccaagttgtccgagctggaggccgccctgcagcgggccaagcaggacatggcgcggcagctgcgtgagtaccaggagctgatgaacgtcaagctggccctggacatcgagatcgccacctacaggaagctgctggagggcgaggagagccggctggagtctgggatgcagaacatgagtattcatacgaagaccaccagcggctatgcaggtggtctgagctcggcctatgggggcctcacaagccccggcctcagctacagcctgggctccagctttggctctggcgcgggctccagctccttcagccgcaccagctcctccagggccgtggttgtgaagaagatcgagacacgtgatgggaagctggtgtctgagtcctctgacgtcctgcccaagtgaacagctgcggcagcccctcccagcctacccctcctgcgctgccccagagcctgggaaggaggccgctatgcagggtagcactgggaacaggagacccacctgaggctcagccctagccctcagcccacctggggagtttactacctggggaccccccttgcccatgcctccagctacaaaacaattcaattgctttttttttttggtccaaaataaaacctcagctagctctgccaatgtcaaaaaaaaaa

SEQ ID NO: 7 - protein, 483 aa, Homo sapiens
MSIRVTQKSYKVSTSGPRAFSSRSYTSGPGSRISSSSFSRVGSSNFRGGLGGGYGGASGMGGITAVTVNQSLLSPLVLEVDPNIQAVRTQEKEQIKTLNNKFASFIDKVRFLEQQNKMLETKWSLLQQQKTARSNMDNMFESYINNLRRQLETLGQEKLKLEAELGNMQGLVEDFKNKYEDEINKRTEMENEFVLIKKDVDEAYMNKVELESRLEGLTDEINFLRQLYEEEIRELQSQISDTSVVLSMDNSRSLDMDSIIAEVKAQYEDIANRSRAEAESMYQIKYEELQSLAGKHGDDLRRTKTEISEMNRNISRLQAEIEGLKGQRASLEAAIADAEQRGELAIKDANAKLSELEAALQRAKQDMARQLREYQELMNVKLALDIEIATYRKLLEGEESRLESGMQNMSIHTKTTSGYAGGLSSAYGGLTSPGLSYSLGSSFGSGAGSSSFSRTSSSRAVVVKKIETRDGKLVSESSDVLPK

SEQ ID NO: 8 - DNA, 1901 bp, Homo sapiens
acaggcctttccttacctccctccatgctgtccacttcctctgtaaagctctcaaccctgtccccttccccctctctcctgggaaagagccctcccatgcctagctgctgctcttagggaccctgtggctaggtgcgcggatggaaatccaggatctccgcctggttcggcccgcctgcctccactcctgcctctaccatgtccatcagggtgacccagaagtcctacaaggtgtccacctctggcccccgggccttcagcagccgctcctacacgagtgggcccggttcccgcatcagctcctcgagcttctcccgagtgggcagcagcaactttcgcggtggcctgggcggcggctatggtggggccagcggcatgggaggcatcaccgcagttacggtcaaccagagcctgctgagcccccttgtcctggaggtggaccccaacatccaggccgtgcgcacccaggagaaggagcagatcaagaccctcaacaacaagtttgcctccttcatagacaaggtacggttcctggagcagcagaacaagatgctggagaccaagtggagcctcctgcagcagcagaagacggctcgaagcaacatggacaacatgttcgagagctacatcaacaaccttaggcggcagctggagactctgggccaggagaagctgaagctggaggcggagcttggcaacatgcaggggctggtggaggacttcaagaacaagtatgaggatgagatcaataagcgtacagagatggagaacgaatttgtcctcatcaagaaggatgtggatgaagcttacatgaacaaggtagagctggagtctcgcctggaagggctgaccgacgagatcaacttcctcaggcagctatatgaagaggagatccgggagctgcagtcccagatctcggacacatctgtggtgctgtccatggacaacagccgctccctggacatggacagcatcattgctgaggtcaaggcacagtacgaggatattgccaaccgcagccgggctgaggctgagagcatgtaccagatcaagtatgaggagctgcagagcctggctgggaagcacggggatgacctgcggcgcacaaagactgagatctctgagatgaaccggaacatcagccggctccaggctgagattgagggcctcaaaggccagagggcttccctggaggccgccattgcagatgccgagcagcgtggagagctggccattaaggatgccaacgccaagttgtccgagctggaggccgccctgcagcgggccaagcaggacatggcgcggcagctgcgtgagtaccaggagctgatgaacgtcaagctggccctggacatcgagatcgccacctacaggaagctgctggagggcgaggagagccggctggagtctgggatgcagaacatgagtattcatacgaagaccaccagcggctatgcaggtggtctgagctcggcctatgggggcctcacaagccccggcctcagctacagcctgggctccagctttggctctggcgcgggctccagctccttcagccgcaccagctcctccagggccgtggttgtgaagaagatcgagacacgtgatgggaagctggtgtctgagtcctctgacgtcctgcccaagtgaacagctgcggcagcccctcccagcctacccctcctgcgctgccccagagcctgggaaggaggccgctatgcagggtagcactgggaacaggagacccacctgaggctcagccctagccctcagcccacctggggagtttactacctggggaccccccttgcccatgcctccagctacaaaacaattcaattgctttttttttttggtccaaaataaaacctcagctagctctgccaatgtcaaaaaaaaaa

SEQ ID NO: 9 - protein, 456 aa, Homo sapiens
MTTTFLQTSSSTFGGGSTRGGSLLAGGGGFGGGSLSGGGGSRSISASSARFVSSGSGGGYGGGMRVCGFGGGAGSVFGGGFGGGVGGGFGGGFGGGDGGLLSGNEKITMQNLNDRLASYLDKVRALEEANADLEVKIHDWYQKQTPTSPECDYSQYFKTIEELRDKIMATTIDNSRVILEIDNARLAADDFRLKYENELALRQGVEADINGLRRVLDELTLARTDLEMQIEGLNEELAYLKKNHEEEMKEFSSQLAGQVNVEMDAAPGVDLTRVLAEMREQYEAMAEKNRRDVEAWFFSKTEELNKEVASNTEMIQTSKTEITDLRRTMQELEIELQSQLSMKAGLENSLAETECRYATQLQQIQGLIGGLEAQLSELRCEMEAQNQEYKMLLDIKTRLEQEIATYRSLLEGQDAKMAGIGIREASSGGGGSSSNFHINVEESVDGQVVSSHKREI

SEQ ID NO: 10 - DNA, 1861 bp, Homo sapiens
cactcaaggtgtgcaggcagctgtgtttgtcaggaaggcagaaggagttggctttgctttaggggaggagacgaggtcccacaacaccctctgaagggtatataaggagccccagcgtgcagcctggcctggtacctcctgccagcatctcttgggtttgctgagaactcacgggctccagctacctggccatgaccaccacatttctgcaaacttcttcctccacctttgggggtggctcaacccgagggggttccctcctggctgggggaggtggctttggtggggggagtctctctgggggaggtggaagccgaagtatctcagcttcttctgctaggtttgtctcttcagggtcaggaggaggatatgggggtggcatgagggtctgtggctttggtggaggggctggtagtgttttcggtggaggctttggagggggcgttggtgggggttttggtggtggctttggtggtggcgatggtggtctcctctctggcaatgagaaaattaccatgcagaacctcaatgaccgcctggcctcctacctggacaaggtacgtgccctggaggaggccaatgctgacctggaggtgaagatccatgactggtaccagaagcagaccccaaccagcccagaatgcgactacagccaatacttcaagaccattgaagagctccgggacaagatcatggccaccaccatcgacaactcccgggtcatcctggagatcgacaatgccaggctggctgcggacgacttcaggctcaagtatgagaatgagctggccctgcgccagggcgttgaggctgacatcaacggcttgcgccgagtcctggatgagctgaccctggccaggactgacctggagatgcagatcgagggcctgaatgaggagctagcctacctgaagaagaaccacgaagaggagatgaaggagttcagcagccagctggccggccaggtcaatgtggagatggacgcagcaccgggtgtggacctgacccgtgtgctggcagagatgagggagcagtacgaggccatggcggagaagaaccgccgggatgtcgaggcctggttcttcagcaagactgaggagctgaacaaagaggtggcctccaacacagaaatgatccagaccagcaagacggagatcacagacctgagacgcacgatgcaggagctggagatcgagctgcagtcccagctcagcatgaaagctgggctggagaactcactggccgagacagagtgccgctatgccacgcagctgcagcagatccaggggctcattggtggcctggaggcccagctgagtgagctccgatgcgagatggaggctcagaaccaggagtacaagatgctgcttgacataaagacacggctggagcaggagatcgctacttaccgcagcctgctcgagggccaggatgccaagatggctggcattggcatcagggaagcctcttcaggaggtggtggtagcagcagcaatttccacatcaatgtagaagagtcagtggatggacaggtggtttcttcccacaagagagaaatctaagtgtctattgcaggagaaacgtcccttgccactccccactctcatcaggccaagtggaggactggccagagggcctgcacatgcaaactccagtccctgccttcagagagctgaaaagggtccctcggtcttttatttcagggctttgcatgcgctctattccccctctgcctctccccaccttctttggagcaaggagatgcagctgtattgtgtaacaagctcatttgtacagtgtctgttcatgtaataaagaattacttttccttttgcaaataaaaaaaaaaaaaaaaaaaaaa

SEQ ID NO: 11 - protein, 430 aa, Homo sapiens
MSFTTRSTFSTNYRSLGSVQAPSYGARPVSSAASVYAGAGGSGSRISVSRSTSFRGGMGSGGLATGIAGGLAGMGGIQNEKETMQSLNDRLASYLDRVRSLETENRRLESKIREHLEKKGPQVRDWSHYFKIIEDLRAQIFANTVDNARIVLQIDNARLAADDFRVKYETELAMRQSVENDIHGLRKVIDDTNITRLQLETEIEALKEELLFMKKNHEEEVKGLQAQIASSGLTVEVDAPKSQDLAKIMADIRAQYDELARKNREELDKYWSQQIEESTTVVTTQSAEVGAAETTLTELRRTVQSLEIDLDSMRNLKASLENSLREVEARYALQMEQLNGILLHLESELAQTRAEGQRQAQEYEALLNIKVKLEAEIATYRRLLEDGEDFNLGDALDSSNSMQTIQKTTTRRIVDGKVVSETNDTKVLRH

SEQ ID NO: 12 - DNA, 1485 bp, Homo sapiens
tccggggcgggggcggggcctcactctgcgatataactcgggtcgcgcggctcgcgcaggccgccaccgtcgtccgcaaagcctgagtcctgtcctttctctctccccggacagcatgagcttcaccactcgctccaccttctccaccaactaccggtccctgggctctgtccaggcgcccagctacggcgcccggccggtcagcagcgcggccagcgtctatgcaggcgctgggggctctggttcccggatctccgtgtcccgctccaccagcttcaggggcggcatggggtccgggggcctggccaccgggatagccgggggtctggcaggaatgggaggcatccagaacgagaaggagaccatgcaaagcctgaacgaccgcctggcctcttacctggacagagtgaggagcctggagaccgagaaccggaggctggagagcaaaatccgggagcacttggagaagaagggaccccaggtcagagactggagccattacttcaagatcatcgaggacctgagggctcagatcttcgcaaatactgtggacaatgcccgcatcgttctgcagattgacaatgcccgtcttgctgctgatgactttagagtcaagtatgagacagagctggccatgcgccagtctgtggagaacgacatccatgggctccgcaaggtcattgatgacaccaatatcacacgactgcagctggagacagagatcgaggctctcaaggaggagctgctcttcatgaagaagaaccacgaagaggaagtaaaaggcctacaagcccagattgccagctctgggttgaccgtggaggtagatgcccccaaatctcaggacctcgccaagatcatggcagacatccgggcccaatatgacgagctggctcggaagaaccgagaggagctagacaagtactggtctcagcagattgaggagagcaccacagtggtcaccacacagtctgctgaggttggagctgctgagacgacgctcacagagctgagacgtacagtccagtccttggagatcgacctggactccatgagaaatctgaaggccagcttggagaacagcctgagggaggtggaggcccgctacgccctacagatggagcagctcaacgggatcctgctgcaccttgagtcagagctggcacagacccgggcagagggacagcgccaggcccaggagtatgaggccctgctgaacatcaaggtcaagctggaggctgagatcgccacctaccgccgcctgctggaagatggcgaggactttaatcttggtgatgccttggacagcagcaactccatgcaaaccatccaaaagaccaccacccgccggatagtggatggcaaagtggtgtctgagaccaatgacaccaaagttctgaggcattaagccagcagaagcagggtaccctttggggagcaggaggccaataaaaagttcagagttcaaaaaaaaaaaaaaaaaaa

SEQ ID NO: 13 - protein, 430 aa, Homo sapiens; identical to SEQ ID NO: 11

SEQ ID NO: 14 - DNA, 1439 bp, Homo sapiens
gcagcctcgagggccaacaacacctgctgtccgtgtccatgcccggttggccaccccgtttctgggggcatgagcttcaccactcgctccaccttctccaccaactaccggtccctgggctctgtccaggcgcccagctacggcgcccggccggtcagcagcgcggccagcgtctatgcaggcgctgggggctctggttcccggatctccgtgtcccgctccaccagcttcaggggcggcatggggtccgggggcctggccaccgggatagccgggggtctggcaggaatgggaggcatccagaacgagaaggagaccatgcaaagcctgaacgaccgcctggcctcttacctggacagagtgaggagcctggagaccgagaaccggaggctggagagcaaaatccgggagcacttggagaagaagggaccccaggtcagagactggagccattacttcaagatcatcgaggacctgagggctcagatcttcgcaaatactgtggacaatgcccgcatcgttctgcagattgacaatgcccgtcttgctgctgatgactttagagtcaagtatgagacagagctggccatgcgccagtctgtggagaacgacatccatgggctccgcaaggtcattgatgacaccaatatcacacgactgcagctggagacagagatcgaggctctcaaggaggagctgctcttcatgaagaagaaccacgaagaggaagtaaaaggcctacaagcccagattgccagctctgggttgaccgtggaggtagatgcccccaaatctcaggacctcgccaagatcatggcagacatccgggcccaatatgacgagctggctcggaagaaccgagaggagctagacaagtactggtctcagcagattgaggagagcaccacagtggtcaccacacagtctgctgaggttggagctgctgagacgacgctcacagagctgagacgtacagtccagtccttggagatcgacctggactccatgagaaatctgaaggccagcttggagaacagcctgagggaggtggaggcccgctacgccctacagatggagcagctcaacgggatcctgctgcaccttgagtcagagctggcacagacccgggcagagggacagcgccaggcccaggagtatgaggccctgctgaacatcaaggtcaagctggaggctgagatcgccacctaccgccgcctgctggaagatggcgaggactttaatcttggtgatgccttggacagcagcaactccatgcaaaccatccaaaagaccaccacccgccggatagtggatggcaaagtggtgtctgagaccaatgacaccaaagttctgaggcattaagccagcagaagcagggtaccctttggggagcaggaggccaataaaaagttcagagttcaaaaaaaaaaaaaaaaaaa

SEQ ID NO: 15 - protein, 400 aa, Homo sapiens
MTSYSYRQSSATSSFGGLGGGSVRFGPGVAFRAPSIHGGSGGRGVSVSSARFVSSSSSGAYGGGYGGVLTASDGLLAGNEKLTMQNLNDRLASYLDKVRALEAANGELEVKIRDWYQKQGPGPSRDYSHYYTTIQDLRDKILGATIENSRIVLQIDNARLAADDFRTKFETEQALRMSVEADINGLRRVLDELTLARTDLEMQIEGLKEELAYLKKNHEEEISTLRGQVGGQVSVEVDSAPGTDLAKILSDMRSQYEVMAEQNRKDAEAWFTSRTEELNREVAGHTEQLQMSRSEVTDLRRTLQGLEIELQSQLSMKAALEDTLAETEARFGAQLAHIQALISGIEAQLGDVRADSERQNQEYQRLMDIKSRLEQEIATYRSLLEGQEDHYNNLSASKVL

SEQ ID NO: 16 - DNA, 1490 bp, Homo sapiens
agatatccgcccctgacaccattcctcccttcccccctccaccggccgcgggcataaaaggcgccaggtgagggcctcgccgctcctcccgcgaatcgcagcttctgagaccagggttgctccgtccgtgctccgcctcgccatgacttcctacagctatcgccagtcgtcggccacgtcgtccttcggaggcctgggcggcggctccgtgcgttttgggccgggggtcgcctttcgcgcgcccagcattcacgggggctccggcggccgcggcgtatccgtgtcctccgcccgctttgtgtcctcgtcctcctcgggggcctacggcggcggctacggcggcgtcctgaccgcgtccgacgggctgctggcgggcaacgagaagctaaccatgcagaacctcaacgaccgcctggcctcctacctggacaaggtgcgcgccctggaggcggccaacggcgagctagaggtgaagatccgcgactggtaccagaagcaggggcctgggccctcccgcgactacagccactactacacgaccatccaggacctgcgggacaagattcttggtgccaccattgagaactccaggattgtcctgcagatcgacaatgcccgtctggctgcagatgacttccgaaccaagtttgagacggaacaggctctgcgcatgagcgtggaggccgacatcaacggcctgcgcagggtgctggatgagctgaccctggccaggaccgacctggagatgcagatcgaaggcctgaaggaagagctggcctacctgaagaagaaccatgaggaggaaatcagtacgctgaggggccaagtgggaggccaggtcagtgtggaggtggattccgctccgggcaccgatctcgccaagatcctgagtgacatgcgaagccaatatgaggtcatggccgagcagaaccggaaggatgctgaagcctggttcaccagccggactgaagaattgaaccgggaggtcgctggccacacggagcagctccagatgagcaggtccgaggttactgacctgcggcgcacccttcagggtcttgagattgagctgcagtcacagctgagcatgaaagctgccttggaagacacactggcagaaacggaggcgcgctttggagcccagctggcgcatatccaggcgctgatcagcggtattgaagcccagctgggcgatgtgcgagctgatagtgagcggcagaatcaggagtaccagcggctcatggacatcaagtcgcggctggagcaggagattgccacctaccgcagcctgctcgagggacaggaagatcactacaacaatttgtctgcctccaaggtcctctgaggcagcaggctctggggcttctgctgtcctttggagggtgtcttctgggtagagggatgggaaggaagggacccttacccccggctcttctcctgacctgccaataaaaatttatggtccaagggaaaaaaaaaaaaaaaaaaaa

SEQ ID NO: 17 - protein, 378 aa, Homo sapiens
MDSVRSGAFGHLFRPDNFIFGQSGAGNNWAKGHYTEGAELVDSVLDVVRKECENCDCLQGFQLTHSLGGGTGSGMGTLLISKVREEYPDRIMNTFSVVPSPKVSDTVVEPYNATLSIHQLVENTDETYCIDNEALYDICFRTLKLATPTYGDLNHLVSATMSGVTTSLRFPGQLNADLRKLAVNMVPFPRLHFFMPGFAPLTARGSQQYRALTVPELTQQMFDAKNMMAACDPRHGRYLTVATVFRGRMSMKEVDEQMLAIQSKNSSYFVEWIPNNVKVAVCDIPPRGLKMSSTFIGNSTAIQELFKRISEQFTAMFRRKAFLHWYTGEGMDEMEFTEAESNMNDLVSEYQQYQDATAEEEGEMYEDDEEESEAQGPK

SEQ ID NO: 18 - DNA, 1851 bp, Homo sapiens
agacactcaccccggactcccttgaacagggacagggaggaaccccaggcagctagaccccagcagcagccacacgagcacactgtggggcagggaggggcatctcttgagaacaaaagatccatttctcgactttccaaactggagagcttcttgagagaaaagagagagacaggtacaggtccacgccacccacacacagccctgtgcacacagaccggacacaggcgtccacagttctgggaagtcatcagtgatgagcatggcatcgaccccagcggcaactacgtgggcgactcggacttgcagctggagcggatcagcgtctactacaacgaggcctcttctcacaagtacgtgcctcgagccattctggtggacctggaacccggaaccatggacagtgtccgctcaggggcctttggacatctcttcaggcctgacaatttcatctttggtcagagtggggccggcaacaactgggccaagggtcactacacggagggggcggagctggtggattcggtcctggatgtggtgcggaaggagtgtgaaaactgcgactgcctgcagggcttccagctgacccactcgctggggggcggcacgggctccggcatgggcacgttgctcatcagcaaggtgcgtgaggagtatcccgaccgcatcatgaacaccttcagcgtcgtgccctcacccaaggtgtcagacacggtggtggagccctacaacgccacgctgtccatccaccagctggtggagaacacggatgagacctactgcatcgacaacgaggcgctctacgacatctgcttccgcaccctcaagctggccacgcccacctacggggacctcaaccacctggtatcggccaccatgagcggagtcaccacctccttgcgcttcccgggccagctcaacgctgacctgcgcaagctggccgtcaacatggtgcccttcccgcgcctgcacttcttcatgcccggcttcgcccccctcacagcccggggcagccagcagtaccgggccctgaccgtgcccgagctcacccagcagatgttcgatgccaagaacatgatggccgcctgcgacccgcgccacggccgctacctgacggtggccaccgtgttccggggccgcatgtccatgaaggaggtggacgagcagatgctggccatccagagcaagaacagcagctacttcgtggagtggatccccaacaacgtgaaggtggccgtgtgtgacatcccgccccgcggcctcaagatgtcctccaccttcatcgggaacagcacggccatccaggagctgttcaagcgcatctccgagcagttcacggccatgttccggcgcaaggccttcctgcactggtacacgggcgagggcatggacgagatggagttcaccgaggccgagagcaacatgaacgacctggtgtccgagtaccagcagtaccaggacgccacggccgaggaagagggcgagatgtacgaagacgacgaggaggagtcggaggcccagggccccaagtgaagctgctcgcagctggagtgagaggcaggtggcggccggggccgaagccagcagtgtctaaacccccggagccatcttgctgccgacaccctgctttcccctcgccctagggctcccttgccgccctcctgcagtatttatggcctcgtcctccccacctaggccacgtgtgagctgctcctgtctctgtcttattgcagctccaggcctgacgttttacggttttgttttttactggtttgtgtttatattttcggggatacttaataaatctattgctgtcagatacccttaaaaaaaaaaaaaaaaaaaaaaaaa

SEQ ID NO: 19 - protein, 450 aa, Homo sapiens
MREIVHIQAGQCGNQIGAKFWEVISDEHGIDPSGNYVGDSDLQLERISVYYNEASSHKYVPRAILVDLEPGTMDSVRSGAFGHLFRPDNFIFGQSGAGNNWAKGHYTEGAELVDSVLDVVRKECENCDCLQGFQLTHSLGGGTGSGMGTLLISKVREEYPDRIMNTFSVVPSPKVSDTVVEPYNATLSIHQLVENTDETYCIDNEALYDICFRTLKLATPTYGDLNHLVSATMSGVTTSLRFPGQLNADLRKLAVNMVPFPRLHFFMPGFAPLTARGSQQYRALTVPELTQQMFDAKNMMAACDPRHGRYLTVATVFRGRMSMKEVDEQMLAIQSKNSSYFVEWIPNNVKVAVCDIPPRGLKMSSTFIGNSTAIQELFKRISEQFTAMFRRKAFLHWYTGEGMDEMEFTEAESNMNDLVSEYQQYQDATAEEEGEMYEDDEEESEAQGPK

SEQ ID NO: 20 - DNA, 1794 bp, Homo sapiens
gacatcagccgatgcgaagggcggggccgcggctataagagcgcgcggccgcggtccccgaccctcagcagccagcccggcccgcccgcgcccgtccgcagccgcccgccagacgcgcccagtatgagggagatcgtgcacatccaggccggccagtgcggcaaccagatcggggccaagttctgggaagtcatcagtgatgagcatggcatcgaccccagcggcaactacgtgggcgactcggacttgcagctggagcggatcagcgtctactacaacgaggcctcttctcacaagtacgtgcctcgagccattctggtggacctggaacccggaaccatggacagtgtccgctcaggggcctttggacatctcttcaggcctgacaatttcatctttggtcagagtggggccggcaacaactgggccaagggtcactacacggagggggcggagctggtggattcggtcctggatgtggtgcggaaggagtgtgaaaactgcgactgcctgcagggcttccagctgacccactcgctggggggcggcacgggctccggcatgggcacgttgctcatcagcaaggtgcgtgaggagtatcccgaccgcatcatgaacaccttcagcgtcgtgccctcacccaaggtgtcagacacggtggtggagccctacaacgccacgctgtccatccaccagctggtggagaacacggatgagacctactgcatcgacaacgaggcgctctacgacatctgcttccgcaccctcaagctggccacgcccacctacggggacctcaaccacctggtatcggccaccatgagcggagtcaccacctccttgcgcttcccgggccagctcaacgctgacctgcgcaagctggccgtcaacatggtgcccttcccgcgcctgcacttcttcatgcccggcttcgcccccctcacagcccggggcagccagcagtaccgggccctgaccgtgcccgagctcacccagcagatgttcgatgccaagaacatgatggccgcctgcgacccgcgccacggccgctacctgacggtggccaccgtgttccggggccgcatgtccatgaaggaggtggacgagcagatgctggccatccagagcaagaacagcagctacttcgtggagtggatccccaacaacgtgaaggtggccgtgtgtgacatcccgccccgcggcctcaagatgtcctccaccttcatcgggaacagcacggccatccaggagctgttcaagcgcatctccgagcagttcacggccatgttccggcgcaaggccttcctgcactggtacacgggcgagggcatggacgagatggagttcaccgaggccgagagcaacatgaacgacctggtgtccgagtaccagcagtaccaggacgccacggccgaggaagagggcgagatgtacgaagacgacgaggaggagtcggaggcccagggccccaagtgaagctgctcgcagctggagtgagaggcaggtggcggccggggccgaagccagcagtgtctaaacccccggagccatcttgctgccgacaccctgctttcccctcgccctagggctcccttgccgccctcctgcagtatttatggcctcgtcctccccacctaggccacgtgtgagctgctcctgtctctgtcttattgcagctccaggcctgacgttttacggttttgttttttactggtttgtgtttatattttcggggatacttaataaatctattgctgtcagatacccttaaaaaaaaaaaaaaaaaaaaaaaaa

SEQ ID NO: 21 - DNA, 170856 bp, Homo sapiens
gagttagacccaggttcaagtccagctttgtccagtcattaccagctgaccaatagcaaatcttatcacttaatcactaatgaggggaacaagcattcaaatatagtcatgtgtacataatgacatttctgtcaacaacagacagcacaacacattactgttgtgtttgtggtgatgctggtgtaatcataaccttctgtgctgcagtccagtaaaaatatagcacaggccgggggcggtggctcacacttgtggagggccacctccacaagttgcagtgagctgagatcgcaccactgcactccagcctgggcaacaagagtgaaactccatctcaaaaaaataaaacaaacaaacaaacaaacaaacaaacactttttattgcctgggtgtggtggctcacgcctgtaatcccagcactttgggaggctgaggcaggaggattgcttgagcccaggaattttagaccagcctgggcaacatggcgaaaccctgtctctacaaaaaatacaaaaattagctgggcatggtggtgcgcccctatagtcccagctactcaggaggctgaagtgggaagataacctgagcccagggaggtcgataataaaattttaaaaatttttagtagagatgggatttcaccgtgttggaccaggctgatctcgaactcctggcctcaggtgatctgtgcacctcgacctcccaaagtgctgggattacaagcgtgagccactgtgcccagccaacatacttgtttattatcaaatattatatactgtacataattgtatgttttatatatgtatgtatgtgtgtgtgtgtatatatatatatatatatatatatattttttttttttttttagacagagtcttgctctgtcacccaggctggagtgcaacggcaccatcttagctcactgcaacctctgcctcctgggttcaaaccattctcccgcctcagcctcccaagtagctgagattacaggcactcgccatcatgccccactaattttttttgtatttttgtagagatggggttccaccgtgttggccaggctggtctcgaactcctgacctcaggtgatccgcctacctcagcctcccaaagtgctgggattagaggcgtaacccaccgtgcctggccaataaaaagttttaaatacagaaaaaagcttacagaataaggatttaaagaaagaaagaatttttgtacagcttataatgtgtttgtgttttaagctgttattacaaaagccaaaaagtcaaagaattaaaaaatatataaaattaaaaaattacagtaagctaaggttaatttcttttttatttttcttttttcttttttttttttttttgagacggagtctcactctattggcaggttggagtgcagtggcgcgatctcggctcactgtaacctccacctcccggattcaagcaactctcctgcctcagccttccgagtagctgggactacaggtgcgtgccaccccacccagctagtttttgtattttcagtagagacagggtttcaccacgttggccaggatggtcttgatctcttgacctcgtgatccacccgcctcagcctcctaaagtgctgggattacaggggtgagccaccgtgcccggcctctaaggttaatttcttattgcagaagaaaaagattaaaaaaataaacttagtatagcctcagtgtacagtgtttataaagtctacagtagtgcacagtaatgtcctaggccttcacagtcacgtaccactcactcactgactcacccagagcaaattccagtgctgcaagctccattcatggcaagtgcccatacaggtagactatttttatctttttatttatttatttagttagttaatttttgagatggagtctctctctgtcttccaggctggagcgcagtggtgcgatcttggctcactgtaacctctgcctcctgggttcaagcaattctcctacccaagcctcccgagtagctgggattacaggcgcctgccaccatgcctggctaatttttgtatttttagtagagaccgagttttgccatgttggtcaggctggtctcgaactcctgatctcaagtgatccacccgccttggcctcccaaagagctgggattacaggtgtgagccaccacgccccgcccaattttatcttttatatcgtatttttattatacccttttaatgtttagattcacaaatacttattgtaacaattgcctacagtatcaatatagtaacttgctgtacaggtttgtagcccaggggcaacaggtgatcccctctaacctggatgtgtggtcgcctgtaccatctaggtctgtgtgaacacactctctggtgttcctatcatgacaaaatcctctagcattcctgttgttaagcaacacatgagtgtagttactgagtccctattgtgagccagggccgggtaatatattctctcccccaggctgttgtgaccatttccagtgagtcagttcatctgtctgaacaaagcactctggcattgattgtatgcaaataacctgttacagaatggttctacccataaactggctggcctcttttgagcaaccctcaaagttgcaagcccttgccctctgtcctggtcaacctctcttcctcagaagcttgcctgctctgaactcctctcccaaaccgggttaggagccccttctctggtatcagggcaccctgtgcctctcttacagacttgcattatggttctaactgtgctgtgtggcctgggcaagccgctcaaccactcggttatttcttctttttttttttttgagacagagtttcactgttattgcccaggctggagtgcaatcttggctcaccacaacctctgcctcctgggttcaagcgattctcctgcctcagcctcccaagtagctgggattacaggcatgcgccaccacgcccagctaattttttgtatttttagtagagctagggttttttcatgttggtcaggctggtctcgaactcctgacctcaggtgatctgcccaccttggcctcccaaggtgctgggattacaggtgtgagccactgcacccgacttgaaagaaattgctttgcactgtgcttggcacagaggaacagcaggtgttcattcaatgcttgctgttgtaattattcaggcttttatcaacagagggctggcctgagactctgccatatctcagaacctagcacagaacctggatgagtacagagtaagtgctcaatgtatgctgtggtaggcagagtaatagcccccaaagacgttcacatcctaactctcaggacctgtgaacattcccttaaatggcaaaggggaattaaggttgcaaacaggattagggttcttaatcggctgattttaaaatagggagatcatgttggactaaccagctggcccaatgtcatcttaagagtccttaaaagggccaggtgtggggaggttgaagctgcagggagccgagattgagtcatagcactccagtttgggagacggagtgagacaaaaaaaaggctgggcaaggtggctcatgcctgtaatcccatcactttgggaggcagaggctggtggatcgcttgaggtcaggagttcaagaccagcctggccaacatggtgaaagcccgtctctattaaaaatacaaaaattagcggagcgtggtggcgggtgcctgtaatcccagccactcaggaggttgaggcaagagaattgcttgaacccaggaggaggaggttgcagtgagccgagattgcaccactggactctagcctgggcaacggagtaagactccatcgcaggaaaaaaaaaaaaaaggaagatgtgcctatggagagaggactgtctgaggtctgagagactccacctgacattgcaggcttgcttttctgttttttttttttttttttttttttttgagacggagttttgctctgtcgcccaggctggagtgcaatggcaccatctcagctcactgtaacctctgcctcccaggttcaagcgattctcctatctcagccttcccagtagctgggattacaggtacgcgccaccacacctggctaatttttgtattttaagtagagatggggttttaccatgttggccaggctggtctcgaactcctgacctcaggtgatccacccaccttggcctcccaaagtgctgggattacaggtgtgagccattgtgcccagcccattgcaggctttcacagagaaaaggggcaggagtcaggcgcgcaggcagcttctggaagttagaaaacacaaggaaacagattcttccctacagcctccagaagggaatgcatcctgccaacactttgtttttagctcagcaagacctgtgtgggccatcgaacctacagaactgaaggataatacatttgtgggtgtgtgttttcaaagacactaagttttggtaacttgttacagcagtaactggaaactaagacatgcaacaagccttattgttcatttttaccaccactactgggctgttggttatggtggaattacacttttctcttccattaggctgtgtgaactccttgaggttgtgcaatacgtttgtctgatttactactggttagcaggctctgagaagaatggctggtacacaggcggagctcaataaaagcccttactgaattttattcaatctatatgtggatgaagacctccgccccgcgcgcccctcccgcaagtcccactgaggcccgacccattctgtccggctcccagcccccgcgggtccccccaccccggggctgaccgggtgattcaggcagccctacatcctgctggggtggtgggcttcgagcgcgggtcccaggacgcagtggggcgcagtgcctgcggcaggcggcaggaggcgagcgtggcccaggaactcccgcgggagggtcgggacggggcggggcttgggggcggggcggctcagcgcgcaggcgcggggccaggcgcctcgcgcggccaggggcgggcggccgcagagcagcaccggccgtggctccggtagcagcaagttcgaaccccgctcccgctccgcttcggttctcgctccttcggcccttgggcctccaaacaccagtccccggcagctcgttgcgcattgcgctctccccgccaccaggatgccggtaaccgagaaggatctagctgaggacgcgccttggaagaagatccagcagaacacgttcacacgctggtgcaacgagcacctcaagtgcgtgaacaaacgcatcggcaacctgcagaccgacctgagcgacgggctgcggctcatcgcgctgctcgaggtgctcagccagaagcgcatgtaccgcaagtaccatcagcggcccacctttcgccagatgcagctcgagaatgtgtccgtggcgctcgagttcctggaccgtgagagcatcaagctcgtgtccatcggtgagttctctggccgggcccaggcgcccactgtggtgccgacccgcccccgcgcgtgcacccctgcggagggcgaggatttcccgcagcgcgcccccacctcggagataagggggagtcgtccccaggggtgggttatagggggcctagaccccctccccggtgtcttcccctgggatgggacctgttgtgatcgctccccgccatccgccccagcagtgcacctttggctggctaagggttgagggtttgggctggggtcacaggaggagaggtggagttgttgcatttctctacacctggggcgcccctatgggagctaggggactagaaaccctcgttcgctgtccccgggggcgggccctagggtcagatgctccgcggagtgctctccctgctgcgcccaggttggtgctctcagaggcagctgaatgggcgttggctcggaggccgggccgtgagacctgaggaggaaccgttctctgcgcctggggcctccctgcccaggtggagacagagacctggtaccttcccctgccgtcgctggaatgggtgtgggccccgaggttgcaagggtaggcgcgggtgtgtgtcctcgctctctctgctcccagctcagctctggccgcgcgccgcaggttgaacccactccttgctgccgaagttataatttagagatggtggtggtaacagtaattgctgtcttgtagggagcccaactagcgtccactgtgtaccgtcagccttctaagttatctccgtccctacgcatcctgccatctggggtgaggctagacccattttacagataagggggtccggagggttaattgacctgtccaaggtcagcaagtagggcccagctgagaactgaaggaagtgggcaacagttagaaggaggctttgttttcctctcctctcccaaacctacaccagggtcttcctgaaaggagggagggaattggtgtctcttgctggactgggccttctggtctggggaggaagaataaggatgaagtctcccttgtggtctgagatagttggaggcttcccagagggccacaaggctactgatagtgtgggctgtgatggtaggggctgtgatgtgtgtgtgcatgtgggcgtttgtgcagagaacgtgtgtacacacatagcatgtgtgtatagcatgtgcatatgcaaagagtttgcatgtacacggaatgtatgcagagaatgtgtatccacctacacgtgtgtatgggtgtgtgtatgtgtgtgtgtgtatgtgggtgggtgggtgtgggttggggcagaggagggttctgggtctggatctcttcctaaggagaaccagggactggccctggcctgtgatttgggtctcttcctgaggaaaccaggtcactatagtgaccctagtgacaggaagaaagggagatgggtgtggctgccaggactttctccagtggaaaagggattccctctaggctgagcctcccctgggccttagggcctcacccttcccttcccccacacctgtcctggcaggtaaggctgcttcctgcttcctgggcccagatggcagccgcaccacccagctgatctccagcagccctccccctccccaagggtggcttccctgcagaagaatctgcatggcacgctgttgtcttctttctggggtccatctcctgtactggggagggagaacctcagaatctcctggaattctttaccattcagaaaccagcctcccctctgaagaatcccaaggcccagctgggctcaatttggatctgttctttgttttaaaaatgtgtatttatttaattaactgaataaagaaacttaaagtaaaccagaagtatccaaatacgacatgaaatctctaaaacaacaacaaaaccaaaccaaaccgcagcactagcaaatcacagactgcctgatctacccactgtttacagaggcagcagctacttccagcactgtctctcatcagtgcccggggctgtgggtctcattctagattttgtctacatttttttacatggttctcctgattccctgctccccctccccaccaccgccccgcctggagatggagccttgctctgtctccaggctggagtacaatggtgccatctctgctcactgcaacctccacctcccgggttcaagcgattcttctgcctcagcctcctgagtagctagaattacaggcacatgccaccacgcccggctaatttttgtattcttagtagagatggggtttcaccatgttggccaggctggtctcgaactcttgacctcatgatatgcccgcctcggcctcccaagtgcgggggttacagccctgagccaccgcgcccagcccggtcctccttttattttcgaatccactcaggccctagctactcccattgtcccgacgttccagggttagttagcttcccttcctctgtgctgggcctgtgggctgttggcagcttcttcctgttcctaccacaacttgcattctatttttttcctttttaatgatttcttggatcatattccccagagtgacattcctgggttaaagggtgtgaccacatttatgacttgtatcattggctgcctaattgctctcccgagagatcttgcaacaaacaggttttccagcctctggagaccacagagagccctggcaagtgccaggactgctgtggggataaagcaggaggcttcttccctaagctcttgaggctgttgtgggtaatggtccttcatccttcaaggcaaagttacctccagcttggactaaggttcatatattcactgcttaggttgtgttacattgtgctgacaatgacactagcttcaatttgggggcacctactgggtgttaagtgtgttctgttgatcaccccattgaattttcatgctaatcattgattgacagcaactactgccctatctctaatgatctgcttctgcaagtcacttagagagttcagggcttaacactgtcctgggcatgtgttgcttagaaaatggcgcctgttaattaaataaggtgctgtctaataattatctcaaaagtaatgccagggctggatgccgtggctcacgcctgtaatcccagcactttaggaggccaaggtgggtggatcacctgaggtcaggagttcgagaccagcctggacaacatggtgaaaccctagctctactaaaaatacaaaaattagctgggcatggtggtgcacacctgtagtcccagctactcgggaggctgaggcaggagaattgcttgaacccgggaggtggaggttgcagtgagccgaggtctttgtgtaactgcactccagcctgggagagcgagactctgactcaaaaaaaaaaaaaaaaaaaaaagtcatgcccgaatggtttgcacaccgaagggacgttcaaaattaggggagaacagcctggttgtttgtttctgtttggttgatcatactcttgccatggttagtattattatctttatttaaagatgggaaacaggagtgaagccacttgtggaggtgacccagctagctagtaaatggtgtctgaaacccaggtctgcccagctgttgaattggagccttaactgacttgccttccagtttcagagatgagtaaaatacagcttttctctccacatcagagggtccctgcaacactaggtttgcaagtcttaggtgttagggtggtggctggatacccacactctgaacctctgaccttggacaaaatagggatgtcagggccttccatgattggcaggatgaatcctctgggctgtgatgaaggtctcacaagttgagagtcagccgggaattaagtgggatcagtttgcctcttgtgttttcctcattgtgttttggttggttggttgagatttcctactacccaatggatgatgttttattccatcgtcagggaaggtatcattgaatgaatacagggttttgtatgctttggataagaccagacagttgtggagtcattagaattgtgtacatgcctccagctctgagataggtggtgtttcaacagctgccagaggactctggcttttctgcctagaattcactgaaagacaaccctggctattgattcacatttgtggttcattgtaaggtaggcccctaggcgccatccaaaagttgaaaatttccttacgtttcttgttatgtgatgggcagttcatagtgaggactcagtgtctttaattccagctgtttgccaggagttggcagttttatttacttgtttttccaaaaacctttctgacatggggcagtccagccagctgggaggaaaaggggtctctcagcccaagaatgatgatcaaggcctagaagtttgggtggtgtgttttgttttgggcctttagagaaaggaattgtttccttttcagaggatgtggtctaaccctaaagtttacttgactgacttaaaccaggccagcgccagagcaggcagggtgcgtgttcccaagacttcgggtcactaggcagcttccagggtggtgggtcactggtccagtcagctccttttccttcctctcccttttgtgctactactaccaaaataatttccaaataaccttaagttctgctctttcttgcatgtctagcagatgccagcatgtcttttgggtagtacagagagtgcttaaaaagtagcaaagttggccggacgtggtggctcatgcctgtaatcccagcaccctgggaggccaaggtgggtggatcacctgaggtctggagtttgagaccagcctgaccaacatggagaaaccccatctctactaaaaatacaaaattagatggccgtggtggtgcatgcctgtaatcccagctacgtgggaggctgaggcaggacaatagcttgaatccaagggcagaggctgtgttgagctgagatcatgccattgcactccagcttgggcaacaggagcaaaactccatctcaaaaaaaagtagcaaagtagcatgctttgtcagaattattaataacaagttgtgggccatgtacaaggtggcacattagcattcaatgtcacttgtgtagtagttaagagcaaggattcttggttcaaatcccacttgccactaagtagctattagaaacttctgtgccttggtttccttatcactaaaatggggataataactaccttcttaaaaggctgttataaagattaaacaagttaataatttttaaagtgcttggcacagtttatggtacatagtaagtgctctgtgaatgcctgttaattaaataaggcactgtttaataatctcaaaagtcatgccggaaaggtttgcacactgaaagggcatttgaaatcagcgcgctctggggagaacagcttggttggctaaggttgatcctacttgctaaaatacggctatggactgcctagagggtgtcacctccttgaaaggggctgccccctgctatgttatggctgcctccagggcccattcacaccagctttgtttccaagctggacagggagctccaggcgtctggtcattccagcctcccacccctttcaggaatctctgggccaaatcacttccagatggtggttgggcctctgtggagttctcccagcaacggcggagccagcatgccagtcggcagccgccttcgttcttggagagtctgagctaaaggagggctttgatttggagccaaattgtgtctcttgggtcctggttttgtgctgtgaggcaggtaccatggagtgggctgctggcttagttgaggatggctgccctgctccttaggggagcagatacccagggcctggagcctttaggccctgcctccagtagctccatggtcagggtgccagtcaccttgcgttttctttttctttttttttgagatggagtcttgctctgtcgcccaggttggagtgcagtggcgtgatctcggctcactgcaacctctgtctcccggggtcaagcaattctcctgcctcagcctcctgagtagctgggattacaggcgtgcgccactatgtctggctaatttttgtatttttagtagagatggggtttcaccttgttggtcaggctggtctcgaactcccaacctcgtgatccacctgcctcggcctcccaaagtgctgggattacaggcgtgagccaccggacccagccaactttgctacatcagtttccaggtagcatatcctaggcaaaactggatgtagcctagtgattcagggcctcggtctgaagctagactgtctggattctaatccgcactctgcctgataccagctgtgcaactctagtccactgctttaacctttctgtgcctgcttccctgtctataaaatgcaagagcaaaatagttgctatcttagagttgctgggagcattatatttgatgaggttaagttatagcacagtgttgtcattatcactatgaatattgtgcttttggacccaagtccaggactttgtcttgtcttctgtctattctctggccagtccagatatttttggaatcctattgctgtcatctggtgtgttagctgttccctttctccaagttcagaacgtctgatgaagatgtctcccaagatcctttcttcctttcctcattcaacaaatatatgaaagcccatctctgaaccaggccctgtgctgggtgctaggacaacaggaatgagaggatcatgtcctttgcttgcctcagatactgctcagaggagaagagacaagcaagcagggagagccatgcagaggagagctgctcaaaccttcaggcccatgctcatcacctggggactttgttaaaaatgcaggtctgattgagtaggtgctggggtgtaggctgggattctgcgtttccagtcagcttcagatcctgctgtctgtgcaccgtgctgtaagtagcaaggatctaggtgccaagccctctgaaaaggaggagcacctgcccctaggctgggtatgggtaatctagaaggttccctggaggaagggacctttcagctaagacctaaagcgtgactagaattaggcaggcaaacagacatttacacaggagcagacgagtgtgtcagtttagaggtcttgatgctcaggtcagaggggcagtggaggggtgggcagggctggtttaccaagggctttctgaaactggaggctgcctatggggtatgctccttgagtttgtttgtttgtttttttttttgagttggagtttcaatcttgtttcctaggctggagtgcagtacagtggcatgatctcggctcactgcagcctccatctcccgggttcaagagattctcctgcctgagcctcccaagtagctggaattataggcatgtgcacacctggctaattttgtatttttagtagatatggtgtttcaccatgttggtcaggctggcctcgaactcctgacctcaggtgatccacccacctagcctcccaaagtgctgggattacaggcgtgagccacggcatccagccccttgtttagtgtagggtagtaaacccagccaaaaggggtcgtttatctcaggggtctcacctgttgctccagtcattcctattagcagaaagttttgtatgtgccccttcctcatatatatatatatttatatatgtatttatatatatttataagttataaacatactctactgtcaatttgtatattaaatattagtaaatcttagtttctttttagatgacaaatccaaatataaaatctgtttttttcctggctctaacggattatcttatgtccccttggggtggacatacctcttttggaggctcccgtgaaggtttgtgtttctacatttagtttttttcttttttccatattcttgttattctgcttttaattttcatctttgagtattctaaattaaggagctggatctgtaattgtaacaccttcccccaacaataagtttaactaatgaaaatattcaatggaatgagccattttaatctaaatggggctatttcctgcttttataatgattacagttgcttttcatgacattctactagaagccatcttacattactgttgtaaatctagttattcattaaacgggcacagtaatccctaaattggctcaggttattgtataataaacaacaatactttcttcttcaggagcttgagaagtgatcttgtatttttaaggtgcctaactaacttttcatgggaaactgagtccatgtactgggaagaaagctttttggggaaaatgattagaaaaccaaatgggtctctttatgactgaagtgatgaaccagcaggtgagagtaggtatagatggtacagaggacggaattactgggtattttaatcaggcccacttagtatcacaatttattattctattctatttttattattattttttgagatggagtttcgctcttgtcatccaggctggagtgcagtggcgctatctcagctcactgcaacctccgcctcccgggttcaagagattctcctgcctcagcctcccaagtagctgggattacaggcatgcgccatcacacctggataatttttttgcatttttagtagagatgaggtttctccatgttggtcaggctggtctcgaactcccgatctcaggtgatccgcccgctttggcctctcaaagtgctgggattgcaggtgtgagccatcgcgcctggccagtgtcaggatttattctgtgggaggggaggaggacaaagaaaaatactgagctatgtttgaagctcctgccctctaagagccttagagcagctgacttaaatgtgttcctttgataaactgtagatggttgttgtaactcttctgcaaactgtttatttttaaaaacaatttgatgagattttacttatgcccattgtttgagtacagcatttaccaaagaacaattttggccagatcccatgcagtagaatgcccttggccaaaattttcttgtactataagcaaagaagcagtttggtttttcacttaggcaagactgcctatcagactgagttattgtgacagagccgctgactctctccctttccccattatcaaaatctggcttttctaagcagcgcatgtaaaaagcttggcaaggaggacccttgtcctcctacatattattctttggctcttcttggtaccaagaatacatacaaataatgctggctgtgtactgaatgttgaggtgtgcactgttgaggatattcatcctctaatataacatctagtatttctcacaccttccgtctgctgagcattggtctatcttacttatactacttctaatcctcgtgaactctgcaaaactagtggctttacatctatgagaaaagaaaagaacttttatcggaagaaggtgagtccttttaaagtatcaggcctggaaagacattaaatgagacagcgaacacatcctgctaccctctttgagctatgtattcattgacttttttttttttttttttttttttttgaggcagagttttgctttgtcaccaggctggagtgtagtggtgcaatcttggctcactgcaacctctgcctccggggttcaagtgattctcatgccacagcctcctgagtagctgggattacaggcgcctgccaccttgcctggctagttttggtatttttatttttatttatttattttaagacagggtctcactctgtcacccaggctggagtacagtggcgcgatcttggctcactgcaacctctgcctcccgggttccagcgattctcctgcctcaacctctccagtagctgggattacaggcgccttggcaccacagccagttaattttttgtatttttagtagaaacggggtttcagcatgttggccaggctggtctcgaactcccaacctcaggtaatccgcctgctttggcctcccaaagtgctgggattacgagtgtgagccattgtgccccgcctatgtattcatttcttaaaattggttgctggctaggtgtggtggtacatgcctgtcctataatcacagcactttggaaggccggtgctggaggatctattgaggccaggagtttaagaccagcctgggtgagatcacatctctacaaaaaaaaaaaaaaaaaaaaaaattatctggatgcagtggcacaagcctacatagttgtagctgcttgggaggctgagttgggaggatagcttgagcccaggagtttgagtctgcagtgagctatgattgcgtcactgcactctagcctgggcgacagagtgagacccgtttctaaaacaaagaaattgctattgtcacaattagttataaattaatctaataatgctgcacgcagtaccataatccacaccctatagcttaacgatggatggccaaccactaatcaatgctatttctgtacgccaatgagaattcctgacaaaaaactttgtatcagccccactccctgtctgtcccctcttttgcttttaaaaacctgcttgtaacaaaggccaaacagagctcatatccaaggttacttgggcctgagtctttcaggcagctgtcttcactttggctcaagtaaactctttaatagtttaaattttaagcctctgcctctttcttttaggttgacatctgtttccattttacagatgagaaaactgaggctcagctctgcctcactttacaggtcaggcttaatccctaatccctgcctgcatcatgctgtaaaggacttttgtgtcaaaactgagtttcacactctgtaaagtaaaatagatatattgtagtgagagggtgtagaagagactgttttctgcttctgtggattttttttcttcctgttttgctttgctccaaactttactcatttgcgcttgattcatgtgaaactgaaatttccttctacagaacaaaactttttgggggctacttaccatatcttttcccacaccgtggagctctgactgggaccttttccagtttttggagacattgctccagttctttccctgcctttggtttccagggggcagtaatgtcaccgcaggtgtggacagtagggaccagctaaaggttgctttggaggaggtgggcagggcttttgtttgtgaggtctagaaaccagaggtgaggaaggaggtgtccctggaactccccctggctgcagggctcacagcacacaccatgacaccacaggggtgtgtgtgtgtgtgtgtgtgtgtgtgtgtgtgtgtgtgtgtgtgtgttgaggggagtgttgttgagagccaactatgccaggagatccttggtgacagcggacataggcacagctatgctctgtcaggaatgagttcacccacacccttttcttctgctaccttgtttaactggtgggagggtgtgctgggttgtgtttgctggtgagcccagcaactgcacccttctttccaggcctagcacccagcctttatcagtctcatggccctggcacaagtgggcagcctgcttccaatccaagcaggcagctttccgctcatctgcaggtagcctcgtgctgtggcagcacaaagttgtgtgagccagagctgaacttgtgatccccacgggcatctcctgaggcgcacctctcctgagagagaaagctggtccgtccagcccattcagggctcagcctccccagccgtcgcagggctggcttgctgaaaggtctgggtgttaacacagcactcctgttctctctctctgaaggccctttatgctggcatgaattccttttctcatagagatctgaaagctcttttgactaaatgggtcacctttctgagtattttcataaggctgtcagcctttaccatgccagacaagttttctggaatttcctttccagaaaaaaaaaaaaaaaaggctactaaagaggttggagttatttggaacacagggtggaattctggcattcgaactatagggaaacgggtggggatttgtggcaggcactatgtaaatttgccgcaagcccataaattcagactttaagatgaaagatggcaagcagcagtcagctttccttcaacaggcaggaacggtgctaccttccgcctgtgctgagtgtgactgagggagaggcaggcctcctagggaggccggggcaggaaaggtttcttggtggctaaaataggatttctcagtttcccccgtgtcccaagaaaataagttcttatcatgcttgtaccacacttcttgtgcgtatcaccctggtttccctgcacctccttgaagtggtttatcagattccagggacacaagaatggtttggcatctacagcctattgtgggagcaggggcccggcctggtgcttcttgcccaggaacaaactgattgttcccttggtgtggggtaaagcaggccagagtatgggaccaggccctgcctcccaggggacctgaggtgcaaggtctttgagctgagaccctaaaaggcctttgtgagtctgtagtgctatcagttgagcagagttcagggttctgtttacaagattccctctcagcagaggcagggaggggtacctgctggaagaccaggaatgtgctgctgctgggatgggggccctcggtggagcttctagccatctggaggcagaacccagaatgtgttctgagtgaggcgccttggcagagttggcttgaaagcacctaggcagtggcttgtcacattccttatctccaccaaaggaggcaagctagcacctgggggatggctctcccatcagggagtcctttacaggatgtgatccaggtgtcacattacacttcctgcaggtgtgcacctcttacctaattgtctctcctatccctttttctcagcactattgtctgacatccatggggagtcacacccaaagttgggcatgaggtcctctcctgggcacccaacaccttgtttttttgtttttgttttttttggagatagagtcttgctctgtcacccaggctagagtgcagtggtgccatcacagctcgctgcagcctcgacctccttggctcaagcgatcctcccacctcagcctcccacgtagtcagaattacaggcacacacaccaacactgctggctaattttgtattttttgtagattcggtttgctatgttgcccaggctggtcttgaactcctgggctcaagcgatctgcctgcctcagcctcccaaagtgtggggattacaggcatgagccacctcacttggccacactgccctcttactgagccgtattggtgttctaaatggccttcttactctcccacgggtcatcagtgctccaggggcaggcgctgtgtctcttgtttacctctgtggctctgaccttggcacttaataggaatttaataaataacttgttaaataaacagtctctagtataatagcttgagtattaagactggtacattgacttatttgcaattcagaaaatgcaaaacagtggttctttgctgcctttagtgaagtgggaattatatgtagtagacaactgggtctggggtcccagtggaacacttcgtttttggactgtgatgctgaacttaaagaactcagcagttcatgttcattctctggacatctgtgatttgcttcaacaactgttagagaacaaggccttttccaggtgaagctcagaaaatgaatttaataggaaattactgaaagtcacaatcatagtaacagtttcattagttacagtgaatatagagagagcccatacaaagtaccaggcattgtgataaacgcttcttactaatagctatacaaaacatcattgcaattctgagaagtagttattgttgtaattcccgttatgcagatgagaaaactgaggcacacccagattggccagtgagtgtgtggttattactcagattcttgtctgagattttaatcttcatattttactgctttcccaaggaaagccatcagctcagcaagtctttgaaatttgcttctttttttttttttgagacagagtcttgctgtgtctcccaggctggagtacagtggcgcaatcttggctcactgcaacctccgcctcctgggttcaagcgattctcttgcctcagcctcccgagtagctgggaatatagttgcatgccaccacacctggctattttgtatttttagtagagacggggtttcaccatgttggccagcctggtcctgaactcctgatctcgagatccacctgcctcggcctcctaaagtgctgggatcaggcttgagccaccgaactcggccttttttttttttttttttgaaatgatgtctccttttgttgcccaaactgcagtcttggctcactgcaacttctgcctcctgggttcaagtgattctcctgcctcagcctcccgagtagctgggactacaggcacgtgccaccatgcccagctaatttttgtatttttatagagacaggctaagcttgtcttgaactcctgacctcaagtgatccacctacctggccctcccaaagtgctgggattacaggagtgagcccctgtgcccagcctgaaattcaattctaataaatttttattggagcattaaaaagttacatctgtagttgttactctttgcaaaaaattgcaagaacacagaaaaatataaagaaaaaaatcacctgtgaagaattttaatgaatctttttctacttttaggggattttgcttacagctgccttttaatcagaatagggaagaaagagattcctttctcaggaaaaaagtgactgtggactggaaatgctttgtgaaataattttggtcatactgatggttataacaagattcgtcttcaattgagttattgctgagctttgtccaacattaaaatgaaaggtctcatttgagtctcattgtggtttgcaagtctcccttggtctagaaatatgtttggtcaaccacggcatggaggtgttccagccactttctgtctcttaaaagtttttaggacctacttttattgggactgccagggtctcttaataatagttattatacttggtaactattgtgaccttgtctcataggcagcccagcatagaaactcatttagcttttagttgctcagctccattagctgtttaaacatgtttcagatgtgagcctgacaatgtacttgggcagcttggttcacccttgactgcctgggaactttgagaagtctgaaaattatatgtagccctaaggtcttcatggtattgtttttttggaggcaccatttcccaatagccctgaggacaccaggcccatgaagccatcctgtctcagccaggaggcagaggagatggaatggaaaccacttctggatacagatccagccacttccggagtgcttcagagcatgggtcagatagaccttgctgctttctagctggcagacttggggaaggttgtttgacctctctgagtttgtgtcccagactatagcagtacccccttactggcgttatcgaagataaaatgatataatcctgataaatcacttgacccagtccttggaggtggtggtgggggctggggtaagtgccccatgaatggtggtcatcatgctccccaccaacctcctttctctcttctcctttcccgtctttcacacccctaattcctggacctgggggtggtctctccagactagatgaagaagcaatctaattatctaggaaggtgaaaggtggttgggaatactcccagaaataggccaaagataccgcctcctacctaacagactctttttagaagaagaggcaacctgggtttttggataactgttgagtaggaaccatcatgagtggcatttctgcatttctggtcttctggccaagcctcctttttttttttttttttttttttttttaaccttgagacagtcttgctttgttgccaggctggattgcaatggtgcagtcttggctcactgcaacctccatctcccaggttcaagcgattctcctgcctcagcctcctgagtagctggtactacaggtgccgccactatgcccagctaatttttgtatttttagtagggacggggtttcatcatattggccaggatggtctcaatctcttgacctcatactctgcccgcctcggcctcccaaagtgccagaattacaagcgtgagccactgagcccagccttccttttttttttttttttttaagtagctccattgccctccctcaccctttcttttgtctcctgtaatgtccttcccttccatttcttttttttcttttttcttttcttctttctttctttcttttttttttttttgagataggatctcattctgtggcaaaggctggagtgtagtggcacattcacggctcattgcagcctcgacctccaggactcaggtgatcctcacatctcagcctcccgagtagctgggaccacaggcacacaccaccacacccggctaatttttgcattttttgtagaggtagtgttttgccatgtttcccaggctggtcttgagctcctgggctcaagtgatactccctcctcagcctcccaaattgctgagattacaggcataagcctctgcacctggccttccctctcatttttttttctttcctggttttgcctgtcccagaccaccctcttggaaagatgctctcccagcagcggcagtaaggtcctggtcttgtgtttgctcctgggcctgagtcttggctttgctgctttgtagctagctggctgacaccagggagctgcttccctccaggagcctgtcgtccatatgctgaatgtgatccttaaatgctctgtcttacaggggccagacattgtggctcatgcacttcagggggctgaggcgtgcagatcacttgaggccaggagtttgagaccagcctggccaacatggcgaaaccctgtctctactaaaaatacaaaaattagccggaggtggtagtgtgtgcctttaattccagctacttggaaggctgaggcaggaaaatcgctagaacctgggaggcggaggttgcagtgagccgagatcatgccactgcactccagcctgatcaacagagcgagattgtctcaaacaaacaaacaaaaaatgttctgccttacagagttcttaggtataaaagagaaggtgcctctaaagctcttggcaccgtgcctggcttatagtaagtgcttggtaaacgtcagctgctgctgttgtggtgttagtatcagcattgttgctgtgagaccctgcacttcccacttagccttggaaaaataagtcttcacgttaatgccatgggctaccgcttctcttttcagggcttcttggaggagggtggagatggagagacaggtgggggactgccagggttacatcctccatgaggctgaggctgtgctgactgccttgtgtgctttcaacctggagtaaagggtggctgtgccagctgctcccatcccccaggagtctgactcgtccctgccttggccctgggcagcactttccctcctagctctttggcatctggggtcatggtggggctgcctgccatctgtcaaaatttttgctgccctgggtgtggtggtaaacccccgcactatccaacttggtgtcatggagctggcgacaatatttttacagtggttagtgcttggaaactggacttctgggttatgccctgtacaaacagcatcaaagtcgctgggctagggtgacagaggaggctgccaacagggaattctgtggctcctgggacaggaatggatatgggaggttgggggccagtattttcggttctcttgaggagttggcgagtattagtctttgccctgatggatagaaggaatctgtctgtgtcttgcatgaaccgtgtacttcccccagttactccttggacaccagctgcctgctgttcataattgggccagatttctaatactgcagcgctaccaaatgtcagttttaggccatctctggtgtagccagggaacgcccaacacctttcccaaaggtagaatttgtgtgggttttacttcactgagtgactaatgcagatctttatgttttaatgatgggaagaaattcgtcagcctgggtactttttccatgtgatggggcaaaaatttaaaacacttgcacaacggcttttgtttctccagctactaaaggtgactgtcatttaggcattatcagtatgatcagctgatgttaacccactccccttctggagacccgtttctgtttctgggaaaggtgtaggacatgctggatttggcaagattgcaggtcccaggcagatgtccggacttagactctggctcttttttttttttccagacagggtctccctctgtcacccagtctggagtgcagtggcgcgatctcggctcaccacaacctccgcctcccaggttcaagggattctcctgcctcagccccctgagtagctgggattacaggcgtgcaccactatgcccagctaattctttttttttttttgagatagaggctcactgtcacccaggttggagtgcggtggcccggtccgcctgcctcagcctcccaaagtgttaggattacaggtgtgagccaccgtgcctggcctcagctaacttttgtatttttagtatcaacgaggtttcaccatgttggccaggctggctttgaattcctggcctcaattgatctgcccacctcggcctcccaaagtgctgggattacaggcatgagccaccgcgcctggcccagaccctggctcttactcctaggtctacctctaccatcactggggccctcgcctgaaccttttgccccatctataaaatgggagaactagactaggtctgtgtcccccaagcttcaatcatttgtaaaggaaccacctttactattttgccatatcccacggctgtctctatttcatttttcacttaatattattttcccctgcagttgactcacttgtaaaacaaatgtatttgaaaaggagactttgtgtcactataataacggaaaaacagcgtcactaggtaaatggaaggtaaccataaataaaccccaaacagttattaaattccagccagcactgttgcctgttcacaacatgaggcatactctcttttggttaaaaagggaaattagcaagagatggagaggtgttgaaggtaacctagcactacattgagccttttccttgacctgctcaggaggattgagaaagaactaggagaactgggaagagaataacgtctttttgtgatgcaaagtgcctgagtgtgaccaagagctcagagtagtaatgtatagatgctttgtttggatacttatgcagccattaccatgtgccaggggtgtagaggggctaggagtatagaggggattgggacttgttcactgacttctggttgcttgtggtctagtagtggggaggtggtcatagaatattgaatacaaacgaagatcgaacaggctgcaggggtttaataggaaaatcacaggactaaattctgtcatgtgtacatggggtctacaaataagagttgtttagaattttttttaatttaaatttcccatgaaatataaatctatttcattccagaatgattctagagaagctctaaatacattaaagttgtgttggctgggtgcagtggctcatgcctgtaatcccagcactttgggaggctgaggctggagaatcacttgtggccaggagtttgagaccagcctgggcaacatgggagaccttatctctaccaaaaaaaatttttttttcttttcttttttttttttttgagacaaagtttcgctcttgttgcccaggctagagtgcaatggcatgatctcagctcactgcaacctccgcctccctggttcaagcaattctcctgcctcagcctcccaagtagctgggattacaggcatgtaccaccacacccagctaattttgtattttttttagtggaggtgggatttcaccatgtcgatcaggctggtcttgaactcctgacctcaggtgatccacccatctcagtctcacaaagtgttgggattacaggcgatagccactgcacctggccaaaaacattttaataaattagctgggtatggtggtatgtgcctgtaatcctagctacttgggaggctggggcaggaggatcccttgagcccaggaattccaagctgcagtgaactataatcaggtcactgcactgaagccggagtgacagagtgagaccttgtctcttaaaataaatttgtgtcattgtttgttgtttttatggtgttatgacaatgatccatcttaaccctttatgtagtggtaactaactttctcttttcctaaaagctgatttgagttttaggttctcttggagtctgtgacaattgtaaatagataagatataacaaaatggcctgaaatactcttgcaacactcatatttcccccctcagattagcatgttctatactctctgcaaagcaagatatacaccagaattaggcctctaaaaagcctcatactgctaatctctgggaatgaatggtgttctttgggataatgggatatgaagctcagtctgatttttctgttctgctggtagcttagggccccctttcttctgttgggttttttgggagaagggaagttgtgattaagaatgagaattctttttttttttttttgtctcaagagtcttgctctgtcgcccaggctggagtgcaatggctcgatctcggctcactgcagtcttcacctcctggtgtcaagcgattctcctgccttagcctccaagtagctgggaatacaggcacctgccaccatgcctggctaattttttgtatttttagtaaagatggggtttcaccatgttggccaggctggtctcgaactactgaccccatgatcccaacccccccgacctccccggcctcccaaagtgctgggattataggggggagccactgcgtccagccaagaatgagaatttgggagtcaggcacctctgggattgaatctggaattgactgagtgtacatgctttctctgaggcctccgtcctcactgctctcatctataaactgggaataatcatagtttctatctgaaacagtgggtgtgaagatttaacgagctaaattgtaaagtgcctgagacatgggaagaagtcaggatgtgctaatgggtaatcttacacttccccaatggaaagggccaggtttatattactctaggctggtagtaagcgaggcaaaggagatatcaggtttcagctttgttagaacatgctaatggcaccaggacactcagaagagatacagagtttgagacaaatggcaccatgagccctgagacattgtgtatggggtgaatcggatagcaagaatagacttcaaggagggaagtagggcagttagaatcctttcagctgcaaggaactgaaaactggctcacatagaaggaaaatgattggctcatgtcagcaagcctagatgcagagcaagttatgggtttcagggatccagcatctaaatgatgtcatcaagaacccaagttttttgggtctctgctctgttggtttctttcatcctaaagctggttctcctgtggtttaccatagtagagttcctgtgagaactccactctgaccaatcaggccttcccagagccagggatggatggagtcgcttcttttgaggcccatgggtcctatctggaggggatggatccagactcctatcaggaatctaggaggggccgggcacggtggctcatgcctgtaatcccagcacttcataatgccaaggtggacagatcacttgaggccaggagttccagatcagcctggccagtatggtgaaaccccatctctactaaaaatacaaaaattagctaggcgtggtagcaggcgcctgttgtcccagctactcgggtggctgaggtgggaggatcacttgagcctgggcacagaggttgcggtgaggttgtggtgagctgtggttgcgctgctgccctccagcctgggcaacagagtgagaccctgtctcaaaaacaacaacaacaaaatcttatgtaccccataaatatatacacctactgtgtatccacaaaagttaaaaattagaaaaggcaaattgcagagatttccatatgctatgataccgtttatatgaagttttacatatgtcataaaaatacagataacctttaggggaatgatcattaccaaacttttggataacggtttctggggatgggcagagagggctatacagtcatgaagaggtgtataggggctttcaactctttgtagtgttttatttcttcagtcccatggtggttatatgattcttcactcccctttttttgtgtggaatatttttcttataaaaagtgtgtcttttatttatttatttatctttttcacatggagtctcactctgtcgcccaggctggagtgcagtgttgcgatctcggctcactgcaagctccgcctcccgggttcgcgccattctcctgcctcagcctcccgagtagctgggactacaggcgcccgccaccacgcctggctaattttttgtatttttagcagagacggggtttcactgtgttagccaggatggtctcaatctgctgaccttgtgatctgcctgcctcggcctcccaaagtgctaggggattacagacgtgagccaccgtgccctgcctttttttttttttttttttttttttaaaggcagagtcttgccctgttggccaggctgcagtgcagtggcctgataatggctcactgcagcttccacctcccaggctcaagcaatcctcccacctcagcctcctgagtagctgggactacaggtatgtgccaccaagcctggctaatttttccatttttaaaggttttgccatgttgcccaggctggtctcgaacccctgggttcaagccatcctcccaccttggcctcccaaattgctgggactatagacgtgaaccactgcacccccatccaaaagtgtcattttaatgctgacatactgcattactaagcttgaccaggggaagagaaaaaaaaataccttgtgtttattattttgtttgtttgtttgtttgagacagggtcttgctctttctcccaggctagagtgcagtggcatgaacatggctcactgcagcctccacttcccagggtcaagccatcctcccacttcagcctcccaagtagctgggattacaggtgtgtgccaccacacctgactaatttttctttttttctttttttgtatttttggtagagacagggttgcccaggctggtcttgaactcctgagctcaagcaatcctctcttcagcctcccaaagtgctgggattacaagtatgagccactgtgcccggcctgtttgtttgttttaaagacaagtttgggcccagtttataagaaaagaaaacagaccatccttagggtgtcaggatgatattttgacaaaggcattcatgcttagcaggatttctctccccctacccccaccccaagtgttgaaacggctgagctaattaccttagaatgtaaggcttcctctgttgcttgtgaacgtggcagacttgggattctcagagacagagggcttcagaagcttgcctctgggagcgtccagtcaatagctttttgtctgagcagaaggagatattgctcaaggtaccatctcaagggactgctgaatcagttgcattgtctctaaaagtaggtaaaagtctagagtagggctggttcaacagtggaatgagtgttaagagagagttgcattctaagaacacctttacactgtggccaaattcaagcaggtccattttgtggtttggtggtccccatctagtgggatgtggtctggtatcccaggcacctgcatatatgagctcagatgggtttaatttttgaaaaactgctttattggctgggtgtggtagctcatgcctgtaatcccaacattttgggaggccaaggcaggaggatctcttgagcctgggaattcaggaccagcctgggcaacattgagagatccccatctctactcccttccccgccaaaaaaaagctaggtgtagtgacatgcacctgtggtcccagctactcaggaggctgaggtgggaggattgcttgagcccgggaagtcaagactgcagtgagctgagattgcatgactgcactccagcctgggcaaaagagtgagacattgtctcaatctccccacccctgccaagaaaacccaaaaaatattgaggtataattgttatacaatgaagaacacattttgattagcttatacacacactcctgtgtacacatgtacactcacacatcaggaaaccatcaccataatcaagacagcgaacctccctatccagccccagaagtttccttgtgcctctttgtaattcttgccttttatctctccatgtcttccacacccatgctcaagcattcactgatctgctttctgtcattatcagtcagttttcatcttttagccttttatataaatggaatcatatagtatgctgttttgtttttttttgagacaagagtctcactctgttacccaggctggagtgcagtggtgcgacctcggctcactacaacctccatctccccagatttaagtgattctcctgccctagcttcccgagtagcagggattacaggcacatgctatcatgcctagctaatttttgtatttttagtaaagatggggattcaccatgttggccaggctggtcccgaactcctgacctcaggtgatcacccgccttggcctcccaaagtgctaggatcacaggcatgagccactacgccctgccagtatgtactctttttgtctggcttcttctagcatagttattctgaaattcatccttgttgcatgtgtcaatagtcctattcctttttattgctgagtagtagtccattgtatggatatactacattttgtttatacatccttctgttgataacatttgggtggtttcttatttatttatttatttttgagacggagtctcactctgttgaacaggctggagtgcagtggtgtgatcttggctcactgcaacctccacctcccgggttcaagcaattctcctgcctcagccttctgagtagctgggattacaggcatttgccaccacacctggctaatttttgtatttttagtagagacggggtttcaccatgttggtcatgctggtctcgaactcctgaccttaggcgatccgctcacctctgcctcccaaagtgcagggattataggtgtgagccaccacgcctggccgggtggtttctaaataaagctatcatgaacatcttttactactctttgtatggatgtatatttctatttttctgagtggaatgttaggatcatacatcataggtgtacgtttaactgttcaagaaactgccaaactgtttcccaaagtggttgtattgttttacatttccacgagcagtgtttgagagctccagttcttgcacatcctagccacaaaaaggttctgttttttaaagacaatttttttttttttttgagagtttcgccctagtcgcccaggctggagtgcagtggtaagcgaatccctgctacaggccagagactgttctcagttggtttttacaccaagtatcgcacttcattctaacactccaccattttacaaatgaggaaaccgaggcactgagaggtttagtaacttgtggcacagccaggaagcagtagagaaagactttgaatataaatgtatccattaggatgtatatggttccaagtcatgggaaacctacctaatcctggtttatccaaaaagggagctcattggctctcgtaactgaaaagtcaaggggtaggcaggcagttggacctggaagtctccagggcatcagagagccttggctctgcttctctgattctgttgtctctccacagacgggtgggtgtagcagtcccaggcccgcagccacaccccacacctcccagaggaagaaggcgggccctgatcccagcagtcccaggaaagccctgaggttcactgtgattggaccagcctatgtcacctgctcacatctcagcccaccactggcaagggtgtttgactcttgggaatgactcttgggactggcttgtcctagatcacatgttctacctgaaattggggacattgcagaggattggtggagtggacctcaaggaggtgtttcacgtggcttcctgtgtcactaggttgccatttattctttagaaagcccctttgtttgatgaaaccctggtgtcacaggctgtgtgacttagggtaatccccttgtccacatctgtgaagtgagattacctcttcacctcacaggcagatcaaacaggaaaacaaaaacaaaaccaaacccaaaatacacgtaaattgcagagtgcttgaggtttcttttaagctgtctatgtaattaaaagctgttacttagacttggatatgaaataaaatctgacttcaaatttaagtggtgtaatttccatgcctcttaaaatatcaggtaacttcatttgtgagcctcagtctgtagacttgagggatttccatctgaagagggggcagaatggtggtttagggaacgcaacatgtaccccacccccaacttttttaagaggaagagttgaaagaaataatgaatgtgtgagaaataaggggtttgattgccttccagggtccatgttgaaggagaggaaaatgtagctcaaccacagtgactctccccaattaaaaactaaaaaaagatccgtggttatagggcttggacttcggacaagccagcagcctcagtcattgtgagtgtgattccagattggaaggttctgctaggaggaaagtggaagttttgagaattcctagttggacagaatgcctcttgatcacggccttagctaaaggagaccactctttgctggatggatcagtcagctacgtgtgaagtttggctcagtacaacattctcggcctggggcggcagcatgggaaagatttttattggaattaactttctacagagatgtactttcaaatgagaccatccttctctcactggtgagctcacccgggctcttattccacaaagcttaattgttttggacccatacatttaaactccttaattaattgactcaagacttaggacagatttgcttttctttataatgactccatggctgtaaatgctgctgattcagatgaaagaggaccctagagcacagaatgagaaggacgtggactcaggatacctgtttctttattctgactgtgctcttcgtcagctctggggctttggaccccagttttgtaaccacctaacgagttcaccttgcctgctgcctagacggagctgatttatcaagacagaggaattgcaatggagaaagagtaagtcacccagagccagctgtgtgggaggctagaattttattgttactgaaatcagtctcccgagcatttgggatcagagtttttaaagataattcggcaggtaggggctcaggaagtggggagtgctgattggtcaagttggagatggagtcacagggggtcgaagtgacgttttcttgctgtcttctgttcctgggtgggatggcagaactggttgagccagattaccgctctgggaggtgtcagctgatccatggagtgcagggtctgcaaactatctcaagcactgatgttaagttttacagtagtgatgttatctccagaagcaatttgtggaggttcagactcttgcagtttctgacccctaaaccttaatttctaatcttgtagctaatttgttagtcctacaaaggcagactgctcccaaggcaagaagagggtctttttgggaaagggctattagcagttttttttcagagtgaaaccataaactaaattcattcccaaggttagtttggcctatgcccaggaatgaacaaggacagcctaaaggttagaagcaagatggagtcggttaggtctgacctctttcactgtctataatttttgcaaaggcagtttcagtttctcacctgtaaacgttgaagactgagccagaatcagggtcatcaaatagcaccccggctatactttcttctcttcatgacaaacattgctggtcagttgatatgatgttctttcccactgggcccagacttgacattagagtcttttttttttttttttttttttttttgagacagtctcgctctatcaccctggctggagtgcagtggcaccatctcagctcactgcaacctccgtctccagagttcaagcaattctcctgcctcagcctctcaggtagctgggattacaggagtgcaccaccacacccagcagatttttgtatttttagtagagacggggtttcgccatgttggccaggcttgtctggaactcctgacctcaggccatccgctcgctttggcctcccaaagtgctaggattataggcgtaagccaccacgcctggccgacatcagagtcattttagcctgcaatgcaagttgtcctcagtgggctgctagcattggcttcaaccttcatatcagccagctaaagccccttgtaatgaatggggaggttccttcacccttgcctcccgctgcctcctcttgaccactcattttttttcttgtagttcaggaaccaattcagatgatttccctcgtgaagtcctctcgaaagcccccaggtagaattattcattttttcccttgcattcccacagcactgtgcacacaaattagaatccttgtaaaatggccatgattctgtttatgaccctggccctccaccagaccagcctctctgccctctggcttttttagatcactggcatggtttctgcctactccaggtgccagtattattttgtgaatgttttttttcttcatatctactcatctttatactactttactcgtaaaaggaaactagagaacatgatcttaaatgaaaaccacgatcacttgccagaaagaacaggtaactaggctttgaaaaaataagttagaggagatagcataagaaaaaattaaaaaataaataaaatcaatgaaaacaacgtgttactaaattcttgaaaagttttttgaagactttgagcctgaggcctgttcttattgtttgtttgtttgtttgtttgtttgtttttatgacagagtttcgctcttgttgcccaggctagagtgcaatggcatgatctcggctcattgcagcatttgcctcctgtgttcaagcgattctcctgcctcagcctcccgagtagctgggattacaggtgcccgccaccatgcccagctaatttttgtattttagtagagatgggtttttgccatgttggccaggctggtctcgaactcctgacctcaggtgatccacctgccttggcctcccaaagtgtggggattacaggcgtgagccaccatgctcggcctgttcttattgttaaaaagagagatttgtgtgaaagctgctgacgtctttttggcaccaagtcaagactgagttagttcttgtcagaatctgattgtttgtgaattgatggcttttttttttttcctgagttgggggtctcgctctgttgcccaggctggagtacgaccactataacctcaaattgctgggctcaagcaatccttccgcctcagctgcccaagtagctgggactactaggcatgctccaccatgcccagttaattaatttttttttttttttgagagacagggtctcactatgttccccaggctggtctcaaattcctggcctcaagtgatctcctgcctcagcctcccaaagctctgggattacaggagcgagccactgtgcctggccggattttaaagttctgcccatgcacctccttagctctggcagttactacttgcaggcatctcctttgtctgccctgccccttgttaggaaaggctgtgctgactgtcagctggcacccagtgcatagaagagatagttctctgtagatgatgttgaacaatgtggtactataatcccaacctgttgtatctttgtttactctcaaaagcaacaattgggctgggcatggtggctcatgcctgtaatcgcagcactttgggaggctaaggtgggagggttgcttgaagttagttcctttttttttttttttttaaaaaaaagacaagatctcgctctgtcaccccggctggaatgcagtggcatgatcatagctcactgcagccttgaccacgtgggctcaaggaatgaaccattgtgccaggagttcaacaccagcctggataacatagcgagaccctgtctctacaggaaaaaaaaaaaaaaagaagaattgcataagtatcatcagaactgttgaatggaaaatcagactttgtgggtttggtttgttaattacttctcgttggattagaatttgataggtaaaaaaaaaaaaaaaggtgtagaaaagtgattccagtcttgagcaaatttttaatggaaaacggtgtcttggttctctgttcactacaacttgtatctaagggaaagcctagtgatgcagacatttcatttcgtgatgggaaaactgatgcccagaggttcacagctgaccaggggctagtctgactggggggatctaggtcaccaccccccttgccttgttttcccagctagtgcatttcctactagacttgactctactgtaattcaagttgctgagtagcaaacaagaactacaatgactagaaggaacagaactagcttttttgtgctctgaaagtggaaacttattgagggttcttttcctcccagagaatgcagaagtgccctgatttgcttttggaaggacaccattcactttattgcctcttttcattgttgcccagaatatcaccatgatttattcatgggtggtggggagggtagcactagtgtatgctcccagcaaagaggaacatctcacgttgtgaagagatgcgcaaaactaagccagggcagggtgtggtggctcatgcctgtaatcccagcactttgggaagctgaggtgggcagatcacctgaggtcaagagttgaagaccaccctggccaacatggtgaaactctgtctgtactaaaaatacaaaaattagctgggtctgattgcaggtgcctctaattgcagctacttgggaggctgaggcaggagaatttcttgaacctgggaggcagaggttgcagtgagctgagactgtgccgttgtactctagcctgggcaacaagagccatctcaaaaaaagaagcaagccagatctttggggtgctgtgacggcaaatcccccagcgctggcctctcaggttctcttgcgggattagtgtttgttgaataataagcaatacaccctgacccagcgagccaaagcaaacaggacagtaactgaaactgcaggggagtgtgagtaaacagttaccttctaccctcatggagctggcctctggccagcaacatgatagctgtttgcatcttactcttatggagccattggccctctcattaaggtgggggcagcttctggtccatgcctgcaagtcctcatgggagtgggtacctgacagggtgtaaagggtaggtctgaggacatggtttcttttttttattgttgttgagatggaatcctgctcttgtcacacagtctggagtgcagtggcctgatctcggctcactgcaacctccgtctcactggttcaagcgattctcctgcctaagcctcctgagtagctgggactataggcgcatcctgccatgcctggctaagttttgtatttttagtagagacggggtttcaccacgttggccaggctggtctcgaactcctgacctcaggtgatccacccacctcagcctcccaaagtgctgggattacaggcgtgagccaccgtccccagccaacatggtttctttaaaatatactccccgctccatcccattcatgtgtgggagttgagctgcatctgggtttttcttttctctttttctgtaaatctttattgtattttttttggatcatagaatggatacatgtttcttaaagtttgatcattatagaaacttaattagactattatttgagtgctaaccatagtgagtgagtgcttactgtgtgctaggtggctttttatgcctcatgtcacttacatgaggtctgaggaacggtgttaatcccgttttgcagctgaggaaactgaggctacatttacggtcacctagctggcaagcaagtggctgagcctggagcagcagcagatctggggaactccacaaaccagatttctgtgtggtatccctgtggacacaaggatttaacttgattctttttgctttcagtatcactttatgatattacaatgagcttgcagtatttattttcagaagaaaagccagattattcccatttatgagagaagcagccaggtgggcagggatttccagcgctgaaccagccagtgtgtgcattgtctcttcccgctgagcggccctggtgtgctgggttagtctgtgagccacaggaaatgttgtcagggcctctgggcttttggatgtcagcaggccttcagtggtgaggaggttgtggctggactcagaggactccttgcttttgctgaacgaccctccccaccaaccaccaccaccaccaccagtgggactagcccatgagctgtaagccaaccttttccttcctaacttaattttccaaagaatagtaacttacccaccaccactgcagtcactgggccgggaagacaagcactcttgccttgaatccatgccttgagccagtagccttgacccagggtaaagcagttatgtgcttgggtcacctgggtcatgtttttgaaattgcctcaagcctaccttacaaatccttcctggaaccctgcttggcttttctttgtgggcttcccttaggagggaagcttcccgagcagcttgtcttgactgtagccagctgggtggtcccagccacagaatttaactgtcaaacagcaccagaagggttcctcatccagctgtcttgccccaagtgccctctttgctttctttttagagagttctgagactcattagagagtttagagattttagcattcttgaagttctttctgtggtcagtttggtgaaccacttcatttctaaagtttctcagttgaccccattcttccccagctttgcattctccatgaagccacctgtgtttggtgtgtatgggttttctgcaacctaggttgaacaagtcctctagaatcctgaacaattggtgattcatgctggcctggtttttctaattggcctggaaatgtggctgtagtggacacaagtggacttggcctcctctttgatgcgggtaaactttagatttgcattagctctgtttgattagaggatcttactggtttttgttgttatttatttaccttttaggagctttagtctctgtaggtttttttttttttttttttaaagtccgggtcttactctgtcacccaggctagggtgcagtggcatgatcacagctcactgcagcccccaccttcctgggctcaggtgatcctgccaccttagtttcctgagtagctgggactacaggcatgtgccaccatgcccagcaaatttatttctactttttgaaaacagggtctcactttgtcacccaggccagaatgcagtagcacgatcatggctcactgcagtctcaacctcccaggcttaagggattctcccacctcagcctcccaagtagctgggaggctacttggcatgcatcacaaggcccagctaatttgtgttttttcttgtagaggcggggttttgccatgttgcccaggctggtctcgaactcctggggtcaagttatactctctcctttgcctccagccatgagccgttcgttgcgcctgggctagtcattatagatttatcccttctttcatctcatgctacaaaagcagttcttgtatttttacccgacttgtgattttctactgggaatgtttgtttgtgatggttagcagggtgctgagagggaattaatcccaggaggcccaatattgggccatgtcgtgctgttgagcacagtcatttgacacctataacttctcatcaattcttctgatagactgaggaggaattgggaaatttcctagagttttgtctgcattattgggttgttttgagaacataaaccttaaactctagctatgtaaactggataagtcattttggtaatttggcattcctttttttttttttttttttttttgagacagagtttcactctgttgcccgggggaatgatctctgctcactgcaacctctgcctcccaggttcaagcaattcttctgcctcagcctcccaagtagttgggactacaggcacactccaccgtgtccggctaatttttgtatttttaatagagacaggatttcatcatgttgaccaggctggtaatttggcattcttttgagtacaagtgagagaaactcacttgagctggcttaagtgaaaaaattctttgtcaggagagttttgtgaatttctgtttagtggcaagttgtagaaaccacttgaaactgcttaaaggcaaaagagggagccacttgtcccagtaactgagacatcccagagccgactgcccccaagcattacttggtcccaagtttcaaacgggtcttcagggtttgatctctctcctcatctccagtctgcttcattcattttggctctatgtggtggcagaagggcttctggcatctctggacctttatgcctcccaggtccaaacccagccagaaaggagagtgagagtgctgagtgcaaaactctcctatagctcctatacaagtccaggatttgctattagactccttgaattatgtgcccagctctgagccaatggctgtgcttaggaggctcctgtctcatgcacccaccccagtactgggcatcagaaacaaccagtgatccctataatgaaccacgggttcacagacttaagtgtaatcctgcagcagggcctcaggaagacttgaaacccaaaatcagaaagccatggtttcttgtcttcctggtgtctgttttgtcccttccctctgtagaggagtcctgctatcactgcaggcaacggggctgccctgcagctcctgctgtttacatttcactcggtgtagccataggcagagacctcagggagaacctgattcggcttggattgagtcaggttccaccccagtccagtcagttgtggactgagaggtgatgaggctgggccctttaagacaaatctgggtgggtggagtctgtgcttaatgaagttgtgatgttagctgatggcccagaagggactggtaggtgcctctcattgtctggttgggaagcattctcttaagtccaagatgatgataaatagtattaggccaggtgccgtgtcatgcctctatacccagcactttgagaggccaaggtgggaggatcgcttgagcccagaagttcaaagccagagtgggcaacataaagagaccctgtctctacaaaaaacaaacaaacaaacaaaccaaaaaaaccccacaacaattagccaggcatgatggcgcacaccagtagtcccagctactcaggaggctgaggtgggaggattgcttgagcctggcgggtcgaggttgcagcaagctgtgatcacacctctgcgctccagcctgggtgacagagtgagaccctgtctcaaaaagtaaaaaattcaaataaataaacaaataatatcaagggcctctctcccaagctaggaagatatcagctgaagctctagcccagctacgtggatggctgcttcctgcctggaagcgatgcccagatcagcaccttgggacccccctgaacttgcctctgctccagtgtgggcccttccttcctgcagaggagacagcactgtctgagaggcatgaatgagaatttcctccttctaggcccaagtcagcatgactcgaggatggctttgactggaaaaactgaatcaaagagtgtgctacagccaaggatttccccaaacactaatcagtgctgattacttccagggtattgcctttggctctgtggagttttgtccactgtggctgcaatgtctggcttctgctgcccagaagatgagaaatgagtttgtagggatgagcctgggtgaagggatgtgccccctcaccatcctgacctctattaggtgtaaaagaccctgattgccaaattcataggtcatgggttggctctgcctccagcattaacacttgggggtggagttggggaatcatagtattacttgcataaatggaatcctaaaagtttgttgggacagtttcataaaaatcctcaccatgatcagtttgaaaatgacgttcccttcacatgtttgtcttctgaactgagttgcaatgctgagtatgagtttgagagtcccaagaccatctaaagcaagcctgtccaacccacagactgcaggctgtaggcagcccaggacagctctgaatgcgccccaacacaaattcgtaaactttcttaaaacattatgagatcctttcgcatttgttttttaaagctcatcagctatcattagtgttagtgtatcttatgtggccaagacaattcttcttcttccagtgtggcccagggaagccaagagattggacacccccgatttaaaggaagtaactcaattttgtgaacctgaaacttgatcttggatgaaccaaatgaaattttatgattctcttaagctcacgaaagttcaataactgtgctgtgtaaaatagaggtaaaagacttgagttggaccaggaatggttgctcatgcctgtaatcccagcactctgggaggctgaggcgggtgcatcacttgaagtcaggagttcaagaccagcccggccaacatggtgaaaccctgtttctactaaaaatataaaaattagccgggcgtggtagtgtacgcctgtagtcttagcttcttgggaggctgaggcaggataatcccttgaacccaggaggtggaggttgcagtgagcaagatcataccactgcactacagcctgggctacagagcgagactccgtctccaaaaaaaaaaaaaaaaaaaaaaaaagacttgagttggttctaatagaataccttggagaacctcaagatgccttctggtccagccaggtttacagattggaagatattctgttaatcagaatctcagagagggacaggccctgatcaaggtaacacagtgagttgtggtagctgggctgggctagaacctgggcctccttggttccaggtcacagggaccaagggatttggcttgtcttagtcctacttgtaactacaatactgccttctgctaggaagaataagagcttgcaggctagaggaatttataggaattttctttctttaaaaaaatccccccaaaaccagctttactgagatataactcacacaccataaaattcacccttttaaagtatgcaatttttagtatattcacagaattatgcaactatcatcactataattttagaattgtttttttttttttggagacggagtcttactcttgcccaggctggagtgcagtggtgcagtcttggctcactgcaacctccatctcccaggttcaagcgattctccttcctcagccttccgagtagctgggattataggtgcatgccaccacacccaactaatttttgtatttttagtagacatggggtttcaccattttggtcaggctggtctcaaactccgcctgccttggcctcccaaagtgttgggattacaggtgtgagccactgtgcctggccaattttagaatatttttattgcctcagaagaacccctgtatccattagcagtcactctccctttcccttccccaaccaggcccaataaaccactaatctactctgtctctatggatctgtccattcagaacatttcatatggtaaaatcatacacgtgttctggtgttactgacttctttcacttagcagaatgttttcaaggttcagccatgttatgtctgtactttattcttttttacggccaagtgttggaatgtgtaggatttgaattttcaaataaagctttaaagttttcagatttatttttactttgcctggtgtgttttttcctggaaagccaacttctacatttggagattaaaagacaaactttctcaaactccctgtacctaagtggttgctgcttttcttaaatgttttgacaccaaagagaaaaattggtttctggaagaaagtgtgttttcttttattgccaagaaaattagtgcatgttaattaatatagatgctcaggacccagagttgtaatgaacttttttcttatatttattttctagatgtttgacttattttaacagttttcattttagcaataatgtttccttcccactcccaaatttattggaaaccctcaatcaaccctatttatttatttattttagagatgggatctcactatgttgtccaggctggtctggaaaccctcactcttatagatagtatgaaagaagattatagccaactcttatataaccttccccagagcctccaattgttaatgttttgccatatttgcttgctctatcacttgctctaaagatgcatatcacacactttttttttttttaatttatttttgagacagagtctggctctgtcgcccaggctgtagtgcagtggcatgatcttggcttactgcatcctctgcctcctgggttcaagcgattctcctgccttagtctcctgagtagctgggattacaggcacgggccaccatgcccagctaatttttgtatttttagtagagatggggttggccaagctggtcgtgaactattgacctcaagtgatcctcctgcctcagcctcccaaagtgctaggattacaggagtgagccaccatgcctggccacatgcgtgttttttattgaatcatttgaaagtactcagctcgtatcatgacccttcacccccacatactccaacaagcatctctaagaaaaaggacattctcctaaccacagtgtctctgcattcccaggacattcttctaaccacagcgtcactgcatacccaagaggttagcaccgatacagtaataacatcttgtgtaaaacttcccaaaatgctcccaagtgtcctttatgacagtttaaaaaaaaatggcattttttgggatccaggaaccaattaacgattactcaattgaatttggtttcaaagtcacatacctcaacttttcctttaatcaagaacagcccccctgccttttacacatttttttgtctttcgtgaccgtgtcatttttgaagaaatcaggcccgttgtcttgtagaactggtgtttctcaagtgtgcttgggagggtcttggtaaaatgcacattctgattctggagaacagggtggagcctgggaatctgcatttccagccagcatcccggtgatgccagtgcagctggtcttcggctgtagaatgttccacattctaggtctgtctgtttccttgtgattaaattcaagttgaatatttttggctagggcacttcctgaggtcataggtacttcccactgcctcacagcacaggctcacaatctcagtttgtcctgttacttcgtggtgctaagtgtggtcacctgcttcaagtggtgtccgcctgctctctgttgaaacaatacctttctcctagtataatgattaggtaacctgtgattgtaattggtaagtaatctttgagactacatgaatatcctgttccccagcagttttcactcattggtgaactgttttgggaaaaataatagcatcttacagttataataccctgctggtaacacatggctcttacataatcagcagttaattgtttgtatgtgtgttaatttttatttttaaaatgtaactagtgactggtaactctcatttgtattttaaacattggcttttacagcttctcagtacatttcactctgtgtatgtttttggtagagcatttgttgtcctgtataatggtttaggaaatcctataggccaaatgaagggctggagactcacctgtgttcccaccactgtgtttcactgtgtattgccagagaaaatacagttaaatttgaatttcagatagacaatgaataactttttagtataagtatgttccaagtgtggcagacagctctcacaagttacaagtcgttgcgtaggacatacctatgctaaacgatttgatgtttatctaaattaatatgtaactgatatcttgtatttttatttgtacgatcttccaagcccacgtcccaccgccttctcggggatggccaccatttgtgtttgctgcctggtggtgtttgcagctgcgagaagggccttggaggaggagcaaagtgtagtggtatctccgtgctgtggccttgggcactggggtgggggttagatgagtaattagctgaatatgacctcacccatgaagaatgtgcccttgctaggtattagcagaggtttaggctccagggagccattgtcagaagcttgtcagtgatgtcatcagctggaagggccagctttcaggcctcaggaaaaagcttgaaagtcagggctccagttttggtaataaatgggaatggagtttcacaggtagggtgtggaggaatttattgtgacaggaagcctgatggagcctcttgcctgtgtgcagcccccagccaggtttctgagttctgatgaactaccagaaacttccaccacggcctgtgattacactgttggcccaatgccctggaaaaattggcttgctctcggggaacactccaggagctgcaaagggggtgtcaggactgttgtgcagctccccttaaattggggaggaggggtggctgatgtggaaactgttcattagactgctcagggtagtgtgagaaaacgtgtaatctgtgggcatctacccctagctgcccctctgatctcacccactactgtgggaggaccccgtggatgggggcagaggagggtcttctggatttagacactcacaaaacttccttttaccttgttcattggaagaaatagaaaatgcctttttttttttttttttctttttttttgagacagagtctcgctctgttgacaggctggagtgcagtggcatgatcttggctcaccgcaacctctgcctcccgggttctaacaattctcctgcctcagcctctggagtagctgggactacagccacgtgccaccacacccagctaatttttgtatttttagtacagacggggtttcaccatgttggccaggacggtcttgagctcttgacctcgttatccacccgcctcggcctcccaaagtgctgggattacaggcgtgagccaccatgcctggtctctttttcatttttaaagggtaatttgctgtgcaggagtgggctctcagaccagaagtggggacctgaatgaaatcaaggactgagtatggtaactacagccatttaattttatttgaagtctcccgtaaaatgttctggaaaaaacaggggttccagggctgggtgggcagtttcaatcatggactggattttgtggttcagatttctctgggcctgttggaggttccccttaagcaattacccaaggcagttctgcccagctgaagtactgattacctgcacactataccagtgaggactcatgggtgagcagatgggaggcactgagcttgattctgaaaccctggcctccatcccacctgacattcaatgtcagattagaatttggaagaccctaagtctccagattggtgcactgggtagctcctgaaatggggtggctgagacaggtcctctgtgcccccttccacagcttcctctggggcccttctgctcactggcatgtgcttctgggcaaataggcctctcccagcatttgttttggctctgtgaaatggggtaatatttgttcctattgcgggtgaagcgctgctgttgggatgctcaggtaactcactccgtgggtagctgatattgcctgggcaagtggcattttagaggaaatctgtgccatcaaaagagttggacctgatcacacttttgcttttgaatatgctttgtcccagcctggccattcgtcacttgggaccccctgagtctctctgaccccactgtaaaatggatatgccatggagttgtcccaggaatcaagggcaggtcctctccagtgagtgatgggcttgcctctcacttctctaacacccttctgcttccttgtgtaagatttcactattagtggctattctcttttacagaagaaaaagggagacgcatgcctcttccagttcactgttcaccattgcagcatatttattccaagggactggccgaatcatccctttctttgttagaatgtggttttgttgccttgagacaagtggcccgcatgtctgcactgaaggaggctttgcgcaatagccttgggcacctccggttctgcaagcatgtacagtacttgctctcctttccctttctttgtatactttttctggtctgctacgtgtccatctgcatgtggataaagggtcgtcgtcttgagtagtgattttgctgtgatgtgattcctgtgaggtctagttgcacacagtgattccgaaggtagacccagctggaaagcttttaaattgctgatactccagccccactccccaagagatgctgattttgttttgttttggggagggcagtttttttgggttttttttttaagctttttgatgtgtagccagggttgagactgaagtgatttttgtgagtaacggagaagtgttaaggcttgagaagttggaagagccatgcttgagataggaccaaggtcatatccccggcattagcacagagcaaccctgacctgttggagagttgggctggatggatgcggtcaggggagagactcgctttattttatttatttagagatacagtttcactcttgtcacccaggctggagtgtaatggcacgatctcggctcactgcaacctctgcctcctgggttcaagtgattctcgtgcctcagcctcctgagtggctgggactccaggcacgcgccgccacaccctgctagtttttgtgtttttactagagacagggtttcaccattgttggccaggctggtcttgaactcctgacctcaggtgatccgcccacctcggcctaccaaagtgctgggattatgggtgtgagccactgtgcccagcctcgactcgctttattatatccacacttggaatacaattcggattgattgtagtggggcattttataattaggaaaaattaatcaggaaaaatcactccatgtagattagtaccaccatatgaggggacaagaatttcttcagattaggaacttcttccaacaggactgacagggtccaaaactactcttggatccagctttaagatggacccagcccactgttgagtcccctctgaggtcttctctctgtggatggatttgattgttaacaatggctgagtcatgtggcacccagcccggtgagtaagacagctgagtaagaggggaaacagggcctttggtcagaaaaaccagactgacttcagtcttatctgtttagagaagccccagaagctgcaaaaattgcagcttccagactttagtgtgccgtggtcatgacatcggtgtggatggcaggttgtcatctgagcagtcagggtggcagcacacagcttgcgggctggctgatggccgaggtgtgtgaactgacctgccccaagtgacttcagtgctgggcacagcataggagcagtactaatgatatggacagtatgctcagaggacgttagggagcacagctttgtgtaaagggcatgccctgccctgtccggatttaaagcagctatagcactgaaaccccatggtcaccctcgcatttctacacttctgcctgtgccaagtctagtttgtgtgcctcctccattttgtgtgtacatgggggtatttttttctgctaggcaactgctatttatgcctctcagtactgtacttagtgtgtaccattcctgcaaggtatagacattgtcagcccattttacagatgaggaaaatggagtttttgagagggtgagatcattcagtggcagaatggaatgttaacccaggtagtctaacctctctgctgtagatctgatgtccatttgaactttagacttcccatctgtgtctacagtctagcccttaaaaaatgtgataaacaggtttttaggtaagtctgttaatttcagaaagacattattattattttttagaaagttagagcttatgttagggctcagtctatcctcctgcctcagctgcctgaatagctgggactgcaggcacatgccaccatgcctggttaatttctgtggtatacatcattgattactgagaagtcacagtccgttgttaaataactgagctattcatagccaaatcatttttaaaaacacaaatataagcaaaaacaaaacatttatttatttatttattgagacggagtctcgctgtcacccgggctggagtgcagtggcgctatctcagctcactgcaacctctgcctcctgggttcaagtgattcttctgcttcagcctccccagtagctgggactacagacacccactaccatgcccggctaattttttttttatttttagtagagacagggtttcactgtgttagtcaggatggtctttatctcctgaccttgtgatctgcccgcctcggcctcccaaagtgctgggattacagacgtgagccactgtacctggcccaaacatgtggtttttttaaatgaaagtgtgttcattttacaaacagtgcattcttactaattttacaggccctgtgctagggacatggcctcgtcttccgctatcttagagtgaagaagtaaagacagagaaagtgttcacaagttgctgcacaagtctcattgcagtgcctcccagaggcgcgaagagcaacacctttcacctgggctgtcctagaaggcccgtggcagggtggggttggtgaacactggggcttaagggggtgaattcagaagacaaaggaccttctgggcaaagaagggcccagtagtgggaagtgcaggagtgtgagagtgcctggaattgcccactcactggctctggagcttggtgctgagtgcttgggaagtgttgggaggatcagttatattgctggctgggttctaaagaacctccaaagtttacataaaagttacctttgatttgactgttctaccctccagtcacgtggctaaattaattaaatcaaatttaaaattaagctcagccataccaagtatatccagtgttcaataggtacatgtggcttgtggctgatgcactggacagtgtacatataaaacatttccatcgttgcagaaacttctattgaacagcagttgtattagtccgttctcaacactgctgtgaagaaatacctgagactgggtaatttataaaggaaagaggtttaattgattcccagttccacagggctggggaagtctcgggaaacttacaatcatggcagaaggggaagcaaacatgtccttcttcacatggaggccgcagcaaggagaagtgcagagagaagagggggaaaagccccttataaaaccatcagatcttgtgagaacagcagcatgggggtaaccattcccctgattcaattacctcccaccaggtccctccaatgacctgtggggattatgggaactacaatttaagatgagatttgggtggggacatagccaagccacatcagtgttgttacacaccacagtggtgctgtggtgtgtaggtgggaaaactatggcatgggggccatatctggtcctctgcctatttttataaagttttattggaacataggccacactcatttatttatgtactgtctatggatgctttcacactgcaacaatagatccaaatagttgcaaagagactgtgtggcccacaaaacctaaatatttactatccaggccaggcatggtggctcatgcctgtaattccagcactttgggaggttgaggtgggcagatcccttgaggtcaggagttcaagaccatcctagccaacatggtgaaatcctgtctctaccaaaaatacaaaaattagctaggcttggtggtgcttgcctgtaatcccagctacttgggtgtcgagacacgagaattgcttgaacccagaaggcagaggttgcagtgagctgggatcatgccactgtactccagcctgggtgacagagtgagattctgtctctcaaaaaaaaaaaacttactctttggccctttatggaaagtttgctgacctcttctgtagatggtagggtacggtagaaggtgttcaagccaggagtaacatgaatgattgtatttatggcctaagaggataactcgtggtggtgggcgggccatatttgtggagagacccattttcagtgacttccaagagtctgcgtgagagatgactgaggtcttgccctggcaggaatggttccattaatctgtgtctcatttgacaaatgaggaactacaaatgggaacagtttaagatgagatttgggtggggacacagccaaaccacatcagtggtgctaatagacagtggtgctgtggtgtgtagtagggaaaactatggcctgtgggccaaattttgaagtccttttactttttggttctaaaaattattaattgtagccagagttgttaacttaatatgtcttggaccccttgggctctctgaagactgtactctttctttccacttaataatatacatggaattgcaaaggaaaccaatgatattgaaatagatatcagaaataaaatttttagatatagcaataaatgcacatctgtattaaaatgtgtaataacaagatctaacagtgagtctaagaactactataattatcatgtagcaatggcataaaggatagtttgtgctatctaaaacagtcaatgacaggagaaaatctgatttctttggtgataaaacgacaggtgctgctaatacacctgtgttttatggtcttcgtttgtaatgaaaagaaatgccattaataaattttatttatttatttatttatttatttatttattttttttttttttgaggtggagtctcactctgtcgcccaggctgaagtgcagtggcatgatctcggctcactactacctcctcctcctgggttcaagggattcttctgcctcaggctcctgagtagctgggattacaggcgcccaccaccatgccaagctaatttttgtatttttaatagaggtgggggtttcaccatgttgaccaggctagtctcgaactcctgaccttgtgatctgcctacctcgggctcccaaagtcctgggattacaggtgtgagccaccgcacccggccagatgctgggatgttttttaagaccttagaccctaagcctatcatatcaaatacaatgaaacacacccacttttcacactttaaaaaaagtgtgttggtgtttattgctgtaaaatagtttgaaactttttaaaaaaagttttggtcttgctcatacttgtgttttaaaaaagtatttggctatgactaactcagttatgtatttatttatttatttttgagacggagtctcgctttgttgcccaggctggagtgcagtggcatgacctcggctcactgcagtcgccgcctcctgggttcaagcctcagcctctcgagtagctagaattacaggcgtgctccaccatacccagctaatttttgtatttttagtagagatggggttttaccatattggtcaggatagtcttgatctcctgacctcctgatctgcctgcctcggcctcccaaagtgctgggattacaggcgtgagccaccacgccctgtgactaactcagttatttaacaattgactgtaatttctcagcaatcagtgtatacttggaaattcttgggatgtgagaaaactaacctataactcattttcttttttctttgaggtgaggtctctctttgttacccaggctggcgtgcagtggcatgaacagggctcactgcagccttgacctcctgggctcaatcctcccacctcagtctcctgagtagctgggactactggcacgtgccaccatgcctggttaatttttgtattttctgtagaaatggggtctcactgtgttgcccaggctgatcctgaactcctgagctcaagcaatccacccactttggcctcccaacataccgggattacaggcatgaatgagccaccatgcctggcctgcaacttctataaatagcaaagttagtaattagtgaagatgatggtttgcaagcactgaattatacttctattaatttcatttcctttcaattttctaatgttttgtgcccaatctgtcctgtctgcctctacctagctttagaagtgttttgttggttcctgagatggagctgtgcctgaagggtatgaggttaccctctgggttcagcggggagatttgggaagagttttgatttgtaggccagtaaaggggcctgacattagatgatggctgctgggctagggaacaacttagaggcagctaacaggattcagggagagtggatttggtgggagagagtagtctaggatgaatccaattgggtttttatgagtagtttggtagttggttgactgggtgggtggtcccttggtaattatttgttgattagtggttgttgggttaggttggttacacttacattatagtcgatggaatctcagatttggatctaataccacatgtaagtcgagtggatttttttttgagacagagttttgctcttgttgctcaggctggagtgcagtggaacagtctcagctcaccacaacctccgcctcccaggttcaagcgattctcctacctcagcctcccgagtagctgggattacaggcatgcgccaccacgccgggctaattttgtatttttaagagttgggggtttcaccatattggtcaggctggtctcgaactcccgacctcaggtgatccgcctgccttggcctcctaaagtgctggcattacaggggtgagccactgtgcctggccagttgagtggatttttttagcactcaagcttcgtggctcattgctattattgtgcatgtgagcgttttatctttcagtagcattagggatgctacttggatgtgttttagttattacagaaatagtttttactaacttttactaagttatctttcctctcctgtgtaggaagtttagagtgaagcggcagttggctggaggttctgaaggtttccccctttcacataatttgatgttccagttgcccacatcaggacgactccctctctttctactgatgtaagcagtgggccaaattatggggctccatccctgcatcttcctacttgtctaaatcttcgtcacagacaacatattgctctaaaggaaacctagaaaggaggagaagctggttttcgcccaaattcctcaaaatcatcgcctgttgtttaagaattacagtttgcactggaacaataagatgttccttaatgtggtttttaagtgagttggttgtcgcctgaatttcataaacactggctaaggattgtgcaaaagggtgtgcttccctttagcatccttaattagggacagcgttttgaaaactgctttttattgtcctttatctgcaaaacttcttgaatccaaatagcgagattctcatttcttaatcactgccacagaaagttgtagattagagaaagctccaattccttatttcctgtcttcctttctttctgtgtgtttattgcctgtgtctcatcctcactcctgccagttttatagaatgtaacctcccagcctctgggaatgtttgggagacttgttcatagaggatctgaagagcagtttaaagtggacttacccaaactatcttctggagaacattagtctctttggagataaaatttttaaacatccgctagtccaatagtgttggcaaattccctgtgacactgtagccctctctttgagattgtcaatgtacgttggcatgttaaaggctctgagaagtcctgcagcagttaaaaaattgtttagtctagtgtgcccccagttgtttggccactgaaacccccttttctggaaaaaccagctaacatctggtagtcttttctaagaggtggtactgaagatgatactcatgttacacatttaaaaattctaacatgtgtttttcatgtgtttataaaatgcaactaatgtatcaaacctgtgatttccaggacataattacttaagctaaggaaaaaagaaaacatgagtgaaggaaaaactttagtaaataggccaggtggtaagaggagagagccttgtctgtgagtgtggtctagggggatgctggacctagcttttcagagctaggttcaggcagagctgctctgagatgtagacactgcagctggggttcttgttgagccgggaagcagcttctgactaaggtgcagactgtttagatgagctggtcataaagagccctgactgtggactgcgtctccagccacggcagcagctggtggatggggtgatgccttggatatttatcgtgtgtttcttgcctggcctgcccttggacagtgcgcctcaggaatgttagaatgtgttccccctttagcagcaaagccgatctgctgtgtacttgttctgtttatcttactgccacgaccgtttatcacgggccagagttcaggggcacactgataaatctcttttaggaggatgatgtaaccctcagcattttccccctacttggttctgagtttttaaagcttttgtaacaccatcatgtccttgtttgggcatcttcctgtgtactcccgtttgggtctccagggtgaaatagccaacagtggattctggagtcatggcctgggttcaaattcctgctctgctgcttatcaactctgactttgggtttaattgacctattcattatttttcttaatctggaaaatggagccaacagcagttcctcataaagcagctgtaaggattcaggggggtaactgcacagggccaagccctcaggtttcacctctcactgggaggtcggacctctgcataatggacaagctctcctagggtgcaagtgaacgggggcgcaagggagttaggaaggtgggtgttttttgtttttgttttttggtggcttgaaaaacatgcccaaggctgggtgtggtggctcatgcctgtaattccagcactttggaaggcagaggcgggagcattgtttgagcccgggagtttgagatcagcctgggcaacatggtgagaccctgtctctctttttttttttttttttttgagatggagtctcgctctgttgcccagactggagtgcagtggcgcaatctcagctcactgcaaccttcacccccaggttcaagtgattctcctgcctcagcctcccaagtagctgggattacaggcgtgtgccattgtgcccagctaatttttgtgcttttagtagagatggggttttgtcatgttggccaggctggtctcgaactcctgatcacaggtgacccatccaccttggcctcccaaagtgctaggattataggcgtgagctactgtgcctggctgacccaaaaaattagctgggcgtggtggcacacacccctgtagtcccagctacttgtgaggctggggcaggaggattgcttgaggccagcctgggcaacagagcaagaccttgtctcaaaaaaaaaaaaaaaaaaaaaaaaaaaaaagaaagaaagaaaagaaaagaaaagaaaagaaaaacatgcccaaaggcaaccaaatgactccatcttttgcaatgtaatcttcaacatcgactcctctggcaagctgtttggaaatggcaaagtccatctcctgaggctgggagattgcttgtccaggacgggtgtgtctggtgaggaatggaaggcatttggatggccactgagaaagctgagccaaggagcatcagaaagacaatcaggcaaacccacagagtctccaggtattcctttgctgataggtaacattgcactagcgatttaaacaaacaggtgaaaggccattgccctaccaccccacctcacctctattccttgctgctctttccagaagcaactgcatggtctgggaacagttttttgtcttgtcaagagacagtctgtacatagatgaattcaattatattacttctgtagtaccctgtactcaaatttgaacctgtcatacacattgcttttatcatttcataatacctgttgattttcccacgttagtacctatagatcctgacaagcaattttgttaagatgaagagttcttcatatgtattgtactatgtttctttttttgatgatgtatgtcaagatttattataaaagtaacagatgggtagggcatggtggctcattcctgtgatcccagcactttgggagaccgagatgggaggattgcttgagcccgggagtttaagacaagcctgggaaacctggcgaaatcctgtctctacaaaaattacgaaaattagccaggcatggtggtgactgtcccagctacttgggacccaaatgtcccagatactcaggaagctgagtcgggagcctgatcctcagaggtcgaggttgcagtgagccgtgattgcaccactgcactccagcctaggtgacagagtgagaccctgtctccccctggcctccaaaaaaaaaaaaaaaagtaacatatgtagtttaaattttaaaaattaaatttttgggggggctgggtgtggtggctcatgcctgtaatcccagcactttgggaggccaaggtgggcagatcacctgagatcaggagttcaagaccagcctggccaacatggtgaaaccctgtctctagaaaaacacaaaaattagctgggcatgatggggggcgcctgtaatcccagctacttgggaggctgaggtgggagaatcgcttgaacctgggaggcggaggttgcagtaagccgaaatcatgccactgcactccagcctgggtgacagagcgagactccattaaaaaataaaaataaaaaatcaagcaatgcagaataaataacaacaataaaatgaaagcccatcttccaccatcagcttcttagttttcttcctagaaggagccagtgaggacagtttggtgtttatgcttccagatctttctgttcagatgcagtcatgacttctgaaaaacaggattgtacaattcatacttttctacaaattatccccttcccttaatacatcatagaagcctattcatattggaacaaacaaacatttcttattcttttcacagcaccctgttttcctcttgcttgaatgtaaagtttatttaaccacttactgtcagggaggcatttgttttcagttctccctccctccccccaccagttgtcttgtaatgaactgctttaatggctaaagatcactttaatatcaaaacctcccccacctcccattagaaaaagaaatcatgttagggaacttcaaattgaatttacggaccttgtgtttaattttctatcagcagtggccccagcctggcccctgcagactgccccggaatctgtgggaggagttggggtggcctgcagactagagcacactgccagttcattcagcagctcaccgagcaagaaacatcttgattctatcagccttaatgctgtgtcccattagggacccagctcttgtggtcattagcagatggaatgctcatctgtgctagaaggcggaattctagggcattcggctctgagcagtcttgaaccagaattgaatggcttgaatccttttcacaatgccaacggggaggcacccttagctcccaaacttgtgtgtgttataatactatggtagtaataacagtggttgtagtagcccccgtgaatttgatgggacagtcgtcaggcagtgctgcttgcttgctttactccatcgtatcaccgcagcctgatgaggcgagggagttacgactctcattttgcaggtgaggacactgagcacagggaatcgacccactcatggtcacacagcttgccaagtcgctgtgcttgggaggtgaaccaggcttctctgacgccccagcaggacgtctgaacttctagctgccccatcactaactgacttaatgcccctgactcctgggtgacttggccaccagttacttcagccagcgacctgccctttctttgagtgggttccacccatccctgcaccatgccttttactttggatgttggtggcatggaattccacccgtaagaaggaggtcggtccctgggctgagagagtttgcagagagctctgttgggattgggtgggacgtgtgtttggaggcctcctcacataattgtgggctgaaaggtccagatttggggatataaagttgagccgtcagctgagctaaagacagggcacagggaggagccatccagaaagtgtcagtgtaggtaaagcaggcagagttccccctatctgtcctctgagggcctcctttcttgtggtttcctcccttttctgtggtgatggtcagagccagcggttataaattatttggaattttcctcagcttggttcctactcaagactttaaattaggagttttgttcccttttatgacttcacaatctttgggcaggctgccatctctacagcaggctaatatgagttgtaacttgaggtgagttacaggggaaaaatggaagctgatttctccccttttaaaccaaggaagccaccttgatctgactttgtaacaaagctcaacttttgtaagtttgcaattaaaggataaatacctatcctatttattattattattaactttttattataaaaggggaaaaaactcccaggaaacatagcctaatatgagggacaaaaagccaaaaggttttttttttcttcctttaaaaggtcctcaatgtcttgccctgtggagacaccagttttcattataataacgccattatctctttgtagagtcatttcaagccaatttaactttctcatttaaaagtataattggtattcagcacagagctgggagctcagtaggcagttagaaaatatgtgtatattttttgagacgaagtttcactcttgtcacctaggctggagtgcagtggtgcgatcttggcttactgcaacctccacctcccgggttcaagcaattctcctgcctcagcctcccaaatagctggaactacaggcactcaccaccacgcccaactaattttcgtatttttagtagagatggggtttcaccatggctggtctcaaactcctgagtttcgccaggctggtttcaaactcctgatttcaggtgatctacctgccttggcctcctaaagtgctggcattataggcatgagccacagcacctggctggcagttaggaaatatttattgaatatgagaaaagaaaaatagagcaaattgaatcttcaagtagtatgtgagtaactctaattcctgttttctggaaaacacacaggctgataggtttgggtaaataagagcagagctgcatcttctctcaagttccctgattccctcaaggagttacctgagaatagctctgtgccaagcagtgcggcatgcataggggacctcttgaatggagggacagtccattatcattagaatccccagttccagccaggtgcagtggctcatgcctgtaatcccagcactttgagaggccaatgtgggcagattgcttgagttcaggagttcaagactagcctgggcaacatggcaaaaccttgtctccccccgccacacacacaccacacagacacacagacacacacacactggctaggcgtggtggcaggtgtctgtagtcccagctacttagaaagctgaggtaggaggattgcttgagacttggaggtcgatactgcagtgagctgtgatcgtgccactgcactccagcttgggtgacagagcaagaccccggaccctgtctcaaaaaaaaaattccccagttctcagggtgtggtagaggccgagtcagtcatggctgagacaaggggactgtgctctgtgtgcttctgtgccctgtgtttatatggttcatacgctgcctgtccaccatgtttttcccgagagcctcggcagcgcaggcatcatgggaatgactgagtcaggtggaaattcagaggccctgccctggtgggcagagaagcctggcttacctcccaagcacagcatgtgtgtggatcacttctgtgcactgtctcctcatctccaaaatgggagtcataactgaactcacctcatcaagttgttatgagatgatgtagattcagcgaagtagcaagagtaggagtttgggctttgataacagagagaagtgagtttccatctagattctccccctgtgtcacttttggcagttggcttcacctctgtgggcctctgttatgtcatctgtaaaatgggattaaccctaaaagccaccctcacagggtcattgtgaggattgcacaaggtgatgcaagtggcacagggtctggcccaggagagggggctggaagagagcgagctgccattgtattttggttgctgtggatctaaggagaagagatgtttaggagtctttccctggcatggttcctcctgccttcacccatcactcttttcctcgagggattccctgtggggtgcacagccccagggtgggccagactgagctcacaggagcatgggctgtgtttcaggtgaggtggcctcaccacatgacaaactgagctggagtcaaagggtcacgaggacctccattcacagccagcatttattatttcagctggaaatgtttgccgagcagttgtagctggaagctgtgagcgagacacagactgccatcaggctgaggcctccagagctcatgctgggctttaacctgagcctcttgggggctgggctctgagctcctccacttctgctcatgcccaggcgtccttgggggccttgaactgtcagttgtccaggagaactgtgtggcagcaacagaatgagtttgtatagcaacctgttgctttgaggtttaaaacttagtttagaacgcaattgctttgaccattttggagtgtctatactttttttcttcttctttaagttttcttttttctttttttcttttttttttttttgagacagagttttgctcttgttgcccagtggcaacaagagtgcaatggcgaaatctcggctcaccacaacctctacctcctgggttcaagctattctcctgcctcggccttctgagtagctgggattacaggcgcccgccaccatgcctgaccaatttttgtatttttagtagagacgggtttcaccgtgttcaccaggctggtctcgaactcctgacctcaggtgattcatctgccttggcctcccaaaatgctgggattacaggcataagccatcaagccctgcttttttgtttcccttcttcgacctttctaacaagaggttggaatcctcgttttgacttttaaaggatttcccagtgctagaaagtggtaagatagttactgtatcctaggccctttagcagacctgtctcattgatcatttatttagtccagtgtggctttgttgttggatattaagtaattctcaaaattttaccttttcaaaagtggcattgaaaataaaggcattgggtgatgaaaatggaacttttaaatacagtgattcctgttaaccagaaatagggtgtttgggataatttatgaagcagtacaccatcatagatactatgagctgaaagttcaccaaactctctatcccaaaataacaataaggtatttatgaagtgattcgttccaactatttgaggcaaaaattgtccagcaagtgagagagaacagaaggaatagttggcaaaatagggaatttgaagtctgaggttatgcataaggaatgtgttatgggcctatagtagaaatctcaaatcagggattagggaatgtttactcagttctgttgcagagaaatcctggccacgactcccccatgccatgcccagggcaggcattgctaatcttcactgcctccattctccatgccctgttcacggaagacatttctaatgcattttagcagtcttttttttttttgctgaatccagatgtggcctcagaatccttctcaacacagtgtactagcaccacttggtgctcctgatctactgtatcatctcttgaaaaactactaacatgaaaagacctgccaagtcaactttatattaactgaacccttgacacagtgatggataaaaattaattcaaacagcttctttgtgatctttgagtagttcatgagcaagaaagagaattggaaatccagccaacttcggcccccttgtctacttgtattttactgtggtttatgttttctcttaccaattgagataggcccatgagacttctggtcttccaaagcccagaacatccccacattatagtttaaccactgtaacaaagaggttttttttgtttgtttttttgttttttttttgttttttttttgggacagaatctcgctctgtcgcccaggctggagtgcagtggcatgatcttggctcactgcaagctccgcctcccaggttcacgccattctcctgcctcagcctcctgagtagctggggttacaggcgcccaccatcacgcccggctaattttttgcattttttaatagagacggggtgtctggatctctgacctcgtgatccgcccacctccgcctcccaaagtgctgggattacaggcgtgagccaccacgcctggccagaggttttcttaaaaacaataacaacaaaaacagttgtggaaagcatgtagagtgtgggttttttcggtcttcaggttggcagggcatctgatactgggacccaggttccttccctcaccttgctgtgcctctcctagtgcaggccaaagccaggtgactgcgctgtctgggctcctggctggcaatcggggaaagagtgcatggagcaggcatgcccactgttcaggtcctgaagccgtggctcatttcatatcatttgttgcttatttgaaagacaggcacagcactgacttccaggggaggctgactgaccatctaggtggaagttgcatgcctgggagggagaaggggacaaaggccacagataggcatcagttatcagggccttaagtctgccttgttggcatgcagccttttattggatcaaggccctggagaaaagccctgagcaggaggagataagccagcttggtccccttcatcctacccaggggcctctggggtacctgagccaaagtgcacagttcattggctgtgtggatggaagggatatgggacttgaaaatgggacactggtcctgggcagctgaccgacatggtcctccttaacctgctgtctggggagatgggttgcatctggctaggttttgactgaggaactgaggagagctgtcagctgtccccgctttggttcagaatgcccttttgtttggacagctgaagcctacaattcagccatggtttgtttgggctcagaaaacaggcaaggatggagagaaactgcaaagctgacctgggctgtcagtgggcaccaggtcctgctggcctggggtctggatgcaggagatctgagctcttcaatgtggggtggtcttgcagcagctcttcacaggctgctgctgctgctgctgtaggctcacccaagcagccaagacggacaggatctattctagttttgtgcagagttggatatagaagaggcattagagggagaggggatggggaaggagttccaggccaggtgagcatggggcacagtaaactgggatgttaaggaggggccagtttgtgaccagcctgggcaacatggcggaaccctgtctctataaaaaattaaattagccaggtgggtggcatgtgcctgtagtcctagctacccaggaggctgaggtggaaggatcgcttgagcccaggaggcggatgttgcagtgagcagagattgtaccattgtattctagcctggatgaccgagaccctgtctttaaaaaaaaaaaaaaaggaggggccagacccctgacccatatgtgctgctcttttctttcagggaggtctgataaaatatcagtagttcaattctttttttttttttttttttttttctgagatggagtcttgctctgttgcccaggctggagtgcaatggagtgatttcggctcactgagacctccgtctcccaggttcaagtgattcttgtgcctcagcctcccaagtagctgggattacaaggtgcccaccgccatgcctggctgatttttgtatttttagtagcgacagggtttcaccatattgtccaggctggtctcgaactcgtgacctcaggaggtcctcctgcctcagcctcccaaagtgctgggattataggcgtgagccaccatgcccggcccatagttcagttctttaggtggttcttggtgctgcatatgagatctctgcaagaaggacacgtctgagccgggtggtttagaagaccagcatggcccaagaccctcagagcaacaccaagaaccacctaaaattctttctcagacgtgtccttcttgcagagatctcacgtgccccaggttcgctgcagcgttaggggtcagcctccctttggagcaggagagcaggggccttggaggtggcagtcatggccctcctaattaattgcttggctcagagaagtgacaaattgaacatttcaaccacctgttaattcacaaggtacttcttttcatttcttgctgcttgcacaaaacacttggagtatggcttgtggatgtctggccctagggaagagtgtttggcacatagcaggtacttaagtattaggaaaatgaggatggaggggagggagggaacattattaagcggccaactgtgagacaggcattgtgcttgactctttctttctttttttttttttttttgagacagagtctctttctgtcacccaggctggagtgcagtggtgtgatctcggatcactgcaaccgcgcctcctgggttcaagtgattttcgtgcctcagcctcccaagtagctgggattacaggcgcctgccattatgccctgctaattttatttttagtggagacagggtttcaccatgttggccaggctggtctcgaactcctgacctcagtgatctgcctgcctcggcctcccaaagtgccaggattacaggcgtgagccactgtgcccggccgacacttggcattctctaacctacctactccttataacagccctgggaagtagttgaccatggccatttctatttggtagatgaggaaaaataaggttcagagatggattgttcaaaccgatgtatctagtcaagctactggttcccgagcctgtgtttgcaacccctctaccatgtagcctctccgggtggtagagatgagggggcagagtgcacagtgcatggcatcctgttccccagatggccaagtcttagtgcgagtgtgtgtggccttggtaacttgtgtcaagcacacaccccatctctctctctctctctttttttttttttttttgaaacggagtctcactcggtcacccaggctggagtgcagtggtgctatcttggctcactgcaacctctgcctcctgggttcaggcgattctcttgcctcagcctcccgagtagctgggactacaggcacatgccaccacgcccagcaaatttttagaagagactgggtttcaccatgttggccaggatggtcttgaactcctgacctcgtgatctgccctccttggcctcccaaagtgctaggattacaggctctcttgctctctctctctcttgtttttttttttttgagacagagtcttactttgttgcccagcttggagtgcagtggcgtgatcatggttcactgcagcctcgatctcctggctcaagcaatcctcctgcctcagcctctcaagtactagttggtactaatgggcatgcaccactacacctgactaattttttttattatttgtagggacagggtgtccctatgttgcccaggctctggtcttgaactcctgggctcgagctatcctcctgtctcagcttcccatagtgctgggattacagagatgaaccgcctggcctacacacccctatctctcctcgattcttttttttttttttttttttttgagacagagtctccctctgtctcccaggctggagtgcagtggggtgatcttggctcactgtagcctatggctcccaggttcaagcgattcttgtgcttcagccacccaagtagctgggattacaggcacacaccaccatgcccagctaatttttgtattttgagtagagacagggtttcaccgtgttagccaggctggcctcgaactcctgaccccaagtgatcctcctgcctcggcctcccaaagtgttgagattataggtgtgagccaccatgcctggcctctccttgattcttacagtcactttgttggctgtttctgactcagcagctacctgcattgtggccaaaggatgacctattccttctcaggagggcaaaaatgtggaatagtgtctgtccatgcctctcctcatgggctaccacctctgccaccgtggttaatcagtaacaaccaggagagaagctgctggaactgacctctgggaactccctggatggtttggtgcaggaatgtagtaggcatacacgtggttgcgtggatctgggccctcctgatgtgagtagagaggtaaaaggccaccatctccttgacctctggggaactcatccacaaagaagatgtttccaagatgcttctgaagattgcctaaaaatagccggtttccacccccgtgaatgcatccattctagaatgctccttcaccaggaccagagaactgatttacagaagtgacatgaaaacattccatcccagaatttgcagtagctcaaattaagtttctagctattaaaaagaaaagaaaacaaaactaaacaaaacacacccaccctgctcacttagaagcaacactgagtaattttaagtagttcgagaaaatgtatgtggtttgagggtcagggttgtccagagccaagaccagttatgtgggaattgttattggctggatttggggaggagaaacccatggcccaattccaacccactgaaatctaagcagattctaggtggttaggcggacctggtaggcgttggtttattttattcccgaaaaaggccctggagcaagtcttcacatggaatcctgctgaaaggcttccggctcatctggccttttcctcctcttaaggttctgctccatgttttaccctcggcgtaaacattgcagagcacgttcagatctgaaaagtgtctcatctacgtgatggtcagacgttgttgaccctgtgatgctgtgtaacatttcattttcgaggcttggggagtctcctatttcatgtggatgggaacctggaggtctttgggcaagtcgccatctttttattgttccaagagtttggtgaagcgtttgaaccttcacctgtcaaaatcagttttggaatgagaactgctctctctctagtccttataatagcagaaggaaggtatcatttatcccaatgagaccataaagggggctttcccgtgtggacacccaccttgaattcaattggaaacagaaattctgggcattgtattttttgtaaatttggctcagacttcaactggatcatatttcccccaaaatcttttcgaaaaagacttgtgtctcattcctttagactagcatgtgtaagctgggtaaaaatagagcaagccgatttcatgttaatgatttcatgttaggtttgtgaatcaaatctgcaagtctgcttttgaaaagcatttaacatataacttgggaaagtttgagttttgcagactaatgcctgtggccggatgagacttcatagctccatccaatccctcctggtgcaagagatcaatgccttgagggtgcctggccaccaccattaccctgacagtatacccactatttatttatttatttatttatttatttacttatttattgtttacccttttgaagattgctcttctccctttaacttaaaggaattggcatggaaacttgtttgatctggaatttctgataatcagtaggtagtaactccgtaatcaatagcacttcaaaacaacaaccaaataacaggataactaatccaaaaaattcagtcatggtcaaggacttccagctcaggaaatgtctggtcccgtggggtggattccttggataaccaagttccgtgcagggcctggagttttatgcagaccattgctccttgattgaccacaggacctcaaaaggagggctggcttcatgaccacatgacccgtgtgctcagaagggccctgtacttggtttattgctctgctgttgctgtcttgaagttcttaattttttttttttttttggcactggggagttgcagtttcaaacaacacttattcattgtctcacagtttctgtgggccaggagtccagccatggcttaagaccaggtcctctgctccgggtctcacgagactacaaggaaggtgccatctagggtgtgttttcatctgaatgcctaactaaggaaaaatccacttcattcaggttcattcaggtttttaaaagaatccatttctgtgtgattgtcccactgacaggtcccagctttttactagctgttgcttggaggctaacctcaggttttacaggctacgctcatatctctgccatgaggccttctgcataggcaattcataacacaggtgcctgtttcctcacagccagcaagagaatctgtctcctgtctgctaaagtggagtttcatgcatcgtaatatggtcatgggagtaatagcccgtcacctctgccatttttctgttggttagaataaaggcacaggttttccccacactcaggaagaacccatgatataaaggctttcagtaaaggagacgacaaacagaatatggaatgatcagaattactcttatgacccagaccaagaacatcagcattacctacgaatttattggaaattcaaattctcctgtttcaccccaggcctgttaaatcagaaactttaaaagcgagcccagcattctgtggtttaacagatccttcaggtgattctgacacctgctgaattttgagaaccactggtctagaggcaggcaggtcttgctcccctaggagttaagtttgatgtatcttctggtaatactgagaaatgagctgggaaatggttccaaaatcagattatcctccccaggattaacaagactcatacttgcaaaagagagtgaagaagagaaactaaaaaaagcaagaggctgtgtgtgaagctagattcaaacagttaaagacagcaacacatggcaaaggatgggaatttgaggaagtgggtagtgaaagcaattcttgagctaaattacaagaaaacacggtgaatttgtatctgtttcctatatttagggggctggcttaaacgttagtgatacatttggggagtagaaaatggatgttggtgtgaagttcttaagttttggacaaggaaccctgtattttcatttttctctgagccccatgaattatgtagacagtcctgcttcgaagttattatttatacaattcattatagagaaagtccttgggaaccttaactttgagtgaggattgcttgagttagtttttcttaccagccactccatgatactctttgttttttccaggttagatgatcgagttttattatgactgaatctgcacctgcaaaattaattctgattaattaatttaataattaaattctgatgatttctctctgatggtttgggtgtgggctcttaaagagggtctttttttgcaagaggatataacaataatcaggttaattaaaaaaataaggctctcaccctttcatttttgagtggcatgccatgcaccccttatcagcatgtgagtatgcttttcatgtggtcgtggttgggtttcattaagtgtaatttggcatgtgttcaaccagcattcaggtggctcttggtgggtggctggggagacaccaagatgcagatagctcagtcactcctcaacaagcggcttagttctggaatgaggtgggaggccaaggaactcacacataaatgctggtgggagtgaagtgccaccagctgtagaatctggtgtcagaatgatgagccaggagttatcccacaggaggatgggtgaaggtcttcccatcaaagggatagagaacatgtgaagaggtccaggggctcagggcaagatgtagtccaggaacaaggagtctttgagcctgcagtatggtgggtggaagtggcaagagtggaaagcggattggatggggtttatgtaggttctgaggtgctgtgtatgtttaaggagctgattgtgtgcagcgggaaccctggtgaatttggaagcacagaggcacctgacgagaaagatggttctggggttatgtgaacagtgattcggcttcaaggctatcaaagacaaaaatgtttattgggagggtatagaaaagggtttgccaaaagagttaggtagggatagaattgacacattgtggaaactatacccagagtttaagaggtggagtccaggatagtgcccatgtttgtagcttggggtcctggtagaatgggagctggctatggagtatctttgttggagagtgggtatagggaaacggagagagagagaaagttgcagggggtgcgggagatggatagctgcagagaaggcaagggcagggaaagtggaaacaaatggcagtgagactcctggaaggtgctggccaggggcatggcatggcatgttctgttaagcaaggaaaggactagaaaggggccatgattttggctgggcacttatcctcctcacaacaggacgcatttgtgtcatggcttactcttaagaatgactgacgtgtcagaatagcaaatatgaaaatgattgataacacctagcattggtgagatttgcagggataactagctggcctcttaaatctatagataggaatgtaaacagaaacaaactttttatagggaaaagatatctaggacataatgattaatgaaaagaaaaaaattcctacctatcgaaaaacgtgaattcaggcagcaaacacacatgcatgtatacacatacacacgtgcacacacgcatacacacacaatctggtaggctgtatactaccagtttagcaggttgttacctctgggatgcagtcactcctttttgttgtgtatatttgtgaaatgatttctttcaatttttgagacagggtctcactctgttgcccaggctggagtgcagtggcgtgacgtcagctctctgcaactttcacttcccgggctcaagcgatcctccaacctcagtctcctgagtagctgggactacaggagtgagccaccatgctcggctaattttttttttttttttgggtagagagggagttttgccatgttgcccaggctggtcttgaactcctaagctcaaagcaatcctcctgcctcggcctcccaaaagtgctggggttacaggagtgtgccactgcacctggccattattatggaaaattttaggcgtatacaaaagtagagacagtggtgtcttacatgctcatgaacccatgatccagtgacatccgttaatggcattttggaatcatatttcatctgtttttgtcctcaaatgttttgaagcaaatttcagcattacatcatttcactcttaaatatctcagtatggttctctaatagttgaagactccatttacatttatataaggagcataatttacacttgtgtaacccaaaggaatgaccaagcctgtgcttctctccccagatagcaaagccattgtggatgggaacctgaagctcatcttgggtctggtgtggacgctgatcctccactactccatctccatgcccgtgtgggaggatgaaggggatgatgatgccaagaagcagacgccaaagcagaggctgctggggtggattcagaacaagatcccctacttgcccatcaccaactttaaccagaactggcaagacggcaaagccctgggagccctggtagacagctgtgctccaggtaagtggccagggctgcctaaaccatctgtccaggatgggggtgtgtgggtcccaaacattctggttttcaacgggaatgctatctttgctttgattagcgtatttctccaggtcttagcccattataagcccattataaggaaactaaaactggctctgtgtacccttccaagggcagattttctaggtatatccatagacatgtttgagcatcaagttgagtcttttatccaaattccaatgaaggagttggtgcttagaagcaagacttgggtttaggttccagactccaaaatcctgtgtcttcccacattggtgctcagtttctcattggatttggagaaacatttggtcctattaggtggcttggcatgaaaatctgaaaacttccatggagtggaaagtacccatttttattaaccactggtttgactatatatggcattctccacccttttctttctgtgttgctgtgaaatagcatttggtcaggatccagttggagccttttccacccttgatgggctgctcatttcttagtggttgagtgtatatgaaggttgtaattattcccactggagggtttagattgatgggtagagtttgctggtacacactcagtagaaagaccagagtcagagtttacacacaccccctaaagttgattttaataaaaaaaaaaggtattaatcatattttccatttactgtgtattctgtatttactgggcacattagtatttagttagttagtggttcttgacatactcaaagcagaactagtgtcagttgggtaggggagggctgaaggcctcattcttacttgagagcctataagttggtgtcatccaggaaaaattcaaagtgcagcattaattgatttcctaatatcctcttctttacttccatttaaggacacattttaggatacctctttccaatttaaacctgggagtttttactctagtcctttacctcatgtgcttacaaaggcttttaagataattctaggtttgtgcctttgagcaagtggatttttgaatcacacaggatgctattctagactttttagatatatccaggaatagagtaaaaaataaaatccctcctgcataaaggcaccaggctttttccaagctttgtttattttttaacaccacttcttcaaggaatggataatccccatcttcatgcaagaacatagcacccggaggagaagtctcagtaatggaggatagtttacaccctggcacactcatacctgtgatactttttgcctattaaatatatgatttgctcagattttaggaaaaaatcattctctgaactaaaagaaaaaatggggttagtttaggcacatggtttcctttaatctctttggtcagctaatgctaaaagaatcttttgtgttctgttaacaggtctgtgcccagactgggaatcctgggacccgcagaagcctgtggataatgcacgagaagccatgcagcaggcagatgactggctgggtgtcccacaggtatgcacaagtgtgccaggtcctgtgaggctgcccccacccactagcttgttctgtggatgccttcccgggtcaggcagcccgaccttcttggcattgagacttcagagagcattgcctgtgatgctctctcatcttcctcagtttacccataataatagtaggttctcattgactcaggtgcttatagatcttagtgtgttggtttaatgtagatcatccagaaattttcatgtcactcttctttgtcacacactggcaaattttctagtatttcttctctaaatattttgaagactacctttaaaccccagactacaaatatggaccctaactattaggttgagccataagaaattgatagtatttgaccatttttcaatctacattttaaaaggtaattttaatccaatagcttaagaaaagtcacaggacttaaaatttttttttttttttgagatggagtctcgctttgtcgcccaggctggagtgcagtggtgtgatctccactcactgcaacctctgcctcccgggttcaagcaattctcctgcctcagcctcctgagtagctgggattataggtgcgcaccaccacacctggctaatttttgtatttttagtagagacagggttttaccatgttggtcaggctagtctcgaactcctgacctcgtgatctgcccgcctcagcctcccaaagtgctgggattacaggcgtgagccactgtgcctggccgacttaaaacttttaaaaacatgtaagccaggataatccaccattaatggaaactgtggaagaatctctatcacccataatcctatcacaggaatataacaagagaactcagaaatcaaataagtcttggataccatctacagtagtcacattgcttagttgaagtctgatcttcctagctgggaggaaaaccagtgttttctttccagaaactccctctaacagttaggcaccatgagtcccgtgtccaaaggctagccagggaagattgcaggtagccagtgccatgggactgatggcgtcactataggctgcattgaggtctgagttcagtgtattttgtaacagggtcccttggaaggtagaacaacatgcctgtttctttggtttggttttggagtcatgtctctcctacatggctcattggtttcttggctcgtccaccctcaggaagtggtgtggtgtgtttttcatctccgcttaaacctaaaccgtctcctttttacgttcacgtgatgttggcatgggtgaagttgttgaaggagctgctgggaagaaatgccaaatcgacacacatcctactttttatggaatgtattgaaggcgactgttcaaacccaagtagctcttttgttcctgcaggctaatggtcagaatgttttctggtgctttttatcacatggggagggaagttggacacatctgttgttcattgcacatggttaacctggtccatgagacagagcctctgttcatctgaggaagtgtgatttacctccttagcaccattactggaggcagggaggactctgcaagctgtttagggctgggtcagatgatggtactgaaactgaggtggtggcaccttcagggaagtcacctgtccaggatgggtctagtcttgctcctaagctgaatatcaagagaagttcacccattccctattttttttttttttttttgagatggagtcttgctctgtcacataggctggagtgcagtggcacgatctcagctcactgcaacctccgcctcctaggtacaagcgattctcctgtctcagcctcccgagtagctgggactgcaggtgtatgccaccatgcctggctaattttgtatttttagtagaaatggggtttcaccatgttggccaggcttgtcttgaactcctgacctcgtgatccacccacctcggcctcccaaagtgctgggattacaggtgtgagctactgcgtctggccttttttttttttttaaagagacagcgtcttactcctctgttacccaggctggagtgcagtggcatgatctcggttcactgaaacctccacctgctgggttcaagccatcctcctgcctcagcctccctagtagctgggattacaggtgtctgccaccacactgggctaatttttgtatttttagtagagactgggttttaccatgttggccaggcttgtctcgaactcctgacctcaagtgatttctcttgtcttggcctcctaaagtgatgggattacagtcatgagctaccacgcctggcttccctatttttttaatggctcctaatatattgagatcacatatctaatatttacatgttatttcttttttatttaccttttttaattagtagagttaatacagatacagaccatgagtatacaagcaaaggaaaaagctggttaacctgtgcacttttttgtaacatgctctaatcccatgtgtgcttgtttcttcattttcctgccttgctatagcttatccttttatcatttttgaaattttgaccagaggagtaaatggacttttggggaatggggaggacaatgaacttttggaagttacatgcagaattttttggagaggggcccctagctttcaaaggggtctgcaatttctcaaaaatggttaaaaacactgatattggtgtgttggtttaaagtaatttcacttaattgagaagctgactcagtttcttaatatttgtagtgcttggtttaagaggcatttgcaaacacttcaatagttgcaaagtgatgtgttctgggtgttcatccaccatgtcattatcctaggtcatcactcctgaagaaatcattcacccggatgtggacgagcactcagttatgacttacctgtcccagttccccaaagccaagctcaagccgggggctcctctcaaacccaaactcaacccgaagaaagccagggcctatggcagaggtgagtgctggtcctctggtgttgtattggagacatgtcctctggtgttggagatgatttcatggcttcaagagtgatgttcttagaatcaaaaatagataggtgtaatcctcaaagagaccccaagcctcctttgtaacacattttatgactgttttattctgccttgtttttctaaggctttaagaaatgtttctgcttagatggaaagggcaagtttgctgcttggtgattttagtgcagtagcccattgctcccatttttcagaagaggaatcgcggggtagggagtcgggggagtttggtcttgccccagatcaccacagtcagtgatgggggtgggccatctggctgctgattcatttctccttctgttacactaagcctgcctcagatttccagccggagtgggagctattgttaacccctggcagatacttccttgctaagacatcctgtttatgactgcgaggcagctgcggaacaccgttttgctcagaacattatagtgggtagaagccatttcaaggcatttggtgttgtgattggcacctgacttcaagcacactagctttgtgaagagaacagttacatggctgcaaagtgtggtttctggtgaagatcaacatggccagatacaacttaatgccttttctatgggggaggggaaggagtgcattttatttctcatttttcataattaagaaaatatcggccgggtgtgatggttcatgcctataatctcagcactttgagaggccgaggcgggcagatcacctgaggtcaggagttggagaccagcctggccaacatggtgaaaccctgtctctacaaaaaatacaaaaattagccaggcatggtggcgggtgcctgtaatcccagctattcaggaggctgaggcaggagaatcgcttgaacccaggaggcagaggttgcatcgagccgagatcttgccactgcactccagcctgggtgacagagtgcgtgagcctccgtctcaaaaaaaaaaaacgagaaagaaaatgttatcccagtgggataatagttatacacacagtattctgtatatcttctcccagaattgacagttgttaccattctagcttaatagttttctcttgccctttgtgtgtgtttgcatatgtgttcatgtgtatgattgctgaattatttgaaaataagttgcaagcatggtgacagttctgtcctcagtacatcactaagcttctcctaagaataggatatcctctagcataaccacagtattcattgccacatgtaagaaaattaacaatagtttcatataatctaatattcagtttgttgtagaatttctctattgtcctaagattatcttttatagttgttgctgttttacaaactaagatctgattaaggttcacttactacatttgtttgttatttctctttagactcttttcatgctaaataatttccccaaacttttttttttttttttttaaatgacactgactttctgaatagttaagggcatgtgtcttgtaggatgttccttccctacaaatgttccctttgaataaagtattttcctgcttggtatcagcttagtctttttttttttttttttttttgagagtcttgctctgtcgcccaggctggagtgcagtggcacgatctcagctcactgcaacctctgcctcctgggttcaagcgatcctcctgcctcagcctcccgagtagctgggattacaggcatccaccaccatgcctggctaatttttgtatttttagtagagatggggtttcaccatgttggccaggctggtctccaactcctggcctcaggtgatctgcccggctcggcctcccaatccgcttattcttaagacgacacatggctagggcagtgatgctgaccacgtgctgttctcacctcagtggtcgagtcttctcatctgactttttgggcatgatttagaccggcagatagttctggaacaaaccccttaccatttgaggttccgtttgcagtgggttgtgaggtgtgtgagacatcacttgtgttatgtagggactagggacttcaaagccctcctcccattcacagtcacttgaaggctggcatgtcctcactttctttaaaagtgctttctttggccgggcttggtggctcacacctgtaatcctagcactttggaggctgaggcaggcagatcacaaggtcagaagattgagaccatcctggctaacaaggtgaaaccccatctctactaaaaatacaaaaattagcttggcgtggtggtacaagcctgtagtcccagctactcgggaggctgaggcaggagaattgcttgaacctgggaggcggaggttgcagtgagccgagatcgcgccactgcactccagcctgggtgacagaacgagactctgtctcaaaaaaaaaaaaaaaaaagtgctttctttaaggcataccacaggtggtggctggaatgaggaatctctgactttaaaggttatgcttccttaatgacaaaacagttgcaaacaaccaattaaatcctttgtcaaccagattggtcaaatggactgaatctaatcaaggcatagtgtatgtttgtaataaccttatcactggccatccggcttccctgttgttaatgtgagacggtttcctttcacggtgctattttctagaaaatgatcacttgttatggttcaggaatgtggctggtcattgccatttccttcatctgcctcttagcaagtgtggtgcacttgtagaggaaacacacccttttaaaaaaaaatttttttttatatgtgtgctttttgcatttttttaattgtgggaaaatatccataacataaaattcactattttaaccatttttaagtgtggcattaagtgtattcacgttgttgtgcaaccgccactgctatccatctccagaactttttcaacttcccaaactgaaactccatactcattaaacaatagcgccccattctcccctctcctctgctcctggtaacctttattctactccctgtctctatgaatttgcttattctagggacctcctagaagtgaaatcatatgctgtctgttaggtacctcctagaagtggaatcatacgctgtctgttaggtacctcctagaagtagaatcatatgctgtctttttttctctggcttacttcatttgtcatatgttttcagggttcaccatgttgtagcatgtgttagaatttcattcctttttaaggctgaataatattcctttgtacgtgtatatcacattttgcttatacattcgtctgctgatagacatttgggttgttacattcttttggctattgtgaataatgctgctatgaaaacatgggtgtacaagtgctgtttgagaccctgctttcaattcttttagggatatacccagaagtggaattggtggatcatatggtaattctatatgcagcttatttttcaggaggaagtggcctcactctgctttttaaagtaggagacaaaatggtcatattaggtgacagggtcacaaggccacatgggtggggctgtgagatatgtccctgtcatgtggttagatgaaagccggggtcagttttggtcttctctgtgtgaccacattgcttcatttctgccacctgagcccaggaagagagaccgtttcatcttctagtttctaaaagatttgaaagtgttgttttattttttatttcctgattgtttaatagatgccagttgccagccagttagcatttgttgatccattcactgagtcccaccttgcttagttctagtgggttgaaaggagagagggctggggtgaggtggacctccagccacaaacagatctttgtggtgggcttccttgcagggttagctatgtgaaaagcattcgtccatgagctaatcagaaatctttgtaaaaatctagttctctatgaagcatttactgtagagcaatccttaagcacccttctatctgagtaatcagaggggtaccagttgtctcctttcatggtaagcaaagctccgcagaagtttacagagttggggtgtggttcaactttctaaccagccatggttagccacgggtgaccaacccaagcccagacctttgacaagctgcagagtacgttgtttcttaggctgctggagtcacacgaagtggaacttttagtattttaggtgcatgtttatttacttacttatttttgttgttgtcgttttcagatagagtctcactctctctctctgtgtgtggagtgtcgtgatgccatcacggctaactgcagccttgaccttctgggctcaagtgattctccctcctcagcttccctagtagttcggaccacaggtgtgcaccaccatgtccagctttttttttttttaatattttagtttgagaccagcctggccatgttgcccaggctggtctcaaaatcctgagctcaagcaatccccctgccttggccccctcaaagtgctgggattacaggcatgagccaccatgcttggctattaggtgtatgtttaaatccatttgcttatatcagttacataacctgagtgttatgtaaatcttaagcaaaagaaaaatatatgaaataaaaattgaaactcacttcccaactgccaatctcattcctgccttcaaagtttcaggtatttatttctagccttttttctatgctgagttaaactgtgtatcttctttgctttgcatttcttactgagcagtgtgggaaggctaccttttaaaatttatttgtagttctttataatttttacctttctttttaggcagaaagattatcttattatataacagtctacggccattttttcttaaactaaattattgggaaatgaatagaaatccagagtatagtaacaaatgacctagtgtctttaacagattggtagctaggaaaaggaagtggtggagagacagccggagattaaatgagacttaagagacttagcaaccatttgtaatatgtgaccttatttggatcctattcaaactaatggttaaaaaaattcatgatagctgggcatggtggctcacgcctgtaatcccagtactttgggaggctgaggtgggtggatcacgaggtcaggagatcgagaccatcctggccaacgtggtgaaaccccctttaccaaaaatacaaaaattagctgggcatggcggcatgtgcctgtagtcccagctacttgggaggctgaggcaggaaaatcgcttgaacctgggaggtggaggttgcagtgaaccgagatggcgccactgcactccaggctggcgacagagctagactctgtctcaaacaaacaaacaaacaaataaaaattcatgataaagcagcagctcaaggtgctgtaagaaattcatgatatttataagataattgaaaatttgaacactgaatatttgacattaaggaattatttttttttatatggtatcgatattgtgggtactttgcaagtatcttttaaggatacatagtgattgtggataaaaaatctgaggtctaggatttgtgtcaaaataatacaggaaggggaggtggcgggagtgaaggtgaaacaagaccagctgtgagttgatagttgttgaagctgggtacaggaggtccactgtgcagtgctctctacatctgtgtttgtaattcttttttttttttgagacggagtctcactctgtcgcccaggctggagtgcagtggcatgatctcggcccactgcaacctctgctgcccgggttcaagcgttctcctgcctcagcctgccaagtagctgggattacaggcgcccaccaccacacccggctaattttgtagttttagtagagatggggtttcaccatcttggccaggctggtcttgaactcctgacctcgtgatccacctgcctcggcctcccgaagtgttgggattacaggtgtgagccactgcgcccagccttttttttgagacagagtttcgctcttgttgcccaggctggagtgcaatggcacgatctcggctcactgcaacctctgcctcctggattcaagtaattctcctgcctcagcctcccaagtagctgggattacaggcatgcaccaccacaccccgccaattttgtatttttagtagagacaaggttacaccatgttggtcaggctggtcttgaactgctgaccttgggtgatctgcccaccttggcctcgaaagtgctgagattacaggtgtgaaccacggcgcccagccttttttttttttttttttttttgctgaagtttcacttctgtttcacaggttggagtgcaatggtatgatcttggctcgctgcaacccccgcctctgcctcctgggttcaagggattctcctgcctcagcctcccgagtagctgagattataggcatctaccatcacacctggctaatttttgtatttttagtagagacggagtttcaccatgttggccaggctggtctcgaactcctgacctcaggtaatccacctgccttggcctcccaaattgctggaattacaggtgtgagccactgtgtccagcctagtttggaattcttcataataaaaagctttttaaaaaggtaatatttggacttctgctcctgggaagatggaataggacttttcctaattctttcttctaactacaactaaaacccctgggctatacataaggaaaacacagggagcctctgaaaaaggatgaggcagaccaaccagggatcttgggactcgaggaatgacacagtactgagttccttgggtttactttgctttatatatcccagacttggagccaaagaaagaagctgacaacctgaaaatgccagtgggcacaaacacagaaagtgccaacaaaagctcccctgtccagccagaagaccaggaaagggcagcccagtgaggcagaaaacttaaagagtcactgctctactccaggtccacaccatagaaaaaactatgcagccccacacttacacccgcagaggtgaatggggagcctaggctttgacaacagtctagcaataaggaagccactctccggggccatggaggagcagtaatgaggcactcctacttcctccagccagaactcccaccttcacgcaccagtaatgagccccccaatcttgagcatcagtcgaggttgaatggagagcctagacttcttcccccactgttagtaacaaggtgtgtacccttccctcccctgccacagtggtatcataaaatgccagctacaacagaacatttacagaagacccagagtctcattacatgataccccaaatatccagtttcaaaaaaaaaaagaaatcacttgtcataccaagaaccaggaagatctcaaactgaatgaaaaagacagttgatgccaacactgaggtgatagagatgttagaatcctatgacaaaaattttaaagcagccattaaaaaaggcttcagtagccaggcgtggtggctcactttgggaggcttgtaatcccaggactttgggaggccgaggcgggcagatcacctgaggtcaggaattcgataccagcctgaccaaccttatgaaacccagtctctactaaaaatacaaaaaattagccaggtgaggtggtgggcacctgtaatcccagctactcgggaggctgaggcaggagaatcgcttgaaactgggaggtggaggttgcagtgagctgaggtcatgccgttgccctccagcctgggcaagaagagtgagactccatctcaaaaaaaaaaaaaaaggcttcggtaggcagttaagaacaatcatgaaaaaaatgaaaaaattaaaaatctcaacaaagaaatacaatgtcccagcaaaataataataaaaatttaggagataaaaagaaccaaatggacattttagaattggaaattgcagtaactgaaataaaaacttattggataagcgcaatagcagggtggaaggacagagaaaagaatccttcaactggacaacaattggttgttttgttctgaggtggagttttgctcttgtcacccaggctagagtacagtggagtgatcttggcttactgcaacctctgcctcctgggttcaagctattctcctgcctcagcctccctagtagctgggcttacaggtgcccaccaccacttctggctaatttttttatttttagtagagacgtagtttcaccctgttggcctggctggtcttgaactcctgaccttaggtgatccacctcggtaatccaccttaggtgatccaaagtgctgggattacaggtgtgagccactggacccggcctctgtaagcttttttctgtgtttaaaacttttcatttttgtacttttaaaacttttttttttttttaaacacacacattagtctagacttacacagggtcaggatcatcattatcactatcttccacctccaaatcctgtcccactgtcccactggtaggtcgtcaagagcagtaatgtgtggaaccgccgtctcctataataacaatgccttcttctagaatatttcctgaaggacttgcttgaggctgctttacagttaacttaatttttaaatagaagatgcccactctaaaatataatgataaaaagtatagcatattaaatacataaaccagtagcattgtcatttatcatcaagtattatgtattgaacataattgtctgtgctatatatgtttctatggccggtagcccagtgggtttgtttataccagcatcatcacaaatacatgagtaatgcgatgcgttactgtgacgtcagtaggcaacaggaattttttggctctatttataatcttacgggaccatcattgtatgtgtggactatttttgactgaaacttcattatttagcaaatgactatattagcaaataaaattgagctgtatataatgaagaagtatgcattataaccaagtggggtttattgcagggatgcaaggcctcgttcactattagaaaatcagtcaacagcctggctcggtggctcacgcctgtaatcccagcactttgggaggccgaggtgggcgatgggcggatcatgaggtcaggagatcaagaccatcctggctaacacggtgaaaccctgtctctactaaaaatacaaaaaattagctgggcgtggtggtgggtgcctgtagtcccagctactcgggaggctgaggcaggagaatggcatgaacccgggaggcagagcttgcagtgagccaagattgtgccaccgcactgtagcctgggcgacagagcgagactccgtctcaaaaaaaaaaaaaaaaagtcaaatagtaaagataccacctctcctcaaattgtcattcaggtttgatgcaattgctgtcaaaatcccagcaagagtttttgcagatagcaagattattattttaaaacctatatgaaaaggcaaaggaattaaagtagcaaaaacaattttgagaaagaagtacaacatggaggaatcagccttcctgatttcaagacttgctgtatagctacagaagtccagattttgtagtattggtcaaaggatagacattatagatcagtgaaacagaattgcagccccacacaaatatgcacaactgattattgacaaaggtgcaaagataagtcattgggggaaaaaaccttttcggcacatggtggcagagaaattgaacatccctaggcaaaacaaaacaaaagcaaaccccaaaccaaaaaacaaaaaacccatataactataaaactttgagaaaaaaacatagaagagaatctttgagatctagagctaggcaaatagttctcagatttgacaccaaaaacatgatccattaaaaaaaaataagttggatttcatcaaaattaaaaactttttaatgttttaagaaggatggtctgtctcaaagactcaacatggtacatggtggttggcctttatgtgctgttgagggttttcctgcattgaagggtgcactcctgggtcacctactgtcctgcaagacaagctgtcttagccctcacactataaaagccacccggacaccgtctcaaacagaactcaaaatgttgctgagactgggatctgggggctggattttacttttacaaacaatttaaaactttttacagttaagaggatgaatatacaggctaaagactgggagaaaaaatttgcaaaccatatgtccaacagaacactagtatctagaacatgtagaaagaactctcaagtcttagtcgttaaaaaacagacaaacatttaaccaaacaacccaataagaaaatgggcaaaagacataaacagtttctgctgaagagaacgtccatatgacaaaaaaacacatcgaaatttgttcagtatcattaaccatgagaaaaatgcgaattaatcctagtacacactatcagaacggctaaaataaaaaatattaatactgataacactaaatgcagaacggatggagagaaactgaatctggatcactcactcatacattgctggtgggaatgtaaaatggtgtagctactttggaacactgtttggtagtttcttaataaagaaataggctgggcacagtgactcccttctgtaatcccagcactttgggaggctgaggctggaggatcacttgagcccaggagtttgagaccagcctgggcaacatagggagattgcatctctacaaataatttttaaaaattatacaggtgtggtggtatgcacctgtggtcccagctactcaggagattgaggcaggaggattgcctgagcctgggaggtcgaggttgcagtgagccgtaattgtgccactgtgctccagcctgggctacagagtgagacttggtctcaaaacaaaaacaaaaacaaaacctcaaaaaacagtacatgcaactaccatatggcccaacaattgcactccttggcatttatcccagaggaatgaaaacttactgtatatgagagccactgtttttccttctatagtctcacagctaaagaaaaaaaacttttctcatcttctctactactcctctcagtatttcgcttccggtcaccaaaatctatggatttctgtcccccatactgacaagttctccaattttatgtggacaacaagtaggtgtcctataatcaattcccttcaattctgacactatctacctgaagttagtgcagacgccattaagggctcggtccctcaaaactgcccctgacttcagaggccagtcagaagtggtgggtcctcaggtaacccacagcttctgtccaggtttgctacaaatcagaaggtcccattaccccttcctcatgttatgttatttgctagagtggctcacagaactcagggaaacacttacctttagcagttgtgtagtgaaggatatgatagaggatacagatgatgccccagatgaagaggtgcacggggcaaagtttagaggcgttttgaacacaggagcgtctgtccccatgaagttggggtgggccatcctcttggcacatggatgtgttcaccaacccagaagctctctaaactccatacttcagggatgtggaggctaagtcacgtaggcgtgattgacattaactgagactacagttcctctcccttccctgtaggatggggagtggggccgaaagttctaagcttctgatcatgacttggtctttctgttgattagccacatcttgaaagctatccgggagcccactaagagttgcctgattagaacagaagatgctcttgtcaccaaggacattccaaggggtttaggaactctggaaccaggggcagagacctatatatataatttcttactattttatacttatgttcacacacacacacacacacacacacacccctatgcacagatgtttacagcagctttattggtaagagacaactagaaacaacccagatgttcttcagtgggcgaatggttaaactgtggtacatctataccatggaatattagctactcagcaataaaaaggaaaaaaaccattgacagaagcaacaacctgggtgaacctgtagacaattatatgtagtgaaaaaggccactcctaaaaggttacatagttatgattccattgatgtgacgttaccgaaataataaaattacagtgtggagaacgggttagtggttatcagggctaaggagagtgtgggtgtggttatgcaagggcagcaggagggctccctgtgctaaagggaatgttctctattttgattgtatcaacgtcaataccctggttgtgagattgagtcatagctttttaccgtgttaccactggggaaactattttgagatggagtcatgctctgccgcctaggatgcgatctgggctcactgcaacctccacctccctggttcaagcaattctcctgcctcagcctcccaagtagctgggattacaggcatgtgccaccacgttgtatttttagtagagacagggtttcaccatgttggccaggctggtcttgaacgcctgacttcaggtgatccacctgcctcagcctcccaaagtgctgggattacaggcatgagccaccgctcccagcaagggcattgtttcttacacctacaggtaaaatctgtctcgatgaatttgctcgatcatcttaaaataaaaaggttaattaaaaaaatgattgaatataatttttaaaaatgtcaggcaatacaataaatgctgtttaatgagaaataagcttcgctcctccctgctgtgttgcttccatcaaggcaagctctgctactacttattaaccacattatttccacaattttatatagactcctgactgaggttctctgaatatcaaaattggatattacttcaataacatgggcaaaattaaggctttcgacctgcctgattttccttgtcaaggcagtttgtccccatttcccacatgggatctgcagggctgggtcccatctctcagttccctgaaagagatgcagtgggcgatggctcatgacacaccctcgcctggcttctaacatgtctgtgtaaacctgtggcaggaatcgagcccactggaaacatggtgaagcagccagccaagttcactgtggacaccatcagcgccgggcaaggagacgtgatggtgtttgttgaggacccagaagggaacaaagaggaggtatgttggaggatgctgcctctcctttccagcacctcatggagcttttggggcttgtaatgcggccagggactgtgcctccattttcatttcagctcacaaccaaaagtgttttttaccaaaaggatactgaggcttatagctgttaaagtaacctgcccaagaggtgagccttgaaatcaaatttaaattgattgccagggacacagtgtttaatgaaataaaggatactttggatttagcaaaggtgccttgtcagttgaggtttatgtatgtatttatttatttatttatttatttattgagacagagtttcactcctgttgcccgggttggagtgcagtggcacaatcttggctcacggcaacattcacctactgggttcaggcgattctcctgcctcagcccggctaatttttgtaacccaagtaactgggattacagggacctgccaccacgcctggctaatttttgtatttttagtagagacagggtttcaccacattggccaggctggtcttgaactcctgacctcaggtgatccacctgcctctgcctcccaaactgctgggattacaggtgtgagccaccgtgcccagcctcagttgaggttttatatactgatggccagaataataagagtcttgccctgctctcttcccacattggccattctttggttcctccctcagagcctttgcacatgctgttctttctgtcacttattttcgtaggaccatattttattcttggcatttagcataatttgcaattctaagtttacagatggatggtccatttcccccaccggggcagggattgtatctgacttgctcatgttttatttttagtacctaacactgggccctgcatttcataagctttcaatgaactattgagtggataaaggtttaagtttcttgcttcatattctctcttacctagagagtgccagcctgacactggacactggagagtcctgactctgttatgcctctgtgctgcatggttttgtttctgtgacttcaagcagtttctctctaggggcgttgtgcaagagggacaggagctcgccagcaccttcagtgtttccgacctggcagctcctgcagaacccctgctgacacagcatgctccttactcacacccggcaccttttctaactgttgcccaccttccctcctaggcacaagtgacccctgacagtgacaagaacaagacatactctgtggagtatctgcccaaggtcaccgggctacacaaagtaagatgaagcagcatggctgtggcttgggctgctctggggctaggagaagaaagatagcccaggaagaagagtgtttttcttaagtgaatttctgattttcctttctgattatagaaggatctatgctcatgatagaaaattggaatcactaggattccctctactagctaggatgagttgtttgcaatgtcgtaagatttttccaactccatctaggtaactaatggttgcagctgtgtgtctggagtgtagatgctgtggtgactacactatagatgggttctttgtccttgattctttttttggagacagggtcttgctctgtcacccaagctggagtgcagtggtgtggtctcagctcactgcaacccccgcctcctgggctcaagcgatcctctcacctcagcctcccaagtaggtgggattataggcacccacaaccactcccagctaatttttgcatttttagtagagaccaggtttcaccaggtcacctagactgttcttgaactcctgacctcaaactatcctcctgcctcagcctcccaaagtgctgggattatagacatgagccaccacaccctgctggctctttgtccttaatgctttcttaagaactctccttggaggtgctctggaggagctgtcagcattgaaggctgaggatggagtagttcagctgaatatagtagagggaaatggccctctcagcacctggagaaatgatagggattgaggcctcaggctctttgtcttggcagcctttcgagttctgtttgagatgacatccaggtgacctatagggcaagggctgagagagcctgtcttgcaggagagtggggtgacccaggagtacacttttcattggaagaaagccctcaacagcacataaaggccaatcccatcatgtacctgcccagactttggaatacagactgtactcaccaccttgggctttagtgaattcacctggaatgatggccttagcgttctcttagactcttagactatgatgcatttggagtaaatgctcttgaagggagcatttataatgtaattaattaattccagtcaagtataggttcacatgaaacccaacccaattaccccccaaaaatttcagagatgagaacagtgactcaagttttagatggaaatcattctactttgtcccaaatccatgtatctaagaatgattttcgtcccttgaaaaaacagtttggctgtggatttgaaatcctggaactgcatattttattctgagggatagtggcccattcagcccccgaaaggactcaatgtccagagattgaaatgtgtttgtttcctattaaagagactaagtgtatataaggtcagcatttttattttgctaaaggtgtgatgtcccagacccagctgtatggctgaaggggccaggtgggagtcccattcaggctgttaaacttggttccagggctccttattctagacaccttgtgtgtgccatcatgggagggtaggagaggtgatcatcaatgtatgtggcttgatgtcagtcttgctgggcacagagaagtgattatgtatttctcacctatctgtcacctataggtcacagtcctctttgcaggacagcacatctccaagagcccatttgaagtgagtgttgacaaggcccagggagatgccagtaaagtcactgcaaaaggtccagggttggaagctgtagggaacatcgccaataagcccacctactttgacatctatacggcaggtaacgtgcctctcctccatggatctgacctttgcgctttcttccagaggctgaaatataatcctcggggacttgaaggcctgaccttttgtcttttaaatcaaataaataatcacaaagacaattttttcaaatgtgttatattagatttttcaaaaccagcttttcttctctaaaatactcaggcttcacttgaataagacatacttcttgaattgttggcttcttttccatgtagtaaatagaaaatgcagaagaaggaaacattcaaccataaacccttcaacccctagaaaatagttgttaacatcttggtgtggacctctctgagggcctgtctcctgtttacttgttttgttgttgttgttgggggaacagagaatcactctattgcccagactggagtgcagtggcgtgatcttggctcaacgcaacctccgcctcctgggttcaagcgattctcatacatcagcctctcaagtagctgggattacaggcgtgcgccaccatgcttggctaatttttgtattttttttagtagagacggatttcaccatgttggccaggctggtctcgaaatcctgacctcaagtgatctacccacctcggcctctcgaagtgctgggattacaagcatgagccaccacactggtcctgtttgcattttgcactcagcagcagtgagctttcagagagggtgacttgggctcatggaatgcttgctttcttgtaggagctggtgtgggtgacattggtgtggaggtggaagatccccaggggaagaacaccgtggagttgctcgtggaagacaaaggaaaccaggtgtatcgatgtgtgtacaaacccatgcagcctggccctcacgtggtcaagatcttctttgctggggacactattcctaagagtcccttcgttgtgcaggttggggaaggtgagtgctgggctgctggccacatgtgcttctcatagggaagctgactgcacagctgggcagggaggccaggaaaacagtcagggcccaacattgaccttatgcctatcccttttctgccagggctacttcagcagtaagtggcttactttgtcctcaatatattaatattaatatcttctatgagccacgcagagacctaaatgctttgcttatattaactcatttacttctctccaaaacacatgtacaggagagtaattatcctcatggagggaggtgggactgaggcagtgggaggactcggtagcataactgaagttagcagcagcaacatgggccctgcagcctccattgcttggcctttactggcccaggcacttaccatgactgcatctaatcattgcaccagcctgtgtgttgcaggtgctattattatccctagcttgcaggtggagatgctgaggcttagatagcgttaggtatcagtactacaaggcatcagcagggctagaaccacagactctgttggccttacccttaactactctgctaaactccctctggcgctgggggtacgcatttttctcaaatgttagactctctccctctgactttgttgcccctttttttctgttttgttttgttttgttttgttttccaactgtactaccttttctaacccacacttgcctttccctgttctgtcctctgaatctgcgtctgcagacgtggcttcctcttccgaatcctacctctgggccagcctggaccctgaagctgttggcttcctagttgagaccactgggccagaggcctcttgcttggtaagggctggttgggtgggacttccttgccagttctttgtgctgcttgtgaatgttagctgggcccgtgttctgtgtgattttaggaaactctgtgcaggtgttattattacagcctgtccagccggaacccaaacccactgtctaattgcctttaaacacatctagggcttttttagatggtgaaggagctggtggtgcccttcagactctagccccatttaatgtttatatgaactcagcaattactcttttgatgttgagactgttgcacatgttcataatttccatgagtgtgtgtgtgtttcttaagacacattaaagccctccgaggaagtcctgtcattgtattgtgactgacttctggtatgaccaacttttctccccttgacaaagaaaaaacaggcaaaaaaaattctaacatattcctaagcaaagctcttttttacataagagagcattttgaatagctttcctaattctactattgttttccaacctttcctcactcgtggacttcctttttcttttctggcctgtacatcctatactatttagcatttaatgaataacctttttcttttaatttactaacatcctctctcccacctaaatgattttacatatgtaaaaaaaaaatatatatatatttgcaggggcgcggtgggaaggatacagggtctcactctgtcttttgggctggagtgcagtggtaccatcatggctcacttgtagcctcgacctcccaggctcaaatgatcctcccacttcagcctcttgagtagctaagactgtagatgtgcgccaccatgcctggttacattttttaccctttttttttctttttctttttctttttttttttgttttgttttgttttgagacagagtctcactctctcacccatgctggagtgtggtggtgtgatcttggctcactgcagcttctgcttccctggttcaagtgattcttgcctcagccacctgagtagctgggactacaggtgcacaccaccacgcctggctaagtttttttgtacttttagcagacacagggtttcactatgttggccaggctggtctcgaactcctgatgtcaagtgatccacctgcctcggcctcccaaaatgctgggtttacaggcataagccaccatgcctgacctaatttttcttttttttgtagaggtggggtctcactctgttgtccagactggtcttaaacccctggactcaagcaatctccccgcctcagcctcccaaagtgctgggtttacagatgtaaattattttatgttaaaagaaactttatatcactttcacaatggaaaaccaaagtcacttgccataaagtgccaccgtaagcttatgttcatccataaaccatctaaaatcatctctaactccaagggtatgtgtatgactctttgggaagcagttgtttgccaaatagccagctaaggccattgcaggaaggaggaaccagaggaggaattaccttccgtctgtggagtagagtcccgtcttctggagtctgtgaccttcctgtatagagatttgtcaaattttcagtgttagatttggaaaggaaaagccacttaataacatgacattttccccactagtctcccgtttctatttactgaaaaggttgtccgtgctgggcagaagatttattctagggcataaaggtatcttttatcaacctctagataccatggaacagtagttctgtggacatttcaagtaaggcatattggaagctatcttcgcccttaacttttagacttacaactctaggttttcaagctagacccggaaatgaaatcagcaatggtgtttactgctaattattgcctttatagccacccacattctgaaggccttgtaacagacagcacgaaaagattggtctgcctcagccaaggtggggctgaactggtctctttccaagctgtgttggttgtttttgcctggttgttcaggcggaagacaacaacatttagacacttaaaaatggctgacccaggttttggaacccagacaggcattttcaagtactgcattttccaagaagacttgaaaaagtccagtctatccaattactgagcccttgagtatggcagtgaggtttgaataatgtccagcactcggccttaactccctttcacaaatgaaaggttaaatgctggaagcaggagcacagcatggatttgctgtgctctcctgttttctttgccaaagtcacttttctccagtccttctgtggtgtcactggacaaagttatattgtgtctgtatttgctagcctggtgtgctccctgagtgggacccctggtcttgggcaactactgcatactatttgtgcaaagcaaatattttcttggcgggtggctccaggttaccttggctttcacgactctgactaaagaatgaaagattgaattgatgtcaaaactgtgcttgcagcctgcaatccaaatgcctgccgggccagtggccgaggcctacaacccaaaggcgtccgtatccgggagaccacagatttcaaggttgacaccaaagctgcaggaagtggggagctcggtgtaaccatgaagggtcctagtaagtgttcctttgtttctctatctcaggtgtggttttggctaactttgcagccatggcatatggatttcatcccacggccagttgtcctcaataatcccagaaggctatgtcaaggatttgaggctatctgggctccttggggaagacggcagtgattgattagtaatgtctgccctggatgcggccagtgggtggcttgacagctttacattacatcaagacttctgggagtagaaaaagcagtgatgtaaaggagttggggaaatgctgctgttggaacaagtggctcattttttattttagacatctgggctcagagaggaaggctcttgcctaaggtcatacagcgtttgtaatcatctgagctggaattcaagcacagtctccaaagccagtgattttcccactacaggttacattttatagagtatgaaattatgtcaagtacttaattactatgatcagtgcttatagaaggagaataaaattccctaagattaagttttctttgtagataaatgccatttgtggaggtacaggttaaaccctgcaacccattctctctccctcttttggggaaggagacagcagatgtggggatgggtgtcttcacttttttcgttggaacagagaagcatttcagcacttctagtctcgggtgtagcagcctttggtggttttactcccatgcctgtggaatcttgagcttcctgtaccaggattgctcttaccttctgtgttcccaacaggctggggcaggagcattctgagctccagaaagttaatatttgacttcacagcaccaggctttgggtcaggctgtgccctgagggtagccgaggttctagactgcccagacctggagtcaagctgcttggggactgtcttccctcccagattattccaacaggagccaaggagggtgtgtgtgtgtgtgtgtgtgtgtgtgtgcacgcgcgtgcatgcctctgcgtatgtgtgcgtacgtgtgtgttttctcctgaccttgaatacttgcttgactcaacggctttcctggccaaacctcagggctcaacacaaaacaagttcctgcctgatggctgggtttggagtttgcagcgtcacatctaaaacctgtcctcttgcagatagcgtctgaggactttcttgcttttgttgtccagctttagatggaaaagtatacgctggaacactgaacctaaaactcataccaaatacttctaaaggtttacttcttccccagtttttgtgggggactaggaagggtagctatgattattgggaaatactgaaatgtgactggatttatctttatgcaggcccagggagttcaggacctcagggcccctcgtagccaagcaagatttctaaagccaattagctgggaaatcctccatttcctcataccttgaagcagagatggctgtgtttttagctttgaaataatctcccaggctttgaggggagaggtcccatactctggggcagcccacttggtttttatgtatggtttatgttttgttcagtgtggctgcctctctgttcttgtccttttgattctcattttgggcctaggattgtgttggaaagattatctccttccttcccacagagggtctggaggagctggtgaagcagaaagactttctggatggggtctacgcattcgagtattaccccagcaccccggggagatacagcattgccatcacatgggggggacaccacattccaaagaggtgaggctcctgctgcagaggggtcttctctggagggtgctcggcccagggcggactcatgggtagttgcttcccgggctgcaggagggaaagagatctgctttgttgaaaactttttttttttttttttcggagcagcacagacatttggcctgttctcaaaagcagcagaaagttgctgtggttttagctgacttgctttaaatcaaatgctggtggttaggggctggtgggaggcaggggaggcagaaggagcagttagagcaaatgggctgtgtgtctagatgcccgcatataaactgagattctctttttcaatgaactcctttgttcatgaatgccacggggcagaatctgctgtggtttacattaagaccgtctacgtgagtgctgtcaggggccaagggacgcagtctacagctttgccttgtgggcattgcacttgcccctctgcgttctgtgttttccagctcccctggaggtgcaactttaaactccgaataaattcagttagccttgagaaatatttgggcattattgggttccgaatacctaccacgcttttttttttaagcctcccatgccaaggttacagcacattcattcatgtatgagataaagcccattcaaccaagttttctggttatagcataagcaggatatagtgtgtggactctctcactttccagggtcatagtctggggaggcctgcacacaaaggtaaagggccaggaggctggtgcaaagcagcgtggcttgagtgccaacccagtggccacctgagctcccagaagcagtcacattacattatattgttgacataacagtagctatgggtgagaggcctgcaggaggaagggcttggctgcagtttgggatgccagatgaaaggatcaggcaagtggaaagaatgtgcaaaggaactgcagcttatggctatagtgacaccttactttactcttctttgatgcttcttctattcctttccctgtagcccctttgaagttcaagttggccctgaagcgggtatgcagaaagtccgtgcttggggccctgggctccatggtgggattgtcgggcggtcagcggacttcgtggtagaatccattggctctgaagtggggtctctgggtaagtggacacagctgaccagcatcttctggaggactgaggattacagggcttccgggctgtgtcaggctggatgttggggccttgcctagcctcaatacctttagcttcctggcctcctggccaccctaagccatctctgcgtgctgctgtacatttgcagttgcctctgataccagcattgattcattcaggagaccttgagggcagaaaccttatgtgggtattgtgcctaaaacaatgcttggaacgtagtaaacacttagcaaatagtgttgactgacctttatagtttagatgaatgaatgaatgaattttgctgaaatttggatttggaagataaatatttcctttggagcacagctgaagtatattttaaatacatgtctaatgtatatatgatcattttatatcaggagtcagccagctttttctataaaaggccagatggcaaatattttccacctgtgggccttatggtctctgtcacagttatttgactctgccgttgtagcctgaaagcagctataggaatacgtaaacaaacgtgtgtggccatgttccagtaaaactttatttgcaaaagtaagcaatgggccagatgtggccttcagactgtcgtttagcaacccgttttaggtaatagcaataagcaaaagagaaaaataagaaatcacatttaattttcccttctagagagatgatatgaatcgtcttgtatattcttagtctagagataatattaagtcttttagtgtatccttctagacttttttctctatatatgcatgcaaatattgatttggtacagaaaatatcttagacaagtctttatatctttatgcgtaaatatagggtatgccttcattttccatagcttccatggaattccattgtatggctctatccattgtcaggctcttcagttatttccagggttttgctataaaaacagtgctgactgtgtatccttggtaattgccttcagataaaaacccagaagtggatttggtggtgctaagagtgggtgttggttcaaggcttttgccacatgttgccacatctccaacagaagggtttgctggttggacttcccctgttggatgatgataaaatacatataatgtatttaatactatatatatatatatatatatatatcctcctggcctcaagtgatccacctgcctcggccctcccaaagtgctgggatgacaggtgtgagccaccacacccagcccaggcctacatttgaaaaaaaaaaaatatatatatattttccaccccttccatctctactgaagacttaatgagcttggttttggaagaaagggatacaaacagatttcaatcttctggccaacacttggcttttagggaggcagcgggaatgagctgtcgtaacatagaataggtgctttccaccatataaccagggagacccttccacctccaccccctagggtttgccattgaaggcccctctcaggcaaagattgagtacaacgaccagaatgatggatcgtgtgatgtcaaatactggcccaaggagcctggcgaatatgctgttcacatcatgtgtgacgacgaagacatcaaggacagcccgtacatggccttcatccacccagccacgggaggctacaaccctgatctggtgaatcagctgctgtgcttctgtcttcttgtccctggcccctggttcctcacccccatgcccgaagttgccttaagcagcatgttgagagatggcagagaggaatcatttggattttaggaaggaaacaggcctgcatttgtttgtttgtttgtttgtttgtttgtttgttttgagacagactcttgctctgtcgcccaggctggggtacggtggcatgatcacagctcactggaacctctgcctcctgggttcaagtgattctcgtgccttagcctcccaagtagctggaactacaggcatgtgccaccacagctggctaatctttgtattgtttagtagagatggggtttcaccatgttggccaggctggtctcgaactcctggcctcaagtgatccacccgcctcggccctcccaaagtgctgggattacaggtgtgagcctccacacccagcccaggcctacatttgaatcctggtagtagcacttagcacttttatagtgttgggcaagtaacttacctatctgactcttggtgtcttcctctataagacaggaatgatagtagtctctgcttctagagagcttctaggatgattcaggaggtggcatgcataaagaccgcctttggcttatgcctggcccatgcagggagctccataagctgttattttcttgcaactccggggatcatatgtcagtcttacagccattttctatagttattatttcaaggtgctccatagataaaggatttttttttcctagttccgtgtctcttaagttggagcaatgtttccaagagtgtcctctcaaacccttagcaggctgataagcatcaagtctgagccagcctggctgacagggagttggccccagaggccacgtgtgctactgttggcccacacgggcagctgtccataggctgatgtcagtctgggctggtagctaccccgttttggccaaatgatattcctttgccctctagggcaaatgttgtccgtggtaaagattctgagtcccctcaaagtgggaacgttgaaactgggcatgactagaggtctctgccccagttgttagaagttctttaggtcaactcagaataaggcagggagcatgggttagtttgggcatggttttagaacaggggtttccaatattttgccttccctgggccacactggaaggagaagaattgtcttgggccacacataaaatactaatgatagccgatgaacaaaaacaaaaacaaaaaaaaaattgcaaaaaattttataacattttaagaaagtttacaaatttgtgttgggctgcattcaaagccatcctgggccgcatgcgggcttcaggccgtgggttggatttgtttagagagttttctcccttatgagggagagacatttgtttttaagttacaacctactttagcactttacttcccataaccaacctcttatgtggatactgtaaaaccagacacaggtcattttgttcttcccccaccccctggttacctgtctttgtataagggtttagttggggcattacacagaaagagacttactatctgcctttgcttcaggttcgagcatacgggccaggtttggagaaatctggatgcattgtcaacaacctggccgagttcactgtggatcctaaggatgctggaaaagctcccttaaagatatttgctcaggtaaatttcagggggccacctgtgcaggtaattgtcaggtaacaagatctgaccacgtaatggcaagttgctgagtccatctgatcttcagtttcctcatctgcaccgtggaaatgataagaagattatcttatagggttatgtgagggttcagtgagactaccatgtagagtactgggctttaaaaaaatcagctttctgatttatattctgtggaaatgaggcttgtttgtttcaggttattctataatgtcttttggtgtggctgaagctgctgaggccatggggggagatttgtaaacaaggatttaaaaagtatgtttatttaatctaattgaatttggccaaaggacttaaatgcaggaattgagtggccaaagctttgtttttgggtcacttgctcttaataactaaaaataaataaatgcatgtcatattttgtcactggttgtcaccgtgttgtgaaaatatggcacattgtagttggtccatgaagttttgttgtataagcaagtggtgacttggctgtcttgggaggccacagtgaccctgtctgatagagacagtgtgagggccacctctggtcctagctctggcttttttgcaggatggggaaggccaacgcattgacatccagatgaagaaccggatggacggcacatatgcatgctcatacaccccggtgaaggccatcaagcacaccattgctgtggtctggggaggcgtgaacatcccgcacagcccctacagggtaggttgtgaggcagaatcctggctgttttatggaaatgcctggtcatacaccaggtctgggatccatgcctgacagccaaggcagacatatggaaggaacccatccctggtgggccttgaatgatggaggggcccgaagggcagagtgctccagcctgctcagaagaactatttctaacaatgttttttaatagtattttactgggtccaagtggaggagaacttgatgaccttctccatgtcttctctaggtcaacatcgggcaaggtagccatcctcagaaggtcaaagtgtttgggccaggtgtggagagaagtggtctgaaggcaaatgaacctacacacttcacggtggactgtactgaggctggggaaggtgagaaagggctttgttcaacccagtgatcattgctccgtggggaaggcagttcttttcataacgtttcaatgccttttgaactaggaagtagtccatctgaataggtaatcatctactgagcctctgagtcattccttagtgatatctttgctaatccatcatccctttccccaaatccttactctttctcaggtttcttactagaaacttcccaattgctttttgagggtgttaacctgagctggaagagattgcacaggacatgctgtttcttgtaagctggtgctaataagctggtctgttccaggtgatgtcagtgttggcattaagtgtgatgcccgggtgttaagtgaagatgaggaagacgtggattttgacattattcacaatgccaatgatacgttcacagtcaaatatgtgcctcctgctgctgggcgatacactatcaaagttctctttgcatctcaggtacgtggtggggcctgggaggagatgggtggagtaggcctggattctctttggccacttgtgtgcatgtctcatctactttttggtgttttgttagtattattatttttgagatggagtctcactctttcacccaagctagagtgcagtggtgtgatcttggctcactgcaacctctgcctcccaggttcaagtgatcctcccacctcagcctcccaagtagctggggactacaggctcataccaccacccagctaatttttttttaatttgtttttatttttttattttttttttgagatggagttttgctcttgttgcccaagctggagtgcaatggcatgatcttggctcactgcaacctctgcctcccgggttcaagtgattctcctgcctcagcctcccaagtagctgggattacaggccaccacgcctggctaatttttttgtatttttatagaaatggggtttcaccatgttagccaggctggtctcaaacttctgacctcagatgatacgcctgccttggcctcccaaagtgctgggattctaggtgtgagccaccgtgcctggccactcagctaattgttttgcatttttagtagagacggttgcccagactgctctcgagctcctgacctcaggcccacctggcctcccaaagtgttgggattataggcatgagccaccacatttggcctcctttttggtgttttactgacagggaagttgtcttgagaacactgctcaatcgttttctctctggctccttacaaccaagaaggaaaaaaaatttacccagagctaaattattaccactttctaacaaaagtgaggcagtgtgttcagtggttaaaagcaggggtctggagagagactagtttgtaataaattttcatcaatattttggttgaaatgcagttagcttctagatatgttctactttgatgcctttgaagcaatgactgtggtctccacccttaaatttttatagagagaggtgatttgaagtttcaggtatgcaatagtgaagatagggtgagcaggatcctgaaagagagaattttgaaatcctagggattaaaattaaccttacataaaaatggaaatcttagtagaatgttctgtgcctaaaggtagtggtcttgacatccatttaacctcttctgcctttattccaatagtctgcaacattctttttgaagaattataatcattctgtctctgatcacttcttgcatttccccagaccttagctctcagctgtccctggaggacatttccttcccccagccccatgtattattgtcgtttttggttttattcttgttggcatttttcatcctgagtactcaacattcagtattaaaggctcaaagtcctcgggtttgtttgtgacatcagggatccaggcattagagagtgacctgttatagaaggccctttcccaatgctgggcccttttggcttatcttacccttctgtttacctgtggtaatagaagtctgctcaccactcgctaagtcagagtgatgctaaggttcaccctttgttgaaggctccctgagctctggctgttgcttcaggggctttcctactaagactgtgtctctgctacaggaaatccccgccagccctttcagagtcaaagttgacccttcccacgatgccagcaaagtgaaggcagaaggcccagggctcagcaaagcaggtaagatggcacgtctaggttgtcctgggcccctctgccagccggtggcactgggcgtgtttcatccacggccttgaggaacttcatctccaccaacaccaacaccaagctggcaggttttctgtgcagctctgatgcagcagtggctggccaggcccgttgctggctgtcataatagacctggtgctgttgaacctgtctgacgggttctcaaagtgaaactactccagctggtctgtctcctcacttcacagtatatctttccaggtgtggaaaatgggaaaccgacccacttcactgtctacaccaagggggctgggaaagccccgctcaacgtgcagttcaacagccctcttcctggcgatgcagtgaaggatttggatatcatcgataattatgactactctcacacggttaaatatacacccacccaacaggtagggtccttctcccctctgctcccctggcccccagccaggcccctttctatgcagtcggtgctgggtcactgtggacaccaaggggtgtgagaggtgctctgccaaagtgctccctgatgggaggcagctcctggcactttgaacccctctgggagcacctataggaagcccaatgggttctatcaggtgaactgcagaattccccaaaagcaagcaggaagctggtcccatatctccacctttggtttgcattttatcagagaaatgctcagttcttgatattcaggccctaatatctatctttctgttacacatgtgcacacatgtgcacacacacacacatacacacacacacgtgcattccctcgcggcctcaccagctgccttttagtcttttcattaattacccacagaaaaagagctgctacacctttgtgtttccttcctggtccttttagcttagtttaccctttttatgaggtgttggaatgaggtcttttctcaaagagccagttcagcctttcgtccctaaggcccagcacactatttagggcagcaaattattcccctttacaaaatgcaggatttcacatgtgatcttaccatctaggctggcttactctgattatttcaggccataagggccttaaaactgcctctctgtacaagttaatgtttatttgtttaaaaacattaaaaaaaatttgtatcgtggtaaaatacacataacacaaaatttaccgtcttaaccatttttaagtgtatagttcattagtgttaagtgcattcattatgtcgtgcacccatcaccaccatccatctccataattctttacatcttgtaaaactgaagccctgtatccattatatttgtttaaaattttgtttcgcttcatgttcacacctctggggtctggagagcagacatcctggcagaaaagtctggattttaatacttaagcctagtgttcgaagtggttgttccaagcctctgagattcctttattcttaagggaaatgatcctgctgtgtttgaaatgccatttgtaggagaagaagggcaacgctttctgcagaagcactgctcagaagccttgctcccgtctgggtcctctcagcgaggagcagtcaagagtcaagtggggaagaaagaggattatagtgaggaaggggtcatggtgtaactgtcccctgagtttgggggctgcactcccttggagatggaatccttactgtgagaacatccctgcagtgggagggattccctgggcgaagggattctgtgtgtcgtgttataaatgtggccccttacatccaggcttgctgctgtttgtgctttcttccccaaatttttatttttatttatttattttttagacaaaagtcttgctctgttgcccaagctggagtgcagtggcatgatctcagctcactgcaacctctgcctcccaggttcaagcgattctcctgcctcagcctcccgagcaggtgggattacaggcacatgccaccacacctggctaatttttgtatttttggtagagacggggtttcgccatgttggccaggctggtctccaactcctgggctgaggcaatcctttcacctcagcctccaaacctgcggatattacaggcatgagccactgcgcctgacctcagtatttgtctttttgtgactgatttatttttcttcctatatgtcctccatgttgtagcacgtgtcagaacttcattccttttcgaggctgcattccactgtatgtatatatgttttgcttctctcttcgtctgttttttgtttgttttttcttgagactcgctctgttcctcaagctggagtggcactgtctcggctcactgcaacctctgtctcctgggttcaagtgattgtcctgcctcagcctaccgagtagctggaagtacaggcacgtgccaccatgcccagctaatttttgtatttttagtatagatgtttcaccatgttggccaaggtttcaccatggggtttcaccatgttggccaggccggtcttgaattcctgatctcaggtgatctgcccacctcagcctccgaaagtgctgggattataggcatgagccaccgcgcccggccatcttcatttgttgaagaacatttgggttgcttccgtcttttgtctgttgtgaataatgctgggtgtacaaatatctctttgagtctctgcatttaattcttgtgattataaacccgaaatggaattgctggatcatatggaaatctctttttaattttttgagaaactactatactgtattccacagtggctgcactactttacagtcctgccaacagcatgcaagggtcctggtttctccacatccttgctaacatttgttttttttctgttttttttttttgttgttgttgttgttgttgatagtgaccatcctgttgagtgtaagatggtgtcttattgtggttttgatttgcattttcctaatgattagtgatgctgatcatcttttcatgtgcttattggtcctttgcatattttctttggagaattatctacttgcccatttttatatcaaccttcttaattttatgttgagttttaggaattctccatgtattctggatattagttccttatcagataaatgatttgcaaatatattctctcactccttggtttgccttttcacgccgttaacagttctcgtgtgcaggttataaacgcggcttcttatctccagacttgctcttcctgtgctttaaaataaaaaatccaaaacaaaacattcattattagtaatgataaaactaacacttttatagatagagcattcttttctcatcaggccactcaatagtaagtaggtaattattttcctgctgatggttctgagggttggtgggagccttactactgggtgcaccacgctgaatcttctttgttgccaaattctccatattctttaggagaaagcaccagaaagccatagctgtctgcgtacaatgactgggatcacaaggccatgacgtcttctaaaaacattttgtgacttctgctttattctatgtctatatgccttttagtgttttggctgagccgttagaaagtaagttgcagatatcaggacagggtcagggtttgacctgcatccttggaaaggactgcagaacccagtaccccagacgtcccctgctgctggttgaggcagaagtggagattaggagcctaggtccggttttgtcccctttgaagtaatgctggagtgggaggctccttacttcagagtcaccccaaggtcacattcatccagttctctgatagcagcaggtttgagaactgctgccatgctgagtactcacttagggctttgtgtccggatgctcccaggatgcattcaaggagccgggtgggccttggtggcggtcgttgccaccaagtggcaacatccaagctgcttgaagccacccacaaccccacaaccaagagaagagaagaccaaagtcctcaggtaaatcacaagtgtgaatgacttgcagggtggcactggggtccttcttgttgtttgttgcttggagctgggtttattgtttcattatttgggcaacttgcaattctgcctatttttctatggcaaagaacacattaaatctctccttagattgaatttccttcccacccccacccccagcacagagcctggccctataagtgctctgtgtggattaatggctgtgagtgagcgaataaatgacatggcgcctggattcacaagcggagatggcctaagaacgttgtaatctggtagaggagtgatgccaacacctcctcattctcctttgaactctgttttctgaagagcagctaaaagctcaagactgggctaaggaagtgtgcccttggatgtggttaagagacctgggtcagcccagaaagccaccccctgacacgggggagggagcatactttgagggctgacacccacaggcacaccttctcatggtagttttagggtataacaggctggaaatccccagaaaggtggctgcttgggcatgggtgtgtcctggcctggtgtgggcgcttccccctcagaacacaggctgtgccacgtggggagccgaggtcctgcctgagtaacccaggtccctgattgctggttttgctccctgacacctgcaggcctgccactccacctcgcaaagtccctgagtgacagcttgcaggtgcttgcctgcctggggtggatgagtgatgtggatggctgtaggatcctgtgagtcccttgaggatgcaaaagtagagcgcgttttgccttagaggaatggacttgttggcttggggcttgaggaccctcccagaggtcaaagactcggttttatagaagggaagtgatttccctgaggactttggtcttctcttctcttggttgtgggtggcttcaagcagcttaaatttctcaccgcacgttcccctgcgcagagcagtttgagaagctggtggcaatgtctccattacgtgctgtgctgggagccactaggattggggaccactccatgtagtactctggcacctttagaaatccctgtgagctcacagaccctcacagagtaacagcttctaccttgaaatgttcttaacgtggtggtcctggctgctcctggagggccctaaaagggatggtgctgagggtggctctctcagtcccatcctcttctgagctgtctggtcagtgtcttgtgtatgtatattttgaagaataagattcaggtttcagaagcatgtagaggagagtgaaactgtcttgcagcctgcgaagtcgtggcgaaatgcactggccatcactacccagacatccctcacttcatagccctgttggggaataaacacagtccattccttagttggggcctcaggggacactttaaaatgctgtaggcattgtaggtgtaaatctccgagattttttccctcccccttcttaggttatttaaggtacagttcattttctatctgagtttttgttttgtttttgactggtaacaagagcatactttcttttatgggatgggtgggcttaactggaagagggtttttccctctcttttttagcacttcagagaagaggccagaaaactttatgcgggtgagggaggaggtatccccaagacctctggttagcctgaggtctgcttagtgagcccctgaattgttaggggctgtggggaaacggaagctcgggaagagttggcacgttgggaatgccacgttggctgaagtagcgagtcagtcctgccttaaacagtacaaaaaggagacctttcctgccccttggctggctcccagctctgttgaatttgacctgtacacattttaccaggaaatgttgttcacatgaggcagggggccaattggttttgtgtgcagtgcttaaaaatgctggaaaattaatcctctcttcattgatgcaaccagtttttttttttttttcttggcctttacccccttccttattacaaaaggaatgtgacaaaatatacataggccaaatgctacacccttttaacacttgatcagcaacagctttcagcagggcctgcattccagcaaggctgctggattcttggggggaactcgtctctccctcacactttcctgttacattatgcctggccgattgtggtgaaggggatcttgatctactgagacagccatgagatttcttggagcctcgatttggagggagggaacttggccaaccatggagagaagaagccggctgtgtgccagcctggaaccggcgagaggagagaaatggcgcacacatggctatcgcgtgccacccggccacccgtgagggtgcctgccaatcctgcaagcaccatctgccttcacacttgcaattttattttctttcacatggaaatggaagttcagatattgtgcgatggtcttagcacaggtctaggtgaactcttgcaaatccctgttgcagcctgggggcctcaaactgattcctaggacagaaatggttctgtttggtgagtggccccaggcccagctgcactggctggcactgggtatgatgatggggaggtggtgtggcagagcagctaggacacagatttgggggccatgggtatgaggcccagctcgcacccttaccaaggtgtgtgacttggggcacgttcctttaccagtctgagccacagtttcctctcctgaaaaaatgagatgacagtaggaactaccccttaggactgttttgatcttgaattgaggaaatgcataaaagcacatagcatggtgcttggtgtgtagaaaatgctcattaagttgcttctgttattattagctgctcttatttgatctaatttttctgttattcttgccttgtggtcaaaagctagaagaaatagatctaagatactttctacattgattggaatcaagtctcccctgtccgtgagaagaatgagggatcttgaggggattttaaatgccaagttagctttttggtacccaaaggtaaactgagttttctctcttgttccagggcaacatgcaggttctggtgacttacggtggcgatcccatccctaaaagccctttcactgtgggtgttgctgcaccgctggatctgagcaagataaaactcaatgggctggaaaacagtaagtgcctgaatggagagcagatgggttgttgatgaccccccaacgtggctgctggttagattttcttcaaaaggtgaaatttgcagagaagcaaattctatgttaagagactttgcagttgcacagactttggttcgaattaaggccgtggtgtgaagtaactgtgactgtgtctgccccttagccacaccgagactcagctttctcatttgtacagtggggggtggtcggcggggagaggttgagaacacccatgggaatattttgaaaattatatgagctaatggttcagaggctggcacgtagtcagccccctggcattgcagtaggaagttttcattaaaaagagaatttgggctatgttgctttctgatgagtttctaactgtgccagctatccttggcaactgaatccgcactaaggttgcgagtcaagcataaatgccaaatccctggcactcagaagtcactaccaccacacctctgccccatcccaatgttcctttagcttgttagggattttactagtataagctcatttcgcttattttcaattttctgattattttttagtagggaaaatttcaaacagaaaaggaaagagaatagtataacatgaacactgatgtacttatcactcagcttcagatgtgcaacacatgctcataaaatgatttttttatacaagtaaaaatatatccatttttcatctaaaaaacattacagttaagggataattccactttaaccctcacctctccttctccctagggttaaccaaagttttcaattcagtttctgttcttccagatcttctctctgcatctatacatatagatgtgcctgtggaacacatttggctgtatttattttgcattaaagttgccctgctgtataaacctacttcttcggcctgccttccaacagtgcatctcgggaatcattcactcctacatcttttccgtctgtgtttactgctgagtggctccagactggatgtacctcagggctcacattcacctggtttcaggcttactgaggcagggctgagtgcatacccccaggacggggcctcctgtattcacctgtgagggtttctccagagtaccactagcagtgccattagtgagcatcttccttcactcgtgacccaagtgcacaagttgcaagcaaggccagctcccagttgcagagatccaaagtgagagctcactgttggcttttgtggctggagcagccagctctgagtgtgtaaacgtccactgcccaaccctgtcatgtgtccccttgtcactcctttccccaagacactgagagctttgactccagaacaggaaaagcagggtgccaattaggaaagcctcttttccggtgggaagtagcgatccgggacctccttgcctgtggttcggcagtgtccatcttgccaggccctatgttccttcagagtcaaggttctctgggttgtggcaggggccctgtgttcccagtgcttttgttttgggtaaagtcctttccctgttcttgtctaatctaacacttgggcttcctgcagccctgctttgcagagaccttttggaaaccatcacggtacagtcagttctcagcacttgcttcaatcggctcgcatttggcagctctgtgacttctgctttcttgagggggaggggtgcctataagatggagttggctgccaagaattagtaaataaaacattgacttatgagggtgtttggatatcaagttaacaccaaaagtaagtaaataagagacgacagtgtcagattacaactttctggtcagcaaagattgtggggtcaggtaaatttcactttgagtcccagcttggcaggctgctgcatatgtcaccctggacaagttacttaacctctctgagcatcagtttccccatctgtgaaagccattggttaataataaataccccataggattgtggtgaaaattaagacaataacctatttgtgcttggcatataaaatgcattcagtaaatgatagccgttattgctgtcatcactaattgattattgtgccgacacttgttgttactgaggctgagatgctgatgatacttactcagctttgctgcttgtcctctgcagcagctgttgcttacagtggaggctgagataagtccccgtgtccaaagaaccattgcttctgtgctctggattgttcctgctgctgaaaagggtcagctcttcacctcagcttgtgtttcttttccaggggtggaagttgggaaggatcaggagttcaccgttgataccaggggggcaggaggccaggggaagctggacgtgacaatcctcagcccctctcggaaggtcgtgccatgcctagtgacacctgtgacaggccgggagaacagcacggccaagttcatccctcgggaggaggggctgtatgctgtagacgtgacctacgatggacaccctgtgcccgggagcccctacacagtggaggcctcgctgccaccagatcccagcaaggtcagcctttgcttttgtcccagaacttgtctcattgctgtcaaacatgacaccatagtccttctctggttcttcctggcaaagaccttctgaaaatcgttttgtgatgaaagttagcacaattcactgtgaaaggtcccctgggtaggtgggtcacaaccctgctcctcctcttgctctctgactacaagactttggtgaggggctccctgtcccagagtcttctttcttcgcttgttagcataatcacagtcctcactacaaagccagcctgtaaggggtaggtgagttagcaaacgtggaggcctctgcccagcacccagctcacagacggagctcaccctccagaagctagaatcatgtaatataaaaatacattattctggccaggcgcggtggctcatgcctgtaatcccagcactttgggaggccgaggcgggcggatcatgaggtcaggagatcaagaccatcctggctaccacggtgaaaccccgtctccactaaaaatacaaaaaattagctgggcatggtggcgggcacctgtagtcccagctactcgggaggctgaggcaggagaatggtgtgaacctgggaggcggagcttgcagtgagctgagatcacaccactgcactccagcctgggcgacagagcaagactccgtctcaaaaaaaaaaaaaaaaaaaccacaaaaaaaaacattattcttggctgggcgcagcggctcacgcctgtaatcactgcactttgggaggccaaggtggatggataacttgaggtcaggagtttgagaccaacctggccaacatggtgaaaccccatctctactaaaaatacaaagattagctgggtgtggtgacgcatgcctgtaatcccagctactcgggaggctgaggtgggataatcgcttgaacctgggaggcagaggttgcagtgagctgagattgtgccactgcactccagcctgggcaacagagtgagattccgtcccctccaaaaaaaaaaaaaaaagttcatcgtcatttcttcatagtaaccctgactcaaggggttttggaagatttccagtggtctcaatggtgtgaatcctatgaaggtgtcttatttgttgaattagaggtgaaagcctccttcctcactcttttttagaaacagtttagttttattattatgcagaatttgttgagcaaattgcaacagcccaagccacagctagctccacaagagcccttccatgagccctcaacctgggatctcgtgtatctttgttggaatggacattaggtttccaagtccaggcctgtgatttagaagggtcaggttgggtaggagagaggagagtcttggaggggctgctccatgggggtcacacctctctcctgtgggttttcgctggtgattgagttctgaggcatttgctgcattgactgttgtagctttaactcgtgtgcacgtgtgacacataaagccccaagagaagggctgcctggctcagatgcacttccatgctgattatatgcatgggtgttgaaagcagtgctggctgagcagcgatcccagtgcagtttgactttattctttgctcaaataggtgaaggcccacggtcccggcctcgaaggtggtctcgtgggcaagcctgccgagttcaccatcgataccaaaggagctggtactggaggtctgggcttaacggtggaaggtccgtgcgaggccaaaatcgagtgctccgacaatggtgatgggacctgctccgtctcttaccttcccacaaaacccggggagtacttcgtcaacatcctctttgaagaagtccacatacctgggtctcccttcaaagctgacattgaaatgccctttgacccctctaaagtcgtggcatcggggccaggtctcgagcacgggaaggtgggtgaagctggcctccttagcgtcgactgctcggaagcgggaccgggggccctgggcctggaagctgtctcggactcgggaacaaaagccgaagtcagtattcagaacaacaaagatggcacctacgcggtgacctacgtgcccctgacggccggcatgtacacgttgaccatgaagtatggtggcgaactcgtgccacacttccccgcccgggtcaaggtggagcccgccgtggacaccagcaggatcaaagtctttggaccaggaatagaagggaaaggtgggtttcatttaaaaaaaaaaaaaaaaaaaaaaagacaagctgggacttaagggctacctgaaacttggagctgcaaactcagccacctgcaggagccaggtgacatataaggcggtgctcacctgttccctctgcctcggggagtagttggggggccctggtgaaggttaagcacattgcatttctggggaccgtgctactcaacccctgttttctgtttctccatggggaacaggacctagcattgtcagcagaatctctagttttttggcaaaggcagaaatcttgatttttctctggaaactcaacatacaacatgttggcatttaattggaaaaaagtttaaaatgtagtgttgtctaacacctgcatgccacacagcaggttagtcttcaacctttaacctgtcctcgagcccggtgtgagcagtcgtgttgtcacttagccgtggctactctagaaaggccttctttgggatggagggggttaatattcttgatttgagagttagaaaaaccagttttccagttactgaaattggacttcatgtgtcctgaagtgccaagaaccttggttctggggtttgcttttgggtctggggtactggtggcagtgttagctatgtgcttgctctgcagatgtgttccgggaagctaccaccgactttacagttgactctcggccgctgacccaggttgggggtgaccacatcaaggcccacattgccaacccctcaggggcctccaccgagtgctttgtcacagacaatgcggatgggacctaccaggtggaatacacaccctttgagaaaggtgagccgccctgtcctcggactggaccctcgttcagagctgcccttggtcattgcctcctggtggctggtactgatgcctgccccatgtgctaggcctgtctcagcagggccacgtgcagagtgacagagtggaagtcagcgtccgctgcagtcacctgcccactcagtgcctggcttgctggccttgtgtaataggtgggctgggtttagcctcagtctcacctcagcaagttatggggtaatgtcatgatgttgctcatttgtgccatttttctttgcgtatgaatttctttcttcttgagtattaggaattataaaaaatttcaataaatagaaaaccataaagaaaaaaaagtgccatgtatatctccactacctggagatcggaagcctgcgatattctgatatagatattttcagtcttcttgtggatgcctgtttcttctgtttcacgggtttcgctttttcttttggttaatggctggatggtgttttcccgaatgagagtagtctgtttaggatgactgacttgaatatttgcttggttggggtggagtggcttatgtgactgcagatagacggtttgtattatttaaaagtcagatcatacctacattactgtgggattgttttgttttgttttgaaacaggatgtcactctgttgcccaggctggagtgcagtggtgtgatcacggctcactgcaggctcaacctcctgggctcaaatgatcctcctgcctcagccccctgagtagctggaactgcaggtgtgcaccaccacactcagctaatttttgtattttttgtagagatggggtctcgccatgttgcccaggctggtcttgaactcctggactcaagtgatctacccacctcggcctcccaaagtgctgggattataggtgtaagccactgcccccagccacattactgtgtttttaacccccttttccaaataacatagtatagcatgcagacttcgatgctagatgaaactctgaagtagagaatcatttttcacaaataggggatttgtatgcaaatatgcgtttctgtttgttgttttgagcaggtctccatgtagtggaggtgacatatgatgacgtgcctatcccaaacagtcccttcaaggtggctgtcactgaaggctgccagccatctagggtgcaagcccaaggacctggattgaaagaggcctttaccaacaagcccaatgtcttcaccgtggttaccaggtaggcaaggccctacatttggtgtcttgagtctcacttttgtggctagattctacctatgtgtcatggtttcctaacttttgataagatgaatttttatttttataacatgtatttccttctgtagagacttatgttacatagaaagaccaagcatacctaaaaaacataccaaagcacttgataatggtcatgaaactatttagcaaaccaggagtcaatcaagctctataacttgataatgtaaaaatttgtagccaaccttgtaagtatttttattaaagttggttgcaaggcatatgcctgcgttgtacttgcagtcctagccagtgcaattagataagaaaaataggctgggtgtggcggctcacacctgtaatctcagcacttcaggtggccgagacgggacaattgcttgaggccaggagtttgagaccagcctggccaacatggcaaaaccccatccctacaagaaatataaaaattagctgggcttggtagtacacgcctgtaatcccagctactacttgggaggctgaggcatgtgaattgcttgaacccaagagacataggttgcagtgagccgagaccgcgccactgcactccagcctgggcaatggagtgagactctgtctcaggaaaaagaaaaataaatgaagcataagcattgaaaatgaggggtcagagtgtctttacttacattatactaatgtgaaattccctatgtgagaggtgtagtaattgagttggggtggctacgtggaatagtttataaagggaatttgcatgaattttggcaataagcagaccagcataaataaatggtgcacatttcactttcttttccactctttccagaggcgcaggaattggtgggcttggcataactgttgagggaccatcagagtcgaagataaattgcagagacaacaaggatggcagctgcagtgctgagtacattcctttcgcaccgggggattacgatgttaatatcacatatggaggagcccacatccccggtgagctattcctcagagaggaccccagagaataattgattttgcaggaaaatgggtttgattttggttatctctctgagtggggaaaacaatctgatatttgtaatagctgcaaaaggagagtttttcttagggctacatctccaagattatctcaactcccagtagaaccggtaacatggcaaaaagcatcggcttagaattttgactggaaacagttgtgcgtgtgttggaggacctagttcttgattcaggggaaagctggttctttacaaagttgaaaatcacagtggctcacacctgtaatccccaaactttgggaggccaaggcatgcagattgcttcaggtcaggagtttgagaccagcccaggcaacatggggaatccccatctttacaagaaatacaaaacttagctgagtgtgatggtgcgtgcctgtaatcctagctatgtggggtgggggctgtgatgggacgatgtctgagatgggagcctgggaggttgagtgagctgagattgcgccactgcgctccagcttgggtgacagaggaagaccctgtctcaaaaaaaaaaaaaaagaaaaagaaagaaaatttctaccttattttgtgcttggctccttattcatgtgtcttggtttcttttttttcactgacaatactagtagctgatcaagatatgcagattcaaattctttcttttgtatttagtgatgtcatgtgtaatcactgtgaaacacggtttctcaactccggcactatgacactttgggctagatgattctttgtggtgtggggctgtcctgttcattgtagacttttgtcagcatccctgccctgtacctgctagatgcccatagcagacttctccttccccattcttatttgtggcaaccaaaaatgtctccatatcttgccagatgtcttaagggacaaaatcacttcagcctgaaccactgctgtaaagattcaaacaataaataaatatatgacttaagtagtgaaagaccctcctccatttgttttggggggaggactctccataggttctagttatctactcaaatgattgtcacccccacacattttatttatttatttcaatagctttggggtacaagtcgtttgtggttacatggatgaattctatagtggtgaattctgagaccacctcccccgcccccatttctaaaagggcaggcaagtgtgtggtgtggacagaagaccgagggctggggctgttctgggccacttatgccttgtcttaggtgtggtgtgaagagggcaaagccccaccccaggaccccaggagcagaaagagcctcagcggggtcttgttcttctttctctgggtcacgctgagaggggaagggcaggttgaggggcccactgctgggttctgggttaactctcaggcagctggagtgtccactgaccacacgctttcctgattccattcctgcttcccccttaccacatggaaatgtgcacacacactcacactcactctctctcacactgatcagaaagtattgacattcaactcagactgattctactcagatactcatttaagcctcaagtcatttaaaacaacatgtttctcctcaaacttgtgcttgcggctcattcaatatagatttaaaaaattcctataatcactagtctaggggacttcagctgtgggcaagacaaagttcctgccctcagggagcttactgtctagggcttttacaactaaaacttgtgatgactgctatgaagaatgagaatggggctcggtgacagaattcagagctacgggcttgttttggagttttgtaacacttgcgttaggagagagttgggcacaggaaacgggtagaaggctgctcccaggaggggtgatgtggctccgacctggcaggcaacagtggagatgaacatctcctgtggcaatgaaactttttgactatggggaaaggctggtgagtgccaccagcttccgaatcccccttacagaaaggggtcagagtttgtcccctgtggccgacctgtgagcttaaagcaaatggtcgtctttgagcataacaacagaaagacactcatttgtggttttcccatcaggtgtggatggtgcctttttatgtttcaggctctctgttgcctcccagagagccaaatgccggcttttccagaaccccagaactttcccaggcagagatatttagtgaagtgttggttggttttctaagcatcaggcttcttagctaaggcaacctatgggggtactgccgggaaacagtcggctacctgccaccttctaatttgctttcatggtaattctgggtgcttaaatattagcctagtttttcctggcctggttaaaaacccggagtggagttatttttaacaacgtgtcctgtcttacccgtaatggcatgttgatttcctgtggtaggccagctgtggttggttggtggcggctccctagaccactggattgactggggttcagagtgcatgaggaagaagatctggcatgagggaatggtgacatgtgtctgggcatggaacaggggagtggcggataatgcttggggtctgccatcttggacagtttatcttacccgggtttgttggtttttggctactctcatgctgagctcagacaacttctagtggaggctctgacttaaagattggcctcagaggtagtcccttgccatcagctgttgacattgaaatcctcaactgtcactctctaaagtaaagcccccttttgttcctctcaccccagtgtggaggcctgtgcttgtttgccagggccagccatttatttcacgtagctaaagacctggatgccgttgaaacccagctgttgttagaaagccagggactcaattctttgtgtgtcttggctgtctaccatctctaattctacaaagtataaattctctgggatgcaaagcagagatccctcagctttcacggcagtcattaactttgccagataccatggggagcaccaggactcccatgcgaggcagaggtgcacgtagccccttggtgatgggcgtggtagcctgaggcatgctgccgttcgctggatggggaggtccccctccacagtggagtccatgagtgtccttggcctagcccttgtttctctgtttagcacttctctagcaaatcactatctcctctcctcgactcctctgtgcttcatctttaaaactgacaccctcaaggagtcagaggccctcagggtcccccggggggtcagccatgtagcaggagctcagcttacactcaggaagacggcaaggcttcaccaggtggccgagtgaccgagaaggctgagtgtggtcagaaggtgccagctgcattggagggagaggagtctgggggacacacaggagccatgtgtgggggacagggctggatgtgggctgcagggcctgcccatctctctccgttctgttgttccaccacttggcttcctccttcagttgctccagcagcctgtctcctccctcgcctctaggctcctgcatgtgctgaggcctctctacttgaagcacctctctgtctgctccctcttgtgccgcaactgagatgttactggaaagctttctctggtctcccgcagaccaggttaattgcctcctgagtgctccaccttccacaccccaaatatgttatgtaggatgttagagtgacttgcttgcctcatccttctcctgcagttgtgggttcctggggggtgttaaccgctcaggatccagcacgtggcacaacatctgcacgtagtaggtgttctgtgagaatggttgacaacaatgagtaggcacatgagcagtgcacacagtgaggcagggggagctgaccgaggcctgcatggccgaggtcccgggggagcagcagtgctattctgggtgtgcacaaggtggtctccaattcccagcttgtgctcagaatcccacaacctctcttccaggcagccccttcagggttcctgtgaaggatgttgtggaccccagcaaggtcaagattgccggccccgggctgggctcaggcgtccgagcccgtgtcctgcagtccttcacggtggacagcagcaaggctggcctggctccgctggaagtgagggttctgggcccacgaggtaagtgtgcaccctgccttcctgcagacattcatctgccccaggcaggggcagctgtaacccagagcagatgctttgcttttgagtttgctcatgagcttaaaattaaattaaaaaaaattattgtttcatttctagttaaacagtagaaattcctgcttacaagtaagcaggcttgttatttctccagtgatctgtccccccatttaataatatggctatcaatttcttagaggaagcagcagtatttgggctgtcatatgtaatatggtggcgactgtttcattatgtgtttcagcatttgtgagggggtgggttgctctggatgtggcagatggtggggtttggaggtgataactcattgagatatcttggtgtccatgtggtacataccagaacctctgggaatgccaggcacatgatgcacgtgatacgtggctttgtcattgtcttagttccccagagagagagtgtgtcttggggaatgggctttgttggcaatttggcctgccttgttggcagcttggaacttgggtttggtaaggctagcgggccatatagggacaaagccctgaagtgcattggaacttgccttttttgataagtgaccatgtttcctcctccagcacttaaaatgtgcctttctcccacatagaggacagtgtgcctaatttcttacgtaatctggattttcctcgccaatgatatgttcttggattcacagaagtggcaaatggggttttccctctttgaagaggaaccttctccttcatggggttcagcaggaggttttatcttttgaagctcagggcagaaatggtttgggggaaattaggtcatgggtctgggatcagattctgtgaagttactgagcttcaggacctgcatgtgtttgtgtgcatgtatgtgtccctgtgtatgtgtgaatgagagagggagaaaaagaagaaagagaagctttacttggatatctgcctctattatgaaggactctcaagtaacagccttttgattttagctgacgacacggattcccagtcatggcgcagccccttgaaagccctttcagagttctttaaaggtgacccgaagggtgactttaataagacaggtttgcattttcccatggctgctgaattatgtaacccaaatgcttcttgctggcctcacttctaaaattgcttacacctgcctcatctgctttgcttaatgagcatgccatcctttgattaacctaccctggagttgacccatccttgactgtcacgttggaagctgggatctggactctgcaacccaacgcgtgccttgattatgttttagcataatctctaacatctccacaggcttcaccttgagggtccccttgccccatgagattggcaccctcacctgccctgcacctatgccccagcatgctggtaccacagtgttctttgctcaaaggtggccacaagtcttgactagccagcccattggttaatttttgctcttcacaattctggactctttggcagtgtctcagctgtagagtaaaattgccacatcctaagcgtgcctaaccagcttgaaaggttatattgtgtcttcaacacacatcatccacatacaccctccagcagcaagcacaggcagtctccttaattatactctagggcagactgagtgtattttagccaacaaaaagctaaaggtgtctctcggggtcatttctgcaaccatgaattggggatcctgtgatttttttcaggcctgtgattatggttgctggcctttttgttactcatcagtggaaaccaatagctcttggggatggatgtggtcctatttcagactcagccaagggtggagtaaaggtgaggccaggcagctccttaaacctctcatctctgtcctcaggcttggtggagccagtgaacgtggtggacaatggagatggcacacacacagtaacctacaccccatctcaggagggaccttacatggtctcagttaaatatgctgatgaagagattcctcgcaggtaagctccatccatctgcccatccattcctccatcagtctatctgtccacccatccattcctccatcagtccatccacccatccgttcctccatcattccatccatccactcatccattcctccatcagtccatccatccacccatccattcctccatcagtccatccatccatccattctttcatcattccatccatccacccatccattcctccatcagtccgtctacccattcatagaggcagcaagtattacatagaacctgcaacttgtcaccacacactagccttgatatttgtggctcccgctctctcactcccccagttcctttcagacatctttagtttaaaggtgagctgaaattaagaagttggaaatcctaaccacgtgtggtgggattcgcctgtaatcccagctacttgggagactgagatgagaggatcacttgagcccaagagtttgaggccagcctgggcaacatagaccctcccctgacatctctggaaaaaaaaaaaaaaaaaaaaaaaaaaaagcaatagtagtagacaatcattgatgaaataaataatttattagtttattagaggcttccttttggtgttttggtgaacctgcaagtagttttctgattgggacaggacaaaggtctttacttcagggtttgcttgataaaagcatttccaaaaggttttacatagaaaccttgttccttgttgatattaatacaaaaaaaaatgttacataagctcttcacctcttggaacaatctctaagggttttcttttctttttttaaaaaatcatgccccttaagatgaaaaactttcacccatatcccctaacacatattttatatagagataagcatattagctctatgtagaaatatgtaatttataaattacatttgtatattgctttactaatataccatgtaccatatgaagcatactatagaataattatagatacagaatatagaataagatgagatataaatattaaaactgaagttccagtattctctttccatttggtgaccatgatcttagcataacaaaagtggggtaaatgtgtttaaccctgtgtttcccaaactaatttgtgaactcttcctccccaaactacttgtatcccttggaacagaggtccccaacccttggagcgtggactggtgtgggtgcacggcatgttaggaattgggccgcacggtggtgggtgagccatcattactgcctgagccctgcctcctgtcagatcagcagctgcattagattctcataggagtgcgaaccctattgtgaactgcacatgagaaggatctagattgcacactccttgtgagaatctaactagtgcctgatgatctgaggtggaacagttttatcctgaaagcattcccccaccaggccccctggtcttctacgaaaccagtccctagtgccaaaaaggttggggaccgctgccttggaacacactcaggacaaaaccagtctgtcatatgatggttactacctcatagttgtaaatttctgctagacttaggcaccttgactaactcactgtcttatctgctgtagaaatccccttttccatcccactcttatgtgtaagaaaagtcagatgcagctgggttgacatgtatctttattgactagggtgtgtgtgtgtgtgtctatcaagtcccttcaaggtcaaggtccttcccacatatgatgccagcaaagtgactgccagtggccccggccttagttcctatggtgtgcctgccagtctacctgtggactttgcaattgatgcccgagatgccggggaaggcctgcttgctgttcaaataacggtaacttggagttattttctgagccaaaccttaatcctaagacttaatttctgggccagatttaagaacaagggtttcaataaccgatttctgactcaatgcaagttgtttgttagattttcccaccaaagagtcagtaaatgtgcagaagcagaagcagctcacctgagagatttgagggtgtagctccaagaaccactttttggtgaattttcatgtttttttactacatctattcctatgtttttatttttattttttttaaagatggggtttcaccatgttgcccaatctggtcttgaactctcttgggttcaagcagtctgcctgcctcaacctcccaaagtgctgggattgcagacatgagacactgtgcccgtcccctatgtttttatttttaaatgttttaaattactctttggttcatttaagactaagttatgctgcatatcacagtaaaccttaaaataagagtggctgaaataaatgagattattctctcttgttaaggaaccccaggctaagccacctgggtgccctgcagctcaccaaggaagtcagctccatctctctgctcctctacctagcatgtggcttctgtccttaaggtctcctcctggaccataaggctgccagtgctctggccatcacatccacatggcaggccagaaggaggaagaaagaagggaaaaaggggtcctcccagctcagtgggctctcttaagcagccctgccaaaagtccatcatagacttccattcccttctgatttgttgggggttggtcacaattcacattacctagtggcaaggatgctaggaagtggattcccatcttctgggagcggtgcacctagctaagagttatggtcctgttaataaagagaaaagggagactggatgtggtggtgtgtgagcagaagcctctgcctcctcccctccctacatttcagaggatttcgagctaaaacactcttggttcacctgacaacaaaattactaaaaattggccatgtctgtcatggtgttaaagggatctgtgaccctctactctccctaccaaaaaacaaaacaaaactagattgtattaagccatcaattctgtctgtttccactagaggcactaattggaaaatatgtcagggttttccatgaatgttttctacatcttgacaacatcctaaatagcatttctctatgatccacaggaccaagaaggaaaacccaaaagagccattgtccatgacaataaagatggcacgtatgctgtcacctacatccccgacaagactgggcgctatatgattggagtcacctacgggggtgacgacatcccactttctccttatcgcatccgagccacacagacgggtgatgccagcaagtgcctggccacgggtgagtacagggcatctcaaggtcaggggcacaggctttgcaatcagaaagccgggccgtagcccttctctgtgacttacaagctacatgatctgggcacgttgctcaacctcactgaacttcagtttgacatagattgaagctctttgtttttatttggagaacatttagatccaagaagctcttctaaggaacagagactgttttacagggttactgcaaagattagatgaggtcaggcatgaaaaatgcttagcacagtgctaggtacatgataactattattatatgcttttgaaatgttgagaacccaactctgatggcggctcccatgaaaagcagcacatttctgccttttatgagtagatagttactcaggattcattcaagagcatttcaggtcagcattagagaaacacatttaaggatctaggtttttttcatcatgcatatgtaaacctctcaggaattctccatgaatatttgagcatcacagtttctttggtttctttctttttttttcccctcctttttccttcagtttctaagacacaactattgactgtcacaggccattctttttttttttttttttttttttgagatggagtcttgctctgttgcccaggctggagtgcagtgacgcaatctcagctcactgcagcctcagcctcctgagtagctgggaccacaggtgcccacgaccatgcccggctaagttttgtatttttagtggattcagggtttcaccataattggccaggctggtctcgaactcctggcctcaagtgatctgccctcctcagcctcccaaagtgctgggattacaggtgtgagcaccacgcctggccggcctttcagtttttaagaacagcccttgggcagctcagtgctgctgctcaagcagattttaaaacacgaatccccatctctaaaatgagacagatttacttctttttaaataagaagactaaacacaggaccacccttgatgtgttctgtttctctcttagcccatctttttttgaatggagaaaatctgggctttcacggcaaggttgtgaattgctcagcgtggccctttttggctcacccatggcaaaaaatggaaaaattttggaatgcaggccaatccaccacctcctaggtctatgcagctgccagcgacaaccagatcatctttactaattgatggcatgttaacgttggatggggacttcccccttgccttgcaggccctatttcctcccccagcttgggcagaagcctgagctgaatacttgccttttggccacacctctgggtctgtcattcagggtcttccacagattgactccagtcttctcttccactcctccctgaacaaactgttcttgccaccctccctattactcctacgcacttggctcatatctaccaatgtgcttttagttcatgcttttctgcatttcctgatatgtggatcctgtgtaaaggggcgccagaaatcaagagagagactggtcactggggagaggttgcaagtctcccttagctaacagcacccatccttcagggttcagccatgtttcctttctttaggaagccctttgtcagtgcggcaaccctgggatataaattcttagaacctttgcctagatatgctgccagacacttctctgaggaacagtttgttattttttctgtaacttagttcctcttcagcatttccactgcagttggaaatgtcgttcttggtgcctggccctgttaacatcttgagagcagggactgtgtcttgcccacctttatgtgtacctggcacttaagaaaatgcccaatatgtttgctattgaaagtcaaccttcattgccatacctttaaatgctggcaaacccaggctaacctttagtcaacactcagagcttacagatgctccttatttagtaagtaattgatgacgtaaccctttgagcaacacctgatcaggggatctttgggatatccctctgaatggcagcagttggaggcctaacatttacaggcacagacaacatggatgggtatgatttgttcttgggcctccaggatgtgtgtccatacttccattctcttcccctgaactcttctccaggtcctggaatcgcctccactgtgaaaactggcgaagaagtaggctttgtggttgatgccaagactgccgggaagggtaaagtgacctgcacggttctgaccccagatggcactgaggccgaggccgatgtcattgagaatgaagatggaacctatgacatcttctacacagctgccaagccgggcacatatgtgatctatgtgcgcttcggtggtgttgatattcctaacagccccttcactgtcatggtaaggaaaattccttctcccgagcatgctgttattggtggaaactgtaacagctgccgtttgttgaaccctgactaggatatcctcttcaccttttttttcctttggaaaaaaatttgttaagcagtcatgaccttgtagagtcccagagtaatctctagaaactcagagaccctttggctgtaagggtttttagggaatcttactggccaccaaggtgtctatcataataagggacttgggcaatatcctggcctaagcccaggcattttgaaagataactcctcagaaaaacacacctttatgaaaatgtttctacataaaacatgacaggtttttaaccggccagctcttccttcttccatcttcatggccattctccatggctggaggagagagcttcctgatgctgttttgtttggagacttgactctgaaatcccaggactcaaagtacctccacttgtgttttggaaagattcacactttatgtatgagggggaaatacctcgtcttttgcagctaggaacatctggaataaaaggaggaaaccattatgcaaacacctgggttagtgaatgaccaaggtctttcattttcagttgtgagttacttatagatcttcctctgtttatttatttttattattacataatagatcttcttctgaatattcttcaaccaggaaaagggttagaaaccttggggacattacctcattgaaccctcaaaaccaagcatcgttggcttttttacaaatgaagcatgcttggtctagacagacaccaaataccatgctgtcatcctcactggtgtcctttgatactgtggtcagcagccgcacttgaccacaaggtttataggcccttaatgacctggccttgtgcacagccgacaaagcaccttctaattatttcattttgtgcagcaatggagaggtgcatgaagactccattccaaactccaaagctcagggactttcttccgaacagtctatactctgttgtagtattattcccttccatcgacgtctgtttatctgtaaacagcatgccagagatctggaggctcttttatgtctcaagtatgtaaatgtaaacacttgtcaacttttgacattgttcatttaagagtgtttttctcctgtaggaagaaagaaatacagctgggaagttgatgtccttattcacagagaagggtaccagttgtagttttcagaatctgtttttagcccatagtgggttttatctggttggttagaattaggtggaaggagggaagagcagccaagcactgagcagtggtcatgggcctgctggtgcaatgatttgggggtaagagaagaccatattgggaaggtctacgtgagaaagtcagagtaaaaaaattgaggaccctttttgcagaagtggaggcttccaaactcagtaataagtgtcttctagcccctgaatacacacaaagcaagaatactttgtgtttacccactgccccctgaccactgctgaaggcagaaagggacgatcacctacagtacctggtttgggtctttattctctcattccagggagagaaccttaactagatggactgactgactgttcattggctttggttgggtagattccctgcttccctctataagtttgacgccaaaaaaggacaccgaccagcactgcagtcatagcaaatgtctcaaggagacccacagggtggtttcttcaaatacactactcacacacagcacatggagtcatggacaaacagcttaactgcccattgcctttgagaagtcctggaccaaaggccatagctcagccattgaaagatcttccttctgactgatatgtccctgcatagctccaacctgtgcaggcagaggatagggctgttccaaatgtcgctcacagagctgcctttgcctttctgcagatcccaagatacacacaaagcagttaacatgggtaaataggccttcctctgtaggagagggcttctgattcttattctttcttatggcggaagagggtgttgagaggggttcccttgctgttggttctgttgaatcaggagcattaaatcttttttgtttttttttgagacagaatctcactctgtcacccaggctggagtacagtggtgcaatctcagctctctgcaacctccacctcctgggtttaagcgattctcctgcctcagcctcccgagtagctgggattataggcacctgccaccacgcctggctattttttgtatatttagtagagatggggtttcaccatgttggccaggctggtaactcctgacctccagtgatccacctgccttggcctcccaaagtgctgggattaccggcatgagccactgcgcccagccatgagcattaaagctaagatttgttgaaaatgaatttataaaaaactttagaaacattaactgctgagcatggtggctcatgcctgaaatctcagcagtttgggaggccaaggtgagagggttgctggatcccaggagtttaagaccagcctgggcaatacagtgagaccccatctctaccaaaaaaaaaaaataataattagcctggtgtggtggtgcacgcctctagtcccaactgctcaggaggctgaggtgggaggatcacctgggcccagaaggttgaggctgtagtaagctgagattgcgccactgcactccagcctggatgacagagcaaaactctgcctcaaaaaaaattaaataattaaccacagtagacatttatcaagtaaaaaaagaactttttcctgattctgtgctgcagagatgccttgtgttagtttttacctacttacacttcacacacctcactttcatgcctggggtcacaccgtacatactgctttcgcaccttgcttccttccctcaatgtgtcataggtacccttacatattgattcattggacctgactgccatgttccactggacagactcaccagaatttatttgaccaaatcccttccagatggacattgggttgctttagttttgcacgaccacagacagcaccagtcaaggtccttacacacatcaattaactatggagtctcccgccagcttaggtctgcgtgctacaagtggggttgtgggctcacagggcatgcgcatctgacagttgaagagaggacaccaactgccttccaaaagggcagtaagaaagtgtccttcgctagagtgagtggctcactgcagttcaagatggagcagtgggggaagcagctctgtggtggtagtctactgagtgtatccttccagtatggttcccaactaatctccatttgccactgaccaggccacagatggggaagtcacagccgtggaggaggcaccggtaaatgcatgtccccctggattcaggccctgggtacaattttggttttttcctttttgtgtttctgtgtttactcagccttcatttcagaaaatctgccatctgcttctgggattgcttaagccctgtgggtgtcctggtcattggtgtgcccctcactgatcagcccatcacgatgatccctgctttttctgtaataagatcacctttgcgtcaccatccgtgctccacgaatcgccagccgtcgtgtctgtgatcacgctcggtgcagtttgtctctgtgtttaaagagaaagacagacagctgtctgcagccctcctgctgcctctcaaagccgccacttgcacattcagtttctgttcagggggaaagccacccactgctactctctgccacttaaaatgcaccttcttttccaggccacaagcaactaaacctttccagatggagcctcttgggactcatagacattgctgtctctcacttttccactttcccgtgggtgctgctgggaattttacaaacagactcccgagtgattgctaacagttggtcagcatgacctctccagtccctcaggttctaccctgggtctggagccacttagacaaagcccataccacaatgggcagccgcattcccaaatcccggcctcactggcttgtagaattcccagcagctctaacccctgtagcttcaccagctcccgctgttgtctgctttacccagtgaccactgccttctgtttttaggtgaccgaagaggcctatgtcccagtgagtgacatgaacggcctgggatttaagccttttgacctggtcattccgtttgctgtcaggaaaggagaaatcactggtaagcacttgccataaaggccgtctcattctcacttgctctcacgagcttcccagaatggtgctggggaggtgtgtccactgtcccccagacccaggctccttaacccagggtcacgagttcttggtctccggtgttgggccgtgggctcctgaaactacagaatatgccacgtgtgtgtttctctgaagaagtggctcactgacaacttgcattactttcttgagcagtcccatgattctctctaggttaaaaactgctgtgtttagatacctcatgactgtcgggttcttgtttgcccctttttcctgccttctcttatttgacttttccagatgtgactttgacactgagtctgtcatacaggagttcctttctcccctcagcctcttttcaatggcccacttctctttggtttgatgctctatgtatccagctggtttcatggtgttctcaagtcctttctgagcttgattttgccagttgtagaaaactctttaagagttgtctgctatattttgtggaagccaaatggaactggaaaaaaaaaaaagaaaagagcaaatggtctctcccattgtgggacttgaatgttttaggcagcaacgaatgttcttgggtctggaaacctttattttgaatacatctgtgccttgggctctgcttctctggggaaggttgctggtgggcttcattgccccgtctctctgtgctccataggagaggtccacatgccttctgggaagacagccacacctgagattgtggacaacaaggacggcacggtcactgttagatatgcccccactgaggtcgggctccatgagatgcacatcaaatacatgggcagccacatccctggtaagctgagtcagcaggcccagcagggctccaccattcaggggcatccgggcagcctgcagacactcctcagccgctttgcagggagcagctctcggcagcaggctggagaatgcagcgttggtacccctgtgaaaccaaacagtctgggaccctagcaggtccagctgatttctggaagggatgatgtagctcagtgtcttgggtcacagtgcaggcctttgggtctgtggttgtttatctttgtcactacgctgagtgtggccagaggtcaagctgggagaaaaatgggaggcatggtgagggactttccagcctggcctgcagagccctgtgtgggctggaggcttggggccaggtcagaggtggaagaagaggaccagcagccctggaagaagaggaccagcagccctctacaagggaagccagcccaggtttcatgggtcaccaaccagcacagtgtcaccagttcattctttctttttgtagttgtatttgttttttaatttagtattttgaataggtaacacattctcatggttcaaaaataaaaatgatacgaagaaagttttccttcctacccctctccttgaactagactatcataaatttttttatgttcgatttcagagtttcagggttttattttttatttttttgtggagatagggtctcactgtgttgcacagattggtctcaaactcctgtcctcaagcagacctcccgcctttgtctcctaaagtgttgggataacaggcatgagccgccacgcctggccaatttcagagtatttttaagactctccatgcaaacggaaatacagatatataagagagtgtcttcccagccttccctcatgtggacgaaccattacatatttgaccatttccctattggagggcattttggttcttcctgccctcgctgtccccagtgttgctgcgcaaatcgacttttcccctagtcacctcacactcacaaagatgtatctgtgagatttagttaccagaggaggcaatgctagggccccagtgcaggcatctatgattttgacagatcttgccaaattgcccttcagaggggctgttgcagttcacacgccctctggccatggagaagagcaccttcttttccacaaaatttgccagtagaatatggtatcaaatttttggagctttgccagtctgatggttggaaagaaacagaatctcagcgttgctttatttgtatttctcttgtgaatgagaccacacaactttccctatgtctatttgtatttctttttctgtgaactgaacatttggatccacggcctgtttttctatttggttattggcctttgtcatatagtttctaagagcaatgtaaacattggagagattagccctttgtggtaggagttgcaaatgtttctctgagattggcatttactttagttgtctgtatgtaatattggtttaaagcaaaaatgtattatctgcttctatttaaatattctaaagcggcagatggagagagaggaaaaaatgtctttctcacatctgccatccacttccactgctggtgtgagttgtgtatcttttcagatgtttctctctgtatctacaaacatacatataattttattctattttgtttttaaaggaatagcataatggtattcatagtttatagcaacttgctttttttctttttaatgcatcatattatggataatttctcaagtcagtaaacatgggtcttcctcactctttttaatggcccatgagtagatcagcatttatttaaccggtcccctgttgtgaacacttaggtcttttcctgatgtgcacccgaacactgcagaaatgaaagtgcttacatagggctaggagtcggggtgggcagagaagaccactgtggggttgattccttacaggttgaatggcatgggcaaatggccttccaaaagccctttccacttaccttccctctggccatgggtcctttcaccacccagtgcaaaagtttcttccttatttgtcaggttgggctggtaccttaccttagcccccttcctcatctggagcagcttccaggattgtttttcttatgttgtgattgaaggaataatactgcgtagaccctctctgatgtcctaggatggcgggggatgggaggtgcatgtgcatctccttctgtctcttcatgcctctgcttaggaggcgccagacctgtagagaggtggacgtcaagatgccagttgtccagggtcttcgttcaccccttaatgagcaccaattttgtttgtgtccttcgtaaacccagagagcccactccagttctacgtgaactaccccaacagtggaagtgtttctgcatacggtccaggcctcgtgtatggagtggccaacaaaactgccaccttcaccatcgtcacagaggatgcaggagaaggtactgtgtggtttacgtgtttatacgcctccagctgtccatttggagggtgaagtggacacggttccagggtggcttttaaaagtgagacaatcgaatggtagtatttgtcttgtcttttctctcgtgtaaatctgtttcttctttagagccgcttcgtcttctacccagacagacatttttgaagtcctttgtgttctaactgaaatcagattcatgctatgaaatactttatgtgacttgtctggaatttaagtgtgttttggttggtgatgtttttgttcttgttgcacatgtatccacaagaccacatgacttactgagtggctctttttgataaagctgtgtgcccattcccgtggtattcatggataatcccaaatctgtggttctaatgggatttccgtgatggcagccagtgcctgatgggcagggacaatccacctctgccctccaccacccaccgtctcctatgtgtaattgatgtacacggctccttccttttctcatcccatgcatcctgagagtagagagagctccagggttacttgcagtgaagaactcagatgtttggggtttcttctcagtgggtgtttttactgcgtggactgcttcattctgacagatgtccctttgcccacagctcacgtggagtgcgtcaatccattgtccccagcatcagggctgccctggatgagttgttaaaaggaaactcttaaaacaaggcaactctctccctaacacccctgcatccctgttcccacttgtaggtggtctggacttggctattgagggcccctcaaaagcagaaatcagctgcattgacaataaagatgggacatgcacagtgacctacctgccgactctgccaggcgactacagcattctggtcaagtacaatgacaagcacatccctggcagccccttcacagccaagatcacaggtagggttgtctggcttctggggtcttcctcgtgggaagtatggctgcctctgactgccaccctccttatcagacccctggcagcaggctagacgtctctttgagtttaggtttcacagagacttgttgaggaggagcaggggatggaatgcaattttggattagctaaatccttctcttgctgataatccaggaaaatgcgagagctagtatttggagcacacttttattgtgccagtgtgactctagggtgcaaagagaaagctctcagatggagtgttcgaatcatacttactgcaatagtgcatgaagtgcatgagcttagacatgcccttcagcgtcactactaggtaaattttctgctatcccttttacagatgggaaaactgaggcttggcaaggtagtggtgtagccaagttcacatataggtaaacagatccaggttatcaaattccaaagcccatgctcctcaccttgctgtgttcaggttatgctttcagtgggttataaggaagatgcacaaggcagatcctgtttccccaccgtatttagacctgtctgtgaagcagccagtagtactgtgtggaatgtggtcattgtttacctagaaatgcccacagccatgccaggcaggtatgaggtgccttcaactaacaaaaattcctatattttattttatttttgagacagagtctcactctatcacccaggctggagttttagtggcatgatctcggctcactgtgacctctacctcctgggttcaagcgattctcctgcctcagcctcctgaatagctgggattacagcacccaccaccacacccagcttatttttgtatttttaatagagatgaagtttcaccatgttggacaggctggtcttgaactcctgacctcaagtgattcgtctgcctcagcctctcaaagtgttgggattaggcacctggcccaaagattcctttaaaatgtggtccatgaggactcaagtctctaggtcctgccagcttcttgtctttgctgcaagcaggcatgaatcccatcattcttcattggttgggtctactcagtgttcaaggctcatttttttttcacttaactttgtgtaattagttcttgcgtgttcatccgtgaacagcatatggcatggcagctctgtgaagccagggtaaccacatgtaacgggagtcctttttgggggatgtttcccagatgacagcaggcggtgctcccaggtgaagttgggctcagccgctgacttcctgctcgacatcagtgagactgacctcagcagcctgacggccagcattaaggccccatctggccgagacgagccctgtctcctgaagaggctgcccaacaaccacattggtgagctaggctacccttcctggctggagccaggacatcttgggtgggagatggggactcttgcagtcctttcttgggaatgggtagcacaatggagtgtgatgtgataaacctgctgggtcacacgcacgataaatgcccaagcgtatttgtgcattgtgatatcgacactctggattgttgggtgtcaggaaagaggacatatttctatttctgagagtgtgtctctctcctgcttcctctccgccatccccttacaagccccaatctgtgttctggtccaggcatctccttcatcccccgggaagtgggcgaacatctggtcagcatcaagaaaaatggcaaccatgtggccaacagccccgtgtctatcatggtggtccagtcggagattggtgacgcccgccgagccaaagtctatggccgcggcctgtcagaaggccggactttcgagatgtctgacttcatcgtggacacaagggatgcaggtctgtgtggtcccaggggagaggcccagagcttgtgggaaccgacttattttgctgaggcagcgtcatcttttcatcctaccaactccttttcctttctgagcatccttcaagctataggtccttctgcctgcattgtcttttatgcctcatgaccattggcaaaaatgggattgtctttgttttttagatgatgaaactgaggcttgcaaggtttagagccccctctgcactaggatctgaacccagagccacaacacctcgcaaacccctgttttcttatctgctctcccacccttgttctcagcttcccagcgtctctccaagcaaagaatgttgggttgattggccaagaccatggtcatctgagcagagcttttgtggaaatgaagcatctctttctgttttctctttgagatggtttgagttagattgtgtctcttccaagcttgccacaccccagtgcctccagtcatctgctttcttgaaggatggccacgctggtgaattctagacaaattctaacccggggagagggctggagaatttctggtcctggttgggagatactccctgttaaaccttcggatatgctgacctagctgaggtagccaggggctatttaaaaattcaaaatctcagatctggctgtggataaacccccaaggtggtacgtgcagtacttggaggcgtgagggcagaaggtcctccccagcagtttgtacgggacacatcatctatgggatattagtaaatatccttaaggaaaggcttctgtggtcaaaaccaggttcagcaggttatttcactatggggcttctcaggacgcttaacctactcatccccctctgggctttgcaaacgaggccgccattgctttctttctgctatgtagaaatagattgaggcgtaagggtcggatgtcctttctccattcatcaggctccctcttcctgaggagctgctgtcagaacagcctggggctgctgtgttgcaggttatggtggcatatccttggcggtggaaggccccagcaaagtggacatccagacggaggacctggaagatggcacctgcaaagtctcctacttccctaccgtgcctggggtttatatcgtctccaccaaattcgctgacgagcacgtgcctggtatgtgcattccattcccctccaggtgggatgcttgggttttctgtaaatgctgtgccttggcctctggcctgctcacaggagccttcttgggtcttgcagggagcccatttaccgtgaagatcagtggggagggaagagtcaaagagagcatcacccgcaccagtcgggccccgtccgtggccactgtcgggagcatttgtgacctgaacctgaaaatcccaggtgggcgtcggggactagtagggtggggaagccttggctccagccttcagggcagtgggtgcctttgggaaccaagtttaggcatggcccagaacacagtatccaagtcggctgtgctgaccttttcatttcacttcatttcattatgttcttctatgtttattttcacagagtctcatccaagaaaaacaaatgtttaccttgctacctttttcctcttccaaataaaaatagctttattgtgtcacatgggggaaacgtagatatgcttttagatttttagattaactatctgtcaaatagaatcatgtcagtgaaagaactggccctgccgatgccagggtctggaagtatttaagaggtggcagcccagcggcatccttctagtatttctctttcattcctgaaattagaacgagggctgtgctgcagaactcgctgggccacatctagccctttggtggtgaattgttcttcttgggccccgattagccagtcaacaggtcacacagtctgtctgaaatgtgttccaagttctttctataaagaatccttccagagggaagccactgtgagtgaaaattttgaggctcctctgcccagaagttggcatgtcctgtggaattgcacaaattctacagagaagggaaatctaaatcgtcttcagatggagcttgtgttgcgagctctggagagggggttgtctttctacactgcatctcccatccttcctaacgagtcacggagctgtcgactccgccttcttggctttagttaacaggttcttcttgtgtagtcacatcaacgtcgggtcacatgggaatgtggtaaagcctcattactgtagagttcagacatgatcacttaaaaagagctttattgggccgggcgcggtggcttactcctataatcccagcactttggggggccgaggcaggcagatcacctgaggtcaggagttcgagaccagcctggctaacatggcaaaaccctatctcttctaaaaatacaaaaataagcagggcgtggtggcgggcacctgtaatcccacctactcaggaggctgaggcacaagaattgcgtaaacctgggaggtggaggttgcagtgagctgaaattgcaccgctgcactccagcctgggcaacaaagtgagactccttctcaaaaaaaaaaaaaaaaaaaaaaaagagctgtactgatcgtttgtagtcataaacagttcgtgtgcctcaaggtggggggaggaagtgtcacctcccagagagagcttggttcacattttaggtacagagttggaccctggctgccccatcctcatagccacgtctgctcactttccagtcacattggtgtactcatccactgtttttgtgggcatcttcccacctcaaaaaatagacatccacatcatctctttcatgaccctgataaaatgccatttcattcaatggaactattggtgatagaaaaagagagattccatttcatgtctagatgcatcaaccttcgttactcatctctgtgcctcagctcccatcatcagggctgctgtgacatttgccaccctgtgctcaggctgtgggctggatgcccaggagtgggctgggctggtgcatttcagatgctgccatgccttggcagaccgccctccacatttctccatactcccccaccagcactggggctgtctctccttctcactttggccaacctgatggaaaaacatggcattcagtgttcagtttcatatcttcgattactagtgatatgtgtactgtgttttcttttcatttgctttacatttctcatttggcaaaatttctgtgctctgcttatttcttgaggaactagcaagtatctgcagtgtggacgtttaccctttctcttaagtctcttccagctcttggccattttgttattcttttagttacttagtaccagatgactctgggtgaggctcgattttccactcattacccaaatgatcctctcggagatcccctcctccttaatggaggacagctcactaacttcagatgtcctccggacccaggttttgcggggcatctttgtcagtttgggctgctgtagcaaaatcacatgaactaggtggcaaccaacagaaatgtatgcctcacagttgtggaggctggaagtccaagatcaggtgccagcatggccagattgtggtgagggcctccttccaggctgcaaaccgacagcgtccccttgtatcctcacatgctggagaacggagggagccagctgtctgggactcttacaaggccactgaccccatcacagggtcgctccactttcatgaccttatctaatcctaattgcctcctcaaggcccatgataatcccatcacattgttgggggtagggtttcaatatttgaattttggagggacacaaacattcagttcattacatgggtgaccctcttttcaacctcccttcccttttctgtcctcaggggtcagagtcatgaactgctctgcccagatcctgtggggctggagggtgcagtttcatactggctctaggtgatggcagtgctccgtgccccgcatgcggccgcctggcctcaccacggcagtgcaggcacagtcgttggcatgacgtgagcagctcacggagagtgatgtggtcttgcgtcctagcactggtgacccgagacattgcttttctgaaagtgtggcccctggtctttggtttgctcaaagctttgctcacgcatggtttcccctctgccattgggacttacatatgttcacctttttctctaactttgtcttgttgcctaaaagaaatgccaaagcttcttgacggtaaaggatgatggctcttgttttctacccttacctatctgtggaaaggagcccgtctgtgcatgatggatgaccacgtcacctttggcaaaaagtctcagtgcccccagcatgggtggcctgaagggccctgcccactccatgctggccacagaagggcaggcacccagcctgaagggaaggaagcctgggcacctcacgtccaccgggctgcacacaccttgctctcggctgcttgccctgcatgtcctgccctgtctcaggcccttgccctaaccctcttctctcccccaacctccctccctctttcagaaatcaacagcagtgatatgtcggcccacgtcaccagcccctctggccgtgtgactgaggcagagattgtgcccatggggaagaactcacactgcgtccggtttgtgccccaggagatgggcgtgcacacggtcagcgtcaagtaccgtgggcagcacgtcaccggcagccccttccagttcaccgtggggccacttggtgaaggaggcgcccacaaggtgcgggcaggaggccctggcctggagagaggagaagcgggagtcccaggtgagcattgcgggcaggattttcacttgggaagaatagagttgagcccaggcagtgtgggcacccacatacttttttgccccatttgaaagagaagacttctgataggtggcattaagggcattatttaaaacaaggcatcatgactaagtctggcacagtttgtaactaagctttgctcacttacgtaaagccaaacaggtttcttactgggagcctccttggagcccgtatcttattagtgtgcacctgagtctctaattggggagcagagtaatacggtttccagagcatctttcagggctgatgttctgtggaacatactagaaagctacaaaactgactgtaagcatcctttcctgtggttgccgctggtgggaagatctgtagggaaaaaatggaacattctcatctttctctggcttggttaaggtgtattcattttttaaattttttatttaatatctttttctctcttgtttgttagagatggggtcccactatcttgctcagactggtcttgaactcctgggctcaagtgatcctcctgccttggcctcctaaagtgctgggattataggcatgagccactgtgcctggccggttaagatgtattcagggctgggcgtggtggctcacacctgtaactctagcactttgcaaggccgaggcaggcagactgcctgagctcaggagttcaagaccagcctgggcaacacggtgaaaccccatctttactaaaatataaaagaaattagctgggcatggcggcatgagcctgtagtctcagctactcgggaggctgagacaggagaattgcttgaacacaggagatggagcttgcagtgagctgagattgcaccactgcactccagcctgggcagcagagcaagactccgtctcaaaaaaaaaaaaaaaaagacatgtcttcagaggactccagatgtcctgtgaatttagttatcactagtgatgcttaggaaacttcagcaatggaccttggaccttgcttgggttctgcttggggttggagaaagaggaaagggctagcaacagacgaaacctagcactgcaggtttgaacaaggatggaagagggacaggggctctgtggggctcagtcactaaccaggtttctctttgctctcagctgagttcagcatttggacccgggaagcaggcgctggaggcctctccatcgctgttgagggccccagtaaggccgagattacattcgatgaccataaaaatgggtcgtgcggtgtatcttatattgcccaagagcctggtatgtattcagggttcacaagaggacattttccttgtttgaacatgattaggttgcaaggaacagaaatccatcaagtttgctgaagtcaatgaggaatctatgtgtatgggcacatgggacagcctcctagaaatccagttgcaagatacatggccagacctcttaagggtgggaacgcttgttctggttgccttttgcctttctccattagcctctctgcttcttgctttcattcaattgctccattctttccaccaaccagcctctgtctgcccacccatggctaccctggctggctgccccagaagagtggccttggcatctgagctccctctagcaggagctcttaaccttttgtgtgccattgactcttgccatctggcgaagcctatggggactgttcttgggataatgttttaaagcacataaaatgaaatatgtcacattataaaagaaatcattgatattatagtacagttaccaaaatcttacaagaacaaatatgcaacatagaaacatgcatatcttcgttaatacattaaatcataagatttggtgacagtatattaactgtcatcaaagtgacaaagtaataagtgaaaatgatacgtcaaaataactgtaaaatgacataaaaatatatgatttttaatggtgatgtaagtcatatgtacttataatgtgctgtgatttcttgtcaacatttctgaagaaaggaaatggtaaatttcagttagagaatggtgaaaattaaaacgtaattttttccccattgaagtccatggatctgctgaattcaatacaggccatttggggaccctgtgagccccggttaagagtccctggccttaccccactaaggaaatcatatcggcccagcctcagccaggcgactcccactcaaccaatcagctgtggccattgaggagggctgggtctctctgaaggcattttagcccttggtgagaagcaagagtccactctgggtccagagtctctgaaatgatgggactttcctgtcctcataggtaactacgaggtgtccatcaagttcaatgatgagcacatcccggaaagcccctacctggtgccggtcatcgcaccctccgacgacgcccgccgcctcactgttatgagccttcaggtgagatgcaaggaagcatccatctccttggccgcaggccaccagtgagacccctggactcctgaggctgcttcaatgtccccttaggtgctgaggccccttttcacattttgaccacagatgtcacccagtcactggggagctttcctgtggcagagtcaactccccatacacttagggcggatgacacttggggcgagcaaaaacagagccacagtcaacaacacaccttaatgtttggggacacgtttgtttttaaaggtttatttaagagaaacaaaggaagcctgttcataactggttaagggataacaagggctttcaaaacaaaaccaacacaaaaataacagtgcagtgatgttttagcctgctgttgttggctgcctttcttcaagaaagtcagttgcaacttactgtgattcattaataagtgtgcagggaactatattaagagctttatcagtgttacctcagtaaatccttgcaatagcctgacaagtaggttctcttgaccccattttaatgatggaaaaacagagatacaaggaggttttgtccactgggaaccagctagtatgaggcagaacaggcacagtgtggctccagaacctgtatttttgtttgtttgttgttgttgttgaggcagagtctcgctctgtcacccaggctggagtgcagtggcatgatctcggctcactgaaacctctgcctcccaggttcaagtgattcttctgcctcagcctcctgagtagctgagactccaggcacgcgccatcacacccggctaatttttggatttttcgtagagatggggttgcaccatgttggccaggctggtctcaaactcctgacctgaggtgatccaccccactcaacctcccaaagtgctgggattacagacgtgagccactgtgcctggccagaacctgtgcccttaacggcaacctctctaacccccacctgatgttgtggcacacggttgcatagtccatcccattaggataccaggagatgcaacatttttcctcgtcctaaacaggtcacttaattcaaggttgtactagcaccttcagccaaactaagaaccatcggggatgcctctgggtttttgcccaggacactgaaaaataattaggtgtctgaactgggagtagcaattaagttgtgaaataacatcgaaatcccaaagtatgatttctgggtaagagtttctaaatagccttgagctgcccccagttcttgaaaatattggattcattaaaatccaatctgatgtctaagattggtgatatcattggctttagttccatacacttggtttacatttgagattctaatcttactctgaggggaactgggatacctccagttgttccaaacattagtctttcatttagagacgtaaacagaacccaaaccagactcagtccacacattgaagcggcctcatccggagaataccaagggtactaactggttactgtggtgtagatgtttttcttgtgtttcatttaaaggcttcttaacagaagtgtcttttgtggccaacttaactaaaacctacggagggagataaacccagcacttattgagggcaggagctgccctcatgcatctcgaagatttctttcaaatctgccgaggcatttatctccctcttgaggatttagcggcaagcggattcaggtaatgtaaatgattctgtctaaaaggagctggtttggaaaaatcccctccaggaaacttctgtagagtgctctcgtcatagctgggtcataaatgtttcagtaagtgcacagcaggctgtttcttaagcttttgtaaccagctgctgccgcaggagaagtgtgttcatcagcatcgccccctgttcttcccgggtcatttgatgccgagtgatatgtaaattattgatcagagattttgcggaggcccacgcaagcaacatctggtgctggttagcaaagagaggcatgtatcgttttgtcttgcttttgagactttttaggaaattggagtaggctggcacttggggtgggggtgggatgggagtgatctggtgatcaaagaccctctaattctgtgttctgtcctccctcctcagtctatatcccctagggcagcacagtccaatagtaggttctgcagtgatcaaaatgcttcaagtctatgctatgcagcatgatagccactaaccatatgtgactattgaacatctgaaatgtggccagaggaaccaaggagctggatgtttagttttatttaagtgcattaagttgaaatatatgtatatatggcctcgtggctggtgactaccaaattagccagtgcagctttaggaccttgccatgaagatgtggttcttgggccagttcttggacctcagcatcacctgagaacttcagtcccagacccactggaaaagaatctgtattttaataagatccccagatggtttgcttacacattaagtgtgagccatgctgcttcagagttattgcctgaggagtggctgtccgaccaagtctaaatcaaaattactgacttgtaaaatgctgctgttcaggattggctagtcttaaaatatctcaaatgttgttgctcagctttgttcttaaccatctgaacttctaatcccctcctcccagaagaggagatagtttccaagacaaagtatggggagtgaaactgatccagggaagagcaaaagctatgtctttctatggcttcttgtggggatacaacctctaaatgcatattaatatttaataataagctgacgttttcgagcctctctgtgtatgggctaggccctgtgataaatgttttgcatgcacagcttcatttgatctttatagtagccctcgagatagatcgttattatgcccattttacagatgaggaaactgagactcgaagaggtttggcaccctagatatatagctaggaaatggtaggaaatccagatccagctgattcttaactgctatggagtactgccttctttgcacacgtagccctttataatatgttcctccaggtctgcccttgagataacaaacagcataacataaaactgtgttcgtgttcgtgagtgcatgactttgttagctgcagtatcctcttaaaagaggacacttttttgacctggaacatactgggttttctggcctgcatgggcattattttggatgctgagatgatagtccttttgaccaggatgtctcaagtatccaagcccagaaatcatctcttctaggctgaatcaagatggtttgcataagagaccatgcagatgcacgtctctgctatcttacattaaaaatgcagaatggctcacctgccctttgttgtcatatgttatatagaaaaacctatttgcatgagaactgtcacccacagttttgggtagggtcagtgtgtgccactgagcaggaacgccgagggccataacctgtctgatgtattaaattctcaggaatcgggattaaaagttaaccagccagcatcctttgctataaggttgaatggcgcaaaaggcaagattgatgcaaaggtgcacagcccctctggagccgtggaggagtgccacgtgtctgagctggagccaggtgagcaggaggcctgctggggggtcccagcaccagcactttccagcagaatgttcctgtaaatgtgtgtcccaagggagggctgatcagtttcattactgccagtgagcctctgaattccctttgctgttgccagatattgtttataaattagggtttaaacatgtgccagggatagggagaccctttatgctaggagagaatgctcattctttctttcttttttaaacaaatgctgggctgggtacagtgccttaacctgagaggtcaaggctgcagtgagctatgatgcagtgagctatgattgtgccactgaactccagcctgggtgacagagtgagaccctgtctccagaaaaaaaacaaaaaaacaaaaaaacacatacacacaacacaaaaacaaatgcttctttgttttctgttagtttttcagattccttttgcatgacattcatcataatttttctttcatattgtaacaacatcttacagatttttattcattgaccttatggcacgagtaagcatattttgatctcactttactctaaaggaaaagtaggttaatgttctgtaaatttaaaaaagaaaatctgggtctctaggccctaatgtcctaagatttttcttgcttggtgccttggtatatggaattctctgatttaatcaactttaaagagacagtgttaccggtgaacataataaatttattaagtgtcagaaacttgaaggaaggtataaggctcaaagagttgctcaaagtttagtgaaggcctggccaaaaagcagatgatgaccccaaatgatcactagtaccacaggagaactgtgaagcaaatggtaaagatggtcagagcaggagagagaaatagtttctgcctcggtgagttcaggagggcttctcagaggaggtgacatttgatgtgggccttgatgtatgaggaggagacctatgattactgccttatagggcatttgttgtgtgcctggctgtatttgtatagtgtagttggaaatctaggctctgaccaggcatggtggctcacacctgtaatctcagcactttgggaggatcagttgagcccaggagtttgggaccaacctgggtaacatagtgagaccccttctctacaaaaaaaagtaaaaaaaaaattagccaggcatggtggcacacacctgtagtctacttgtgggggatgaggtgggaggattgcttatgtccaggaggtcgagactgctgtgagctgtgatcatgccattgcactccagcctgggtaacacagcaagaccctgtctcaaaaagaaagaaaaaggaatgtaggctctgtgtgaacatttagatctatgtttcctagtaggcagaaaggcagtggggagcctcaggaggaacaagtgtaaaggatggggtcagatcctggttttagtctgaaaggccaagtggcaagctggtgctcccagagtggtccatttgaggaagcagtggcactggaaatggagaggagggacttgaggccagagatctatggtggctatagagagtgagagagagaatccattccaaaatgttccacgtagcttagtgattgggtcggaagatgacagtgcagttatcagaactagggccagccaggcagagggtgggtgaggattggtcagggccttaaagggtttaatattttactttgaggggttttgaaggatccccaatacccaaatggagatgtttactagatcactgtgaggtttggtggcctcagccccaacagtccctcactgggtaccctccctcttctcttaaagccaatgtgcttcaggggaagctaactccaccccagacaggatttgaacccctacagatgtatgagatcattagcatgacacagttactattgattgcaaattacagaatacccagctcaagccaactcacacaataaaggggcccagtaagttgcataactagaaagttcaagacatccaagacaggtttcagcaatttgatttggtcattgagctgcgccctgcaaggcgtcaaatatttctgctgttctgctttgtgggcctggttctggccttcctcttggtggcaggatggccttcctcttggtggcaggatggctgcagcagcaccagatgtcccaccttcacgccacatcaattaagagagacaccctctcaggattcttagaagtcgagagcctcctttcccagaagtctccagcacgtctgccttcccctctcactgacctggacacatgcccactgctgagtcatttcctgtggctaaagaaatgccatgtgctcattgactaaggcttagtgaagaaggatttttccctgatccactcagggaccacacctggacatggcggtggagccagcttcccctacaacacattggctttaagggaggcggatggggactgttggaggatgttcagtgccaaaggacgtagggtgcacagcttcatggaggtgcacctctgtggagacgtccagaggcagggagaagagctttggggaacacaaattctgagagggatgaagagtactaggcaccagggagagaccgagagactacctggagaggtaggaggagaacaggctctgcaccctgggcaggagggcttcaaggaggaagcggcagtcaggtggtgcacaatgggtagatgttctaggtgcccacttcagttaacagattaccttgctacatgctgtgacccaaacgcacagccacaaacctgccctgtgggggcagttcctagctttgagcttaattaaggagcattaatgccagttggaaccgttttttttccccttcaagtggccaaatagagaaacatagaagaagtgaggttttcttttttcccttcatatatattcctttttatttcttgttatgccttcccaaaacagagacattgaacagtagttagaatggccatctcccaatgtttaaaaacaaactgaactccccaatgggtgaacaaagtaaagagtagtaacctggagttcagctgagtaagccgctgcggagccttaagtggtgaggtcttccaatttcagagtgctgtgtcttcaacttgtatcatcattttagtggaaaaacataatttaattttggtgaaatgagattcatctcgtgacaggattagtaacagcattcacagaatttcacactgaagaagtgaggttttctaaagaaaggaagtgttcttctgaggcaggggtcagagtcttgtcctgtgtttataggatttgcaatgtggatgcgtttcccttggggctgatgagggatacccagggggtctgtctggttctgaaatccaggatgctgagtgccaggctccctgtagaactgttgattttaaatgggccatctcagcttggcctccatcctttatcctcactgaactcaggggtgtccatttgcttgatttcaccctgtgcctttgctcattctcctagataagtatgctgttcgcttcatccctcatgagaatggtgtccacaccatcgatgtcaagttcaatgggagccacgtggttggaagccccttcaaagtgcgcgttggggagcctggacaagcggggaaccctgccctggtgtccgcctatggcacgggactcgaagggggcaccacaggtaacccactcttctgcttcttgaagccttaactgaaccagctccagggaccaagccagatggaaatcctcaagccccatgaaagctttttacacgtactccccgtggaaactggggtcatgcacacttcggaggcgcttgctgtccaaagctgttttgggagttgcggtttgacccacgataaatccagagtgagagctcgatggccgtgttatcacacctcattactgttagttgtgattcagattccttcctctgccaagtttcttgactttcagaacaggatgctgatagtcagggaacacagcacagtgtcattaattttgagggtttctttgcctgcacagaattcatgatgcgtccaagtgggctcctacccgtctgttctttcatggtaccaggctcccagaaatgcactgaagcagcaataagacctgtcccagcctatctcctcctctttttactctcagatcttaatggaggaggagaaaagactgaaatgttcaaagaattctgaagctttttagacccgttacaatttacttttattctttgccacagatgggacatgtttgattatgaaagatacaggcagtgaagaagtaaataaagtgagactcactccatcttctctcctcctcccccacctgggtctggaagcaaacggctctgggaagggaggaccttcaccctgtctgtcatctcattgtctgtcttcattcttggttgctgggttggttagctaattggttcattagacaagcagacacagagttttgcttttgtcttacagaaagaatcttactgtatccactgtgtggtatagcttgtgtttttgctttgacatcttaaagatctttccatgtcagaacagatcttcccctccttttcctggctgtagtgagaattcctgctgtgaatcgcagttatttgaacaggtggcatcgggtggtgcgcagtgagtgcgtcactgttatggaggctgccagggtggagagtcagtccttagtctttgcaggggaagtgcgcagtgtggactcactggggcatgtttgcatttggtgttactttggaccctcttgggaaagcagtatgtcctggtttcttgagtctcttgtgtgtgtacccccaccccgcataaggagagtgggatggagcagacttgcctcccaggggtgaggggtgagtggctgcatggttgcctggcatccagccctaggagcaagtgacctgtgtggccaaggggccctctccgggtgcaggagtgactggtgggctggcaggctgcccgggactctggccaaagcagtggcctcagcaaagccacccacaggggtggtgtgagtgctgccagactccccaggcaaatccagcccggctccacgctgaactctgggcctgcggcttgccttttgtgaaaggcatggtatcattttaccgtaagtgatgtccattttacagatgtggaaagtgagatgcagaggttgagtcactccccaaacaacactcccccaaaaagcagtcagctgggaggaggcagaaccaggaatcagtctacatccgtgacctcagagcctatgcgctgaacccccgagcttggccccctctctaagtggctggctcacccagaggcagtgactgcatccccagcccactttggggatgtcctaaaccaggacccctgtcctcccagccactcaggagtactttccaggcagcagtgctggcacttgggccctgacaaggtactcacctttgagggcccaggtggggtcctctcggcacttggagcgcgtggcaggcttcaggccaggcctcacagcagctgctggggtctcccacactggccaggaagcatctcaccctcctgctggctcatgccgctgtgcctgggccctctcccatttccttttggctgttcgcacacctttttgggagcttgggtttcaggctgtgctctgcaagtgctggacgctgctgagagaaggagttgctcttgcagggaagctcctagccaggaggggagaggtacagaaccgcctgcttcaaaccctgtgtaaatattgctcttgtcacagggaaggcgccttgtttttccagccctcctgctcccaagcctttccctaaatatccattctgagattacacagctgcagtgtgcatggaatgaaaaggtatctgtgcttggccgccagagcgcccagtatcctgaccttctgaacaaagcaaacctccctctgtttttaatgggtgagtttgctgtatctcttggctcaagctttaaatggtccattctgtagattttggagtaggggaatgtggagaatttggggcgggaccctgctggaggcggcttgagaggctgggagatagaccagggagctccagattctttggagccgctgagcaattttcctaatgaaatggtccaggaaccccagtgtgctcggggtataccagaagggcctccttccttaactgccttgaagaacaagcagtgctgcgtttaacatgcattaaactcacaggaactgagctggacatatttgagggggtgggggaagaccgccacgcccagagatgttttgtggtgtcagatacaggttatagctagaggcagtggtgagagacttctgcttgtggatttttttccttccatcttctctcaggtaagtgctttagctccaagttggacagactttatgtttaaatcccagttctgctggtccccagctgtgtgactccagatgaattatctgacttcactgtgcctctgcttcctttcctgtaaaacaggattaataacaggacccacctaataggcttgtttggagctgtagaggaggtaacagccaagtagtagctcttgtcccataacccctgctttctcttttcccacctcgtcttccctgcccttttgggccctcacagtcaagatgaactgatttttggttggtcaaaatattgcattagggccaaatgggtgcggtggctcatgcctgtaatcaaagcactttggaaggccaaggcagaaagattgtttgaggccaagagtttgagaccagcctgggtgacatagtaaaactccatctctaccaaaaaaaaaaatttttaaagacgaacttaggaatgaaacagcttgttaaaaaatggtggaactttcccctgcagccacatcatttcaacttcactttaaaaatatctttttggcctggcacagtggctcacacctgtaatcccagcactttgggaggtggaggtgggaggatcacttgagcctaggagtttgagaccagcccaggcaacacagcaaaaccccatctctacaaaaaaatttaaaaattagccaggcgtggtggtgcatgcctgaagtcccagctactttggaggctgaggcaggaggatggcttgagcctggaagattgacgctgtggtgagctgtgatcatgccaccgtactccagcctgggcaacagaggaagactttatctaaaaaaaaaaatattagtaataaggccgggtgcgttggctcatgcctgtaatcctagcactttgggagaccaaggtgggcagatcacttgaggtcaggagctcaagaccagcctggccaacatggtgagaccccatctctactaaagaaatacaaaaattagctgggcatggtggcgagtgcctgtaatcccagctaatcaggaagctgaagcaggagaatcgcttgaacctgggaggcggaggttgcaataagccaagatcatggtactgcactccagcctgggcaacagagcgagactctatctcaatcaatcaatcaataaaatatctttccttatcatcaccttacagctgcttcctggatggacacactgtctccttgttgctcacctcccgcttcttccctacgtagccccaggcctcagagctgctgcttgaggggcttcttggctgcacagattagataccatgatgaggttgagatagtgttgggggtggaccttggggcaggagcctcaagagcttccaggaacagctgggttgtgtttgagagttgcacgatagcagctcttttgtttttattgatatccagaacaataattctttctctggactaggagctataattaaaccaaaatatttcccagctggggcagtgtctagggctctggcagaagcatagccctgcatggggatgctatgccaggcatgccccatagagggcactgtagcaggcatgcgccagacctgatgactgaaggaggctctccctgggccagctaagttgtctcagggctgcagttaggggatctgaggcagctccactgcccatccaggggtcaagagatgagcctggcaccagagccatgcagacatggttcaaacccggctctaccactttctggttgtgtagcgtgactggccccctccctgagccgcagagtcatttgtgaagcaggaatcacggaaaggattccataccacatgcgtaaatggtgctgtgcacaggacctggagccggagtggggtacgcatgccccgtcagcgggagctgctgttctgttcctgtgcttgttgctggaattcacggcaaagtgggtgggctggcaggtcacagtggctgcacccggtctgcagcacagtgcctggggtgagggctgaggaggaagggaggagatgcttggcctccctggcttctccaagtctacccggagaagaaaggacagtcagaggggcccacgcctcccccacacccctggagggagagctggactctggtggctgaagcagcacttcaggctcacagtgtgactcaggcttcttgccctcagccacaatggctcatgcccagaggagagaacagggtgtccaggctgttggtgcttgtgggcgaaatgtcagccatgctcctcctgccttggcctagaaaagggagcccccaccccgcagggcctgaggttctctctgccagaagttcagagctagtgccagtgggttcccatgccaccagggtgagccctctgtaaggggatctatgtgtgtccctcaccacggcctcagtgctcccaggaaagccctccaagtcatcaacacagcattttctattcctttctcccaggtatccagtcggaattctttattaacaccacccgagcaggtccagggacattatccgtcaccatcgaaggcccatccaaggttaaaatggattgccaggaaacacctgaagggtacaaagtcatgtacacccccatggctcctggtaactacctgatcagcgtcaaatacggtgggcccaaccacatcgtgggcagtcccttcaaggccaaggtgacaggtaacgaacaaccaccttcggagttactctcccttcctggggagctggttgtgtcagatcaatcatagtggaaactatggatggttttagatgtgttaaagctactttgaactttgaatgtcagtaaatagtatgagatgtcagagggcagtgtttgaaacttacaaaagtccacagagtggagccgtgcagaagttgagaaagcatgttaggatgttaggtggttttctatctctaacaggaaagaatacatattgaaatcttacgtatttgtttagatcagggtctgaaaaatcccctgatttctaattttcacttgaaaaataatcaaaaagttttcctatacttataaaaatgtgtctcctccaaaacactggaaaaaataccaaactatgaaaaccacttcacagccaccacccaaggtaaccaccataaacactgtagtaaatcccttccacacgtcatgattcactgttacataaagaatgtaggttcatcgcaggaaaattagaaaattcagatagaaaaatcatcctttctcatccacagaatcattttttgatatttcattatatgtcatcccaaacttttacactgcttatacatagactattttatgtcaatagaaagatgtgaattccacaggcacatctttggtgggtagggggtggggggattgggagggtccttggccttgtcagccaaggccagactcatccatttgcccagaaagccagatcctagttgtatgggggtgggatcctaggggtttagaagacattatgggtgtgagatacaggtgtggtggcttttgtgttggggtgcgcgggctctcctggggttactgtgtagggtactcgcctgtcctctggctgagagacccctcttgatctggccattcatgcctgtccccctccctcctgtatcttaggccagcgtctagttagccctggctcagccaacgagacctcatccatcctggtggagtcagtgaccaggtcgtctacagagacctgctatagcgccattcccaaggcatcctcggacgccagcaaggtgacctctaagggggcagggctctcaaaggcctttgtgggccagaagagttccttcctggtggactgcagcaaagctggtaggtgtctgggccttttcaagggtggggtggggcaggggcaggctgggcaccctgggtacactggccttccctgctgaggtctcctgcagtgcccacccccatgtaggccagccgtttgcaagtaaccatcgtcatgaccctgttctcctgcacttaatatttttaaatgatttccttctcttttgccttttgaacttgggtatttatttgggtttcaagggtcggttgcctgggttctggcatccagtacacctgggctggaaacctagtaccgccacttcattcattcattcgtttgttctaaaacttatttagccatgtgaccttggaaagttattaaatctctttccaaaagtcagtttcctcttctcggaagtaccttccttaaggtgcttgtgagagtaaacaagaagattctcatagccaacacttagaatagcccttactgtgtgctaggttttgacacccataactcttaaacctcacaactagttcgtgaggtatgtgctgttctcattccctgtttacagatggggaagctgagctagggagaggtgagattccagtccaaggtcacccaggtagcaagtggcagggcagggattcgaacccacaccgtcaggctctatgagcctctgcttgtaattgccacgctctcccacctcttaggggccccagcattatcgtggaagcaccttacctttggctctcatatttcctcttcttcctgtgcctgtcctgatgcatccgggtggagtaaccaccttttgcctcctaggctccaacatgctgctgatcggggtccatgggcccaccaccccctgcgaggaggtctccatgaagcatgtaggcaaccagcaatacaacgtcacatacgtcgtcaaggagaggggcgattatgtgctggctgtgaagtggggggaggaacacatccctggcagcccttttcatgtcacagtgccttaaaacagttttctcaaatcctggagagagttcttgtggttgcttttgttgcttgtttgtaattcattttatacaaagccctccagcctgtttgtggggctgaaaccccatccctaaaatattgctgttgtaaaatgccttcagaaataagtcctagactggactcttgagggacatattggagaatcttaagaaatgcaagcttgttcagggggctgagaagatcctgagtacactaggtgcaaaccagaactcttggtggaacagaccagccactgcagcagacagaccaggaacacaatgagactgacatttcaaaaaaacaaaactggctagcctgagctgctggttcactcttcagcatttatgaaacaaggctaggggaagatgggcagagaaaaaggggacacctagtttggttgtcatttggcaaaggagatgacttaaaatccgcttaatctcttccagtgtccgtgttaatgtatttggctattagatcactagcactgctttaccgctcctcatcgccaacacccccatgctctgtggccttcttacacttctcagagggcagagtggcagccgggcaccctacagaaactcagagggcagagtggcagccaggcccacatgtctctcaagtacctgtcccctcgctctggtgattatttcttgcagaatcaccacacgagaccatcccggcagtcatggttttgctttagttttccaagtccgtttcagtcccttccttggtctgaagaaattctgcagtggcgagcagtttcccacttgccaaagatcccttttaaccaacactagcccttgtttttaacacacgctccagcccttcatcagcctgggcagtcttaccaaaatgtttaaagtgatctcagaggggcccatggattaacgccctcatcccaaggtccgtcccatgacataacactccacacccgccccagccaacttcatgggtcactttttctggaaaataatgatctgtacagacaggacagaatgaaactcctgcgggtctttggcctgaaagttgggaatggttgggggagagaagggcagcagcttattggtggtcttttcaccattggcagaaacagtgagagctgtgtggtgcagaaatccagaaatgaggtgtagggaattttgcctgccttcctgcagacctgagctggctttggaatgaggttaaagtgtcagggacgttgcctgagcccaaatgtgtagtgtggtctgggcaggcagacctttaggttttgctgcttagtcctgaggaagtggccactcttgtggcaggtgtagtatctggggcgagtgttgggggtaaaagcccaccctacagaaagtggaacagcccggagcctgatgtgaaaggaccacgggtgttgtaagctgggacacggaagccaaactggaatcaaacgccgactgtaaattgtatcttataacttattaaataaaacatttgctccgtaaagttgccttggtgttcttggatgatgtcgcttctgaataaattgtttaatcctaggagttcaacaccctcagcctgggtaacagcaagacccagcctctacaaaaaattaaaaaattagccagcatggtgatgcatgcctgcagtcccagctactcaggaggcggaggcaggaggattgcttgagcctgagaggccaaggttgcagtgagctgtgtttgcaaccctgcactctagcctgggcaacagagcaagacagtgtaacacacacacacacacacacacacacacacacacacacacaggcacatcgttggagccccagatcagctctcccaaccccttaagggacacaaaactagcaacttgttttgacaatgaacctgggctccttttgtgggggtggggtggggctggtaaacaagctgtcacctgtcaccctgctgtgcttattgttgctgctgcctctgtttctcttttttttttttttttaattttccttttttgagacagagtctcactctgttgcccaggctggagtgcagtggcaggatctctgctcactgcagcctccgcctcccaggttcaagtgattcttctgcctcagcttcccaagtagctgggactacaggcgtgcaccaccatgcctggctaatttttgtctttttagtagagatgtggtttcgccgtgttggccaggctggtcttgaactcctgacctcaagtgatccgccctgccttggtcttccaaagtgctgtattacaggcgtcaaccactgcgactggcctgtttctcctttttctagaagagcttttgattgctgaatgcttacgaggtacctagcacccctcctccgcccccacctcctcctcctctgtctccgcctcctccccaccccacagcagtgataccgctttacagatggcactaccacctcaggtgctgcaatgacatgtttgcagatgcaaagctcacttgggggaagaccctaggcccctgccttcttgaccccagggtgctagctctaccccctggtgataccgctgtggaaacaggagtccccagataggccccggcaggtgccacggtgatgggaaatcacggctgggcccccagccctccagatgggggttgggggtggagagaaaagcagggaagggagactggattcttctgacacctggctgtcaattgggatcaattgtttgcctctgagaggagggaggaagagagtggaggaaaggtcctctcctcccggagggagcagccttatctgtggcctgcaccaggaagcactgcttcctggactcctatctgagaaggtccgtgggcttcgggattctgcagtggcgggcagttcccccacttgccaaagagtccattcaggctctgcccggtggggtctggccgggccacagtatcatgctagtttgcccacagaggagcacagggcgcagccattggtctctccactgtgaagcctggcggctttctgttgggggaggcagcatttgtaaattaacagcatgggctttggtgtcaggcaccccagagcttcaacgctggctctgccgttcattagctgtgtggccctggggaagtcgccttgcctcacctctctgggtggtcgtgaggatcaaataagagcccacagggagctgtaaggaacaattccctgccagagtctcagccactgctgtctgtgaccaacacctgctggaagtgatgttcctggcagaaggccgccccctggctgcttgttggcatctggggctacacttggttgtcccctgcatgggagcgatggtgatgttaccctggggtaaatttccccactagaagccactgcctcctgttacatcaaagacatcccagggtgggatgcacctctttatcagtcaatggctaggaccacagggcaacccttacctgcacctgggcttggctgctatggaaaccagctgtttgtgcaaataccttgaaaactttgaaacttgaccccggac

SEQ ID NO: 22 - protein, 2633 aa, Homo sapiens
MPVTEKDLAEDAPWKKIQQNTFTRWCNEHLKCVNKRIGNLQTDLSDGLRLIALLEVLSQKRMYRKYHQRPTFRQMQLENVSVALEFLDRESIKLVSIDSKAIVDGNLKLILGLVWTLILHYSISMPVWEDEGDDDAKKQTPKQRLLGWIQNKIPYLPITNFNQNWQDGKALGALVDSCAPGLCPDWESWDPQKPVDNAREAMQQADDWLGVPQVITPEEIIHPDVDEHSVMTYLSQFPKAKLKPGAPLKPKLNPKKARAYGRGIEPTGNMVKQPAKFTVDTISAGQGDVMVFVEDPEGNKEEAQVTPDSDKNKTYSVEYLPKVTGLHKVTVLFAGQHISKSPFEVSVDKAQGDASKVTAKGPGLEAVGNIANKPTYFDIYTAGAGVGDIGVEVEDPQGKNTVELLVEDKGNQVYRCVYKPMQPGPHVVKIFFAGDTIPKSPFVVQVGEACNPNACRASGRGLQPKGVRIRETTDFKVDTKAAGSGELGVTMKGPKGLEELVKQKDFLDGVYAFEYYPSTPGRYSIAITWGGHHIPKSPFEVQVGPEAGMQKVRAWGPGLHGGIVGRSADFVVESIGSEVGSLGFAIEGPSQAKIEYNDQNDGSCDVKYWPKEPGEYAVHIMCDDEDIKDSPYMAFIHPATGGYNPDLVRAYGPGLEKSGCIVNNLAEFTVDPKDAGKAPLKIFAQDGEGQRIDIQMKNRMDGTYACSYTPVKAIKHTIAVVWGGVNIPHSPYRVNIGQGSHPQKVKVFGPGVERSGLKANEPTHFTVDCTEAGEGDVSVGIKCDARVLSEDEEDVDFDIIHNANDTFTVKYVPPAAGRYTIKVLFASQEIPASPFRVKVDPSHDASKVKAEGPGLSKAGVENGKPTHFTVYTKGAGKAPLNVQFNSPLPGDAVKDLDIIDNYDYSHTVKYTPTQQGNMQVLVTYGGDPIPKSPFTVGVAAPLDLSKIKLNGLENRVEVGKDQEFTVDTRGAGGQGKLDVTILSPSRKVVPCLVTPVTGRENSTAKFIPREEGLYAVDVTYDGHPVPGSPYTVEASLPPDPSKVKAHGPGLEGGLVGKPAEFTIDTKGAGTGGLGLTVEGPCEAKIECSDNGDGTCSVSYLPTKPGEYFVNILFEEVHIPGSPFKADIEMPFDPSKVVASGPGLEHGKVGEAGLLSVDCSEAGPGALGLEAVSDSGTKAEVSIQNNKDGTYAVTYVPLTAGMYTLTMKYGGELVPHFPARVKVEPAVDTSRIKVFGPGIEGKDVFREATTDFTVDSRPLTQVGGDHIKAHIANPSGASTECFVTDNADGTYQVEYTPFEKGLHVVEVTYDDVPIPNSPFKVAVTEGCQPSRVQAQGPGLKEAFTNKPNVFTVVTRGAGIGGLGITVEGPSESKINCRDNKDGSCSAEYIPFAPGDYDVNITYGGAHIPGSPFRVPVKDVVDPSKVKIAGPGLGSGVRARVLQSFTVDSSKAGLAPLEVRVLGPRADDTDSQSWRSPLKALSEFFKGDPKGDFNKTGLVEPVNVVDNGDGTHTVTYTPSQEGPYMVSVKYADEEIPRSPFKVKVLPTYDASKVTASGPGLSSYGVPASLPVDFAIDARDAGEGLLAVQITDQEGKPKRAIVHDNKDGTYAVTYIPDKTGRYMIGVTYGGDDIPLSPYRIRATQTGDASKCLATGPGIASTVKTGEEVGFVVDAKTAGKGKVTCTVLTPDGTEAEADVIENEDGTYDIFYTAAKPGTYVIYVRFGGVDIPNSPFTVMATDGEVTAVEEAPVNACPPGFRPWVTEEAYVPVSDMNGLGFKPFDLVIPFAVRKGEITGEVHMPSGKTATPEIVDNKDGTVTVRYAPTEVGLHEMHIKYMGSHIPESPLQFYVNYPNSGSVSAYGPGLVYGVANKTATFTIVTEDAGEGGLDLAIEGPSKAEISCIDNKDGTCTVTYLPTLPGDYSILVKYNDKHIPGSPFTAKITDDSRRCSQVKLGSAADFLLDISETDLSSLTASIKAPSGRDEPCLLKRLPNNHIGISFIPREVGEHLVSIKKNGNHVANSPVSIMVVQSEIGDARRAKVYGRGLSEGRTFEMSDFIVDTRDAGYGGISLAVEGPSKVDIQTEDLEDGTCKVSYFPTVPGVYIVSTKFADEHVPGSPFTVKISGEGRVKESITRTSRAPSVATVGSICDLNLKIPEINSSDMSAHVTSPSGRVTEAEIVPMGKNSHCVRFVPQEMGVHTVSVKYRGQHVTGSPFQFTVGPLGEGGAHKVRAGGPGLERGEAGVPAEFSIWTREAGAGGLSIAVEGPSKAEITFDDHKNGSCGVSYIAQEPGNYEVSIKFNDEHIPESPYLVPVIAPSDDARRLTVMSLQESGLKVNQPASFAIRLNGAKGKIDAKVHSPSGAVEECHVSELEPDKYAVRFIPHENGVHTIDVKFNGSHVVGSPFKVRVGEPGQAGNPALVSAYGTGLEGGTTGIQSEFFINTTRAGPGTLSVTIEGPSKVKMDCQETPEGYKVMYTPMAPGNYLISVKYGGPNHIVGSPFKAKVTGQRLVSPGSANETSSILVESVTRSSTETCYSAIPKASSDASKVTSKGAGLSKAFVGQKSSFLVDCSKAGSNMLLIGVHGPTTPCEEVSMKHVGNQQYNVTYVVKERGDYVLAVKWGEEHIPGSPFHVTVP

SEQ ID NO: 23 - DNA, 9560 bp, Homo sapiens
gcggccaggggcgggcggccgcagagcagcaccggccgtggctccggtagcagcaagttcgaaccccgctcccgctccgcttcggttctcgctccttcggcccttgggcctccaaacaccagtccccggcagctcgttgcgcattgcgctctccccgccaccaggatgccggtaaccgagaaggatctagctgaggacgcgccttggaagaagatccagcagaacacgttcacacgctggtgcaacgagcacctcaagtgcgtgaacaaacgcatcggcaacctgcagaccgacctgagcgacgggctgcggctcatcgcgctgctcgaggtgctcagccagaagcgcatgtaccgcaagtaccatcagcggcccacctttcgccagatgcagctcgagaatgtgtccgtggcgctcgagttcctggaccgtgagagcatcaagctcgtgtccatcgatagcaaagccattgtggatgggaacctgaagctcatcttgggtctggtgtggacgctgatcctccactactccatctccatgcccgtgtgggaggatgaaggggatgatgatgccaagaagcagacgccaaagcagaggctgctggggtggattcagaacaagatcccctacttgcccatcaccaactttaaccagaactggcaagacggcaaagccctgggagccctggtagacagctgtgctccaggtctgtgcccagactgggaatcctgggacccgcagaagcctgtggataatgcacgagaagccatgcagcaggcagatgactggctgggtgtcccacaggtcatcactcctgaagaaatcattcacccggatgtggacgagcactcagttatgacttacctgtcccagttccccaaagccaagctcaagccgggggctcctctcaaacccaaactcaacccgaagaaagccagggcctatggcagaggaatcgagcccactggaaacatggtgaagcagccagccaagttcactgtggacaccatcagcgccgggcaaggagacgtgatggtgtttgttgaggacccagaagggaacaaagaggaggcacaagtgacccctgacagtgacaagaacaagacatactctgtggagtatctgcccaaggtcaccgggctacacaaagtcacagtcctctttgcaggacagcacatctccaagagcccatttgaagtgagtgttgacaaggcccagggagatgccagtaaagtcactgcaaaaggtccagggttggaagctgtagggaacatcgccaataagcccacctactttgacatctatacggcaggagctggtgtgggtgacattggtgtggaggtggaagatccccaggggaagaacaccgtggagttgctcgtggaagacaaaggaaaccaggtgtatcgatgtgtgtacaaacccatgcagcctggccctcacgtggtcaagatcttctttgctggggacactattcctaagagtcccttcgttgtgcaggttggggaagcctgcaatccaaatgcctgccgggccagtggccgaggcctacaacccaaaggcgtccgtatccgggagaccacagatttcaaggttgacaccaaagctgcaggaagtggggagctcggtgtaaccatgaagggtcctaagggtctggaggagctggtgaagcagaaagactttctggatggggtctacgcattcgagtattaccccagcaccccggggagatacagcattgccatcacatgggggggacaccacattccaaagagcccctttgaagttcaagttggccctgaagcgggtatgcagaaagtccgtgcttggggccctgggctccatggtgggattgtcgggcggtcagcggacttcgtggtagaatccattggctctgaagtggggtctctggggtttgccattgaaggcccctctcaggcaaagattgagtacaacgaccagaatgatggatcgtgtgatgtcaaatactggcccaaggagcctggcgaatatgctgttcacatcatgtgtgacgacgaagacatcaaggacagcccgtacatggccttcatccacccagccacgggaggctacaaccctgatctggttcgagcatacgggccaggtttggagaaatctggatgcattgtcaacaacctggccgagttcactgtggatcctaaggatgctggaaaagctcccttaaagatatttgctcaggatggggaaggccaacgcattgacatccagatgaagaaccggatggacggcacatatgcatgctcatacaccccggtgaaggccatcaagcacaccattgctgtggtctggggaggcgtgaacatcccgcacagcccctacagggtcaacatcgggcaaggtagccatcctcagaaggtcaaagtgtttgggccaggtgtggagagaagtggtctgaaggcaaatgaacctacacacttcacggtggactgtactgaggctggggaaggtgatgtcagtgttggcattaagtgtgatgcccgggtgttaagtgaagatgaggaagacgtggattttgacattattcacaatgccaatgatacgttcacagtcaaatatgtgcctcctgctgctgggcgatacactatcaaagttctctttgcatctcaggaaatccccgccagccctttcagagtcaaagttgacccttcccacgatgccagcaaagtgaaggcagaaggcccagggctcagcaaagcaggtgtggaaaatgggaaaccgacccacttcactgtctacaccaagggggctgggaaagccccgctcaacgtgcagttcaacagccctcttcctggcgatgcagtgaaggatttggatatcatcgataattatgactactctcacacggttaaatatacacccacccaacagggcaacatgcaggttctggtgacttacggtggcgatcccatccctaaaagccctttcactgtgggtgttgctgcaccgctggatctgagcaagataaaactcaatgggctggaaaacagggtggaagttgggaaggatcaggagttcaccgttgataccaggggggcaggaggccaggggaagctggacgtgacaatcctcagcccctctcggaaggtcgtgccatgcctagtgacacctgtgacaggccgggagaacagcacggccaagttcatccctcgggaggaggggctgtatgctgtagacgtgacctacgatggacaccctgtgcccgggagcccctacacagtggaggcctcgctgccaccagatcccagcaaggtgaaggcccacggtcccggcctcgaaggtggtctcgtgggcaagcctgccgagttcaccatcgataccaaaggagctggtactggaggtctgggcttaacggtggaaggtccgtgcgaggccaaaatcgagtgctccgacaatggtgatgggacctgctccgtctcttaccttcccacaaaacccggggagtacttcgtcaacatcctctttgaagaagtccacatacctgggtctcccttcaaagctgacattgaaatgccctttgacccctctaaagtcgtggcatcggggccaggtctcgagcacgggaaggtgggtgaagctggcctccttagcgtcgactgctcggaagcgggaccgggggccctgggcctggaagctgtctcggactcgggaacaaaagccgaagtcagtattcagaacaacaaagatggcacctacgcggtgacctacgtgcccctgacggccggcatgtacacgttgaccatgaagtatggtggcgaactcgtgccacacttccccgcccgggtcaaggtggagcccgccgtggacaccagcaggatcaaagtctttggaccaggaatagaagggaaagatgtgttccgggaagctaccaccgactttacagttgactctcggccgctgacccaggttgggggtgaccacatcaaggcccacattgccaacccctcaggggcctccaccgagtgctttgtcacagacaatgcggatgggacctaccaggtggaatacacaccctttgagaaaggtctccatgtagtggaggtgacatatgatgacgtgcctatcccaaacagtcccttcaaggtggctgtcactgaaggctgccagccatctagggtgcaagcccaaggacctggattgaaagaggcctttaccaacaagcccaatgtcttcaccgtggttaccagaggcgcaggaattggtgggcttggcataactgttgagggaccatcagagtcgaagataaattgcagagacaacaaggatggcagctgcagtgctgagtacattcctttcgcaccgggggattacgatgttaatatcacatatggaggagcccacatccccggcagccccttcagggttcctgtgaaggatgttgtggaccccagcaaggtcaagattgccggccccgggctgggctcaggcgtccgagcccgtgtcctgcagtccttcacggtggacagcagcaaggctggcctggctccgctggaagtgagggttctgggcccacgagctgacgacacggattcccagtcatggcgcagccccttgaaagccctttcagagttctttaaaggtgacccgaagggtgactttaataagacaggcttggtggagccagtgaacgtggtggacaatggagatggcacacacacagtaacctacaccccatctcaggagggaccttacatggtctcagttaaatatgctgatgaagagattcctcgcagtcccttcaaggtcaaggtccttcccacatatgatgccagcaaagtgactgccagtggccccggccttagttcctatggtgtgcctgccagtctacctgtggactttgcaattgatgcccgagatgccggggaaggcctgcttgctgttcaaataacggaccaagaaggaaaacccaaaagagccattgtccatgacaataaagatggcacgtatgctgtcacctacatccccgacaagactgggcgctatatgattggagtcacctacgggggtgacgacatcccactttctccttatcgcatccgagccacacagacgggtgatgccagcaagtgcctggccacgggtcctggaatcgcctccactgtgaaaactggcgaagaagtaggctttgtggttgatgccaagactgccgggaagggtaaagtgacctgcacggttctgaccccagatggcactgaggccgaggccgatgtcattgagaatgaagatggaacctatgacatcttctacacagctgccaagccgggcacatatgtgatctatgtgcgcttcggtggtgttgatattcctaacagccccttcactgtcatggccacagatggggaagtcacagccgtggaggaggcaccggtaaatgcatgtccccctggattcaggccctgggtgaccgaagaggcctatgtcccagtgagtgacatgaacggcctgggatttaagccttttgacctggtcattccgtttgctgtcaggaaaggagaaatcactggagaggtccacatgccttctgggaagacagccacacctgagattgtggacaacaaggacggcacggtcactgttagatatgcccccactgaggtcgggctccatgagatgcacatcaaatacatgggcagccacatccctgagagcccactccagttctacgtgaactaccccaacagtggaagtgtttctgcatacggtccaggcctcgtgtatggagtggccaacaaaactgccaccttcaccatcgtcacagaggatgcaggagaaggtggtctggacttggctattgagggcccctcaaaagcagaaatcagctgcattgacaataaagatgggacatgcacagtgacctacctgccgactctgccaggcgactacagcattctggtcaagtacaatgacaagcacatccctggcagccccttcacagccaagatcacagatgacagcaggcggtgctcccaggtgaagttgggctcagccgctgacttcctgctcgacatcagtgagactgacctcagcagcctgacggccagcattaaggccccatctggccgagacgagccctgtctcctgaagaggctgcccaacaaccacattggcatctccttcatcccccgggaagtgggcgaacatctggtcagcatcaagaaaaatggcaaccatgtggccaacagccccgtgtctatcatggtggtccagtcggagattggtgacgcccgccgagccaaagtctatggccgcggcctgtcagaaggccggactttcgagatgtctgacttcatcgtggacacaagggatgcaggttatggtggcatatccttggcggtggaaggccccagcaaagtggacatccagacggaggacctggaagatggcacctgcaaagtctcctacttccctaccgtgcctggggtttatatcgtctccaccaaattcgctgacgagcacgtgcctgggagcccatttaccgtgaagatcagtggggagggaagagtcaaagagagcatcacccgcaccagtcgggccccgtccgtggccactgtcgggagcatttgtgacctgaacctgaaaatcccagaaatcaacagcagtgatatgtcggcccacgtcaccagcccctctggccgtgtgactgaggcagagattgtgcccatggggaagaactcacactgcgtccggtttgtgccccaggagatgggcgtgcacacggtcagcgtcaagtaccgtgggcagcacgtcaccggcagccccttccagttcaccgtggggccacttggtgaaggaggcgcccacaaggtgcgggcaggaggccctggcctggagagaggagaagcgggagtcccagctgagttcagcatttggacccgggaagcaggcgctggaggcctctccatcgctgttgagggccccagtaaggccgagattacattcgatgaccataaaaatgggtcgtgcggtgtatcttatattgcccaagagcctggtaactacgaggtgtccatcaagttcaatgatgagcacatcccggaaagcccctacctggtgccggtcatcgcaccctccgacgacgcccgccgcctcactgttatgagccttcaggaatcgggattaaaagttaaccagccagcatcctttgctataaggttgaatggcgcaaaaggcaagattgatgcaaaggtgcacagcccctctggagccgtggaggagtgccacgtgtctgagctggagccagataagtatgctgttcgcttcatccctcatgagaatggtgtccacaccatcgatgtcaagttcaatgggagccacgtggttggaagccccttcaaagtgcgcgttggggagcctggacaagcggggaaccctgccctggtgtccgcctatggcacgggactcgaagggggcaccacaggtatccagtcggaattctttattaacaccacccgagcaggtccagggacattatccgtcaccatcgaaggcccatccaaggttaaaatggattgccaggaaacacctgaagggtacaaagtcatgtacacccccatggctcctggtaactacctgatcagcgtcaaatacggtgggcccaaccacatcgtgggcagtcccttcaaggccaaggtgacaggccagcgtctagttagccctggctcagccaacgagacctcatccatcctggtggagtcagtgaccaggtcgtctacagagacctgctatagcgccattcccaaggcatcctcggacgccagcaaggtgacctctaagggggcagggctctcaaaggcctttgtgggccagaagagttccttcctggtggactgcagcaaagctggctccaacatgctgctgatcggggtccatgggcccaccaccccctgcgaggaggtctccatgaagcatgtaggcaaccagcaatacaacgtcacatacgtcgtcaaggagaggggcgattatgtgctggctgtgaagtggggggaggaacacatccctggcagcccttttcatgtcacagtgccttaaaacagttttctcaaatcctggagagagttcttgtggttgcttttgttgcttgtttgtaattcattttatacaaagccctccagcctgtttgtggggctgaaaccccatccctaaaatattgctgttgtaaaatgccttcagaaataagtcctagactggactcttgagggacatattggagaatcttaagaaatgcaagcttgttcagggggctgagaagatcctgagtacactaggtgcaaaccagaactcttggtggaacagaccagccactgcagcagacagaccaggaacacaatgagactgacatttcaaaaaaacaaaactggctagcctgagctgctggttcactcttcagcatttatgaaacaaggctaggggaagatgggcagagaaaaaggggacacctagtttggttgtcatttggcaaaggagatgacttaaaatccgcttaatctcttccagtgtccgtgttaatgtatttggctattagatcactagcactgctttaccgctcctcatcgccaacacccccatgctctgtggccttcttacacttctcagagggcagagtggcagccgggcaccctacagaaactcagagggcagagtggcagccaggcccacatgtctctcaagtacctgtcccctcgctctggtgattatttcttgcagaatcaccacacgagaccatcccggcagtcatggttttgctttagttttccaagtccgtttcagtcccttccttggtctgaagaaattctgcagtggcgagcagtttcccacttgccaaagatcccttttaaccaacactagcccttgtttttaacacacgctccagcccttcatcagcctgggcagtcttaccaaaatgtttaaagtgatctcagaggggcccatggattaacgccctcatcccaaggtccgtcccatgacataacactccacacccgccccagccaacttcatgggtcactttttctggaaaataatgatctgtacagacaggacagaatgaaactcctgcgggtctttggcctgaaagttgggaatggttgggggagagaagggcagcagcttattggtggtcttttcaccattggcagaaacagtgagagctgtgtggtgcagaaatccagaaatgaggtgtagggaattttgcctgccttcctgcagacctgagctggctttggaatgaggttaaagtgtcagggacgttgcctgagcccaaatgtgtagtgtggtctgggcaggcagacctttaggttttgctgcttagtcctgaggaagtggccactcttgtggcaggtgtagtatctggggcgagtgttgggggtaaaagcccaccctacagaaagtggaacagcccggagcctgatgtgaaaggaccacgggtgttgtaagctgggacacggaagccaaactggaatcaaacgccgactgtaaattgtatcttataacttattaaataaaacatttgctccgtaaagttg

SEQ ID NO: 24 - protein, 2591 aa, Homo sapiens
MPVTEKDLAEDAPWKKIQQNTFTRWCNEHLKCVNKRIGNLQTDLSDGLRLIALLEVLSQKRMYRKYHQRPTFRQMQLENVSVALEFLDRESIKLVSIDSKAIVDGNLKLILGLVWTLILHYSISMPVWEDEGDDDAKKQTPKQRLLGWIQNKIPYLPITNFNQNWQDGKALGALVDSCAPGLCPDWESWDPQKPVDNAREAMQQADDWLGVPQVITPEEIIHPDVDEHSVMTYLSQFPKAKLKPGAPLKPKLNPKKARAYGRGIEPTGNMVKQPAKFTVDTISAGQGDVMVFVEDPEGNKEEAQVTPDSDKNKTYSVEYLPKVTGLHKVTVLFAGQHISKSPFEVSVDKAQGDASKVTAKGPGLEAVGNIANKPTYFDIYTAGAGVGDIGVEVEDPQGKNTVELLVEDKGNQVYRCVYKPMQPGPHVVKIFFAGDTIPKSPFVVQVGEACNPNACRASGRGLQPKGVRIRETTDFKVDTKAAGSGELGVTMKGPKGLEELVKQKDFLDGVYAFEYYPSTPGRYSIAITWGGHHIPKSPFEVQVGPEAGMQKVRAWGPGLHGGIVGRSADFVVESIGSEVGSLGFAIEGPSQAKIEYNDQNDGSCDVKYWPKEPGEYAVHIMCDDEDIKDSPYMAFIHPATGGYNPDLVRAYGPGLEKSGCIVNNLAEFTVDPKDAGKAPLKIFAQDGEGQRIDIQMKNRMDGTYACSYTPVKAIKHTIAVVWGGVNIPHSPYRVNIGQGSHPQKVKVFGPGVERSGLKANEPTHFTVDCTEAGEGDVSVGIKCDARVLSEDEEDVDFDIIHNANDTFTVKYVPPAAGRYTIKVLFASQEIPASPFRVKVDPSHDASKVKAEGPGLSKAGVENGKPTHFTVYTKGAGKAPLNVQFNSPLPGDAVKDLDIIDNYDYSHTVKYTPTQQGNMQVLVTYGGDPIPKSPFTVGVAAPLDLSKIKLNGLENRVEVGKDQEFTVDTRGAGGQGKLDVTILSPSRKVVPCLVTPVTGRENSTAKFIPREEGLYAVDVTYDGHPVPGSPYTVEASLPPDPSKVKAHGPGLEGGLVGKPAEFTIDTKGAGTGGLGLTVEGPCEAKIECSDNGDGTCSVSYLPTKPGEYFVNILFEEVHIPGSPFKADIEMPFDPSKVVASGPGLEHGKVGEAGLLSVDCSEAGPGALGLEAVSDSGTKAEVSIQNNKDGTYAVTYVPLTAGMYTLTMKYGGELVPHFPARVKVEPAVDTSRIKVFGPGIEGKDVFREATTDFTVDSRPLTQVGGDHIKAHIANPSGASTECFVTDNADGTYQVEYTPFEKGLHVVEVTYDDVPIPNSPFKVAVTEGCQPSRVQAQGPGLKEAFTNKPNVFTVVTRGAGIGGLGITVEGPSESKINCRDNKDGSCSAEYIPFAPGDYDVNITYGGAHIPGSPFRVPVKDVVDPSKVKIAGPGLGSGVRARVLQSFTVDSSKAGLAPLEVRVLGPRGLVEPVNVVDNGDGTHTVTYTPSQEGPYMVSVKYADEEIPRSPFKVKVLPTYDASKVTASGPGLSSYGVPASLPVDFAIDARDAGEGLLAVQITDQEGKPKRAIVHDNKDGTYAVTYIPDKTGRYMIGVTYGGDDIPLSPYRIRATQTGDASKCLATGPGIASTVKTGEEVGFVVDAKTAGKGKVTCTVLTPDGTEAEADVIENEDGTYDIFYTAAKPGTYVIYVRFGGVDIPNSPFTVMATDGEVTAVEEAPVTEEAYVPVSDMNGLGFKPFDLVIPFAVRKGEITGEVHMPSGKTATPEIVDNKDGTVTVRYAPTEVGLHEMHIKYMGSHIPESPLQFYVNYPNSGSVSAYGPGLVYGVANKTATFTIVTEDAGEGGLDLAIEGPSKAEISCIDNKDGTCTVTYLPTLPGDYSILVKYNDKHIPGSPFTAKITDDSRRCSQVKLGSAADFLLDISETDLSSLTASIKAPSGRDEPCLLKRLPNNHIGISFIPREVGEHLVSIKKNGNHVANSPVSIMVVQSEIGDARRAKVYGRGLSEGRTFEMSDFIVDTRDAGYGGISLAVEGPSKVDIQTEDLEDGTCKVSYFPTVPGVYIVSTKFADEHVPGSPFTVKISGEGRVKESITRTSRAPSVATVGSICDLNLKIPEINSSDMSAHVTSPSGRVTEAEIVPMGKNSHCVRFVPQEMGVHTVSVKYRGQHVTGSPFQFTVGPLGEGGAHKVRAGGPGLERGEAGVPAEFSIWTREAGAGGLSIAVEGPSKAEITFDDHKNGSCGVSYIAQEPGNYEVSIKFNDEHIPESPYLVPVIAPSDDARRLTVMSLQESGLKVNQPASFAIRLNGAKGKIDAKVHSPSGAVEECHVSELEPDKYAVRFIPHENGVHTIDVKFNGSHVVGSPFKVRVGEPGQAGNPALVSAYGTGLEGGTTGIQSEFFINTTRAGPGTLSVTIEGPSKVKMDCQETPEGYKVMYTPMAPGNYLISVKYGGPNHIVGSPFKAKVTGQRLVSPGSANETSSILVESVTRSSTETCYSAIPKASSDASKVTSKGAGLSKAFVGQKSSFLVDCSKAGSNMLLIGVHGPTTPCEEVSMKHVGNQQYNVTYVVKERGDYVLAVKWGEEHIPGSPFHVTVP

SEQ ID NO: 25 - DNA, 9434 bp, Homo sapiens
gcggccaggggcgggcggccgcagagcagcaccggccgtggctccggtagcagcaagttcgaaccccgctcccgctccgcttcggttctcgctccttcggcccttgggcctccaaacaccagtccccggcagctcgttgcgcattgcgctctccccgccaccaggatgccggtaaccgagaaggatctagctgaggacgcgccttggaagaagatccagcagaacacgttcacacgctggtgcaacgagcacctcaagtgcgtgaacaaacgcatcggcaacctgcagaccgacctgagcgacgggctgcggctcatcgcgctgctcgaggtgctcagccagaagcgcatgtaccgcaagtaccatcagcggcccacctttcgccagatgcagctcgagaatgtgtccgtggcgctcgagttcctggaccgtgagagcatcaagctcgtgtccatcgatagcaaagccattgtggatgggaacctgaagctcatcttgggtctggtgtggacgctgatcctccactactccatctccatgcccgtgtgggaggatgaaggggatgatgatgccaagaagcagacgccaaagcagaggctgctggggtggattcagaacaagatcccctacttgcccatcaccaactttaaccagaactggcaagacggcaaagccctgggagccctggtagacagctgtgctccaggtctgtgcccagactgggaatcctgggacccgcagaagcctgtggataatgcacgagaagccatgcagcaggcagatgactggctgggtgtcccacaggtcatcactcctgaagaaatcattcacccggatgtggacgagcactcagttatgacttacctgtcccagttccccaaagccaagctcaagccgggggctcctctcaaacccaaactcaacccgaagaaagccagggcctatggcagaggaatcgagcccactggaaacatggtgaagcagccagccaagttcactgtggacaccatcagcgccgggcaaggagacgtgatggtgtttgttgaggacccagaagggaacaaagaggaggcacaagtgacccctgacagtgacaagaacaagacatactctgtggagtatctgcccaaggtcaccgggctacacaaagtcacagtcctctttgcaggacagcacatctccaagagcccatttgaagtgagtgttgacaaggcccagggagatgccagtaaagtcactgcaaaaggtccagggttggaagctgtagggaacatcgccaataagcccacctactttgacatctatacggcaggagctggtgtgggtgacattggtgtggaggtggaagatccccaggggaagaacaccgtggagttgctcgtggaagacaaaggaaaccaggtgtatcgatgtgtgtacaaacccatgcagcctggccctcacgtggtcaagatcttctttgctggggacactattcctaagagtcccttcgttgtgcaggttggggaagcctgcaatccaaatgcctgccgggccagtggccgaggcctacaacccaaaggcgtccgtatccgggagaccacagatttcaaggttgacaccaaagctgcaggaagtggggagctcggtgtaaccatgaagggtcctaagggtctggaggagctggtgaagcagaaagactttctggatggggtctacgcattcgagtattaccccagcaccccggggagatacagcattgccatcacatgggggggacaccacattccaaagagcccctttgaagttcaagttggccctgaagcgggtatgcagaaagtccgtgcttggggccctgggctccatggtgggattgtcgggcggtcagcggacttcgtggtagaatccattggctctgaagtggggtctctggggtttgccattgaaggcccctctcaggcaaagattgagtacaacgaccagaatgatggatcgtgtgatgtcaaatactggcccaaggagcctggcgaatatgctgttcacatcatgtgtgacgacgaagacatcaaggacagcccgtacatggccttcatccacccagccacgggaggctacaaccctgatctggttcgagcatacgggccaggtttggagaaatctggatgcattgtcaacaacctggccgagttcactgtggatcctaaggatgctggaaaagctcccttaaagatatttgctcaggatggggaaggccaacgcattgacatccagatgaagaaccggatggacggcacatatgcatgctcatacaccccggtgaaggccatcaagcacaccattgctgtggtctggggaggcgtgaacatcccgcacagcccctacagggtcaacatcgggcaaggtagccatcctcagaaggtcaaagtgtttgggccaggtgtggagagaagtggtctgaaggcaaatgaacctacacacttcacggtggactgtactgaggctggggaaggtgatgtcagtgttggcattaagtgtgatgcccgggtgttaagtgaagatgaggaagacgtggattttgacattattcacaatgccaatgatacgttcacagtcaaatatgtgcctcctgctgctgggcgatacactatcaaagttctctttgcatctcaggaaatccccgccagccctttcagagtcaaagttgacccttcccacgatgccagcaaagtgaaggcagaaggcccagggctcagcaaagcaggtgtggaaaatgggaaaccgacccacttcactgtctacaccaagggggctgggaaagccccgctcaacgtgcagttcaacagccctcttcctggcgatgcagtgaaggatttggatatcatcgataattatgactactctcacacggttaaatatacacccacccaacagggcaacatgcaggttctggtgacttacggtggcgatcccatccctaaaagccctttcactgtgggtgttgctgcaccgctggatctgagcaagataaaactcaatgggctggaaaacagggtggaagttgggaaggatcaggagttcaccgttgataccaggggggcaggaggccaggggaagctggacgtgacaatcctcagcccctctcggaaggtcgtgccatgcctagtgacacctgtgacaggccgggagaacagcacggccaagttcatccctcgggaggaggggctgtatgctgtagacgtgacctacgatggacaccctgtgcccgggagcccctacacagtggaggcctcgctgccaccagatcccagcaaggtgaaggcccacggtcccggcctcgaaggtggtctcgtgggcaagcctgccgagttcaccatcgataccaaaggagctggtactggaggtctgggcttaacggtggaaggtccgtgcgaggccaaaatcgagtgctccgacaatggtgatgggacctgctccgtctcttaccttcccacaaaacccggggagtacttcgtcaacatcctctttgaagaagtccacatacctgggtctcccttcaaagctgacattgaaatgccctttgacccctctaaagtcgtggcatcggggccaggtctcgagcacgggaaggtgggtgaagctggcctccttagcgtcgactgctcggaagcgggaccgggggccctgggcctggaagctgtctcggactcgggaacaaaagccgaagtcagtattcagaacaacaaagatggcacctacgcggtgacctacgtgcccctgacggccggcatgtacacgttgaccatgaagtatggtggcgaactcgtgccacacttccccgcccgggtcaaggtggagcccgccgtggacaccagcaggatcaaagtctttggaccaggaatagaagggaaagatgtgttccgggaagctaccaccgactttacagttgactctcggccgctgacccaggttgggggtgaccacatcaaggcccacattgccaacccctcaggggcctccaccgagtgctttgtcacagacaatgcggatgggacctaccaggtggaatacacaccctttgagaaaggtctccatgtagtggaggtgacatatgatgacgtgcctatcccaaacagtcccttcaaggtggctgtcactgaaggctgccagccatctagggtgcaagcccaaggacctggattgaaagaggcctttaccaacaagcccaatgtcttcaccgtggttaccagaggcgcaggaattggtgggcttggcataactgttgagggaccatcagagtcgaagataaattgcagagacaacaaggatggcagctgcagtgctgagtacattcctttcgcaccgggggattacgatgttaatatcacatatggaggagcccacatccccggcagccccttcagggttcctgtgaaggatgttgtggaccccagcaaggtcaagattgccggccccgggctgggctcaggcgtccgagcccgtgtcctgcagtccttcacggtggacagcagcaaggctggcctggctccgctggaagtgagggttctgggcccacgaggcttggtggagccagtgaacgtggtggacaatggagatggcacacacacagtaacctacaccccatctcaggagggaccttacatggtctcagttaaatatgctgatgaagagattcctcgcagtcccttcaaggtcaaggtccttcccacatatgatgccagcaaagtgactgccagtggccccggccttagttcctatggtgtgcctgccagtctacctgtggactttgcaattgatgcccgagatgccggggaaggcctgcttgctgttcaaataacggaccaagaaggaaaacccaaaagagccattgtccatgacaataaagatggcacgtatgctgtcacctacatccccgacaagactgggcgctatatgattggagtcacctacgggggtgacgacatcccactttctccttatcgcatccgagccacacagacgggtgatgccagcaagtgcctggccacgggtcctggaatcgcctccactgtgaaaactggcgaagaagtaggctttgtggttgatgccaagactgccgggaagggtaaagtgacctgcacggttctgaccccagatggcactgaggccgaggccgatgtcattgagaatgaagatggaacctatgacatcttctacacagctgccaagccgggcacatatgtgatctatgtgcgcttcggtggtgttgatattcctaacagccccttcactgtcatggccacagatggggaagtcacagccgtggaggaggcaccggtgaccgaagaggcctatgtcccagtgagtgacatgaacggcctgggatttaagccttttgacctggtcattccgtttgctgtcaggaaaggagaaatcactggagaggtccacatgccttctgggaagacagccacacctgagattgtggacaacaaggacggcacggtcactgttagatatgcccccactgaggtcgggctccatgagatgcacatcaaatacatgggcagccacatccctgagagcccactccagttctacgtgaactaccccaacagtggaagtgtttctgcatacggtccaggcctcgtgtatggagtggccaacaaaactgccaccttcaccatcgtcacagaggatgcaggagaaggtggtctggacttggctattgagggcccctcaaaagcagaaatcagctgcattgacaataaagatgggacatgcacagtgacctacctgccgactctgccaggcgactacagcattctggtcaagtacaatgacaagcacatccctggcagccccttcacagccaagatcacagatgacagcaggcggtgctcccaggtgaagttgggctcagccgctgacttcctgctcgacatcagtgagactgacctcagcagcctgacggccagcattaaggccccatctggccgagacgagccctgtctcctgaagaggctgcccaacaaccacattggcatctccttcatcccccgggaagtgggcgaacatctggtcagcatcaagaaaaatggcaaccatgtggccaacagccccgtgtctatcatggtggtccagtcggagattggtgacgcccgccgagccaaagtctatggccgcggcctgtcagaaggccggactttcgagatgtctgacttcatcgtggacacaagggatgcaggttatggtggcatatccttggcggtggaaggccccagcaaagtggacatccagacggaggacctggaagatggcacctgcaaagtctcctacttccctaccgtgcctggggtttatatcgtctccaccaaattcgctgacgagcacgtgcctgggagcccatttaccgtgaagatcagtggggagggaagagtcaaagagagcatcacccgcaccagtcgggccccgtccgtggccactgtcgggagcatttgtgacctgaacctgaaaatcccagaaatcaacagcagtgatatgtcggcccacgtcaccagcccctctggccgtgtgactgaggcagagattgtgcccatggggaagaactcacactgcgtccggtttgtgccccaggagatgggcgtgcacacggtcagcgtcaagtaccgtgggcagcacgtcaccggcagccccttccagttcaccgtggggccacttggtgaaggaggcgcccacaaggtgcgggcaggaggccctggcctggagagaggagaagcgggagtcccagctgagttcagcatttggacccgggaagcaggcgctggaggcctctccatcgctgttgagggccccagtaaggccgagattacattcgatgaccataaaaatgggtcgtgcggtgtatcttatattgcccaagagcctggtaactacgaggtgtccatcaagttcaatgatgagcacatcccggaaagcccctacctggtgccggtcatcgcaccctccgacgacgcccgccgcctcactgttatgagccttcaggaatcgggattaaaagttaaccagccagcatcctttgctataaggttgaatggcgcaaaaggcaagattgatgcaaaggtgcacagcccctctggagccgtggaggagtgccacgtgtctgagctggagccagataagtatgctgttcgcttcatccctcatgagaatggtgtccacaccatcgatgtcaagttcaatgggagccacgtggttggaagccccttcaaagtgcgcgttggggagcctggacaagcggggaaccctgccctggtgtccgcctatggcacgggactcgaagggggcaccacaggtatccagtcggaattctttattaacaccacccgagcaggtccagggacattatccgtcaccatcgaaggcccatccaaggttaaaatggattgccaggaaacacctgaagggtacaaagtcatgtacacccccatggctcctggtaactacctgatcagcgtcaaatacggtgggcccaaccacatcgtgggcagtcccttcaaggccaaggtgacaggccagcgtctagttagccctggctcagccaacgagacctcatccatcctggtggagtcagtgaccaggtcgtctacagagacctgctatagcgccattcccaaggcatcctcggacgccagcaaggtgacctctaagggggcagggctctcaaaggcctttgtgggccagaagagttccttcctggtggactgcagcaaagctggctccaacatgctgctgatcggggtccatgggcccaccaccccctgcgaggaggtctccatgaagcatgtaggcaaccagcaatacaacgtcacatacgtcgtcaaggagaggggcgattatgtgctggctgtgaagtggggggaggaacacatccctggcagcccttttcatgtcacagtgccttaaaacagttttctcaaatcctggagagagttcttgtggttgcttttgttgcttgtttgtaattcattttatacaaagccctccagcctgtttgtggggctgaaaccccatccctaaaatattgctgttgtaaaatgccttcagaaataagtcctagactggactcttgagggacatattggagaatcttaagaaatgcaagcttgttcagggggctgagaagatcctgagtacactaggtgcaaaccagaactcttggtggaacagaccagccactgcagcagacagaccaggaacacaatgagactgacatttcaaaaaaacaaaactggctagcctgagctgctggttcactcttcagcatttatgaaacaaggctaggggaagatgggcagagaaaaaggggacacctagtttggttgtcatttggcaaaggagatgacttaaaatccgcttaatctcttccagtgtccgtgttaatgtatttggctattagatcactagcactgctttaccgctcctcatcgccaacacccccatgctctgtggccttcttacacttctcagagggcagagtggcagccgggcaccctacagaaactcagagggcagagtggcagccaggcccacatgtctctcaagtacctgtcccctcgctctggtgattatttcttgcagaatcaccacacgagaccatcccggcagtcatggttttgctttagttttccaagtccgtttcagtcccttccttggtctgaagaaattctgcagtggcgagcagtttcccacttgccaaagatcccttttaaccaacactagcccttgtttttaacacacgctccagcccttcatcagcctgggcagtcttaccaaaatgtttaaagtgatctcagaggggcccatggattaacgccctcatcccaaggtccgtcccatgacataacactccacacccgccccagccaacttcatgggtcactttttctggaaaataatgatctgtacagacaggacagaatgaaactcctgcgggtctttggcctgaaagttgggaatggttgggggagagaagggcagcagcttattggtggtcttttcaccattggcagaaacagtgagagctgtgtggtgcagaaatccagaaatgaggtgtagggaattttgcctgccttcctgcagacctgagctggctttggaatgaggttaaagtgtcagggacgttgcctgagcccaaatgtgtagtgtggtctgggcaggcagacctttaggttttgctgcttagtcctgaggaagtggccactcttgtggcaggtgtagtatctggggcgagtgttgggggtaaaagcccaccctacagaaagtggaacagcccggagcctgatgtgaaaggaccacgggtgttgtaagctgggacacggaagccaaactggaatcaaacgccgactgtaaattgtatcttataacttattaaataaaacatttgctccgtaaagttg

SEQ ID NO: 26 - protein, 2578 aa, Homo sapiens
MPVTEKDLAEDAPWKKIQQNTFTRWCNEHLKCVNKRIGNLQTDLSDGLRLIALLEVLSQKRMYRKYHQRPTFRQMQLENVSVALEFLDRESIKLVSIDSKAIVDGNLKLILGLVWTLILHYSISMPVWEDEGDDDAKKQTPKQRLLGWIQNKIPYLPITNFNQNWQDGKALGALVDSCAPGLCPDWESWDPQKPVDNAREAMQQADDWLGVPQVITPEEIIHPDVDEHSVMTYLSQFPKAKLKPGAPLKPKLNPKKARAYGRGIEPTGNMVKQPAKFTVDTISAGQGDVMVFVEDPEGNKEEAQVTPDSDKNKTYSVEYLPKVTGLHKVTVLFAGQHISKSPFEVSVDKAQGDASKVTAKGPGLEAVGNIANKPTYFDIYTAGAGVGDIGVEVEDPQGKNTVELLVEDKGNQVYRCVYKPMQPGPHVVKIFFAGDTIPKSPFVVQVGEACNPNACRASGRGLQPKGVRIRETTDFKVDTKAAGSGELGVTMKGPKGLEELVKQKDFLDGVYAFEYYPSTPGRYSIAITWGGHHIPKSPFEVQVGPEAGMQKVRAWGPGLHGGIVGRSADFVVESIGSEVGSLGFAIEGPSQAKIEYNDQNDGSCDVKYWPKEPGEYAVHIMCDDEDIKDSPYMAFIHPATGGYNPDLVRAYGPGLEKSGCIVNNLAEFTVDPKDAGKAPLKIFAQDGEGQRIDIQMKNRMDGTYACSYTPVKAIKHTIAVVWGGVNIPHSPYRVNIGQGSHPQKVKVFGPGVERSGLKANEPTHFTVDCTEAGEGDVSVGIKCDARVLSEDEEDVDFDIIHNANDTFTVKYVPPAAGRYTIKVLFASQEIPASPFRVKVDPSHDASKVKAEGPGLSKAGVENGKPTHFTVYTKGAGKAPLNVQFNSPLPGDAVKDLDIIDNYDYSHTVKYTPTQQGNMQVLVTYGGDPIPKSPFTVGVAAPLDLSKIKLNGLENRVEVGKDQEFTVDTRGAGGQGKLDVTILSPSRKVVPCLVTPVTGRENSTAKFIPREEGLYAVDVTYDGHPVPGSPYTVEASLPPDPSKVKAHGPGLEGGLVGKPAEFTIDTKGAGTGGLGLTVEGPCEAKIECSDNGDGTCSVSYLPTKPGEYFVNILFEEVHIPGSPFKADIEMPFDPSKVVASGPGLEHGKVGEAGLLSVDCSEAGPGALGLEAVSDSGTKAEVSIQNNKDGTYAVTYVPLTAGMYTLTMKYGGELVPHFPARVKVEPAVDTSRIKVFGPGIEGKDVFREATTDFTVDSRPLTQVGGDHIKAHIANPSGASTECFVTDNADGTYQVEYTPFEKGLHVVEVTYDDVPIPNSPFKVAVTEGCQPSRVQAQGPGLKEAFTNKPNVFTVVTRGAGIGGLGITVEGPSESKINCRDNKDGSCSAEYIPFAPGDYDVNITYGGAHIPGSPFRVPVKDVVDPSKVKIAGPGLGSGVRARVLQSFTVDSSKAGLAPLEVRVLGPRGLVEPVNVVDNGDGTHTVTYTPSQEGPYMVSVKYADEEIPRSPFKVKVLPTYDASKVTASGPGLSSYGVPASLPVDFAIDARDAGEGLLAVQITDQEGKPKRAIVHDNKDGTYAVTYIPDKTGRYMIGVTYGGDDIPLSPYRIRATQTGDASKCLATGPGIASTVKTGEEVGFVVDAKTAGKGKVTCTVLTPDGTEAEADVIENEDGTYDIFYTAAKPGTYVIYVRFGGVDIPNSPFTVMVTEEAYVPVSDMNGLGFKPFDLVIPFAVRKGEITGEVHMPSGKTATPEIVDNKDGTVTVRYAPTEVGLHEMHIKYMGSHIPESPLQFYVNYPNSGSVSAYGPGLVYGVANKTATFTIVTEDAGEGGLDLAIEGPSKAEISCIDNKDGTCTVTYLPTLPGDYSILVKYNDKHIPGSPFTAKITDDSRRCSQVKLGSAADFLLDISETDLSSLTASIKAPSGRDEPCLLKRLPNNHIGISFIPREVGEHLVSIKKNGNHVANSPVSIMVVQSEIGDARRAKVYGRGLSEGRTFEMSDFIVDTRDAGYGGISLAVEGPSKVDIQTEDLEDGTCKVSYFPTVPGVYIVSTKFADEHVPGSPFTVKISGEGRVKESITRTSRAPSVATVGSICDLNLKIPEINSSDMSAHVTSPSGRVTEAEIVPMGKNSHCVRFVPQEMGVHTVSVKYRGQHVTGSPFQFTVGPLGEGGAHKVRAGGPGLERGEAGVPAEFSIWTREAGAGGLSIAVEGPSKAEITFDDHKNGSCGVSYIAQEPGNYEVSIKFNDEHIPESPYLVPVIAPSDDARRLTVMSLQESGLKVNQPASFAIRLNGAKGKIDAKVHSPSGAVEECHVSELEPDKYAVRFIPHENGVHTIDVKFNGSHVVGSPFKVRVGEPGQAGNPALVSAYGTGLEGGTTGIQSEFFINTTRAGPGTLSVTIEGPSKVKMDCQETPEGYKVMYTPMAPGNYLISVKYGGPNHIVGSPFKAKVTGQRLVSPGSANETSSILVESVTRSSTETCYSAIPKASSDASKVTSKGAGLSKAFVGQKSSFLVDCSKAGSNMLLIGVHGPTTPCEEVSMKHVGNQQYNVTYVVKERGDYVLAVKWGEEHIPGSPFHVTVP

SEQ ID NO: 27 - DNA, 9395 bp, Homo sapiens
gcggccaggggcgggcggccgcagagcagcaccggccgtggctccggtagcagcaagttcgaaccccgctcccgctccgcttcggttctcgctccttcggcccttgggcctccaaacaccagtccccggcagctcgttgcgcattgcgctctccccgccaccaggatgccggtaaccgagaaggatctagctgaggacgcgccttggaagaagatccagcagaacacgttcacacgctggtgcaacgagcacctcaagtgcgtgaacaaacgcatcggcaacctgcagaccgacctgagcgacgggctgcggctcatcgcgctgctcgaggtgctcagccagaagcgcatgtaccgcaagtaccatcagcggcccacctttcgccagatgcagctcgagaatgtgtccgtggcgctcgagttcctggaccgtgagagcatcaagctcgtgtccatcgatagcaaagccattgtggatgggaacctgaagctcatcttgggtctggtgtggacgctgatcctccactactccatctccatgcccgtgtgggaggatgaaggggatgatgatgccaagaagcagacgccaaagcagaggctgctggggtggattcagaacaagatcccctacttgcccatcaccaactttaaccagaactggcaagacggcaaagccctgggagccctggtagacagctgtgctccaggtctgtgcccagactgggaatcctgggacccgcagaagcctgtggataatgcacgagaagccatgcagcaggcagatgactggctgggtgtcccacaggtcatcactcctgaagaaatcattcacccggatgtggacgagcactcagttatgacttacctgtcccagttccccaaagccaagctcaagccgggggctcctctcaaacccaaactcaacccgaagaaagccagggcctatggcagaggaatcgagcccactggaaacatggtgaagcagccagccaagttcactgtggacaccatcagcgccgggcaaggagacgtgatggtgtttgttgaggacccagaagggaacaaagaggaggcacaagtgacccctgacagtgacaagaacaagacatactctgtggagtatctgcccaaggtcaccgggctacacaaagtcacagtcctctttgcaggacagcacatctccaagagcccatttgaagtgagtgttgacaaggcccagggagatgccagtaaagtcactgcaaaaggtccagggttggaagctgtagggaacatcgccaataagcccacctactttgacatctatacggcaggagctggtgtgggtgacattggtgtggaggtggaagatccccaggggaagaacaccgtggagttgctcgtggaagacaaaggaaaccaggtgtatcgatgtgtgtacaaacccatgcagcctggccctcacgtggtcaagatcttctttgctggggacactattcctaagagtcccttcgttgtgcaggttggggaagcctgcaatccaaatgcctgccgggccagtggccgaggcctacaacccaaaggcgtccgtatccgggagaccacagatttcaaggttgacaccaaagctgcaggaagtggggagctcggtgtaaccatgaagggtcctaagggtctggaggagctggtgaagcagaaagactttctggatggggtctacgcattcgagtattaccccagcaccccggggagatacagcattgccatcacatgggggggacaccacattccaaagagcccctttgaagttcaagttggccctgaagcgggtatgcagaaagtccgtgcttggggccctgggctccatggtgggattgtcgggcggtcagcggacttcgtggtagaatccattggctctgaagtggggtctctggggtttgccattgaaggcccctctcaggcaaagattgagtacaacgaccagaatgatggatcgtgtgatgtcaaatactggcccaaggagcctggcgaatatgctgttcacatcatgtgtgacgacgaagacatcaaggacagcccgtacatggccttcatccacccagccacgggaggctacaaccctgatctggttcgagcatacgggccaggtttggagaaatctggatgcattgtcaacaacctggccgagttcactgtggatcctaaggatgctggaaaagctcccttaaagatatttgctcaggatggggaaggccaacgcattgacatccagatgaagaaccggatggacggcacatatgcatgctcatacaccccggtgaaggccatcaagcacaccattgctgtggtctggggaggcgtgaacatcccgcacagcccctacagggtcaacatcgggcaaggtagccatcctcagaaggtcaaagtgtttgggccaggtgtggagagaagtggtctgaaggcaaatgaacctacacacttcacggtggactgtactgaggctggggaaggtgatgtcagtgttggcattaagtgtgatgcccgggtgttaagtgaagatgaggaagacgtggattttgacattattcacaatgccaatgatacgttcacagtcaaatatgtgcctcctgctgctgggcgatacactatcaaagttctctttgcatctcaggaaatccccgccagccctttcagagtcaaagttgacccttcccacgatgccagcaaagtgaaggcagaaggcccagggctcagcaaagcaggtgtggaaaatgggaaaccgacccacttcactgtctacaccaagggggctgggaaagccccgctcaacgtgcagttcaacagccctcttcctggcgatgcagtgaaggatttggatatcatcgataattatgactactctcacacggttaaatatacacccacccaacagggcaacatgcaggttctggtgacttacggtggcgatcccatccctaaaagccctttcactgtgggtgttgctgcaccgctggatctgagcaagataaaactcaatgggctggaaaacagggtggaagttgggaaggatcaggagttcaccgttgataccaggggggcaggaggccaggggaagctggacgtgacaatcctcagcccctctcggaaggtcgtgccatgcctagtgacacctgtgacaggccgggagaacagcacggccaagttcatccctcgggaggaggggctgtatgctgtagacgtgacctacgatggacaccctgtgcccgggagcccctacacagtggaggcctcgctgccaccagatcccagcaaggtgaaggcccacggtcccggcctcgaaggtggtctcgtgggcaagcctgccgagttcaccatcgataccaaaggagctggtactggaggtctgggcttaacggtggaaggtccgtgcgaggccaaaatcgagtgctccgacaatggtgatgggacctgctccgtctcttaccttcccacaaaacccggggagtacttcgtcaacatcctctttgaagaagtccacatacctgggtctcccttcaaagctgacattgaaatgccctttgacccctctaaagtcgtggcatcggggccaggtctcgagcacgggaaggtgggtgaagctggcctccttagcgtcgactgctcggaagcgggaccgggggccctgggcctggaagctgtctcggactcgggaacaaaagccgaagtcagtattcagaacaacaaagatggcacctacgcggtgacctacgtgcccctgacggccggcatgtacacgttgaccatgaagtatggtggcgaactcgtgccacacttccccgcccgggtcaaggtggagcccgccgtggacaccagcaggatcaaagtctttggaccaggaatagaagggaaagatgtgttccgggaagctaccaccgactttacagttgactctcggccgctgacccaggttgggggtgaccacatcaaggcccacattgccaacccctcaggggcctccaccgagtgctttgtcacagacaatgcggatgggacctaccaggtggaatacacaccctttgagaaaggtctccatgtagtggaggtgacatatgatgacgtgcctatcccaaacagtcccttcaaggtggctgtcactgaaggctgccagccatctagggtgcaagcccaaggacctggattgaaagaggcctttaccaacaagcccaatgtcttcaccgtggttaccagaggcgcaggaattggtgggcttggcataactgttgagggaccatcagagtcgaagataaattgcagagacaacaaggatggcagctgcagtgctgagtacattcctttcgcaccgggggattacgatgttaatatcacatatggaggagcccacatccccggcagccccttcagggttcctgtgaaggatgttgtggaccccagcaaggtcaagattgccggccccgggctgggctcaggcgtccgagcccgtgtcctgcagtccttcacggtggacagcagcaaggctggcctggctccgctggaagtgagggttctgggcccacgaggcttggtggagccagtgaacgtggtggacaatggagatggcacacacacagtaacctacaccccatctcaggagggaccttacatggtctcagttaaatatgctgatgaagagattcctcgcagtcccttcaaggtcaaggtccttcccacatatgatgccagcaaagtgactgccagtggccccggccttagttcctatggtgtgcctgccagtctacctgtggactttgcaattgatgcccgagatgccggggaaggcctgcttgctgttcaaataacggaccaagaaggaaaacccaaaagagccattgtccatgacaataaagatggcacgtatgctgtcacctacatccccgacaagactgggcgctatatgattggagtcacctacgggggtgacgacatcccactttctccttatcgcatccgagccacacagacgggtgatgccagcaagtgcctggccacgggtcctggaatcgcctccactgtgaaaactggcgaagaagtaggctttgtggttgatgccaagactgccgggaagggtaaagtgacctgcacggttctgaccccagatggcactgaggccgaggccgatgtcattgagaatgaagatggaacctatgacatcttctacacagctgccaagccgggcacatatgtgatctatgtgcgcttcggtggtgttgatattcctaacagccccttcactgtcatggtgaccgaagaggcctatgtcccagtgagtgacatgaacggcctgggatttaagccttttgacctggtcattccgtttgctgtcaggaaaggagaaatcactggagaggtccacatgccttctgggaagacagccacacctgagattgtggacaacaaggacggcacggtcactgttagatatgcccccactgaggtcgggctccatgagatgcacatcaaatacatgggcagccacatccctgagagcccactccagttctacgtgaactaccccaacagtggaagtgtttctgcatacggtccaggcctcgtgtatggagtggccaacaaaactgccaccttcaccatcgtcacagaggatgcaggagaaggtggtctggacttggctattgagggcccctcaaaagcagaaatcagctgcattgacaataaagatgggacatgcacagtgacctacctgccgactctgccaggcgactacagcattctggtcaagtacaatgacaagcacatccctggcagccccttcacagccaagatcacagatgacagcaggcggtgctcccaggtgaagttgggctcagccgctgacttcctgctcgacatcagtgagactgacctcagcagcctgacggccagcattaaggccccatctggccgagacgagccctgtctcctgaagaggctgcccaacaaccacattggcatctccttcatcccccgggaagtgggcgaacatctggtcagcatcaagaaaaatggcaaccatgtggccaacagccccgtgtctatcatggtggtccagtcggagattggtgacgcccgccgagccaaagtctatggccgcggcctgtcagaaggccggactttcgagatgtctgacttcatcgtggacacaagggatgcaggttatggtggcatatccttggcggtggaaggccccagcaaagtggacatccagacggaggacctggaagatggcacctgcaaagtctcctacttccctaccgtgcctggggtttatatcgtctccaccaaattcgctgacgagcacgtgcctgggagcccatttaccgtgaagatcagtggggagggaagagtcaaagagagcatcacccgcaccagtcgggccccgtccgtggccactgtcgggagcatttgtgacctgaacctgaaaatcccagaaatcaacagcagtgatatgtcggcccacgtcaccagcccctctggccgtgtgactgaggcagagattgtgcccatggggaagaactcacactgcgtccggtttgtgccccaggagatgggcgtgcacacggtcagcgtcaagtaccgtgggcagcacgtcaccggcagccccttccagttcaccgtggggccacttggtgaaggaggcgcccacaaggtgcgggcaggaggccctggcctggagagaggagaagcgggagtcccagctgagttcagcatttggacccgggaagcaggcgctggaggcctctccatcgctgttgagggccccagtaaggccgagattacattcgatgaccataaaaatgggtcgtgcggtgtatcttatattgcccaagagcctggtaactacgaggtgtccatcaagttcaatgatgagcacatcccggaaagcccctacctggtgccggtcatcgcaccctccgacgacgcccgccgcctcactgttatgagccttcaggaatcgggattaaaagttaaccagccagcatcctttgctataaggttgaatggcgcaaaaggcaagattgatgcaaaggtgcacagcccctctggagccgtggaggagtgccacgtgtctgagctggagccagataagtatgctgttcgcttcatccctcatgagaatggtgtccacaccatcgatgtcaagttcaatgggagccacgtggttggaagccccttcaaagtgcgcgttggggagcctggacaagcggggaaccctgccctggtgtccgcctatggcacgggactcgaagggggcaccacaggtatccagtcggaattctttattaacaccacccgagcaggtccagggacattatccgtcaccatcgaaggcccatccaaggttaaaatggattgccaggaaacacctgaagggtacaaagtcatgtacacccccatggctcctggtaactacctgatcagcgtcaaatacggtgggcccaaccacatcgtgggcagtcccttcaaggccaaggtgacaggccagcgtctagttagccctggctcagccaacgagacctcatccatcctggtggagtcagtgaccaggtcgtctacagagacctgctatagcgccattcccaaggcatcctcggacgccagcaaggtgacctctaagggggcagggctctcaaaggcctttgtgggccagaagagttccttcctggtggactgcagcaaagctggctccaacatgctgctgatcggggtccatgggcccaccaccccctgcgaggaggtctccatgaagcatgtaggcaaccagcaatacaacgtcacatacgtcgtcaaggagaggggcgattatgtgctggctgtgaagtggggggaggaacacatccctggcagcccttttcatgtcacagtgccttaaaacagttttctcaaatcctggagagagttcttgtggttgcttttgttgcttgtttgtaattcattttatacaaagccctccagcctgtttgtggggctgaaaccccatccctaaaatattgctgttgtaaaatgccttcagaaataagtcctagactggactcttgagggacatattggagaatcttaagaaatgcaagcttgttcagggggctgagaagatcctgagtacactaggtgcaaaccagaactcttggtggaacagaccagccactgcagcagacagaccaggaacacaatgagactgacatttcaaaaaaacaaaactggctagcctgagctgctggttcactcttcagcatttatgaaacaaggctaggggaagatgggcagagaaaaaggggacacctagtttggttgtcatttggcaaaggagatgacttaaaatccgcttaatctcttccagtgtccgtgttaatgtatttggctattagatcactagcactgctttaccgctcctcatcgccaacacccccatgctctgtggccttcttacacttctcagagggcagagtggcagccgggcaccctacagaaactcagagggcagagtggcagccaggcccacatgtctctcaagtacctgtcccctcgctctggtgattatttcttgcagaatcaccacacgagaccatcccggcagtcatggttttgctttagttttccaagtccgtttcagtcccttccttggtctgaagaaattctgcagtggcgagcagtttcccacttgccaaagatcccttttaaccaacactagcccttgtttttaacacacgctccagcccttcatcagcctgggcagtcttaccaaaatgtttaaagtgatctcagaggggcccatggattaacgccctcatcccaaggtccgtcccatgacataacactccacacccgccccagccaacttcatgggtcactttttctggaaaataatgatctgtacagacaggacagaatgaaactcctgcgggtctttggcctgaaagttgggaatggttgggggagagaagggcagcagcttattggtggtcttttcaccattggcagaaacagtgagagctgtgtggtgcagaaatccagaaatgaggtgtagggaattttgcctgccttcctgcagacctgagctggctttggaatgaggttaaagtgtcagggacgttgcctgagcccaaatgtgtagtgtggtctgggcaggcagacctttaggttttgctgcttagtcctgaggaagtggccactcttgtggcaggtgtagtatctggggcgagtgttgggggtaaaagcccaccctacagaaagtggaacagcccggagcctgatgtgaaaggaccacgggtgttgtaagctgggacacggaagccaaactggaatcaaacgccgactgtaaattgtatcttataacttattaaataaaacatttgctccgtaaagttg

SEQ ID NO: 28 - protein, 2602 aa, Homo sapiens
MPVTEKDLAEDAPWKKIQQNTFTRWCNEHLKCVNKRIGNLQTDLSDGLRLIALLEVLSQKRMYRKYHQRPTFRQMQLENVSVALEFLDRESIKLVSIDSKAIVDGNLKLILGLVWTLILHYSISMPVWEDEGDDDAKKQTPKQRLLGWIQNKIPYLPITNFNQNWQDGKALGALVDSCAPGLCPDWESWDPQKPVDNAREAMQQADDWLGVPQVITPEEIIHPDVDEHSVMTYLSQFPKAKLKPGAPLKPKLNPKKARAYGRGIEPTGNMVKQPAKFTVDTISAGQGDVMVFVEDPEGNKEEAQVTPDSDKNKTYSVEYLPKVTGLHKVTVLFAGQHISKSPFEVSVDKAQGDASKVTAKGPGLEAVGNIANKPTYFDIYTAGAGVGDIGVEVEDPQGKNTVELLVEDKGNQVYRCVYKPMQPGPHVVKIFFAGDTIPKSPFVVQVGEACNPNACRASGRGLQPKGVRIRETTDFKVDTKAAGSGELGVTMKGPKGLEELVKQKDFLDGVYAFEYYPSTPGRYSIAITWGGHHIPKSPFEVQVGPEAGMQKVRAWGPGLHGGIVGRSADFVVESIGSEVGSLGFAIEGPSQAKIEYNDQNDGSCDVKYWPKEPGEYAVHIMCDDEDIKDSPYMAFIHPATGGYNPDLVRAYGPGLEKSGCIVNNLAEFTVDPKDAGKAPLKIFAQDGEGQRIDIQMKNRMDGTYACSYTPVKAIKHTIAVVWGGVNIPHSPYRVNIGQGSHPQKVKVFGPGVERSGLKANEPTHFTVDCTEAGEGDVSVGIKCDARVLSEDEEDVDFDIIHNANDTFTVKYVPPAAGRYTIKVLFASQEIPASPFRVKVDPSHDASKVKAEGPGLSKAGVENGKPTHFTVYTKGAGKAPLNVQFNSPLPGDAVKDLDIIDNYDYSHTVKYTPTQQGNMQVLVTYGGDPIPKSPFTVGVAAPLDLSKIKLNGLENRVEVGKDQEFTVDTRGAGGQGKLDVTILSPSRKVVPCLVTPVTGRENSTAKFIPREEGLYAVDVTYDGHPVPGSPYTVEASLPPDPSKVKAHGPGLEGGLVGKPAEFTIDTKGAGTGGLGLTVEGPCEAKIECSDNGDGTCSVSYLPTKPGEYFVNILFEEVHIPGSPFKADIEMPFDPSKVVASGPGLEHGKVGEAGLLSVDCSEAGPGALGLEAVSDSGTKAEVSIQNNKDGTYAVTYVPLTAGMYTLTMKYGGELVPHFPARVKVEPAVDTSRIKVFGPGIEGKDVFREATTDFTVDSRPLTQVGGDHIKAHIANPSGASTECFVTDNADGTYQVEYTPFEKGLHVVEVTYDDVPIPNSPFKVAVTEGCQPSRVQAQGPGLKEAFTNKPNVFTVVTRGAGIGGLGITVEGPSESKINCRDNKDGSCSAEYIPFAPGDYDVNITYGGAHIPGSPFRVPVKDVVDPSKVKIAGPGLGSGVRARVLQSFTVDSSKAGLAPLEVRVLGPRGLVEPVNVVDNGDGTHTVTYTPSQEGPYMVSVKYADEEIPRSPFKVKVLPTYDASKVTASGPGLSSYGVPASLPVDFAIDARDAGEGLLAVQITDQEGKPKRAIVHDNKDGTYAVTYIPDKTGRYMIGVTYGGDDIPLSPYRIRATQTGDASKCLATGPGIASTVKTGEEVGFVVDAKTAGKGKVTCTVLTPDGTEAEADVIENEDGTYDIFYTAAKPGTYVIYVRFGGVDIPNSPFTVMATDGEVTAVEEAPVNACPPGFRPWVTEEAYVPVSDMNGLGFKPFDLVIPFAVRKGEITGEVHMPSGKTATPEIVDNKDGTVTVRYAPTEVGLHEMHIKYMGSHIPESPLQFYVNYPNSGSVSAYGPGLVYGVANKTATFTIVTEDAGEGGLDLAIEGPSKAEISCIDNKDGTCTVTYLPTLPGDYSILVKYNDKHIPGSPFTAKITDDSRRCSQVKLGSAADFLLDISETDLSSLTASIKAPSGRDEPCLLKRLPNNHIGISFIPREVGEHLVSIKKNGNHVANSPVSIMVVQSEIGDARRAKVYGRGLSEGRTFEMSDFIVDTRDAGYGGISLAVEGPSKVDIQTEDLEDGTCKVSYFPTVPGVYIVSTKFADEHVPGSPFTVKISGEGRVKESITRTSRAPSVATVGSICDLNLKIPEINSSDMSAHVTSPSGRVTEAEIVPMGKNSHCVRFVPQEMGVHTVSVKYRGQHVTGSPFQFTVGPLGEGGAHKVRAGGPGLERGEAGVPAEFSIWTREAGAGGLSIAVEGPSKAEITFDDHKNGSCGVSYIAQEPGNYEVSIKFNDEHIPESPYLVPVIAPSDDARRLTVMSLQESGLKVNQPASFAIRLNGAKGKIDAKVHSPSGAVEECHVSELEPDKYAVRFIPHENGVHTIDVKFNGSHVVGSPFKVRVGEPGQAGNPALVSAYGTGLEGGTTGIQSEFFINTTRAGPGTLSVTIEGPSKVKMDCQETPEGYKVMYTPMAPGNYLISVKYGGPNHIVGSPFKAKVTGQRLVSPGSANETSSILVESVTRSSTETCYSAIPKASSDASKVTSKGAGLSKAFVGQKSSFLVDCSKAGSNMLLIGVHGPTTPCEEVSMKHVGNQQYNVTYVVKERGDYVLAVKWGEEHIPGSPFHVTVP

SEQ ID NO: 29 - DNA, 9467 bp, Homo sapiens
gcggccaggggcgggcggccgcagagcagcaccggccgtggctccggtagcagcaagttcgaaccccgctcccgctccgcttcggttctcgctccttcggcccttgggcctccaaacaccagtccccggcagctcgttgcgcattgcgctctccccgccaccaggatgccggtaaccgagaaggatctagctgaggacgcgccttggaagaagatccagcagaacacgttcacacgctggtgcaacgagcacctcaagtgcgtgaacaaacgcatcggcaacctgcagaccgacctgagcgacgggctgcggctcatcgcgctgctcgaggtgctcagccagaagcgcatgtaccgcaagtaccatcagcggcccacctttcgccagatgcagctcgagaatgtgtccgtggcgctcgagttcctggaccgtgagagcatcaagctcgtgtccatcgatagcaaagccattgtggatgggaacctgaagctcatcttgggtctggtgtggacgctgatcctccactactccatctccatgcccgtgtgggaggatgaaggggatgatgatgccaagaagcagacgccaaagcagaggctgctggggtggattcagaacaagatcccctacttgcccatcaccaactttaaccagaactggcaagacggcaaagccctgggagccctggtagacagctgtgctccaggtctgtgcccagactgggaatcctgggacccgcagaagcctgtggataatgcacgagaagccatgcagcaggcagatgactggctgggtgtcccacaggtcatcactcctgaagaaatcattcacccggatgtggacgagcactcagttatgacttacctgtcccagttccccaaagccaagctcaagccgggggctcctctcaaacccaaactcaacccgaagaaagccagggcctatggcagaggaatcgagcccactggaaacatggtgaagcagccagccaagttcactgtggacaccatcagcgccgggcaaggagacgtgatggtgtttgttgaggacccagaagggaacaaagaggaggcacaagtgacccctgacagtgacaagaacaagacatactctgtggagtatctgcccaaggtcaccgggctacacaaagtcacagtcctctttgcaggacagcacatctccaagagcccatttgaagtgagtgttgacaaggcccagggagatgccagtaaagtcactgcaaaaggtccagggttggaagctgtagggaacatcgccaataagcccacctactttgacatctatacggcaggagctggtgtgggtgacattggtgtggaggtggaagatccccaggggaagaacaccgtggagttgctcgtggaagacaaaggaaaccaggtgtatcgatgtgtgtacaaacccatgcagcctggccctcacgtggtcaagatcttctttgctggggacactattcctaagagtcccttcgttgtgcaggttggggaagcctgcaatccaaatgcctgccgggccagtggccgaggcctacaacccaaaggcgtccgtatccgggagaccacagatttcaaggttgacaccaaagctgcaggaagtggggagctcggtgtaaccatgaagggtcctaagggtctggaggagctggtgaagcagaaagactttctggatggggtctacgcattcgagtattaccccagcaccccggggagatacagcattgccatcacatgggggggacaccacattccaaagagcccctttgaagttcaagttggccctgaagcgggtatgcagaaagtccgtgcttggggccctgggctccatggtgggattgtcgggcggtcagcggacttcgtggtagaatccattggctctgaagtggggtctctggggtttgccattgaaggcccctctcaggcaaagattgagtacaacgaccagaatgatggatcgtgtgatgtcaaatactggcccaaggagcctggcgaatatgctgttcacatcatgtgtgacgacgaagacatcaaggacagcccgtacatggccttcatccacccagccacgggaggctacaaccctgatctggttcgagcatacgggccaggtttggagaaatctggatgcattgtcaacaacctggccgagttcactgtggatcctaaggatgctggaaaagctcccttaaagatatttgctcaggatggggaaggccaacgcattgacatccagatgaagaaccggatggacggcacatatgcatgctcatacaccccggtgaaggccatcaagcacaccattgctgtggtctggggaggcgtgaacatcccgcacagcccctacagggtcaacatcgggcaaggtagccatcctcagaaggtcaaagtgtttgggccaggtgtggagagaagtggtctgaaggcaaatgaacctacacacttcacggtggactgtactgaggctggggaaggtgatgtcagtgttggcattaagtgtgatgcccgggtgttaagtgaagatgaggaagacgtggattttgacattattcacaatgccaatgatacgttcacagtcaaatatgtgcctcctgctgctgggcgatacactatcaaagttctctttgcatctcaggaaatccccgccagccctttcagagtcaaagttgacccttcccacgatgccagcaaagtgaaggcagaaggcccagggctcagcaaagcaggtgtggaaaatgggaaaccgacccacttcactgtctacaccaagggggctgggaaagccccgctcaacgtgcagttcaacagccctcttcctggcgatgcagtgaaggatttggatatcatcgataattatgactactctcacacggttaaatatacacccacccaacagggcaacatgcaggttctggtgacttacggtggcgatcccatccctaaaagccctttcactgtgggtgttgctgcaccgctggatctgagcaagataaaactcaatgggctggaaaacagggtggaagttgggaaggatcaggagttcaccgttgataccaggggggcaggaggccaggggaagctggacgtgacaatcctcagcccctctcggaaggtcgtgccatgcctagtgacacctgtgacaggccgggagaacagcacggccaagttcatccctcgggaggaggggctgtatgctgtagacgtgacctacgatggacaccctgtgcccgggagcccctacacagtggaggcctcgctgccaccagatcccagcaaggtgaaggcccacggtcccggcctcgaaggtggtctcgtgggcaagcctgccgagttcaccatcgataccaaaggagctggtactggaggtctgggcttaacggtggaaggtccgtgcgaggccaaaatcgagtgctccgacaatggtgatgggacctgctccgtctcttaccttcccacaaaacccggggagtacttcgtcaacatcctctttgaagaagtccacatacctgggtctcccttcaaagctgacattgaaatgccctttgacccctctaaagtcgtggcatcggggccaggtctcgagcacgggaaggtgggtgaagctggcctccttagcgtcgactgctcggaagcgggaccgggggccctgggcctggaagctgtctcggactcgggaacaaaagccgaagtcagtattcagaacaacaaagatggcacctacgcggtgacctacgtgcccctgacggccggcatgtacacgttgaccatgaagtatggtggcgaactcgtgccacacttccccgcccgggtcaaggtggagcccgccgtggacaccagcaggatcaaagtctttggaccaggaatagaagggaaagatgtgttccgggaagctaccaccgactttacagttgactctcggccgctgacccaggttgggggtgaccacatcaaggcccacattgccaacccctcaggggcctccaccgagtgctttgtcacagacaatgcggatgggacctaccaggtggaatacacaccctttgagaaaggtctccatgtagtggaggtgacatatgatgacgtgcctatcccaaacagtcccttcaaggtggctgtcactgaaggctgccagccatctagggtgcaagcccaaggacctggattgaaagaggcctttaccaacaagcccaatgtcttcaccgtggttaccagaggcgcaggaattggtgggcttggcataactgttgagggaccatcagagtcgaagataaattgcagagacaacaaggatggcagctgcagtgctgagtacattcctttcgcaccgggggattacgatgttaatatcacatatggaggagcccacatccccggcagccccttcagggttcctgtgaaggatgttgtggaccccagcaaggtcaagattgccggccccgggctgggctcaggcgtccgagcccgtgtcctgcagtccttcacggtggacagcagcaaggctggcctggctccgctggaagtgagggttctgggcccacgaggcttggtggagccagtgaacgtggtggacaatggagatggcacacacacagtaacctacaccccatctcaggagggaccttacatggtctcagttaaatatgctgatgaagagattcctcgcagtcccttcaaggtcaaggtccttcccacatatgatgccagcaaagtgactgccagtggccccggccttagttcctatggtgtgcctgccagtctacctgtggactttgcaattgatgcccgagatgccggggaaggcctgcttgctgttcaaataacggaccaagaaggaaaacccaaaagagccattgtccatgacaataaagatggcacgtatgctgtcacctacatccccgacaagactgggcgctatatgattggagtcacctacgggggtgacgacatcccactttctccttatcgcatccgagccacacagacgggtgatgccagcaagtgcctggccacgggtcctggaatcgcctccactgtgaaaactggcgaagaagtaggctttgtggttgatgccaagactgccgggaagggtaaagtgacctgcacggttctgaccccagatggcactgaggccgaggccgatgtcattgagaatgaagatggaacctatgacatcttctacacagctgccaagccgggcacatatgtgatctatgtgcgcttcggtggtgttgatattcctaacagccccttcactgtcatggccacagatggggaagtcacagccgtggaggaggcaccggtaaatgcatgtccccctggattcaggccctgggtgaccgaagaggcctatgtcccagtgagtgacatgaacggcctgggatttaagccttttgacctggtcattccgtttgctgtcaggaaaggagaaatcactggagaggtccacatgccttctgggaagacagccacacctgagattgtggacaacaaggacggcacggtcactgttagatatgcccccactgaggtcgggctccatgagatgcacatcaaatacatgggcagccacatccctgagagcccactccagttctacgtgaactaccccaacagtggaagtgtttctgcatacggtccaggcctcgtgtatggagtggccaacaaaactgccaccttcaccatcgtcacagaggatgcaggagaaggtggtctggacttggctattgagggcccctcaaaagcagaaatcagctgcattgacaataaagatgggacatgcacagtgacctacctgccgactctgccaggcgactacagcattctggtcaagtacaatgacaagcacatccctggcagccccttcacagccaagatcacagatgacagcaggcggtgctcccaggtgaagttgggctcagccgctgacttcctgctcgacatcagtgagactgacctcagcagcctgacggccagcattaaggccccatctggccgagacgagccctgtctcctgaagaggctgcccaacaaccacattggcatctccttcatcccccgggaagtgggcgaacatctggtcagcatcaagaaaaatggcaaccatgtggccaacagccccgtgtctatcatggtggtccagtcggagattggtgacgcccgccgagccaaagtctatggccgcggcctgtcagaaggccggactttcgagatgtctgacttcatcgtggacacaagggatgcaggttatggtggcatatccttggcggtggaaggccccagcaaagtggacatccagacggaggacctggaagatggcacctgcaaagtctcctacttccctaccgtgcctggggtttatatcgtctccaccaaattcgctgacgagcacgtgcctgggagcccatttaccgtgaagatcagtggggagggaagagtcaaagagagcatcacccgcaccagtcgggccccgtccgtggccactgtcgggagcatttgtgacctgaacctgaaaatcccagaaatcaacagcagtgatatgtcggcccacgtcaccagcccctctggccgtgtgactgaggcagagattgtgcccatggggaagaactcacactgcgtccggtttgtgccccaggagatgggcgtgcacacggtcagcgtcaagtaccgtgggcagcacgtcaccggcagccccttccagttcaccgtggggccacttggtgaaggaggcgcccacaaggtgcgggcaggaggccctggcctggagagaggagaagcgggagtcccagctgagttcagcatttggacccgggaagcaggcgctggaggcctctccatcgctgttgagggccccagtaaggccgagattacattcgatgaccataaaaatgggtcgtgcggtgtatcttatattgcccaagagcctggtaactacgaggtgtccatcaagttcaatgatgagcacatcccggaaagcccctacctggtgccggtcatcgcaccctccgacgacgcccgccgcctcactgttatgagccttcaggaatcgggattaaaagttaaccagccagcatcctttgctataaggttgaatggcgcaaaaggcaagattgatgcaaaggtgcacagcccctctggagccgtggaggagtgccacgtgtctgagctggagccagataagtatgctgttcgcttcatccctcatgagaatggtgtccacaccatcgatgtcaagttcaatgggagccacgtggttggaagccccttcaaagtgcgcgttggggagcctggacaagcggggaaccctgccctggtgtccgcctatggcacgggactcgaagggggcaccacaggtatccagtcggaattctttattaacaccacccgagcaggtccagggacattatccgtcaccatcgaaggcccatccaaggttaaaatggattgccaggaaacacctgaagggtacaaagtcatgtacacccccatggctcctggtaactacctgatcagcgtcaaatacggtgggcccaaccacatcgtgggcagtcccttcaaggccaaggtgacaggccagcgtctagttagccctggctcagccaacgagacctcatccatcctggtggagtcagtgaccaggtcgtctacagagacctgctatagcgccattcccaaggcatcctcggacgccagcaaggtgacctctaagggggcagggctctcaaaggcctttgtgggccagaagagttccttcctggtggactgcagcaaagctggctccaacatgctgctgatcggggtccatgggcccaccaccccctgcgaggaggtctccatgaagcatgtaggcaaccagcaatacaacgtcacatacgtcgtcaaggagaggggcgattatgtgctggctgtgaagtggggggaggaacacatccctggcagcccttttcatgtcacagtgccttaaaacagttttctcaaatcctggagagagttcttgtggttgcttttgttgcttgtttgtaattcattttatacaaagccctccagcctgtttgtggggctgaaaccccatccctaaaatattgctgttgtaaaatgccttcagaaataagtcctagactggactcttgagggacatattggagaatcttaagaaatgcaagcttgttcagggggctgagaagatcctgagtacactaggtgcaaaccagaactcttggtggaacagaccagccactgcagcagacagaccaggaacacaatgagactgacatttcaaaaaaacaaaactggctagcctgagctgctggttcactcttcagcatttatgaaacaaggctaggggaagatgggcagagaaaaaggggacacctagtttggttgtcatttggcaaaggagatgacttaaaatccgcttaatctcttccagtgtccgtgttaatgtatttggctattagatcactagcactgctttaccgctcctcatcgccaacacccccatgctctgtggccttcttacacttctcagagggcagagtggcagccgggcaccctacagaaactcagagggcagagtggcagccaggcccacatgtctctcaagtacctgtcccctcgctctggtgattatttcttgcagaatcaccacacgagaccatcccggcagtcatggttttgctttagttttccaagtccgtttcagtcccttccttggtctgaagaaattctgcagtggcgagcagtttcccacttgccaaagatcccttttaaccaacactagcccttgtttttaacacacgctccagcccttcatcagcctgggcagtcttaccaaaatgtttaaagtgatctcagaggggcccatggattaacgccctcatcccaaggtccgtcccatgacataacactccacacccgccccagccaacttcatgggtcactttttctggaaaataatgatctgtacagacaggacagaatgaaactcctgcgggtctttggcctgaaagttgggaatggttgggggagagaagggcagcagcttattggtggtcttttcaccattggcagaaacagtgagagctgtgtggtgcagaaatccagaaatgaggtgtagggaattttgcctgccttcctgcagacctgagctggctttggaatgaggttaaagtgtcagggacgttgcctgagcccaaatgtgtagtgtggtctgggcaggcagacctttaggttttgctgcttagtcctgaggaagtggccactcttgtggcaggtgtagtatctggggcgagtgttgggggtaaaagcccaccctacagaaagtggaacagcccggagcctgatgtgaaaggaccacgggtgttgtaagctgggacacggaagccaaactggaatcaaacgccgactgtaaattgtatcttataacttattaaataaaacatttgctccgtaaagttg

SEQ ID NO: 30 - protein, 193 aa, Homo sapiens
MVAPKSHTDDWAPGPFSSKPQRSQLQIFSSVLQTSLLFLLMGLRASGKDSAPTVVSGILGGSVTLPLNISVDTEIENVIWIGPKNALAFARPKENVTIMVKSYLGRLDITKWSYSLCISNLTLNDAGSYKAQINQRNFEVTTEEEFTLFVYAPFIEKLSVHVIEGDHRTLLEGSGLESIISTLAEPRVSVREG

SEQ ID NO: 31 - DNA, 1525 bp, Homo sapiens
acatacacatacacatgcacacacacactcatatacacatgcagaagctgtgacacgtgcggaagctgtggtaagtgcatcctccttcagtctcagttctgaaaatagatcatcatggtggcaccaaagagtcacacagatgactgggctcctgggcctttctccagtaagccacagaggagtcagctgcaaatattctcttctgttctacagacctctctcctcttcctgctcatgggactaagagcctctggaaaggactcagccccaacagtggtgtcagggatcctagggggttccgtgactctccccctaaacatctcagtagacacagagattgagaacgtcatctggattggtcccaaaaatgctcttgctttcgcacgtcccaaagaaaatgtaaccattatggtcaaaagctacctgggccgactagacatcaccaagtggagttactccctgtgcatcagcaatctgactctgaatgatgcaggatcctacaaagcccagataaaccaaaggaattttgaagtcaccactgaggaggaattcaccctgttcgtctatgcaccatttattgaaaagttgtccgtccacgtcatcgagggtgaccaccgcacactcctggagggcagcggcctggagtccatcatcagcaccctggctgagccacgtgtgagcgtgcgggagggctaggccctcgcccccacctgccactggagaccgctccgccatccccacctcaccgccgcgcagcagagctggaagggtcctgccgatgggaccctgccaggcccagtgccactgccccccgaggctgctagacgtgggcgttaggcgtgtcccacccacccgccgcctcccatggcacgtcgggaacaccggagccgccaacttggagactcctggtctgtgaagagccgctgacgcccgcaggaaccgggctgggccttgtgtgccagtggggtttgtgcttggtctttctccgcttggatttgcttatttattgcattgctggtagagactcccaagcctgtccaccctgcaaagactcctcgggcagcatgcgggtcccgcacactgcacccatttcctggatgtcccctgcaggcgcgggaggccatccgggcctgctggctgcggccccctctcagccaggcctggctcagcccactgcgtgggaggtcaccggccactccccgaggagctgggatccccgggatgcaggcccacagtgcggggctgcacccatgatgcggagctggcctccaaccctgcgggccgcgccaggcaccaactcagtgtttgtcagtgtttgtttttccaagaaatggttcaaattgctgctcagatttttaaatttactgtagctgccagtgtacacgtgtggaccccattttatttttacaccaatttggtgaaaatgctgctttcctcagcctccccacaattaaactgcacatggtctctaaaaaaataaaaataaataaataaataaataaataaaaagtatcttttctcccca

SEQ ID NO: 32 - protein, 641 aa, Homo sapiens
MVAPKSHTDDWAPGPFSSKPQRSQLQIFSSVLQTSLLFLLMGLRASGKDSAPTVVSGILGGSVTLPLNISVDTEIENVIWIGPKNALAFARPKENVTIMVKSYLGRLDITKWSYSLCISNLTLNDAGSYKAQINQRNFEVTTEEEFTLFVYEQLQEPQVTMKSVKVSENFSCNITLMCSVKGAEKSVLYSWTPREPHASESNGGSILTVSRTPCDPDLPYICTAQNPVSQRSSLPVHVGQFCTDPGASRGGTTGETVVGVLGEPVTLPLALPACRDTEKVVWLFNTSIISKEREEAATADPLIKSRDPYKNRVWVSSQDCSLKISQLKIEDAGPYHAYVCSEASSVTSMTHVTLLIYRRLRKPKITWSLRHSEDGICRISLTCSVEDGGNTVMYTWTPLQKEAVVSQGESHLNVSWRSSENHPNLTCTASNPVSRSSHQFLSENICSGPERNTKLWIGLFLMVCLLCVGIFSWCIWKRKGRCSVPAFCSSQAEAPADTPGYEKLDTPLRPARQQPTPTSDSSSDSNLTTEEDEDRPEVHKPISGRYEVFDQVTQEGAGHDPAPEGQADYDPVTPYVTEVESVVGENTMYAQVFNLQGKTPVSQKEESSATIYCSIRKPQVVPPPQQNDLEIPESPTYENFT

SEQ ID NO: 33 - DNA, 2508 bp, Homo sapiens
acatacacatacacatgcacacacacactcatatacacatgcagaagctgtgacacgtgcggaagctgtggtaagtgcatcctccttcagtctcagttctgaaaatagatcatcatggtggcaccaaagagtcacacagatgactgggctcctgggcctttctccagtaagccacagaggagtcagctgcaaatattctcttctgttctacagacctctctcctcttcctgctcatgggactaagagcctctggaaaggactcagccccaacagtggtgtcagggatcctagggggttccgtgactctccccctaaacatctcagtagacacagagattgagaacgtcatctggattggtcccaaaaatgctcttgctttcgcacgtcccaaagaaaatgtaaccattatggtcaaaagctacctgggccgactagacatcaccaagtggagttactccctgtgcatcagcaatctgactctgaatgatgcaggatcctacaaagcccagataaaccaaaggaattttgaagtcaccactgaggaggaattcaccctgttcgtctatgagcagctgcaggagccccaagtcaccatgaagtctgtgaaggtgtctgagaacttctcctgtaacatcactctaatgtgctccgtgaagggggcagagaaaagtgttctgtacagctggaccccaagggaaccccatgcttctgagtccaatggaggctccattcttaccgtctcccgaacaccatgtgacccagacctgccatacatctgcacagcccagaaccccgtcagccagagaagctccctccctgtccatgttgggcagttctgtacagatccaggagcctccagaggaggaacaacgggggagactgtggtaggggtcctgggagagccagtcaccctgccacttgcactcccagcctgccgggacacagagaaggttgtctggttgtttaacacatccatcattagcaaagagagggaagaagcagcaacggcagatccactcattaaatccagggatccttacaagaacagggtgtgggtctccagccaggactgctccctgaagatcagccagctgaagatagaggacgccggcccctaccatgcctacgtgtgctcagaggcctccagcgtcaccagcatgacacatgtcaccctgctcatctaccgcaggctgaggaagcccaaaatcacgtggagcctcaggcacagtgaggatggcatctgcaggatcagcctgacctgctccgtggaggacgggggaaacactgtcatgtacacatggaccccgctgcagaaggaagctgttgtgtcccaaggggaatcacacctcaatgtctcatggagaagcagtgaaaatcaccccaacctcacatgcacagccagcaaccctgtcagcaggagttcccaccagtttctttctgagaacatctgttcaggacctgagagaaacacaaagctttggattgggttgttcctgatggtttgccttctgtgcgttgggatcttcagctggtgcatttggaagcgaaaaggacggtgttcagtcccagccttctgttccagccaagctgaggccccagcggatacaccaggatatgagaagctggacactcccctcaggcctgccaggcaacagcctacacccacctcagacagcagctctgacagcaacctcacaactgaggaggatgaggacaggcctgaggtgcacaagcccatcagtggaagatatgaggtatttgaccaggtcactcaggagggcgctggacatgacccagcccctgagggccaagcagactatgatcccgtcactccatatgtcacggaagttgagtctgtggttggagagaacaccatgtatgcacaagtgttcaacttacagggaaagaccccagtttctcagaaggaagagagctcagccacaatctactgctccatacggaaacctcaggtggtgccaccaccacaacagaatgatcttgagattcctgaaagtcctacctatgaaaatttcacctgaaaggaaaagcagctgctgcctctctcctgggaccgtggggttggaaagtcagctggacctcatggggcctggggctcacagacagaagcacctcagaatttccttcagtgcctcagagatgcctggatgtggcccctccccctccttctcacccttaaggactcccaaacccattaatagttcagacacaggctccttcttggagcctatgggcttcagatgtctttgccccatttgtcacctcgcacacttatagcgtttcctcctcgaaattctaccaagactggtcaaatgttgctgaggggcctggaccagctgtcctttacaccaccttctcaacactgctgaaaagaacccaagagaattgtcacacatgacacaagatgtacataatatcatgctcactgcagtgttatttaaaataaaaggcaggaaataaaaaaaaaaaaaaaaaaaaaaaaaaaaaaa

SEQ ID NO: 34 - protein, 565 aa, Homo sapiens
MVAPKSHTDDWAPGPFSSKPQRSQLQIFSSVLQTSLLFLLMGLRASGKDSAPTVVSGILGGSVTLPLNISVDTEIENVIWIGPKNALAFARPKENVTIMVKSYLGRLDITKWSYSLCISNLTLNDAGSYKAQINQRNFEVTTEEEFTLFVYEQLQEPQVTMKSVKVSENFSCNITLMCSVKGAEKSVLYSWTPREPHASESNGGSILTVSRTPCDPDLPYICTAQNPVSQRSSLPVHVGQFCTDPGASRGGTTGETVVGVLGEPVTLPLALPACRDTEKVVWLFNTSIISKEREEAATADPLIKSRDPYKNRVWVSSQDCSLKISQLKIEDAGPYHAYVCSEASSVTSMTHVTLLIYRPERNTKLWIGLFLMVCLLCVGIFSWCIWKRKGRCSVPAFCSSQAEAPADTPEPTAGHTLYSVLSQGYEKLDTPLRPARQQPTPTSDSSSDSNLTTEEDEDRPEVHKPISGRYEVFDQVTQEGAGHDPAPEGQADYDPVTPYVTEVESVVGENTMYAQVFNLQGKTPVSQKEESSATIYCSIRKPQVVPPPQQNDLEIPESPTYENFT

SEQ ID NO: 35 - DNA, 2280 bp, Homo sapiens
acatacacatacacatgcacacacacactcatatacacatgcagaagctgtgacacgtgcggaagctgtggtaagtgcatcctccttcagtctcagttctgaaaatagatcatcatggtggcaccaaagagtcacacagatgactgggctcctgggcctttctccagtaagccacagaggagtcagctgcaaatattctcttctgttctacagacctctctcctcttcctgctcatgggactaagagcctctggaaaggactcagccccaacagtggtgtcagggatcctagggggttccgtgactctccccctaaacatctcagtagacacagagattgagaacgtcatctggattggtcccaaaaatgctcttgctttcgcacgtcccaaagaaaatgtaaccattatggtcaaaagctacctgggccgactagacatcaccaagtggagttactccctgtgcatcagcaatctgactctgaatgatgcaggatcctacaaagcccagataaaccaaaggaattttgaagtcaccactgaggaggaattcaccctgttcgtctatgagcagctgcaggagccccaagtcaccatgaagtctgtgaaggtgtctgagaacttctcctgtaacatcactctaatgtgctccgtgaagggggcagagaaaagtgttctgtacagctggaccccaagggaaccccatgcttctgagtccaatggaggctccattcttaccgtctcccgaacaccatgtgacccagacctgccatacatctgcacagcccagaaccccgtcagccagagaagctccctccctgtccatgttgggcagttctgtacagatccaggagcctccagaggaggaacaacgggggagactgtggtaggggtcctgggagagccagtcaccctgccacttgcactcccagcctgccgggacacagagaaggttgtctggttgtttaacacatccatcattagcaaagagagggaagaagcagcaacggcagatccactcattaaatccagggatccttacaagaacagggtgtgggtctccagccaggactgctccctgaagatcagccagctgaagatagaggacgccggcccctaccatgcctacgtgtgctcagaggcctccagcgtcaccagcatgacacatgtcaccctgctcatctaccgacctgagagaaacacaaagctttggattgggttgttcctgatggtttgccttctgtgcgttgggatcttcagctggtgcatttggaagcgaaaaggacggtgttcagtcccagccttctgttccagccaagctgaggccccagcggatacaccagaacccacagctggccacacgctatactctgtgctctcccaaggatatgagaagctggacactcccctcaggcctgccaggcaacagcctacacccacctcagacagcagctctgacagcaacctcacaactgaggaggatgaggacaggcctgaggtgcacaagcccatcagtggaagatatgaggtatttgaccaggtcactcaggagggcgctggacatgacccagcccctgagggccaagcagactatgatcccgtcactccatatgtcacggaagttgagtctgtggttggagagaacaccatgtatgcacaagtgttcaacttacagggaaagaccccagtttctcagaaggaagagagctcagccacaatctactgctccatacggaaacctcaggtggtgccaccaccacaacagaatgatcttgagattcctgaaagtcctacctatgaaaatttcacctgaaaggaaaagcagctgctgcctctctcctgggaccgtggggttggaaagtcagctggacctcatggggcctggggctcacagacagaagcacctcagaatttccttcagtgcctcagagatgcctggatgtggcccctccccctccttctcacccttaaggactcccaaacccattaatagttcagacacaggctccttcttggagcctatgggcttcagatgtctttgccccatttgtcacctcgcacacttatagcgtttcctcctcgaaattctaccaagactggtcaaatgttgctgaggggcctggaccagctgtcctttacaccaccttctcaacactgctgaaaagaacccaagagaattgtcacacatgacacaagatgtacataatatcatgctcactgcagtgttatttaaaataaaaggcaggaaataaaaaaaaaaaaaaaaaaaaaaaaaaaaaaa

SEQ ID NO: 36 - protein, 655 aa, Homo sapiens
MVAPKSHTDDWAPGPFSSKPQRSQLQIFSSVLQTSLLFLLMGLRASGKDSAPTVVSGILGGSVTLPLNISVDTEIENVIWIGPKNALAFARPKENVTIMVKSYLGRLDITKWSYSLCISNLTLNDAGSYKAQINQRNFEVTTEEEFTLFVYEQLQEPQVTMKSVKVSENFSCNITLMCSVKGAEKSVLYSWTPREPHASESNGGSILTVSRTPCDPDLPYICTAQNPVSQRSSLPVHVGQFCTDPGASRGGTTGETVVGVLGEPVTLPLALPACRDTEKVVWLFNTSIISKEREEAATADPLIKSRDPYKNRVWVSSQDCSLKISQLKIEDAGPYHAYVCSEASSVTSMTHVTLLIYRRLRKPKITWSLRHSEDGICRISLTCSVEDGGNTVMYTWTPLQKEAVVSQGESHLNVSWRSSENHPNLTCTASNPVSRSSHQFLSENICSGPERNTKLWIGLFLMVCLLCVGIFSWCIWKRKGRCSVPAFCSSQAEAPADTPEPTAGHTLYSVLSQGYEKLDTPLRPARQQPTPTSDSSSDSNLTTEEDEDRPEVHKPISGRYEVFDQVTQEGAGHDPAPEGQADYDPVTPYVTEVESVVGENTMYAQVFNLQGKTPVSQKEESSATIYCSIRKPQVVPPPQQNDLEIPESPTYENFT

SEQ ID NO: 37 - DNA, 2550 bp, Homo sapiens
acatacacatacacatgcacacacacactcatatacacatgcagaagctgtgacacgtgcggaagctgtggtaagtgcatcctccttcagtctcagttctgaaaatagatcatcatggtggcaccaaagagtcacacagatgactgggctcctgggcctttctccagtaagccacagaggagtcagctgcaaatattctcttctgttctacagacctctctcctcttcctgctcatgggactaagagcctctggaaaggactcagccccaacagtggtgtcagggatcctagggggttccgtgactctccccctaaacatctcagtagacacagagattgagaacgtcatctggattggtcccaaaaatgctcttgctttcgcacgtcccaaagaaaatgtaaccattatggtcaaaagctacctgggccgactagacatcaccaagtggagttactccctgtgcatcagcaatctgactctgaatgatgcaggatcctacaaagcccagataaaccaaaggaattttgaagtcaccactgaggaggaattcaccctgttcgtctatgagcagctgcaggagccccaagtcaccatgaagtctgtgaaggtgtctgagaacttctcctgtaacatcactctaatgtgctccgtgaagggggcagagaaaagtgttctgtacagctggaccccaagggaaccccatgcttctgagtccaatggaggctccattcttaccgtctcccgaacaccatgtgacccagacctgccatacatctgcacagcccagaaccccgtcagccagagaagctccctccctgtccatgttgggcagttctgtacagatccaggagcctccagaggaggaacaacgggggagactgtggtaggggtcctgggagagccagtcaccctgccacttgcactcccagcctgccgggacacagagaaggttgtctggttgtttaacacatccatcattagcaaagagagggaagaagcagcaacggcagatccactcattaaatccagggatccttacaagaacagggtgtgggtctccagccaggactgctccctgaagatcagccagctgaagatagaggacgccggcccctaccatgcctacgtgtgctcagaggcctccagcgtcaccagcatgacacatgtcaccctgctcatctaccgcaggctgaggaagcccaaaatcacgtggagcctcaggcacagtgaggatggcatctgcaggatcagcctgacctgctccgtggaggacgggggaaacactgtcatgtacacatggaccccgctgcagaaggaagctgttgtgtcccaaggggaatcacacctcaatgtctcatggagaagcagtgaaaatcaccccaacctcacatgcacagccagcaaccctgtcagcaggagttcccaccagtttctttctgagaacatctgttcaggacctgagagaaacacaaagctttggattgggttgttcctgatggtttgccttctgtgcgttgggatcttcagctggtgcatttggaagcgaaaaggacggtgttcagtcccagccttctgttccagccaagctgaggccccagcggatacaccagaacccacagctggccacacgctatactctgtgctctcccaaggatatgagaagctggacactcccctcaggcctgccaggcaacagcctacacccacctcagacagcagctctgacagcaacctcacaactgaggaggatgaggacaggcctgaggtgcacaagcccatcagtggaagatatgaggtatttgaccaggtcactcaggagggcgctggacatgacccagcccctgagggccaagcagactatgatcccgtcactccatatgtcacggaagttgagtctgtggttggagagaacaccatgtatgcacaagtgttcaacttacagggaaagaccccagtttctcagaaggaagagagctcagccacaatctactgctccatacggaaacctcaggtggtgccaccaccacaacagaatgatcttgagattcctgaaagtcctacctatgaaaatttcacctgaaaggaaaagcagctgctgcctctctcctgggaccgtggggttggaaagtcagctggacctcatggggcctggggctcacagacagaagcacctcagaatttccttcagtgcctcagagatgcctggatgtggcccctccccctccttctcacccttaaggactcccaaacccattaatagttcagacacaggctccttcttggagcctatgggcttcagatgtctttgccccatttgtcacctcgcacacttatagcgtttcctcctcgaaattctaccaagactggtcaaatgttgctgaggggcctggaccagctgtcctttacaccaccttctcaacactgctgaaaagaacccaagagaattgtcacacatgacacaagatgtacataatatcatgctcactgcagtgttatttaaaataaaaggcaggaaataaaaaaaaaaaaaaaaaaaaaaaaaaaaaaa

SEQ ID NO: 38 - protein, 238 aa, Homo sapiens
MWVPVVFLTLSVTWIGAAPLILSRIVGGWECEKHSQPWQVLVASRGRAVCGGVLVHPQWVLTAAHCIRNKSVILLGRHSLFHPEDTGQVFQVSHSFPHPLYDMSLLKNRFLRPGDDSSHDLMLLRLSEPAELTDAVKVMDLPTQEPALGTTCYASGWGSIEPEEFLTPKKLQCVDLHVISNDVCAQVHPQKVTKFMLCAGRWTGGKSTCSWVILITELTMPALPMVLHGSLVPWRGGV

SEQ ID NO: 39 - DNA, 1906 bp, Homo sapiens
agccccaagcttaccacctgcacccggagagctgtgtcaccatgtgggtcccggttgtcttcctcaccctgtccgtgacgtggattggtgctgcacccctcatcctgtctcggattgtgggaggctgggagtgcgagaagcattcccaaccctggcaggtgcttgtggcctctcgtggcagggcagtctgcggcggtgttctggtgcacccccagtgggtcctcacagctgcccactgcatcaggaacaaaagcgtgatcttgctgggtcggcacagcctgtttcatcctgaagacacaggccaggtatttcaggtcagccacagcttcccacacccgctctacgatatgagcctcctgaagaatcgattcctcaggccaggtgatgactccagccacgacctcatgctgctccgcctgtcagagcctgccgagctcacggatgctgtgaaggtcatggacctgcccacccaggagccagcactggggaccacctgctacgcctcaggctggggcagcattgaaccagaggagttcttgaccccaaagaaacttcagtgtgtggacctccatgttatttccaatgacgtgtgtgcgcaagttcaccctcagaaggtgaccaagttcatgctgtgtgctggacgctggacagggggcaaaagcacctgctcgtgggtcattctgatcaccgaactgaccatgccagccctgccgatggtcctccatggctccctagtgccctggagaggaggtgtctagtcagagagtagtcctggaaggtggcctctgtgaggagccacggggacagcatcctgcagatggtcctggcccttgtcccaccgacctgtctacaaggactgtcctcgtggaccctcccctctgcacaggagctggaccctgaagtcccttccccaccggccaggactggagcccctacccctctgttggaatccctgcccaccttcttctggaagtcggctctggagacatttctctcttcttccaaagctgggaactgctatctgttatctgcctgtccaggtctgaaagataggattgcccaggcagaaactgggactgacctatctcactctctccctgcttttacccttagggtgattctgggggcccacttgtctgtaatggtgtgcttcaaggtatcacgtcatggggcagtgaaccatgtgccctgcccgaaaggccttccctgtacaccaaggtggtgcattaccggaagtggatcaaggacaccatcgtggccaacccctgagcacccctatcaaccccctattgtagtaaacttggaaccttggaaatgaccaggccaagactcaagcctccccagttctactgacctttgtccttaggtgtgaggtccagggttgctaggaaaagaaatcagcagacacaggtgtagaccagagtgtttcttaaatggtgtaattttgtcctctctgtgtcctggggaatactggccatgcctggagacatatcactcaatttctctgaggacacagataggatggggtgtctgtgttatttgtggggtacagagatgaaagaggggtgggatccacactgagagagtggagagtgacatgtgctggacactgtccatgaagcactgagcagaagctggaggcacaacgcaccagacactcacagcaaggatggagctgaaaacataacccactctgtcctggaggcactgggaagcctagagaaggctgtgagccaaggagggagggtcttcctttggcatgggatggggatgaagtaaggagagggactggaccccctggaagctgattcactatggggggaggtgtattgaagtcctccagacaaccctcagatttgatgatttcctagtagaactcacagaaataaagagctgttatactgtg

SEQ ID NO: 40 - protein, 218 aa, Homo sapiens
MWVPVVFLTLSVTWIGAAPLILSRIVGGWECEKHSQPWQVLVASRGRAVCGGVLVHPQWVLTAAHCIRKPGDDSSHDLMLLRLSEPAELTDAVKVMDLPTQEPALGTTCYASGWGSIEPEEFLTPKKLQCVDLHVISNDVCAQVHPQKVTKFMLCAGRWTGGKSTCSGDSGGPLVCNGVLQGITSWGSEPCALPERPSLYTKVVHYRKWIKDTIVANP

SEQ ID NO: 41 - DNA, 1335 bp, Homo sapiens
agccccaagcttaccacctgcacccggagagctgtgtcaccatgtgggtcccggttgtcttcctcaccctgtccgtgacgtggattggtgctgcacccctcatcctgtctcggattgtgggaggctgggagtgcgagaagcattcccaaccctggcaggtgcttgtggcctctcgtggcagggcagtctgcggcggtgttctggtgcacccccagtgggtcctcacagctgcccactgcatcaggaagccaggtgatgactccagccacgacctcatgctgctccgcctgtcagagcctgccgagctcacggatgctgtgaaggtcatggacctgcccacccaggagccagcactggggaccacctgctacgcctcaggctggggcagcattgaaccagaggagttcttgaccccaaagaaacttcagtgtgtggacctccatgttatttccaatgacgtgtgtgcgcaagttcaccctcagaaggtgaccaagttcatgctgtgtgctggacgctggacagggggcaaaagcacctgctcgggtgattctgggggcccacttgtctgtaatggtgtgcttcaaggtatcacgtcatggggcagtgaaccatgtgccctgcccgaaaggccttccctgtacaccaaggtggtgcattaccggaagtggatcaaggacaccatcgtggccaacccctgagcacccctatcaaccccctattgtagtaaacttggaaccttggaaatgaccaggccaagactcaagcctccccagttctactgacctttgtccttaggtgtgaggtccagggttgctaggaaaagaaatcagcagacacaggtgtagaccagagtgtttcttaaatggtgtaattttgtcctctctgtgtcctggggaatactggccatgcctggagacatatcactcaatttctctgaggacacagataggatggggtgtctgtgttatttgtggggtacagagatgaaagaggggtgggatccacactgagagagtggagagtgacatgtgctggacactgtccatgaagcactgagcagaagctggaggcacaacgcaccagacactcacagcaaggatggagctgaaaacataacccactctgtcctggaggcactgggaagcctagagaaggctgtgagccaaggagggagggtcttcctttggcatgggatggggatgaagtaaggagagggactggaccccctggaagctgattcactatggggggaggtgtattgaagtcctccagacaaccctcagatttgatgatttcctagtagaactcacagaaataaagagctgttatactgtg

SEQ ID NO: 42 - protein, 69 aa, Homo sapiens
MWVPVVFLTLSVTWIGAAPLILSRIVGGWECEKHSQPWQVLVASRGRAVCGGVLVHPQWVLTAAHCIRK

SEQ ID NO: 43 - DNA, 555 bp, Homo sapiens
agccccaagcttaccacctgcacccggagagctgtgtcaccatgtgggtcccggttgtcttcctcaccctgtccgtgacgtggattggtgctgcacccctcatcctgtctcggattgtgggaggctgggagtgcgagaagcattcccaaccctggcaggtgcttgtggcctctcgtggcagggcagtctgcggcggtgttctggtgcacccccagtgggtcctcacagctgcccactgcatcaggaagtgagtaggggcctggggtctggggagcaggtgtctgtgtcccagaggaataacagctgggcattttccccaggataacctctaaggccagccttgggactgggggagagagggaaagttctggttcaggtcacatggggaggcagggttggggctggaccaccctccccatggctgcctgggtctccatctgtgttcctctatgtctctttgtgtcgctttcattatgtctcttggtaactggcttcggttgtgtctctccgtgtgactattttgttctctctctccctctcttctctgtcttcagt

SEQ ID NO: 44 - protein, 261 aa, Homo sapiens
MWVPVVFLTLSVTWIGAAPLILSRIVGGWECEKHSQPWQVLVASRGRAVCGGVLVHPQWVLTAAHCIRNKSVILLGRHSLFHPEDTGQVFQVSHSFPHPLYDMSLLKNRFLRPGDDSSHDLMLLRLSEPAELTDAVKVMDLPTQEPALGTTCYASGWGSIEPEEFLTPKKLQCVDLHVISNDVCAQVHPQKVTKFMLCAGRWTGGKSTCSGDSGGPLVCNGVLQGITSWGSEPCALPERPSLYTKVVHYRKWIKDTIVANP

SEQ ID NO: 45 - DNA, 1464 bp, Homo sapiens
agccccaagcttaccacctgcacccggagagctgtgtcaccatgtgggtcccggttgtcttcctcaccctgtccgtgacgtggattggtgctgcacccctcatcctgtctcggattgtgggaggctgggagtgcgagaagcattcccaaccctggcaggtgcttgtggcctctcgtggcagggcagtctgcggcggtgttctggtgcacccccagtgggtcctcacagctgcccactgcatcaggaacaaaagcgtgatcttgctgggtcggcacagcctgtttcatcctgaagacacaggccaggtatttcaggtcagccacagcttcccacacccgctctacgatatgagcctcctgaagaatcgattcctcaggccaggtgatgactccagccacgacctcatgctgctccgcctgtcagagcctgccgagctcacggatgctgtgaaggtcatggacctgcccacccaggagccagcactggggaccacctgctacgcctcaggctggggcagcattgaaccagaggagttcttgaccccaaagaaacttcagtgtgtggacctccatgttatttccaatgacgtgtgtgcgcaagttcaccctcagaaggtgaccaagttcatgctgtgtgctggacgctggacagggggcaaaagcacctgctcgggtgattctgggggcccacttgtctgtaatggtgtgcttcaaggtatcacgtcatggggcagtgaaccatgtgccctgcccgaaaggccttccctgtacaccaaggtggtgcattaccggaagtggatcaaggacaccatcgtggccaacccctgagcacccctatcaaccccctattgtagtaaacttggaaccttggaaatgaccaggccaagactcaagcctccccagttctactgacctttgtccttaggtgtgaggtccagggttgctaggaaaagaaatcagcagacacaggtgtagaccagagtgtttcttaaatggtgtaattttgtcctctctgtgtcctggggaatactggccatgcctggagacatatcactcaatttctctgaggacacagataggatggggtgtctgtgttatttgtggggtacagagatgaaagaggggtgggatccacactgagagagtggagagtgacatgtgctggacactgtccatgaagcactgagcagaagctggaggcacaacgcaccagacactcacagcaaggatggagctgaaaacataacccactctgtcctggaggcactgggaagcctagagaaggctgtgagccaaggagggagggtcttcctttggcatgggatggggatgaagtaaggagagggactggaccccctggaagctgattcactatggggggaggtgtattgaagtcctccagacaaccctcagatttgatgatttcctagtagaactcacagaaataaagagctgttatactgtg

SEQ ID NO: 46 - DNA, 8533 bp, Homo sapiens
attcgcgtggaggcgcgtcgcgcgcagcggacgccgacagaatccccgaggcgcctggcgcgggcgcgggcgcgaaggcgatccgggcgccaccccgcggtcatcggtcaccggtcgctctcaggaacagcagcgcaacctctgctccctgcctcgcctcccgcgcgcctaggtgcctgcgactttaattaaagggccgtcccctcgccgaggctgcagcaccgcccccccggcttctcgcgcctcaaaatgagtagctcccactctcgggcgggccagagcgcagcaggcgcggctccgggcggcggcgtcgacacgcgggacgccgagatgccggccaccgagaaggacctggcggaggacgcgccgtggaagaagatccagcagaacactttcacgcgctggtgcaacgagcacctgaagtgcgtgagcaagcgcatcgccaacctgcagacggacctgagcgacgggctgcggcttatcgcgctgttggaggtgctcagccagaagaagatgcaccgcaagcacaaccagcggcccactttccgccaaatgcagcttgagaacgtgtcggtggcgctcgagttcctggaccgcgagagcatcaaactggtgtccatcgacagcaaggccatcgtggacgggaacctgaagctgatcctgggcctcatctggaccctgatcctgcactactccatctccatgcccatgtgggacgaggaggaggatgaggaggccaagaagcagacccccaagcagaggctcctgggctggatccagaacaagctgccgcagctgcccatcaccaacttcagccgggactggcagagcggccgggccctgggcgccctggtggacagctgtgccccgggcctgtgtcctgactgggactcttgggacgccagcaagcccgttaccaatgcgcgagaggccatgcagcaggcggatgactggctgggcatcccccaggtgatcacccccgaggagattgtggaccccaacgtggacgagcactctgtcatgacctacctgtcccagttccccaaggccaagctgaagccaggggctcccttgcggcccaaactgaacccgaagaaagcccgtgcctacgggccaggcatcgagcccacaggcaacatggtgaagaagcgggcagagttcactgtggagaccagaagtgctggccagggagaggtgctggtgtacgtggaggacccggccggacaccaggaggaggcaaaagtgaccgccaataacgacaagaaccgcaccttctccgtctggtacgtccccgaggtgacggggactcataaggttactgtgctctttgctggccagcacatcgccaagagccccttcgaggtgtacgtggataagtcacagggtgacgccagcaaagtgacagcccaaggtcccggcctggagcccagtggcaacatcgccaacaagaccacctactttgagatctttacggcaggagctggcacgggcgaggtcgaggttgtgatccaggaccccatgggacagaagggcacggtagagcctcagctggaggcccggggcgacagcacataccgctgcagctaccagcccaccatggagggcgtccacaccgtgcacgtcacgtttgccggcgtgcccatccctcgcagcccctacactgtcactgttggccaagcctgtaacccgagtgcctgccgggcggttggccggggcctccagcccaagggtgtgcgggtgaaggagacagctgacttcaaggtgtacacaaagggcgctggcagtggggagctgaaggtcaccgtgaagggccccaagggagaggagcgcgtgaagcagaaggacctgggggatggcgtgtatggcttcgagtattaccccatggtccctggaacctatatcgtcaccatcacgtggggtggtcagaacatcgggcgcagtcccttcgaagtgaaggtgggcaccgagtgtggcaatcagaaggtacgggcctggggccctgggctggagggcggcgtcgttggcaagtcagcagactttgtggtggaggctatcggggacgacgtgggcacgctgggcttctcggtggaagggccatcgcaggctaagatcgaatgtgacgacaagggcgacggctcctgtgatgtgcgctactggccgcaggaggctggcgagtatgccgttcacgtgctgtgcaacagcgaagacatccgcctcagccccttcatggctgacatccgtgacgcgccccaggacttccacccagacagggtgaaggcacgtgggcctggattggagaagacaggtgtggccgtcaacaagccagcagagttcacagtggatgccaagcacggtggcaaggccccacttcgggtccaagtccaggacaatgaaggctgccctgtggaggcgttggtcaaggacaacggcaatggcacttacagctgctcctacgtgcccaggaagccggtgaagcacacagccatggtgtcctggggaggcgtcagcatccccaacagccccttcagggtgaatgtgggagctggcagccaccccaacaaggtcaaagtatacggccccggagtagccaagacagggctcaaggcccacgagcccacctacttcactgtggactgcgccgaggctggccagggggacgtcagcatcggcatcaagtgtgcccctggagtggtaggccccgccgaagctgacatcgacttcgacatcatccgcaatgacaatgacaccttcacggtcaagtacacgccccggggggctggcagctacaccattatggtcctctttgctgaccaggccacgcccaccagccccatccgagtcaaggtggagccctctcatgacgccagtaaggtgaaggccgagggccctggcctcagtcgcactggtgtcgagcttggcaagcccacccacttcacagtaaatgccaaagctgctggcaaaggcaagctggacgtccagttctcaggactcaccaagggggatgcagtgcgagatgtggacatcatcgaccaccatgacaacacctacacagtcaagtacacgcctgtccagcagggtccagtaggcgtcaatgtcacttatggaggggatcccatccctaagagccctttctcagtggcagtatctccaagcctggacctcagcaagatcaaggtgtctggcctgggagagaaggtggacgttggcaaagaccaggagttcacagtcaaatcaaagggtgctggtggtcaaggcaaagtggcatccaagattgtgggcccctcgggtgcagcggtgccctgcaaggtggagccaggcctgggggctgacaacagtgtggtgcgcttcctgccccgtgaggaagggccctatgaggtggaggtgacctatgacggcgtgcccgtgcctggcagcccctttcctctggaagctgtggcccccaccaagcctagcaaggtgaaggcgtttgggccggggctgcagggaggcagtgcgggctcccccgcccgcttcaccatcgacaccaagggcgccggcacaggtggcctgggcctgacggtggagggcccctgtgaggcgcagctcgagtgcttggacaatggggatggcacatgttccgtgtcctacgtgcccaccgagcccggggactacaacatcaacatcctcttcgctgacacccacatccctggctccccattcaaggcccacgtggttccctgctttgacgcatccaaagtcaagtgctcaggccccgggctggagcgggccaccgctggggaggtgggccaattccaagtggactgctcgagcgcgggcagcgcggagctgaccattgagatctgctcggaggcggggcttccggccgaggtgtacatccaggaccacggtgatggcacgcacaccattacctacattcccctctgccccggggcctacaccgtcaccatcaagtacggcggccagcccgtgcccaacttccccagcaagctgcaggtggaacctgcggtggacacttccggtgtccagtgctatgggcctggtattgagggccagggtgtcttccgtgaggccaccactgagttcagtgtggacgcccgggctctgacacagaccggagggccgcacgtcaaggcccgtgtggccaacccctcaggcaacctgacggagacctacgttcaggaccgtggcgatggcatgtacaaagtggagtacacgccttacgaggagggactgcactccgtggacgtgacctatgacggcagtcccgtgcccagcagccccttccaggtgcccgtgaccgagggctgcgacccctcccgggtgcgtgtccacgggccaggcatccaaagtggcaccaccaacaagcccaacaagttcactgtggagaccaggggagctggcacgggcggcctgggcctggctgtagagggcccctccgaggccaagatgtcctgcatggataacaaggacggcagctgctcggtcgagtacatcccttatgaggctggcacctacagcctcaacgtcacctatggtggccatcaagtgccaggcagtcctttcaaggtccctgtgcatgatgtgacagatgcgtccaaggtcaagtgctctgggcccggcctgagcccaggcatggttcgtgccaacctccctcagtccttccaggtggacacaagcaaggctggtgtggccccattgcaggtcaaagtgcaagggcccaaaggcctggtggagccagtggacgtggtagacaacgctgatggcacccagaccgtcaattatgtgcccagccgagaagggccctacagcatctcagtactgtatggagatgaagaggtaccccggagccccttcaaggtcaaggtgctgcctactcatgatgccagcaaggtgaaggccagtggccccgggctcaacaccactggcgtgcctgccagcctgcccgtggagttcaccatcgatgcaaaggacgccggggagggcctgctggctgtccagatcacggatcccgaaggcaagccgaagaagacacacatccaagacaaccatgacggcacgtatacagtggcctacgtgccagacgtgacaggtcgctacaccatcctcatcaagtacggtggtgacgagatccccttctccccgtaccgcgtgcgtgccgtgcccaccggggacgccagcaagtgcactgtcacaggtgctggcatcggccccaccattcagattggggaggagacggtgatcactgtggacactaaggcggcaggcaaaggcaaagtgacgtgcaccgtgtgcacgcctgatggctcagaggtggatgtggacgtggtggagaatgaggacggcactttcgacatcttctacacggccccccagccgggcaaatacgtcatctgtgtgcgctttggtggcgagcacgtgcccaacagccccttccaagtgacggctctggctggggaccagccctcggtgcagccccctctacggtctcagcagctggccccacagtacacctacgcccagggcggccagcagacttgggccccggagaggcccctggtgggtgtcaatgggctggatgtgaccagcctgaggccctttgaccttgtcatccccttcaccatcaagaagggcgagatcacaggggaggttcggatgccctcaggcaaggtggcgcagcccaccatcactgacaacaaagacggcaccgtgaccgtgcggtatgcacccagcgaggctggcctgcacgagatggacatccgctatgacaacatgcacatcccaggaagccccttgcagttctatgtggattacgtcaactgtggccatgtcactgcctatgggcctggcctcacccatggagtagtgaacaagcctgccaccttcaccgtcaacaccaaggatgcaggagaggggggcctgtctctggccattgagggcccgtccaaagcagaaatcagctgcactgacaaccaggatgggacatgcagcgtgtcctacctgcctgtgctgccgggggactacagcattctagtcaagtacaatgaacagcacgtcccaggcagccccttcactgctcgggtcacaggtgacgactccatgcgtatgtcccacctaaaggtcggctctgctgccgacatccccatcaacatctcagagacggatctcagcctgctgacggccactgtggtcccgccctcgggccgggaggagccctgtttgctgaagcggctgcgtaatggccacgtggggatttcattcgtgcccaaggagacgggggagcacctggtgcatgtgaagaaaaatggccagcacgtggccagcagccccatcccggtggtgatcagccagtcggaaattggggatgccagtcgtgttcgggtctctggtcagggccttcacgaaggccacacctttgagcctgcagagtttatcattgatacccgcgatgcaggctatggtgggctcagcctgtccattgagggccccagcaaggtggacatcaacacagaggacctggaggacgggacgtgcagggtcacctactgccccacagagccaggcaactacatcatcaacatcaagtttgccgaccagcacgtgcctggcagccccttctctgtgaaggtgacaggcgagggccgggtgaaagagagcatcacccgcaggcgtcgggctccttcagtggccaacgttggtagtcattgtgacctcagcctgaaaatccctgaaattagcatccaggatatgacagcccaggtgaccagcccatcgggcaagacccatgaggccgagatcgtggaaggggagaaccacacctactgcatccgctttgttcccgctgagatgggcacacacacagtcagcgtgaagtacaagggccagcacgtgcctgggagccccttccagttcaccgtggggcccctaggggaagggggagcccacaaggtccgagctgggggccctggcctggagagagctgaagctggagtgccagccgaattcagtatctggacccgggaagctggtgctggaggcctggccattgctgtcgagggccccagcaaggctgagatctcttttgaggaccgcaaggacggctcctgtggtgtggcttatgtggtccaggagccaggtgactacgaagtctcagtcaagttcaacgaggaacacattcccgacagccccttcgtggtgcctgtggcttctccgtctggcgacgcccgccgcctcactgtttctagccttcaggagtcagggctaaaggtcaaccagccagcctcttttgcagtcagcctgaacggggccaagggggcgatcgatgccaaggtgcacagcccctcaggagccctggaggagtgctatgtcacagaaattgaccaagataagtatgctgtgcgcttcatccctcgggagaatggcgtttacctgattgacgtcaagttcaacggcacccacatccctggaagccccttcaagatccgagttggggagcctgggcatggaggggacccaggcttggtgtctgcttacggagcaggtctggaaggcggtgtcacagggaacccagctgagttcgtcgtgaacacgagcaatgcgggagctggtgccctgtcggtgaccattgacggcccctccaaggtgaagatggattgccaggagtgccctgagggctaccgcgtcacctatacccccatggcacctggcagctacctcatctccatcaagtacggcggcccctaccacattgggggcagccccttcaaggccaaagtcacaggcccccgtctcgtcagcaaccacagcctccacgagacatcatcagtgtttgtagactctctgaccaaggccacctgtgccccccagcatggggccccgggtcctgggcctgctgacgccagcaaggtggtggccaagggcctggggctgagcaaggcctacgtaggccagaagagcagcttcacagtagactgcagcaaagcaggcaacaacatgctgctggtgggggttcatggcccaaggaccccctgcgaggagatcctggtgaagcacgtgggcagccggctctacagcgtgtcctacctgctcaaggacaagggggagtacacactggtggtcaaatggggggacgagcacatcccaggcagcccctaccgcgttgtggtgccctgagtctggggcccgtgccagccggcagcccccaagcctgccccgctacccaagcagccccgccctcttcccctcaaccccggcccaggccgccctggccgcccgcctgtcactgcagccgcccctgccctgtgccgtgctgcgctcacctgcctccccagccagccgctgacctctcggctttcacttgggcagagggagccatttggtggcgctgcttgtcttctttggttctgggaggggtgagggatgggggtcctgtacacaaccacccactagttctcttctccagccaagaggaataaagttttgcttccattaaaaaaaaaaaaaaaaaaaaaaaaaaaaaaaaaaaaaaaaaaaaaaa

SEQ ID NO: 47 - protein, 2639 aa, Homo sapiens
MSSSHSRAGQSAAGAAPGGGVDTRDAEMPATEKDLAEDAPWKKIQQNTFTRWCNEHLKCVSKRIANLQTDLSDGLRLIALLEVLSQKKMHRKHNQRPTFRQMQLENVSVALEFLDRESIKLVSIDSKAIVDGNLKLILGLIWTLILHYSISMPMWDEEEDEEAKKQTPKQRLLGWIQNKLPQLPITNFSRDWQSGRALGALVDSCAPGLCPDWDSWDASKPVTNAREAMQQADDWLGIPQVITPEEIVDPNVDEHSVMTYLSQFPKAKLKPGAPLRPKLNPKKARAYGPGIEPTGNMVKKRAEFTVETRSAGQGEVLVYVEDPAGHQEEAKVTANNDKNRTFSVWYVPEVTGTHKVTVLFAGQHIAKSPFEVYVDKSQGDASKVTAQGPGLEPSGNIANKTTYFEIFTAGAGTGEVEVVIQDPMGQKGTVEPQLEARGDSTYRCSYQPTMEGVHTVHVTFAGVPIPRSPYTVTVGQACNPSACRAVGRGLQPKGVRVKETADFKVYTKGAGSGELKVTVKGPKGEERVKQKDLGDGVYGFEYYPMVPGTYIVTITWGGQNIGRSPFEVKVGTECGNQKVRAWGPGLEGGVVGKSADFVVEAIGDDVGTLGFSVEGPSQAKIECDDKGDGSCDVRYWPQEAGEYAVHVLCNSEDIRLSPFMADIRDAPQDFHPDRVKARGPGLEKTGVAVNKPAEFTVDAKHGGKAPLRVQVQDNEGCPVEALVKDNGNGTYSCSYVPRKPVKHTAMVSWGGVSIPNSPFRVNVGAGSHPNKVKVYGPGVAKTGLKAHEPTYFTVDCAEAGQGDVSIGIKCAPGVVGPAEADIDFDIIRNDNDTFTVKYTPRGAGSYTIMVLFADQATPTSPIRVKVEPSHDASKVKAEGPGLSRTGVELGKPTHFTVNAKAAGKGKLDVQFSGLTKGDAVRDVDIIDHHDNTYTVKYTPVQQGPVGVNVTYGGDPIPKSPFSVAVSPSLDLSKIKVSGLGEKVDVGKDQEFTVKSKGAGGQGKVASKIVGPSGAAVPCKVEPGLGADNSVVRFLPREEGPYEVEVTYDGVPVPGSPFPLEAVAPTKPSKVKAFGPGLQGGSAGSPARFTIDTKGAGTGGLGLTVEGPCEAQLECLDNGDGTCSVSYVPTEPGDYNINILFADTHIPGSPFKAHVVPCFDASKVKCSGPGLERATAGEVGQFQVDCSSAGSAELTIEICSEAGLPAEVYIQDHGDGTHTITYIPLCPGAYTVTIKYGGQPVPNFPSKLQVEPAVDTSGVQCYGPGIEGQGVFREATTEFSVDARALTQTGGPHVKARVANPSGNLTETYVQDRGDGMYKVEYTPYEEGLHSVDVTYDGSPVPSSPFQVPVTEGCDPSRVRVHGPGIQSGTTNKPNKFTVETRGAGTGGLGLAVEGPSEAKMSCMDNKDGSCSVEYIPYEAGTYSLNVTYGGHQVPGSPFKVPVHDVTDASKVKCSGPGLSPGMVRANLPQSFQVDTSKAGVAPLQVKVQGPKGLVEPVDVVDNADGTQTVNYVPSREGPYSISVLYGDEEVPRSPFKVKVLPTHDASKVKASGPGLNTTGVPASLPVEFTIDAKDAGEGLLAVQITDPEGKPKKTHIQDNHDGTYTVAYVPDVTGRYTILIKYGGDEIPFSPYRVRAVPTGDASKCTVTGAGIGPTIQIGEETVITVDTKAAGKGKVTCTVCTPDGSEVDVDVVENEDGTFDIFYTAPQPGKYVICVRFGGEHVPNSPFQVTALAGDQPSVQPPLRSQQLAPQYTYAQGGQQTWAPERPLVGVNGLDVTSLRPFDLVIPFTIKKGEITGEVRMPSGKVAQPTITDNKDGTVTVRYAPSEAGLHEMDIRYDNMHIPGSPLQFYVDYVNCGHVTAYGPGLTHGVVNKPATFTVNTKDAGEGGLSLAIEGPSKAEISCTDNQDGTCSVSYLPVLPGDYSILVKYNEQHVPGSPFTARVTGDDSMRMSHLKVGSAADIPINISETDLSLLTATVVPPSGREEPCLLKRLRNGHVGISFVPKETGEHLVHVKKNGQHVASSPIPVVISQSEIGDASRVRVSGQGLHEGHTFEPAEFIIDTRDAGYGGLSLSIEGPSKVDINTEDLEDGTCRVTYCPTEPGNYIINIKFADQHVPGSPFSVKVTGEGRVKESITRRRRAPSVANVGSHCDLSLKIPEISIQDMTAQVTSPSGKTHEAEIVEGENHTYCIRFVPAEMGTHTVSVKYKGQHVPGSPFQFTVGPLGEGGAHKVRAGGPGLERAEAGVPAEFSIWTREAGAGGLAIAVEGPSKAEISFEDRKDGSCGVAYVVQEPGDYEVSVKFNEEHIPDSPFVVPVASPSGDARRLTVSSLQESGLKVNQPASFAVSLNGAKGAIDAKVHSPSGALEECYVTEIDQDKYAVRFIPRENGVYLIDVKFNGTHIPGSPFKIRVGEPGHGGDPGLVSAYGAGLEGGVTGNPAEFVVNTSNAGAGALSVTIDGPSKVKMDCQECPEGYRVTYTPMAPGSYLISIKYGGPYHIGGSPFKAKVTGPRLVSNHSLHETSSVFVDSLTKATCAPQHGAPGPGPADASKVVAKGLGLSKAYVGQKSSFTVDCSKAGNNMLLVGVHGPRTPCEEILVKHVGSRLYSVSYLLKDKGEYTLVVKWGDEHIPGSPYRVVVP

SEQ ID NO: 48 - DNA, 8557 bp, Homo sapiens
attcgcgtggaggcgcgtcgcgcgcagcggacgccgacagaatccccgaggcgcctggcgcgggcgcgggcgcgaaggcgatccgggcgccaccccgcggtcatcggtcaccggtcgctctcaggaacagcagcgcaacctctgctccctgcctcgcctcccgcgcgcctaggtgcctgcgactttaattaaagggccgtcccctcgccgaggctgcagcaccgcccccccggcttctcgcgcctcaaaatgagtagctcccactctcgggcgggccagagcgcagcaggcgcggctccgggcggcggcgtcgacacgcgggacgccgagatgccggccaccgagaaggacctggcggaggacgcgccgtggaagaagatccagcagaacactttcacgcgctggtgcaacgagcacctgaagtgcgtgagcaagcgcatcgccaacctgcagacggacctgagcgacgggctgcggcttatcgcgctgttggaggtgctcagccagaagaagatgcaccgcaagcacaaccagcggcccactttccgccaaatgcagcttgagaacgtgtcggtggcgctcgagttcctggaccgcgagagcatcaaactggtgtccatcgacagcaaggccatcgtggacgggaacctgaagctgatcctgggcctcatctggaccctgatcctgcactactccatctccatgcccatgtgggacgaggaggaggatgaggaggccaagaagcagacccccaagcagaggctcctgggctggatccagaacaagctgccgcagctgcccatcaccaacttcagccgggactggcagagcggccgggccctgggcgccctggtggacagctgtgccccgggcctgtgtcctgactgggactcttgggacgccagcaagcccgttaccaatgcgcgagaggccatgcagcaggcggatgactggctgggcatcccccaggtgatcacccccgaggagattgtggaccccaacgtggacgagcactctgtcatgacctacctgtcccagttccccaaggccaagctgaagccaggggctcccttgcggcccaaactgaacccgaagaaagcccgtgcctacgggccaggcatcgagcccacaggcaacatggtgaagaagcgggcagagttcactgtggagaccagaagtgctggccagggagaggtgctggtgtacgtggaggacccggccggacaccaggaggaggcaaaagtgaccgccaataacgacaagaaccgcaccttctccgtctggtacgtccccgaggtgacggggactcataaggttactgtgctctttgctggccagcacatcgccaagagccccttcgaggtgtacgtggataagtcacagggtgacgccagcaaagtgacagcccaaggtcccggcctggagcccagtggcaacatcgccaacaagaccacctactttgagatctttacggcaggagctggcacgggcgaggtcgaggttgtgatccaggaccccatgggacagaagggcacggtagagcctcagctggaggcccggggcgacagcacataccgctgcagctaccagcccaccatggagggcgtccacaccgtgcacgtcacgtttgccggcgtgcccatccctcgcagcccctacactgtcactgttggccaagcctgtaacccgagtgcctgccgggcggttggccggggcctccagcccaagggtgtgcgggtgaaggagacagctgacttcaaggtgtacacaaagggcgctggcagtggggagctgaaggtcaccgtgaagggccccaagggagaggagcgcgtgaagcagaaggacctgggggatggcgtgtatggcttcgagtattaccccatggtccctggaacctatatcgtcaccatcacgtggggtggtcagaacatcgggcgcagtcccttcgaagtgaaggtgggcaccgagtgtggcaatcagaaggtacgggcctggggccctgggctggagggcggcgtcgttggcaagtcagcagactttgtggtggaggctatcggggacgacgtgggcacgctgggcttctcggtggaagggccatcgcaggctaagatcgaatgtgacgacaagggcgacggctcctgtgatgtgcgctactggccgcaggaggctggcgagtatgccgttcacgtgctgtgcaacagcgaagacatccgcctcagccccttcatggctgacatccgtgacgcgccccaggacttccacccagacagggtgaaggcacgtgggcctggattggagaagacaggtgtggccgtcaacaagccagcagagttcacagtggatgccaagcacggtggcaaggccccacttcgggtccaagtccaggacaatgaaggctgccctgtggaggcgttggtcaaggacaacggcaatggcacttacagctgctcctacgtgcccaggaagccggtgaagcacacagccatggtgtcctggggaggcgtcagcatccccaacagccccttcagggtgaatgtgggagctggcagccaccccaacaaggtcaaagtatacggccccggagtagccaagacagggctcaaggcccacgagcccacctacttcactgtggactgcgccgaggctggccagggggacgtcagcatcggcatcaagtgtgcccctggagtggtaggccccgccgaagctgacatcgacttcgacatcatccgcaatgacaatgacaccttcacggtcaagtacacgccccggggggctggcagctacaccattatggtcctctttgctgaccaggccacgcccaccagccccatccgagtcaaggtggagccctctcatgacgccagtaaggtgaaggccgagggccctggcctcagtcgcactggtgtcgagcttggcaagcccacccacttcacagtaaatgccaaagctgctggcaaaggcaagctggacgtccagttctcaggactcaccaagggggatgcagtgcgagatgtggacatcatcgaccaccatgacaacacctacacagtcaagtacacgcctgtccagcagggtccagtaggcgtcaatgtcacttatggaggggatcccatccctaagagccctttctcagtggcagtatctccaagcctggacctcagcaagatcaaggtgtctggcctgggagagaaggtggacgttggcaaagaccaggagttcacagtcaaatcaaagggtgctggtggtcaaggcaaagtggcatccaagattgtgggcccctcgggtgcagcggtgccctgcaaggtggagccaggcctgggggctgacaacagtgtggtgcgcttcctgccccgtgaggaagggccctatgaggtggaggtgacctatgacggcgtgcccgtgcctggcagcccctttcctctggaagctgtggcccccaccaagcctagcaaggtgaaggcgtttgggccggggctgcagggaggcagtgcgggctcccccgcccgcttcaccatcgacaccaagggcgccggcacaggtggcctgggcctgacggtggagggcccctgtgaggcgcagctcgagtgcttggacaatggggatggcacatgttccgtgtcctacgtgcccaccgagcccggggactacaacatcaacatcctcttcgctgacacccacatccctggctccccattcaaggcccacgtggttccctgctttgacgcatccaaagtcaagtgctcaggccccgggctggagcgggccaccgctggggaggtgggccaattccaagtggactgctcgagcgcgggcagcgcggagctgaccattgagatctgctcggaggcggggcttccggccgaggtgtacatccaggaccacggtgatggcacgcacaccattacctacattcccctctgccccggggcctacaccgtcaccatcaagtacggcggccagcccgtgcccaacttccccagcaagctgcaggtggaacctgcggtggacacttccggtgtccagtgctatgggcctggtattgagggccagggtgtcttccgtgaggccaccactgagttcagtgtggacgcccgggctctgacacagaccggagggccgcacgtcaaggcccgtgtggccaacccctcaggcaacctgacggagacctacgttcaggaccgtggcgatggcatgtacaaagtggagtacacgccttacgaggagggactgcactccgtggacgtgacctatgacggcagtcccgtgcccagcagccccttccaggtgcccgtgaccgagggctgcgacccctcccgggtgcgtgtccacgggccaggcatccaaagtggcaccaccaacaagcccaacaagttcactgtggagaccaggggagctggcacgggcggcctgggcctggctgtagagggcccctccgaggccaagatgtcctgcatggataacaaggacggcagctgctcggtcgagtacatcccttatgaggctggcacctacagcctcaacgtcacctatggtggccatcaagtgccaggcagtcctttcaaggtccctgtgcatgatgtgacagatgcgtccaaggtcaagtgctctgggcccggcctgagcccaggcatggttcgtgccaacctccctcagtccttccaggtggacacaagcaaggctggtgtggccccattgcaggtcaaagtgcaagggcccaaaggcctggtggagccagtggacgtggtagacaacgctgatggcacccagaccgtcaattatgtgcccagccgagaagggccctacagcatctcagtactgtatggagatgaagaggtaccccggagccccttcaaggtcaaggtgctgcctactcatgatgccagcaaggtgaaggccagtggccccgggctcaacaccactggcgtgcctgccagcctgcccgtggagttcaccatcgatgcaaaggacgccggggagggcctgctggctgtccagatcacggatcccgaaggcaagccgaagaagacacacatccaagacaaccatgacggcacgtatacagtggcctacgtgccagacgtgacaggtcgctacaccatcctcatcaagtacggtggtgacgagatccccttctccccgtaccgcgtgcgtgccgtgcccaccggggacgccagcaagtgcactgtcacagtgtcaatcggaggtcacgggctaggtgctggcatcggccccaccattcagattggggaggagacggtgatcactgtggacactaaggcggcaggcaaaggcaaagtgacgtgcaccgtgtgcacgcctgatggctcagaggtggatgtggacgtggtggagaatgaggacggcactttcgacatcttctacacggccccccagccgggcaaatacgtcatctgtgtgcgctttggtggcgagcacgtgcccaacagccccttccaagtgacggctctggctggggaccagccctcggtgcagccccctctacggtctcagcagctggccccacagtacacctacgcccagggcggccagcagacttgggccccggagaggcccctggtgggtgtcaatgggctggatgtgaccagcctgaggccctttgaccttgtcatccccttcaccatcaagaagggcgagatcacaggggaggttcggatgccctcaggcaaggtggcgcagcccaccatcactgacaacaaagacggcaccgtgaccgtgcggtatgcacccagcgaggctggcctgcacgagatggacatccgctatgacaacatgcacatcccaggaagccccttgcagttctatgtggattacgtcaactgtggccatgtcactgcctatgggcctggcctcacccatggagtagtgaacaagcctgccaccttcaccgtcaacaccaaggatgcaggagaggggggcctgtctctggccattgagggcccgtccaaagcagaaatcagctgcactgacaaccaggatgggacatgcagcgtgtcctacctgcctgtgctgccgggggactacagcattctagtcaagtacaatgaacagcacgtcccaggcagccccttcactgctcgggtcacaggtgacgactccatgcgtatgtcccacctaaaggtcggctctgctgccgacatccccatcaacatctcagagacggatctcagcctgctgacggccactgtggtcccgccctcgggccgggaggagccctgtttgctgaagcggctgcgtaatggccacgtggggatttcattcgtgcccaaggagacgggggagcacctggtgcatgtgaagaaaaatggccagcacgtggccagcagccccatcccggtggtgatcagccagtcggaaattggggatgccagtcgtgttcgggtctctggtcagggccttcacgaaggccacacctttgagcctgcagagtttatcattgatacccgcgatgcaggctatggtgggctcagcctgtccattgagggccccagcaaggtggacatcaacacagaggacctggaggacgggacgtgcagggtcacctactgccccacagagccaggcaactacatcatcaacatcaagtttgccgaccagcacgtgcctggcagccccttctctgtgaaggtgacaggcgagggccgggtgaaagagagcatcacccgcaggcgtcgggctccttcagtggccaacgttggtagtcattgtgacctcagcctgaaaatccctgaaattagcatccaggatatgacagcccaggtgaccagcccatcgggcaagacccatgaggccgagatcgtggaaggggagaaccacacctactgcatccgctttgttcccgctgagatgggcacacacacagtcagcgtgaagtacaagggccagcacgtgcctgggagccccttccagttcaccgtggggcccctaggggaagggggagcccacaaggtccgagctgggggccctggcctggagagagctgaagctggagtgccagccgaattcagtatctggacccgggaagctggtgctggaggcctggccattgctgtcgagggccccagcaaggctgagatctcttttgaggaccgcaaggacggctcctgtggtgtggcttatgtggtccaggagccaggtgactacgaagtctcagtcaagttcaacgaggaacacattcccgacagccccttcgtggtgcctgtggcttctccgtctggcgacgcccgccgcctcactgtttctagccttcaggagtcagggctaaaggtcaaccagccagcctcttttgcagtcagcctgaacggggccaagggggcgatcgatgccaaggtgcacagcccctcaggagccctggaggagtgctatgtcacagaaattgaccaagataagtatgctgtgcgcttcatccctcgggagaatggcgtttacctgattgacgtcaagttcaacggcacccacatccctggaagccccttcaagatccgagttggggagcctgggcatggaggggacccaggcttggtgtctgcttacggagcaggtctggaaggcggtgtcacagggaacccagctgagttcgtcgtgaacacgagcaatgcgggagctggtgccctgtcggtgaccattgacggcccctccaaggtgaagatggattgccaggagtgccctgagggctaccgcgtcacctatacccccatggcacctggcagctacctcatctccatcaagtacggcggcccctaccacattgggggcagccccttcaaggccaaagtcacaggcccccgtctcgtcagcaaccacagcctccacgagacatcatcagtgtttgtagactctctgaccaaggccacctgtgccccccagcatggggccccgggtcctgggcctgctgacgccagcaaggtggtggccaagggcctggggctgagcaaggcctacgtaggccagaagagcagcttcacagtagactgcagcaaagcaggcaacaacatgctgctggtgggggttcatggcccaaggaccccctgcgaggagatcctggtgaagcacgtgggcagccggctctacagcgtgtcctacctgctcaaggacaagggggagtacacactggtggtcaaatggggggacgagcacatcccaggcagcccctaccgcgttgtggtgccctgagtctggggcccgtgccagccggcagcccccaagcctgccccgctacccaagcagccccgccctcttcccctcaaccccggcccaggccgccctggccgcccgcctgtcactgcagccgcccctgccctgtgccgtgctgcgctcacctgcctccccagccagccgctgacctctcggctttcacttgggcagagggagccatttggtggcgctgcttgtcttctttggttctgggaggggtgagggatgggggtcctgtacacaaccacccactagttctcttctccagccaagaggaataaagttttgcttccattaaaaaaaaaaaaaaaaaaaaaaaaaaaaaaaaaaaaaaaaaaaaaaa

SEQ ID NO: 49 - protein, 2647 aa, Homo sapiens
MSSSHSRAGQSAAGAAPGGGVDTRDAEMPATEKDLAEDAPWKKIQQNTFTRWCNEHLKCVSKRIANLQTDLSDGLRLIALLEVLSQKKMHRKHNQRPTFRQMQLENVSVALEFLDRESIKLVSIDSKAIVDGNLKLILGLIWTLILHYSISMPMWDEEEDEEAKKQTPKQRLLGWIQNKLPQLPITNFSRDWQSGRALGALVDSCAPGLCPDWDSWDASKPVTNAREAMQQADDWLGIPQVITPEEIVDPNVDEHSVMTYLSQFPKAKLKPGAPLRPKLNPKKARAYGPGIEPTGNMVKKRAEFTVETRSAGQGEVLVYVEDPAGHQEEAKVTANNDKNRTFSVWYVPEVTGTHKVTVLFAGQHIAKSPFEVYVDKSQGDASKVTAQGPGLEPSGNIANKTTYFEIFTAGAGTGEVEVVIQDPMGQKGTVEPQLEARGDSTYRCSYQPTMEGVHTVHVTFAGVPIPRSPYTVTVGQACNPSACRAVGRGLQPKGVRVKETADFKVYTKGAGSGELKVTVKGPKGEERVKQKDLGDGVYGFEYYPMVPGTYIVTITWGGQNIGRSPFEVKVGTECGNQKVRAWGPGLEGGVVGKSADFVVEAIGDDVGTLGFSVEGPSQAKIECDDKGDGSCDVRYWPQEAGEYAVHVLCNSEDIRLSPFMADIRDAPQDFHPDRVKARGPGLEKTGVAVNKPAEFTVDAKHGGKAPLRVQVQDNEGCPVEALVKDNGNGTYSCSYVPRKPVKHTAMVSWGGVSIPNSPFRVNVGAGSHPNKVKVYGPGVAKTGLKAHEPTYFTVDCAEAGQGDVSIGIKCAPGVVGPAEADIDFDIIRNDNDTFTVKYTPRGAGSYTIMVLFADQATPTSPIRVKVEPSHDASKVKAEGPGLSRTGVELGKPTHFTVNAKAAGKGKLDVQFSGLTKGDAVRDVDIIDHHDNTYTVKYTPVQQGPVGVNVTYGGDPIPKSPFSVAVSPSLDLSKIKVSGLGEKVDVGKDQEFTVKSKGAGGQGKVASKIVGPSGAAVPCKVEPGLGADNSVVRFLPREEGPYEVEVTYDGVPVPGSPFPLEAVAPTKPSKVKAFGPGLQGGSAGSPARFTIDTKGAGTGGLGLTVEGPCEAQLECLDNGDGTCSVSYVPTEPGDYNINILFADTHIPGSPFKAHVVPCFDASKVKCSGPGLERATAGEVGQFQVDCSSAGSAELTIEICSEAGLPAEVYIQDHGDGTHTITYIPLCPGAYTVTIKYGGQPVPNFPSKLQVEPAVDTSGVQCYGPGIEGQGVFREATTEFSVDARALTQTGGPHVKARVANPSGNLTETYVQDRGDGMYKVEYTPYEEGLHSVDVTYDGSPVPSSPFQVPVTEGCDPSRVRVHGPGIQSGTTNKPNKFTVETRGAGTGGLGLAVEGPSEAKMSCMDNKDGSCSVEYIPYEAGTYSLNVTYGGHQVPGSPFKVPVHDVTDASKVKCSGPGLSPGMVRANLPQSFQVDTSKAGVAPLQVKVQGPKGLVEPVDVVDNADGTQTVNYVPSREGPYSISVLYGDEEVPRSPFKVKVLPTHDASKVKASGPGLNTTGVPASLPVEFTIDAKDAGEGLLAVQITDPEGKPKKTHIQDNHDGTYTVAYVPDVTGRYTILIKYGGDEIPFSPYRVRAVPTGDASKCTVTVSIGGHGLGAGIGPTIQIGEETVITVDTKAAGKGKVTCTVCTPDGSEVDVDVVENEDGTFDIFYTAPQPGKYVICVRFGGEHVPNSPFQVTALAGDQPSVQPPLRSQQLAPQYTYAQGGQQTWAPERPLVGVNGLDVTSLRPFDLVIPFTIKKGEITGEVRMPSGKVAQPTITDNKDGTVTVRYAPSEAGLHEMDIRYDNMHIPGSPLQFYVDYVNCGHVTAYGPGLTHGVVNKPATFTVNTKDAGEGGLSLAIEGPSKAEISCTDNQDGTCSVSYLPVLPGDYSILVKYNEQHVPGSPFTARVTGDDSMRMSHLKVGSAADIPINISETDLSLLTATVVPPSGREEPCLLKRLRNGHVGISFVPKETGEHLVHVKKNGQHVASSPIPVVISQSEIGDASRVRVSGQGLHEGHTFEPAEFIIDTRDAGYGGLSLSIEGPSKVDINTEDLEDGTCRVTYCPTEPGNYIINIKFADQHVPGSPFSVKVTGEGRVKESITRRRRAPSVANVGSHCDLSLKIPEISIQDMTAQVTSPSGKTHEAEIVEGENHTYCIRFVPAEMGTHTVSVKYKGQHVPGSPFQFTVGPLGEGGAHKVRAGGPGLERAEAGVPAEFSIWTREAGAGGLAIAVEGPSKAEISFEDRKDGSCGVAYVVQEPGDYEVSVKFNEEHIPDSPFVVPVASPSGDARRLTVSSLQESGLKVNQPASFAVSLNGAKGAIDAKVHSPSGALEECYVTEIDQDKYAVRFIPRENGVYLIDVKFNGTHIPGSPFKIRVGEPGHGGDPGLVSAYGAGLEGGVTGNPAEFVVNTSNAGAGALSVTIDGPSKVKMDCQECPEGYRVTYTPMAPGSYLISIKYGGPYHIGGSPFKAKVTGPRLVSNHSLHETSSVFVDSLTKATCAPQHGAPGPGPADASKVVAKGLGLSKAYVGQKSSFTVDCSKAGNNMLLVGVHGPRTPCEEILVKHVGSRLYSVSYLLKDKGEYTLVVKWGDEHIPGSPYRVVVP